European Patent Application EP 4 595 770 A2, published August 6, 2025. Title: Low Fiber Pennycress Meal and Methods of Making. Applicant: CoverCress, Inc. The sequence listing filed with the application follows.

SEQUENCE LISTING (197 sequences)

SEQ ID NO: 1 - DNA, 795 bp, Thlaspi arvense
  source 1..795: mol_type = other DNA
atggggaagagaacaagtaacagtttgaagaaagatgagttaaacagaggagcttggactgatcaagaagacaagatccttaaagattatatcatgatccatggcgaaggcaaatggagcactctcccaaaccaagccggtctcaagaggtgtggcaaaagctgcagactcaggtggaagaactacttgagaccggggataaagcgcggaaacatctcatctgatgaagaagaactcataatccgcctccataatctccttggaaacagatggtctctgatagctgggaggcttccggggcgaacagacaatgaaataaagaaccattggaactcaaacctccgcaaaagacttcccaaaacaaaaaccaaccaaccaaaacttcgaaaacattcaaccaacatcaagaacaatgtctgtgttatacgcacaaaggcgattaggtgctcaaaggctctgacttttcagaaccagagtagtagtggtagtaccaatcttcttcctatgaaagaacaagtgagctctatgatggatcatgaagctggttcttcgttgttggaagatcttgaaattgattttgataaaatccaatcagagtttctcttccctgatctgatggatttggaaggtttgggttgtggaaacgtaacatcacttgtttcatctgaggagattttaggagattatgttcgtgctgatgaatcttctcagggtaatcttgatctcaatagacctttcactccttgtcttcatcgtggcaacgatgaagattggctccgagttttcaattgttag

SEQ ID NO: 2 - protein, 264 aa, Thlaspi arvense
MGKRTSNSLKKDELNRGAWTDQEDKILKDYIMIHGEGKWSTLPNQAGLKRCGKSCRLRWKNYLRPGIKRGNISSDEEELIIRLHNLLGNRWSLIAGRLPGRTDNEIKNHWNSNLRKRLPKTKTNQPKLRKHSTNIKNNVCVIRTKAIRCSKALTFQNQSSSGSTNLLPMKEQVSSMMDHEAGSSLLEDLEIDFDKIQSEFLFPDLMDLEGLGCGNVTSLVSSEEILGDYVRADESSQGNLDLNRPFTPCLHRGNDEDWLRVFNC

SEQ ID NO: 3 - DNA, 3512 bp, Thlaspi arvense
  source 1..3512: mol_type = genomic DNA
tctcagccaaattgacaaataaaaatcacatttagaaaacatttcacggttttgtatgtaaactagtaaaaaaaaaaaaagagaacatgttatttcaatatataacattggaaagtatagtatattgattctctcactaatctaaaaatttatgcatcaataatttttaatagattaaaaatctaaagttaatcttattggaaattaaatataattattaagtttcaatatatatagacatgttatctctttcatttttaaccaactagtgatatgggacaaagtacaaaatgttagttacatcagttttaatctgatataaaatttgtatcaatttttttaatgttaacaaaattattgattacattgattatttaaatagtgtaaatttataattttatatcagttttgtttaactgatgtaaactaatataagtttgtatcaattttattgaacggaagtcaaataatcaataaaaatatcaattttcagaactgatgttaaatcacatattttatatcatttattaataagtaattcaccttttttgtagtgtgatatgagttattggcgtttaataataattttaaaaaattatagtttcatgttaaatcttacaaaattatataaatcttttaaaatcaaaaattatttatttgagcatttgcaataatgaacagttgcgaatgaataattaataaaatatttaaaaattaaaaatgtaaataacaaaatgtatttaaactctgaatatatgtatataataacataaattgacttaaaaaataataaatcatatgtacaaagttgacgccttcttaaatactgtttttataatttctaatataataattattcaaatggaaaaattaaacttgaatatgaaccttttaactctttgattgtcaaaaataaaaagttttcatgaaatagagttccgaacttaaaaaagagacatttgaaacttgggaccccaaatttatgtaacactgaaagatcttaaggagttttattttttgtttgttcatgacgcaggactatgtgtactgtgtaggcatgaagaccatgtgttaccgtcttaactgtatcaaatgatgattgcttacatactagaatgtggctagcaatgactattttcactctgtatacatacttataccccatatgcaatacaataatgatcaaggtcgttttaggacctatatgattggagtctaaggcacgagagactagactagcgatcatcgtgtgaagtgagttcaaaggatttcagatccttagtaataagtacaaaagtatattcttgatgacaaaattcggtagagttaaatctcaccaaaactgatacactattattaccaggtgagaaaaggattgatatttcaaagtgtgtgtgtgtgacagaagttttggaaagcgacatgtgtacggacattgcaacaactccatataaagttactttgttaacacaaaaagaatctattctctactcaacactaaagacaattgtaccaaccaaacaaccacaagagagagaaagagagtatggggaagagaacaagtaacagtttgaagaaagatgagttaaacagaggagcttggactgatcaagaagacaagatccttaaagattatatcatgatccatggcgaaggcaaatggagcactctcccaaaccaagccggtacatatccatctatctattgatctatccgtctttaaatgcaaatcttcatctacttacaataattgcacataaaggtctcaagaggtgtggcaaaagctgcagactcaggtggaagaactacttgagaccggggataaagcgcggaaacatctcatctgatgaagaagaactcataatccgcctccataatctccttggaaacaggttaattaacttcctctttcaccgaaacacagattgttttcttttcaagttaagtttttccataatttttgcggcgtaatgcagatggtctctgatagctgggaggcttccggggcgaacagacaatgaaataaagaaccattggaactcaaacctccgcaaaagacttcccaaaacaaaaaccaaccaaccaaaacttcgaaaacattcaaccaacatcaagaacaatgtctgtgttatacgcacaaaggcgattaggtgctcaaaggctctgacttttcagaaccagagtagtagtggtagtaccaatcttcttcctatgaaagaacaagtgagctctatgatggatcatgaagctggttcttcgttgttggaagatcttgaaattgattttgataaaatccaatcagagtttctcttccctgatctgatggatttggaaggtttgggttgtggaaacgtaacatcacttgtttcatctgaggagattttaggagattatgttcgtgctgatgaatcttctcagggtaatcttgatctcaatagacctttcactccttgtcttcatcgtggcaacgatgaagattggctccgagttttcaattgttagagcgtatcactagtctacataattacatacatatatatctgtacgaacaaaattatatttgtattttgtttgaaagcttctaatttctaattactaattttgttgtgttttctaatccatagattatcaattttgcactctttttcaattaaagacttatggaaatggcttttgtctttagaataaaatacaaattgcaaaatatcgcaaatacgcaatgaagattatttattttcgatagattttattcaattattatgtgcatgcataaatgatagagcttttattatagcctaactaccgcttaactaccctaccaataaattatacgagggtcattgttcttggtaatacgaaaaaaatctttgcaatattgtcttaacgaaattgaattttaatatacacacatatccatttataggcagacacggtcatacatctaaggatttattgttttttgtttcttatcattcttcggaatcattgtataaatggttattgttgtaacaagagaaaggacatcgggttataattttatagaggaaacctaaatttgtgattgtcgactgtggccgctgacggcggttcagtgtcactagtttatggtcttttatctatgctattgtgggtgcgaatatgtccttttgttaaccttcttaaatattgaaataaggttgttttcggattgtcaatgttattaaacaaatccattctcaatagtttgacaaaaaaaaaaaaaaaatccattctcaataaatagctgatgcaggaaagactattggtttttctgtattttaagttatcggatcttttatatgatataatccattacaaatagacactaattagacaagtgttaaaaatagttcttattatcaatttggcagtgatacataaataaacctattacacctacctattaggtgattatctgcgtatacatacatacacacggatttacattttattatagattttaaaatgtataaataatataccatattttattt

SEQ ID NO: 4 - DNA, 795 bp, Thlaspi arvense
  source 1..795: mol_type = genomic DNA
atggggaagagaacaagtaacagtttgaagaaagatgagttaaacagaggagcttggactgatcaagaagacaagatccttaaagattatatcatgatccatggcgaaggcaaatggagcactctcccaaaccaagccggtctcaagaggtgtggcaaaagctgcagactcaggtggaagaactacttgagaccggggataaagcgcggaaacatctcatctgatgaagaagaactcataatccgcctccataatctccttggaaacagatggtctctgatagctgggaggcttccggggcgaacagacaatgaaataaagaaccattgaaactcaaacctccgcaaaagacttcccaaaacaaaaaccaaccaaccaaaacttcgaaaacattcaaccaacatcaagaacaatgtctgtgttatacgcacaaaggcgattaggtgctcaaaggctctgacttttcagaaccagagtagtagtggtagtaccaatcttcttcctatgaaagaacaagtgagctctatgatggatcatgaagctggttcttcgttgttggaagatcttgaaattgattttgataaaatccaatcagagtttctcttccctgatctgatggatttggaaggtttgggttgtggaaacgtaacatcacttgtttcatctgaggagattttaggagattatgttcgtgctgatgaatcttctcagggtaatcttgatctcaatagacctttcactccttgtcttcatcgtggcaacgatgaagattggctccgagttttcaattgttag

SEQ ID NO: 5 - protein, 109 aa, Thlaspi arvense
MGKRTSNSLKKDELNRGAWTDQEDKILKDYIMIHGEGKWSTLPNQAGLKRCGKSCRLRWKNYLRPGIKRGNISSDEEELIIRLHNLLGNRWSLIAGRLPGRTDNEIKNH

SEQ ID NO: 6 - DNA, 813 bp, Thlaspi arvense
  source 1..813: mol_type = other DNA
atgagagattcaaactcaatccttgatctgtctcttcagatcagccttcctaactctcacgccggagaacttcttcacggcggtgaccgaagctccaccacaagtagtgattctggaagcagtctcagtgagttgggccatgagaacaacttcttcaacaaacctctcctaagcttaggttttgatcatcattatcgttatcaaaggcactcaaacatgatccaaccacaaatctacggtcgagatttcaagagaagctcatcatcaatggtttgtcttaaacgaagcattcgagctccaagaatgagatggacttctactctccatgcgcactttgtccatgctgttcagcttcttggcggccatgaaagagctacgcctaaatcagtgttggagttgatgaatgtgaaggatctaaccctagctcatgtcaagagtcacttgcagatgtatagaacagtgaaatgcactgataaaggatcatcaggagaaggaaaggtagagaaagatacagagctgatgacagaggacaataataataatgaagaagctgacgaaggaactgacacaaattcgccaaactcatcatctgtgcaaaagacccaaagggcttcttgttcatccaaaaagagagtgtgtatgaacatatctacacaagcagaacctcacttgggatcaactcgtcacactaatgatgatgggaagaaagaggcgatcaacgctcatctcaatttggaattcacattaggccggcaaagttgggggatggactattcggaacccttaagagatctaactcttctcaagtgctaa

SEQ ID NO: 7 - protein, 270 aa, Thlaspi arvense
MRDSNSILDLSLQISLPNSHAGELLHGGDRSSTTSSDSGSSLSELGHENNFFNKPLLSLGFDHHYRYQRHSNMIQPQIYGRDFKRSSSSMVCLKRSIRAPRMRWTSTLHAHFVHAVQLLGGHERATPKSVLELMNVKDLTLAHVKSHLQMYRTVKCTDKGSSGEGKVEKDTELMTEDNNNNEEADEGTDTNSPNSSSVQKTQRASCSSKKRVCMNISTQAEPHLGSTRHTNDDGKKEAINAHLNLEFTLGRQSWGMDYSEPLRDLTLLKC

SEQ ID NO: 8 - DNA, 4752 bp, Thlaspi arvense
  source 1..4752: mol_type = genomic DNA
gaggtcggtcgattcaaacttcttttccctttttgtcttttgtgtatatttccatatctatcctttattctccgagtaataaggaaattcttctttatcttttgaattagtccgatgtttccggtcttcaaaggttatccttaagagatttccttaaatccgaactaggtcggcacggtcttcctagtcttgatgggcttaagttattgcgagggaaaaccttttaggaaatgtattcattttccctctaacaatgttttaagtatgtattaacaaaataaaaattaatatatgaaaacaattaataaaaataagtaagatgcttatgtgaagcagaatattcccgaccgtgtgtctacttaccgtggccaaagacatcgcatgaaaaaacaaaccaaagagtaaggtaaattaaatagaatgtatttaactagattgaacttggagtaattagttgtctttctctttttgcacttttgaaaagataaacaaaatttccttttggagctactttgtggttcaaacaagaatccccatggcaaaacggcagttactttgtcagtcaacttttgaaatctgaggctttcaaggattgtaagaaatattaaatacaaaactctgttgtattttccatcgaccctaagagacaggccttttcaagcctatctttttagcattggaaattttaaagtgttttattttatttatttaaaatagtaaaaacatgcaaatcatagggtactcattatctaattatcacactcactctctttcctcggcttggtttaacctttttaaccactgatcaaataatacgtagccaatttgtccaaaatcttccaacttcttttcctcctttcttacttctttaaattattttagtattcgtcataaatcaaaagatacgttgtcttgaacatgtacacaggttgtagtatttgtgtgaaacacaaaagtgtatactagtattttagttaggaaatctacaccatatatttacttttcttataaattaagtatatgactttgacattattttaatgatacataatcttttgattactttcatcagttattttttttgctaaaaattaatttaaatgttgtttttaacctactaaagatttcatgcgtacgtcagagactattttttgtttctcatatcatgatatgtaatcagaaaagtgaaaacaggttgccatgtacattcatttatgatacacaattgattttttttttctttttaccaaataacaggttattcatcagttgccacattggcgaaagatgaaaatactattttcattgatccgcataaataaaaaatcctttgattttaccactttgttatggtagtcatttacgtagttttaattcggttatctacccgaattacgttttttttgcttaaaagttgaaaatgttattctacgtagggactaacatctggtaatacagtactacgataagagtgaataattaagagttttataaataggttatatatttaaatcatttgtacacgtagaaaataaaacatattattcttaaaaaaagacgatagactatgtttattgagataaagacaatagttacgtcgttgcttttcttgctctctctctctccatttctttctctctccgctatttaaatagacaaaggattaatgaaaaagtagagagatgatgatgttagactccagaagcagtatgagagattcaaactcaatccttgatctgtctcttcagatcagccttcctaactctcacgccggagaacttcttcacggcggtgaccgaagctccaccacaagtagtgattctggaagcagtctcagtgagttgggccatgagaacaacttcttcaacaaacctctcctaagcttaggttttgatcatcattatcgttatcaaaggcactcaaacatgatccaaccacaaatctacggtcgagatttcaagagaagctcatcatcaatggtttgtcttaaacgaagcattcgagctccaagaatgagatggacttctactctccatgcgcactttgtccatgctgttcagcttcttggcggccatgaaagtattttgctttcacattttcctttttaaaagaaataatcaagatttatgtcaagtaaaatgttttgaaaccaaagtactaagatttgttgcttatttgctggtctcaggagctacgcctaaatcagtgttggagttgatgaatgtgaaggatctaaccctagctcatgtcaagagtcacttgcaggtccatctctattttaatttatttttcttatatattttattataaaaatagtaatggaatctcataagaatgcaataggtttaagtaaacatttatgaaagtgtatctatttggtccactagctaacacatgattgcgtagttgaaataaacttgtattagctatactttttttattttttatttggttttgatttttaaaggatgtgtgtttgttgatgcagatgtatagaacagtgaaatgcactgataaaggatcatcaggtatgcattcaaaccggattggctgatttttgaattcctactggatgtaaatgtaactatctcatttttttttttttgttttaatttgtatttgtttcttcttgggaataacaggagaaggaaaggtagagaaagatacagagctgatgacagaggacaataataataatgaagaagctgacgaaggaactgacacaaattcgccaaactcatcatctgtgcaaaagacccaaaggttactcttttatctattctattttgtaaaaactttgcatttaatctctttgcctttgttatgcgcgaattttgatgaatccctcttctagtcgtatgtgaccctgcttgtccatttttataaatagaaaaaatttctatgatctcagttaaattgtgtgtattcactgttgatagtaaataagtaggttcaaataaaacaatatatgaatatgaatgtccaacaatatgaattattattagtagatttctcaaatgtgttttttatcatttaaatttgaacagggcttcttgttcatccaaaaagagagtgtgtatgaacatatctacacaagcagaacctcacttgggatcaactcgtcacactaatgtacattctttaacaaattgttacaatgttattatagatgtgcactctcacatatacgtacatatacccttctgtatactgtttctaaaatgtgaaatctttggaaataggatgatgggaagaaagaggcgatcaacgctcatctcaatttggaattcacattaggccggcaaagttgggggatggactattcggaacccttaagagatctaactcttctcaagtgctaatcgtttagcttggagaactacaacaaataagtcagcttaggttatcaatttaacataattaacttgtttgatcgtaatagacattggaagaatcattatcatcatatatgaatttcttacaaaaaatgttctcatttttttttttgggatgtaaacaagagattcggattaagtagtagctatgttatggttgtagtggatgagaagggagtgcaagttcaagtagagatgaacttatgattggttgccaccaaatatgcatggtggatttgttggtagtttttttttatgttttcattgactgctattcatattgtcgcagtgaatatatatttaaatgattttgttttgattctttgtcttgatttggattagaaagtagaattcggcaaaactagaggtttttttactgatattctgcatgacaataaaactctcagttctatttaaatttttcgctttgttattgatacatataccgtttaaaaggatacattaaacaatactgaatagtactctcaaattctgtttttcgaaggatatgagttggtagatatttcacaacatcaaaaaacgaaggtgaaaataccttcttcagattgcaaagaattacagaaattttgtgccaggtttcgcagaccgcctgttgtaagagatcgcaacatatatcttgaaccaatccctcgaaagcataaataaacaaagtagacactaagaaatgattatataaataatataatatgtttaatttattaattatatgtagctgcaattgcttcatgaatattatgtggtagagactgacaaaaataaatggaaagagacacttcatcacaacatggtaatcataactcttcatccagaaaacttccatacctcttcatttatatgagaatttaatgttataggcaatctaataaatactctccctttgaaggtgcatccaactgaaaagcagggaccgatgccttccctttctaggaaacttgtcgcgccttaccagaacagtactctgccaagtccaatctagacttcatattgtcctttgtcttcctttgacattgagaacggtgttgattatgttgtctataaaattcttcgtattgtgcataacatctagattatgccttatcaaatggtccttccaaaaagacaattcccaaaatatactcatcttatacaaactatgttggtcaccacaagcgttcacatgataatgataaccttccatgcattggccatcagaataacatgccatatgctggaaaaaggctaatagtccacattaatactgaccccatgacaatattctgctgacaagaaacatgaaatgcctgaacactatgctcctataatatttgcagctcataaaacaatgattggagaaatt

SEQ ID NO: 9 - DNA, 1041 bp, Thlaspi arvense
  source 1..1041: mol_type = other DNA
atgacaatcttggatcagaccgttgtaacaaccggatcgaagaaggcttgtgtcatcggtggcacaggaaacttagcttctactctcatcaagcatttgcttcaaagtggctacaaagttaacactacagttagagatccagagaatgagaagaaaatggctcacttaagggtacttcaagaacttggggacctcaagatcttcaaggcggaatttactgatgaagagagtttcgattcaccagtttcgggctgtgattacgttttccatgtcgcaacgcctatcaactttacatctgaagatcccgagaaagacatgatcaagccagggatacaaggagtgaccaatgtgttgaaatcttgcttaaaatcgaaatcagtcaagcgtgtgatctacacttcttcagctgctgcggtttccatcaacaatctttctggacctggacttgtgatgaacgaagaaaactggactgaccttgattatctcacaaaggagaagccgtttaactggggctacccagtgtcaaagatactagcagaaaaggcagcttgtaaatttgcggaagagaacaagatcgatctagttaccgtgattccggcactcatatccggaaaatctctcctctcggatcctcctccgagcagctcatttctctctatgtctttaatcaccgggaatgaaatgtatctgaaaggtctcaaggaaatgcagaagcaatctggctccatctcgttcagccacgtgaaggatttggctcgtgcccatttgtttcttgcggagaaagaaactgcgtctggtcgttacatttgctgtacttacaacacaagtgttccggagattgcagattttctcaggcagagatatcctaagtacaatgtgctgtctgaattcgaagagtgcttatcaagtgcgaagctgacgctatcttcggaaaaactcatcaatgaaggctttcgattcgaatatgggattaatgagatctatgatgagatgatagagcacttcgagtccaaaggattaatcaaagctaaagaatcttga

SEQ ID NO: 10 - protein, 346 aa, Thlaspi arvense
MTILDQTVVTTGSKKACVIGGTGNLASTLIKHLLQSGYKVNTTVRDPENEKKMAHLRVLQELGDLKIFKAEFTDEESFDSPVSGCDYVFHVATPINFTSEDPEKDMIKPGIQGVTNVLKSCLKSKSVKRVIYTSSAAAVSINNLSGPGLVMNEENWTDLDYLTKEKPFNWGYPVSKILAEKAACKFAEENKIDLVTVIPALISGKSLLSDPPPSSSFLSMSLITGNEMYLKGLKEMQKQSGSISFSHVKDLARAHLFLAEKETASGRYICCTYNTSVPEIADFLRQRYPKYNVLSEFEECLSSAKLTLSSEKLINEGFRFEYGINEIYDEMIEHFESKGLIKAKES

SEQ ID NO: 11 - DNA, 4124 bp, Thlaspi arvense
  source 1..4124: mol_type = genomic DNA
gccgccgccgccgcgaaggccaagaagaaggatgtggaggctccgctgacaattgctttaggcttacaggcgccgaaatcgggaacgaagcggccgagtgaagggacttcaagggaggctaattcaaagcgagctaagaaggttacttcaggggacgacgagaagaagatcggcgaagactcaaagaaacctgcttttcagagactgtggtctgaggaagacgaaatcactgtgcttcaaggtatgatcgatttcaatgctgatacaggcaagtctccttacgaagacacgaatgtgtattacgatttcatcaagaaaaagattagctttgaggttagcaagaaccagttcatggataagattaggagcttgaagaagaagtatataggcaaaggaaagactgccttcacgaaacctcacgatcagagatctttcaagctgtgccaacacatatggggacctgaaggaatggctctcgagtcagcggttaagtccaatggcgtatcgagaaagagccagaagaagaagaagcttgactctgtgaagcaagagctgtcttttgcttcttcccctaatggcaaaacggttgatgatgataaaaaagtgttgatccatggaggagatgtggagtcttcggttgctgcgaagaagcatgattggttcgagagctcgtttcttgttcgcgccattgccggtttgggagttgatgagtatactgtgaaacagaggtggagcttggtgcctgttgagacgaagaagaaggttgaagagaagatgaagatgttgcaggccaaggagattgattttgtgttggagaagacacagtttttgcatgaggttacatcgatgatcgctgaagcatctaagaagaagacattagatatatagatttgatccgaaaatgccaatgccaatgcctctctcttttgttttttgaatcttaggaattatctcttttacttcccttttatgatctatcaatctatgtaatttttctggtttttctggtggtttttaatatggaactctctctcttttggatttgttgcttatacataaaagcaccatggaagtaaattctacatggtgaaatatgaagaagatccaaacaaactgttttttttttttttatgaaatgggtttattcaggatgaattttgttgaattgaggctaaaaaattttggtgttctctaaaacaaaaagttaaatgaaactttcagctcaaagatcaaattggttgaagaaagcaaaactcttttcacaagtagatgatatcaaatcagcaagtcaattaaaagtttgactctttttttgattcttaggtgagagagttagttattaaagaagaggaaggtaacacaaaattagttgcttcaaaactcacgtgcttaccttctaaaaagactttttgatcaatggttgtaccaaatgtgcaagaccataagctttgccactataaaaacgagtgctaaggccataaactcataacagtcagatctaaatatctgtgtttaagaactagtatcagatgacaatcttggatcagaccgttgtaacaaccggatcgaagaaggcttgtgtcatcggtggcacaggaaacttagcttctactctcatcaagcatttgcttcaaagtggctacaaagttaacactacagttagagatccaggttcttcatttcttctttctttcttctcttgaggttctttgagtgtttagtgactcttttattctgaatttgcagagaatgagaagaaaatggctcacttaagggtacttcaagaacttggggacctcaagatcttcaaggcggaatttactgatgaagagagtttcgattcaccagtttcgggctgtgattacgttttccatgtcgcaacgcctatcaactttacatctgaagatcccgaggtctgattttcaacagattgtgtatgtttttttttctctgactcttaagagaaacgttttcagctatcctttgtttgtgtttccatgtacagaaagacatgatcaagccagggatacaaggagtgaccaatgtgttgaaatcttgcttaaaatcgaaatcagtcaagcgtgtgatctacacttcttcagctgctgcggtttccatcaacaatctttctggacctggacttgtgatgaacgaagaaaactggactgaccttgattatctcacaaaggagaagccgtttaactgggtaatttacaatttcttgcgagccaagatagggtttacttggaccagtttacttactacatctctgttcttttctagggctacccagtgtcaaagatactagcagaaaaggcagcttgtaaatttgcggaagagaacaagatcgatctagttaccgtgattccggcactcatatccggaaaatctctcctctcggatcctcctccgagcagctcatttctctctatgtctttaatcaccggtaaacaccaattttactgtttgactccttctgttaaagtttcacaataagaaagtcaaagatgaatggtttttttttgttagggaatgaaatgtatctgaaaggtctcaaggaaatgcagaagcaatctggctccatctcgttcagccacgtgaaggatttggctcgtgcccatttgtttcttgcggagaaagaaactgcgtctggtcgttacatttgctgtacttacaacacaagtgttccggagattgcagattttctcaggcagagatatcctaagtacaatgtgctgtctgagtaagcatttatatccacagaaactgaaaatcttaatggaaaattctgaattttctcgttaattttcgctgtgaaatttggcagattcgaagagtgcttatcaagtgcgaagctgacgctatcttcggaaaaactcatcaatgaaggctttcgattcgaatatgggattaatgagatctatgatgagatgatagagcacttcgagtccaaaggattaatcaaagctaaagaatcttgaaatttataatgtgaagatatggatttatgagtatatgagtctttgttctcattctcattctataaatggcattaaataataagttggttgatttgatatgtattttgatatacacacctagaaaatgaaaaacaagatttttcaagctttatattactctacgaagctgattagtaattttacttctaagtttctcacatttcacaactaccttttttctttcccatgttataaatatataacttttttttcagcataaaaagaagttgtggaaagaatgcgacgaactattttaccaaaaaaaaaggtgacaatctacatggaaaaaagtaaataaaatgtgttaataaactttcgatttaaacaagttgtgtatttacatacaattgatatatatatatataatactttataatactgtattcttttatcaaaaggatatatactgtaatatttagcaaattatacataaaactatcaaattaaagagtatgatgtattccactgaaaacataaaaaatgatatatgtagaaaccaacctgagtgtatgcgcgtggatattcgtttagtaataatgataatgatatgagtagactatattacctaaagccaatcaacatatgaccaatctacaagctcgagctttattagatcaaaacataaaaattggtatatgtagaaatgttgtctaaattaaaccaagatgaaaaacatgagaaaacattaaaacatcactttttattcttggtgatttgttattagaactccgagcaaagaacgaatctgtgaggacatcatgcatgtatgtcttactcagcgtaatagggacattgtgcaagtcactgcaagagatctccaatgatgatctaacggatccaagaaagtaaaggaaaagaagaaggaagagcagattggtgagactcggatccaagaattagaggaagatctgaaggatctgaagcggatgtgcactgttctagaaacctttctagggaaagaaaaggcaaatgtgtttgaagccagagcccctgctatgacgttagatgagttgtataatgacttaggttctgcatgatgcgttgtggtattgtatgttcagggccggctctaagattatgggagtttgaaacaaaataaaaaat

SEQ ID NO: 12 - DNA, 1461 bp, Thlaspi arvense
  source 1..1461: mol_type = other DNA
atggatccgacgacgccgtttctcggtggcgaggtcgaagaggattatgctccggcgaggacatggagcgacgtcaagcgagtttttgctacggagtcggccaaaatgtggatgatcgccgctcccattggtttcaacatcatctgtcagtacggagttacctccatcaccaatattttcgtcggccatatcggcgaggtcgagctctccgccgtcgccatctccctctccgtcatcggcaccttttccttcggcttcctgcttggcatgggaagtgcacttgaaacactctgtggacaagcatttggagctggtcaagtccatatgttaggcgtttacatgcagagatcttggattatcttattcgtctcctgcatctttctccttcctatttacatattcgccacgccgattctgagactcctcggccaagcagaggagatcgccgttccagctggagaattcactcttttaaccatccctcagctattctcactcgccatcaacttcccaacctccaagttccttcaagcgcagagcaaagtcatcgcgattgcttggatcgggttcatcgctttcgtcctacacgtcggtatgctctggctgtttataatcgtgtttggttggggaacaaacggtgctgccttggcgtttaatctcaccaactggggaacagcgatctctcaagtcgtttatgtgattggttggtgtaatgaaggctggtctggtttgtcttggttggcatttaaagagatttgggctttcgttagactctccatagcatctgctgttatgctttgtcttgagatctggtacatgatgagtatcatcgtccttactggtcgccttgacaacgctgttatcgctgttgattccctttccatatgcatgaatctcaatggtctggaggccatgttgttcatcggaataaacgctgctataagtgtccgtgtctccaatgagcttggcttaggccgtccacgagcagcgaaatactctgtctatgtcacggtgttcgagtctctcctcatcggtcttgtctttatggtggctatcatcataggcagagaccattttgcgatcatcttcacgagcagcaaagtacttcaacgcgcagtgtctaagctagcttatcttcttggtataaccatggttctcaacagcgtgcagccagtcatttccggtgtggctgttggaggaggttggcaaagtttggtggcttatataaacttgggttgttactacattttcggccttccctttggatatcttcttggttacaaagcaaacttaggagtgatgggactttggtcgggaatgatagccgggacagcgcttcaaacgttgctactgatgtttgtcttgtacaagacaaactggaataaagaggttgaagagacgatggaacgtatgaagaaatggggagggagcgagacgacatcgaatgatgtaactgcgtga

SEQ ID NO: 13 - protein, 486 aa, Thlaspi arvense
MDPTTPFLGGEVEEDYAPARTWSDVKRVFATESAKMWMIAAPIGFNIICQYGVTSITNIFVGHIGEVELSAVAISLSVIGTFSFGFLLGMGSALETLCGQAFGAGQVHMLGVYMQRSWIILFVSCIFLLPIYIFATPILRLLGQAEEIAVPAGEFTLLTIPQLFSLAINFPTSKFLQAQSKVIAIAWIGFIAFVLHVGMLWLFIIVFGWGTNGAALAFNLTNWGTAISQVVYVIGWCNEGWSGLSWLAFKEIWAFVRLSIASAVMLCLEIWYMMSIIVLTGRLDNAVIAVDSLSICMNLNGLEAMLFIGINAAISVRVSNELGLGRPRAAKYSVYVTVFESLLIGLVFMVAIIIGRDHFAIIFTSSKVLQRAVSKLAYLLGITMVLNSVQPVISGVAVGGGWQSLVAYINLGCYYIFGLPFGYLLGYKANLGVMGLWSGMIAGTALQTLLLMFVLYKTNWNKEVEETMERMKKWGGSETTSNDVTA

SEQ ID NO: 14 - DNA, 4540 bp, Thlaspi arvense
  source 1..4540: mol_type = genomic DNA
gcagttcacatttaaatagtccaatatgttattattggcaagcaacccgaattgaaatgagacagtggaaacattagcaatccaaaacatcatacgaacctacttctacttataccttagagaagaataatcagattacgagtaacaagaatgaagaacctgagtcgcttagccttaatgttctaaatcaaataactaatctgagctcatttgcaaaacattggcccattttaaaattcttggcactgatacgcagcacaaaaggaggttactgtaaaagcccaatgtgcgtacattcattattcacaaaaaaaaatcttgtttgacttaaaattgtggccccctttttgggtttgtcttttaatttcatgtattttttaattaattgttttctattttggcattaatatggctctattaattataatttatgatacaaaatcagaatggaccgggctgggcctttggtgaagttggtgggctcggtttaagaattttatttttttcattattttgacttgcattaaataaaacaagtcaatgggaaatgtcatcatttatctgactggtttaatgacaaaggtttaatgatgaaacagggaaataaatacaaacgatgacgtaaactgaaaggggaccacaggaccctgtcgtttccgatgaaaaagaagaagaaaattccctctccgattcttcttcctgttcatattcattttacaaacggtacgtaactcactttttaatacttcacttaaggacatcaacctattttcggaaacgacaacttttccactcttggttcgagcttagattgattcaacatttttttcctaattaacttacatatactgtattcattttactgtctaacagtaaactcgagctatcctggcaagtttaatcttctcgacaacttactatatagttgatactatatcactaggatcaattttataaaaaaaaaaacaaattaatcacgtgaaaataattctcacacatgataaataaactaggagtaacaagtttgatgtgacattacactaacaaactttcacaacactaccctatcaatattaaatgtcaaatgatggaaaagagaaaagcagttttatgcttttgaataatcttgtatgcatatttctgatatgtcaaagtacgtggtgtctcatgcaccacccgttagcctcacctacctaatctacttctcaattccatgccgaattcggtaataaatttctcgtacgttttgtttttcctttccgctaattacccaaaaactaaaataggctaataactccttcaatttttattattgttattatttgattagtatggcaaaacaaggggagagagaagtgcgtgattcaacggttttgttatataaaccaaaaccccataattccgcaacaaacattgactcagagtgagagagagagagagagagagagagaagtctgtctgtgtgagctttgggtttaacattttgagactcgcacggagatggatccgacgacgccgtttctcggtggcgaggtcgaagaggattatgctccggcgaggacatggagcgacgtcaagcgagtttttgctacggagtcggccaaaatgtggatgatcgccgctcccattggtttcaacatcatctgtcagtacggagttacctccatcaccaatattttcgtcggccatatcggcgaggtcgagctctccgccgtcgccatctccctctccgtcatcggcaccttttccttcggcttcctggtatgcttttctcttcttctaactgatatctttcatgtaactctgctatgtatcaatcaagagcatcttcttgtgacaaatcgacaagaaacagagtctaatttaggtttgaaaactgcagcttggcatgggaagtgcacttgaaacactctgtggacaagcatttggagctggtcaagtccatatgttaggcgtttacatgcagagatcttggattatcttattcgtctcctgcatctttctccttcctatttacatattcgccacgccgattctgagactcctcggccaagcagaggagatcgccgttccagctggagaattcactcttttaaccatccctcagctattctcactcgccatcaacttcccaacctccaagttccttcaagcgcagagcaaagtcatcgcgattgcttggatcgggttcatcgctttcgtcctacacgtcggtatgctctggctgtttataatcgtgtttggttggggaacaaacggtgctgccttggcgtttaatctcaccaactggggaacagcgatctctcaagtcgtttatgtgattggttggtgtaatgaaggctggtctggtttgtcttggttggcatttaaagagatttgggctttcgttagactctccatagcatctgctgttatgctttgtcttgagatctggtacatgatgagtatcatcgtccttactggtcgccttgacaacgctgttatcgctgttgattccctttccatatggtgagttttgatcaacattttacaatgcttcttgtatcatcaacatctttcccactctttttttttgcatttcatttcagcatgaatctcaatggtctggaggccatgttgttcatcggaataaacgctgctataaggtagtactatcattatctgacacaacttttgtttaacccattgttcagcttgtaaactgatcatgtgtctacctacttgtgtactatatattagtgtccgtgtctccaatgagcttggcttaggccgtccacgagcagcgaaatactctgtctatgtcacggtgttcgagtctctcctcatcggtcttgtctttatggtggctatcatcataggcagagaccattttgcgatcatcttcacgagcagcaaagtacttcaacgcgcagtgtctaagctagcttatcttcttggtataaccatggttctcaacagcgtgcagccagtcatttccggtaacaaaaatctaaaattctcatgttccatcaaaacaaaaaccagaggtctcataagaccataaccgtcccggtttgttcatcttgttttaggtgtggctgttggaggaggttggcaaagtttggtggcttatataaacttgggttgttactacattttcggccttccctttggatatcttcttggttacaaagcaaacttaggagtgatggtaagcgaatacaaagaatgacatgaataatgtagatctttcggacatgcatgtttcataaactgatacgtgagagattataacgttttcagggactttggtcgggaatgatagccgggacagcgcttcaaacgttgctactgatgtttgtcttgtacaagacaaactggaataaagaggtaaagaacacctgagacacaaaaccgtagtatatacactggttcattgagatcgattgacttatggaaatataaaattgtaaaaactgtgatgaacaggttgaagagacgatggaacgtatgaagaaatggggagggagcgagacgacatcgaatgatgtaactgcgtgactatttcttttgttaatattaattaattaattattgtttagctttatatatatgaacatgtaggtctcagcttttttgtttgttttccattggtttggcagcaccagtaactctctatttactatttacgctgtaggaaacttttcattcagtgatgtaacgatgcatgcttttgtcactttgtttctcttggagtaaactaaatgttaggtacattttctcgtgtaacacaaattttattagacggcttttagtcttcaatgcaaattcaagtgacttgtacatagattcctgtcttctacttccatttccttcagaagtcaattgtatgtttccattttattcttctaccggtggaaaataatatagtatcagtacgtaatttttagcgtgcttgtaacacaggatggccgagcggtctaagccacgagactcaagttcttgtcctcctataggaggatatggattcaaatccctcttgtgacataataatttctttaaaaaaaaaatcattttgctatactttgcatatttttctttttctttttaagaatgcatgcatgtcttactttctcgtttctgcttgataggtcgtagtgtcctaataagctcttctgagaaatctcttatttttcttcttgaacgttggattcagcatttcttcattgtgatttttgacttgcgaagatacgcacacttatacattgattagggtcatcctcgtctcaagtgttattgcaatgtctaggtttggacatagcacactagtctttgctatttcatcacccaaaatccattaaatcatggtgatgatttgatttaaagctaatggttttgctaatttgattttttttatgtgtattttttgttctgtaataggtggcgtgagtggaacaacagaagggtggaacacaaacacttattaggtctccctgttttcaacatgatgcatttgattttgttggttatatctcctcaaatgcttgttgcattgcctaaa

SEQ ID NO: 15 - DNA, 2322 bp, Thlaspi arvense
  source 1..2322: mol_type = other DNA
atgtcaatggccgtcgaaatgtcatcgaaacaacccaccaaagatttcttctcctctccagccctctccctctctctcgctggtatattccggaatgcatcctccggcagcaggaaccctgaggaggactttttggggagaagggtagttgacgatgaggatcggacggtggagatgagcagcgagaactcgggacccacgagatccagatcagaggaagacttggaggatcaagaggaggaggaggaggatgaggaggaagacggagcaggaaacaagggcaacaagaggaagaggaagaagtatcaccgccacaccaccgatcagattagacacatggaagcgctgttcaaagagacgccccatccagacgagaagcaaagacagcagctgagcaagcaattagggctggctcctcgccaggtcaaattctggttccaaaaccgccgcacccagatcaaggctattcaagaacggcacgagaactcgctgctgaaagcggaactagagaagctgagggaggaaaacaaaggcatgagagagtcttttgccaaggctaattcttgctgcccaaactgcggaggaggcaccgatgatgtccacatcgagaactccaaactgaaggcggagctggataagcttcgtgcggctctcggacgcactccctacccactccaggcctcatgctccgatgatcaaccacaccgtctcgacttctacacgggcgtctttgccctcgacaagtcccgcatcgtggagattgccagccgagccacccttgagctccagaagatggcctcctccggccaacctctttggctccgcagccttgagactggccgtgacattctcaactacgacgagtatctcaaggacttccctcaagctcaggcctctcccctccatgcaaggagatccatcgaagcatccagggatgtggggatcgtgtttatggacgcacacaaacttgctcagagttttatggacgtggggcaatggaaagagatgtttgcgtgcttgatctcaaaggcggcgacggttgatgtaatccggcagggtgaagggccttcaaggatcgacggtgcgattcagttgatgtttggggagatgcaactgctcactccggttgtccccacaagagaagtgtacttcgtgagaagctgccggcagcttagccctgagaaatgggccatcgtggacgtatcagtctctctggaggaagacgacaacaacaacaacacggaggacaaggaggcttcgctgcttaaatgccggaaacgcccctcaggttgcatcatcgaggacacctccaacggccactccaaggtcacctgggtggagcacctcgacttgtctgcctccaccgttcagcctctcttccgctcctttgtcaacaccggtttggcctttggggctcgacactgggtcgccaccctccagctccactgcgaacgcctcgtcttcttcatggctaccaacgtccctaccaaggactctctcggtccgtccattatttacactctctctctccctctctctctttctccctctcaccttttcttaaccccaatcctcctctcaggagttacaacgcttgccgggagaaagagcgtgctcaagatggcccagaggatgacacaaagcttctaccgcgccattgctgcttccagctaccaccaatggaccaaaatcaccaccaaaactggacaagacatgagggtttcttccaggaagaacctccatgatcctggtgagcccaccggagtcatcgtctgcgcttcttcctccctctggttacctgtttctcccactctcctcttcgatttctttagagatgaagctcgtcgccatgagtgggatgctttgtcaaacggagctcatgttcagtctatcgcaagcttatccaagggacaagacagaggcaactcagtgtctatccagacagtgaaatcgagagaaaagagcatatgggtgctgcaggacagcagcacaaactcatatgagtcggtggtcgtatacgctcccgtagatataaacacgacacagctggtgattgcaggacatgatccaagcaacatccaaatcctgccttgtggattctcaatcatacccgatggagtagaatcaagaccactggtaatcacgtctgcacaagaggacagaaacagccaaggagggtctctgctcacactggccctccaaacgctcatcaacacttctcctgcagcaaagctgaatatggagtccgtggaatccgtcacaaacctcgtctctctcaccctccacaacattaagagaagcctccaaatcgaagattgttga

SEQ ID NO: 16 - protein, 773 aa, Thlaspi arvense
MSMAVEMSSKQPTKDFFSSPALSLSLAGIFRNASSGSRNPEEDFLGRRVVDDEDRTVEMSSENSGPTRSRSEEDLEDQEEEEEDEEEDGAGNKGNKRKRKKYHRHTTDQIRHMEALFKETPHPDEKQRQQLSKQLGLAPRQVKFWFQNRRTQIKAIQERHENSLLKAELEKLREENKGMRESFAKANSCCPNCGGGTDDVHIENSKLKAELDKLRAALGRTPYPLQASCSDDQPHRLDFYTGVFALDKSRIVEIASRATLELQKMASSGQPLWLRSLETGRDILNYDEYLKDFPQAQASPLHARRSIEASRDVGIVFMDAHKLAQSFMDVGQWKEMFACLISKAATVDVIRQGEGPSRIDGAIQLMFGEMQLLTPVVPTREVYFVRSCRQLSPEKWAIVDVSVSLEEDDNNNNTEDKEASLLKCRKRPSGCIIEDTSNGHSKVTWVEHLDLSASTVQPLFRSFVNTGLAFGARHWVATLQLHCERLVFFMATNVPTKDSLGPSIIYTLSLPLSLSPSHLFLTPILLSGVTTLAGRKSVLKMAQRMTQSFYRAIAASSYHQWTKITTKTGQDMRVSSRKNLHDPGEPTGVIVCASSSLWLPVSPTLLFDFFRDEARRHEWDALSNGAHVQSIASLSKGQDRGNSVSIQTVKSREKSIWVLQDSSTNSYESVVVYAPVDINTTQLVIAGHDPSNIQILPCGFSIIPDGVESRPLVITSAQEDRNSQGGSLLTLALQTLINTSPAAKLNMESVESVTNLVSLTLHNIKRSLQIEDC

SEQ ID NO: 17 - DNA, 5982 bp, Thlaspi arvense
  source 1..5982: mol_type = genomic DNA
aacccataaagagcattcatttccttttaaggtcgctgaaattaatgagtaacgatcagtcaatgcgtctcgttgaccttccaaaacatccgacgtctctttccgttgcatatccctcggctctgtccctgcagctcccacgtcatccatatttcccctctatccaatttttaactttctaacttattcaacaactcttcctccatgcatttacctcattatctaatcgtattgtttactagtagtaatatagcatactagagtagtagattcggattcccggaataatatatattagcataagttattggagcacaaggcatttcaggtttccatgtagctccaataatatcctcttcactctctcttaccaatgcttttccactttcctatgtcacgcaattactagcttgcttgctttacaaccaagttttattaaccaacataaaatatagagatttaatgttgcattttgtaatcataagttactaattgcttgaagaaagagatcacaataacagacaatacgtacacattacatcataaccaggtaagtatatagtatataataaataaataaatagaagtcataataagagaaatgatgatgataatcaaggaggaaagaagaaagcagaaaatgcggttggagaattaggtgcttaaagttagttgagtccatcccagtatctaacggtcaactctctcctctttcgtccttatttgtattttattttgtttttgaaacaataaactgacatacaatatgtctttctctcactactctctctctctctctctctatacacaaattcaattaaagaagagacagagaagttcgccttttgtctgtatacccttaaatcatgcaacccccttattctcattccttctctctgcctacagtaaactctaggaacgacattatgtggtttaaaccgattcaattcatgattagtggcaaaattctatatgattttcaaccacatgatatatgattttcaacagtaatattgtgcggaaaaataatgcacagcattttattctatatacaaaaggtaaattggaaaggagaattttccagatgcaatagcgaatttgctcgaatatttttataaaaaaaaacgaagtcgatatcgacgcctgcaaataatgtagctggccatgtttgcaaagtaatcaagtgtgaataaaattgtaaaactaatggagtatatatagatattaaaaagaagaaggggttggttaaatataattaaatgaagcacctaaaagtcaagcaatagagaaatatctgaaaaacgaccgtttgtatgtataattagaattgaagggctagcttagctatatagccatatacagtatatgtgaaagagtacattttggtacacacacacacaaaaaaaaagaaataaggaaaatatatagagatatataaatagcacaaggaagaaggaggagagggaagataaagcaaataaaaaaattgggagcgttcgtatgtcaatggccgtcgaaatgtcatcgaaacaacccaccaaagatttcttctcctctccagccctctccctctctctcgtacgcgtactctctgttctactactctcgtaaactcatctaaataaaaatttactgtattgtatatatgtatctatttgtgaatggtactgatataaatacaggctggtatattccggaatgcatcctccggcagcaggaaccctgaggaggactttttggggagaagggtagttgacgatgaggatcggacggtggagatgagcagcgagaactcgggacccacgagatccagatcagaggaagacttggaggatcaagaggaggaggaggaggatgaggaggaagacggagcaggaaacaagggcaacaagaggaagaggaagaagtatcaccgccacaccaccgatcagattagacacatggaagcgtacgttcttccttccttaattattattctttatatttcatctgtagctctaatggattaccatttaatcaaattagggtttcaaaacatggaacatttcgattaattggtcttgatgatatatgaatttgatgacctcaactcctccatatatacttcaattatgactagtcatcatcatcatgccctacacatagggattagagtatatagtagtcagtctgtgctgaacagtaggcctcttcatttctactgccatataaaaaggaagaatgcatatttcatgtatttattagtagtgatgaacaaattaatatatattgcagatcgatgatccagcaatagttaattatttgaatgcgtttaattacatatcttgctctttaattttctctcgtactccctagtatatacatgtgtttatactataacataggacgggacaagtgtttccattcaatcaccctatgattaaactaaaaccaagttctttcaaaacaaaaaactaaaaccaagagcactaatgtgtatagctagttagggctcatataattaagagtttaattcatactatgttttcgaataggaggataaaaaaaagatatgaaagaattaattaaatatgaagaatgatcatggagctatgaatgagaaaactgagggttgcattgcaggctgttcaaagagacgccccatccagacgagaagcaaagacagcagctgagcaagcaattagggctggctcctcgccaggtcaaattctggttccaaaaccgccgcacccagatcaaggtatgtatatcgacgtacgtgatgatgatgatatatatggatttcttaagacaaaaagactattcgcttggagctacatatgtatatagttatagtgaaatactgaaatgtaactgaacaggctattcaagaacggcacgagaactcgctgctgaaagcggaactagagaagctgagggaggaaaacaaaggcatgagagagtcttttgccaaggctaattcttgctgcccaaactgcggaggaggcaccgatgatgtccacatcgagaactccaaactgaaggcggagctggataagcttcgtgcggctctcggacgcactccctacccactccaggcctcatgctccgatgatcaaccacaccgtctcgacttctacacgggcgtctttgccctcgacaagtcccgcatcgtggagattgccagccgagccacccttgagctccagaagatggcctcctccggccaacctctttggctccgcagccttgagactggccgtgacattctcaactacgacgagtatctcaaggacttccctcaagctcaggcctctcccctccatgcaaggagatccatcgaagcatccagggatgtggggatcgtgtttatggacgcacacaaacttgctcagagttttatggacgtggtactctttttctttcatttcctccaaatatttacgaatatacttttgtgtatcacatgtaggcaatataaagatatatatacaacgtgcaggggcaatggaaagagatgtttgcgtgcttgatctcaaaggcggcgacggttgatgtaatccggcagggtgaagggccttcaaggatcgacggtgcgattcagttggttagtgaatcaccttttgatagatagtgatgacacgcgagagatgagagctaatataatacattgatggacatattggcagatgtttggggagatgcaactgctcactccggttgtccccacaagagaagtgtacttcgtgagaagctgccggcagcttagccctgagaaatgggccatcgtggacgtatcagtctctctggaggaagacgacaacaacaacaacacggaggacaaggaggcttcgctgcttaaatgccggaaacgcccctcaggttgcatcatcgaggacacctccaacggccactccaaggtcacctgggtggagcacctcgacttgtctgcctccaccgttcagcctctcttccgctcctttgtcaacaccggtttggcctttggggctcgacactgggtcgccaccctccagctccactgcgaacgcctcgtcttcttcatggctaccaacgtccctaccaaggactctctcggtccgtccattatttacactctctctctccctctctctctttctccctctcaccttttcttaaccccaatcctcctctcaggagttacaacgcttgccgggagaaagagcgtgctcaagatggcccagaggatgacacaaagcttctaccgcgccattgctgcttccagctaccaccaatggaccaaaatcaccaccaaaactggacaagacatgagggtttcttccaggaagaacctccatgatcctggtgagcccaccggagtcatcgtctgcgcttcttcctccctctggttacctgtttctcccactctcctcttcgatttctttagagatgaagctcgtcgccatgaggtaccttgtggcatacacttccttcgcacacacagaaccaataaaaccgttttaaatctaactatacatacgtattattatcatcagtgggatgctttgtcaaacggagctcatgttcagtctatcgcaagcttatccaagggacaagacagaggcaactcagtgtctatccagacagtgaaatcgagagaaaagagcatatgggtgctgcaggacagcagcacaaactcatatgagtcggtggtcgtatacgctcccgtagatataaacacgacacagctggtgattgcaggacatgatccaagcaacatccaaatcctgccttgtggattctcaatcatacccgatggagtagaatcaagaccactggtaatcacgtctgcacaagaggacagaaacagccaaggagggtctctgctcacactggccctccaaacgctcatcaacacttctcctgcagcaaagctgaatatggagtccgtggaatccgtcacaaacctcgtctctctcaccctccacaacattaagagaagcctccaaatcgaagattgttgatgacaactcacagcaggtgtgatgattgttgttacatatataagtatatcataatgtatagcagtgcattaagttttgtacaaaaacaaccctctctctctctcccgcaatcatactgttatccaacactttttgcagcattaagagagcatcatactcgactaagaacccaatacacaaaactttaccgaaacaaaagtgggatcagatgaaccaaatgcataaccctgatttagatacacagtaattggatcagaaacgaaggcctgatcaaattccacaacttaaacaatacgcaattcgagcaggaaaacaaaatgcattccataaacagagagaattacacttgattgcaatacacaacaaacagaaacgaaaaacagtaaaaaagacagctttttttttttaccaaaacaaacaaacactcagtgagtcgcattctcctctacgccggctgctgagattccaagggaatgccgaggtcgttcccagcttctcctccgccttccgctttcctgctgctccttgagacgacagcaagcgccacgaatgacttagtcttactgatgggtctgctcttctccagcctcaccacatcgcccaccttgaactgattatccgggtcatgcgcctggtacttcttcttcttcctcacgcgcctcttgtacttgggatgcggagccagcctcaccacctccaccgccacggtcttgtcgttggttgcgcacaccacgcgcccctgcatcgttttcatggctctgatgaccggaaccaatgccggccttcgagggttcgggaataaattgggcttagagagagatgagagtggagtcgagccatgggcgaatggagacgaaagcttcagagcttgcagagatgaggttattagcgacgtcatcgttatccccctcctctatgggatcgatttggaagacgatgaagaagataaggcgatagatcatgttattataatattggcttttgctaaatgggttaacaa

SEQ ID NO: 18 - DNA, 2007 bp, Thlaspi arvense
  source 1..2007: mol_type = other DNA
atggctactacgtataagcctaagaacattctcatcactggagctgctggattcattgcctctcatgttgccaacagattaatccgtagctatccagattacaagatcgttgtgttggacaagcttgattactgttcagatctgaagaatctcgatccttcgttttcttctccaaatttcaagtttgtgaaaggagatatcgcgagtgatgacctcgttaactacctcctcatcactgaaaacatcgacaccatcatgcactttgctgctcaaacccatgttgataactcctttggtaatagctttgagttcaccaagaacaacatttatggtactcatgtcctcttggaagcctgtaaagtaacaggacagatcaggaggtttattcatgtgagcaccgatgaagtctatggagaaaccgatgaggatgctgctgtaggaaaccatgaggcgtctcagcttttacccacaaacccatactcagccactaaggctggtgctgagatgcttgtgatggcttacggtagatcatacggactgccggttattacaactcgtgggaacaatgtttacggtcctaaccagtttcccgaaaaactgattcctaagttcatcttgttggctatgagtgggaagccgcttccgatccacggagatggatctaacgtaaggagttacttatactgtgaagacgttgctgaagcgtttgaggttgttcttcacaaaggagaagtcggtcacgtctacaacatcgggacaaagagagaaagaagagtgatcgatgtggcgacagacatctgcaaacttttcgggaaagatcctgagtcgagcatcgagttcgtggagaatcgaccgtttaacgatcaaaggtacttccttgatgatcagaagctgaagaatctgggttggtcagagcgaaccgcgtgggaagatggactgaagaagacaatggaatggtacattcagaatcctgagtggtggggtgatgtttctggagctttgcttcctcatccgagaatgcttatgatgcccggaggaagagttcctgacggctccgatgagaagaatgactcgtcaagcaacgcggtccagacattcacggttgtaacaccgaacaacaagactggtggttctagtgacaaagctttcttgaagtttttgatctacggtaagactggttggatcggtggtctcttagggaaactatgtgagaagcaagggattacttatgagtatgggaaaggacgtttagaagatagagcctctctcgtcgcggatattcgcagtatcaaaccgacccatgtgtttaacgctgctggtttaactggcagaccaaacgttgactggtgtgaatctcacaaaccagagaccattcgtgtcaatgtcgctggtactttgactctcgctgatgtttgcagagagaatgatctcttgatgatgaacttcgccaccggttgcatattcgagtacgatgctgcacatccagagcgttcgggtattggtttcaaggaagaagacaagccgaatttcactggctctttctactcaaaaaccaaagccatggtcgaggagcttctgagagaatttgacaatgtgtgtaccttgagagtgcggatgccgatctcatcagacctaaacaacccgagaaacttcatcacgaagatctcgcggtacaacaaagtggtgaacatcccgaacagcatgaccatactggacgagcttctgccgatctccatcgagatggcgaagagaaacctaagagggatatggaacttcaccaacccaggggtggtgagccacaacgagatactggagatgtacaagagttacatcgagccagggtttaaatggtccaacttcacagtggaagaacaagcaaaggtcattgttgctcctcgaagcaacaatgaaatggatgggactaaactaagcaaggagttcccagagatgctaccaattaaagaggcgctgatcaaatacgtcttcgaacctaacaagagaacctga

SEQ ID NO: 19 - protein, 668 aa, Thlaspi arvense
MATTYKPKNILITGAAGFIASHVANRLIRSYPDYKIVVLDKLDYCSDLKNLDPSFSSPNFKFVKGDIASDDLVNYLLITENIDTIMHFAAQTHVDNSFGNSFEFTKNNIYGTHVLLEACKVTGQIRRFIHVSTDEVYGETDEDAAVGNHEASQLLPTNPYSATKAGAEMLVMAYGRSYGLPVITTRGNNVYGPNQFPEKLIPKFILLAMSGKPLPIHGDGSNVRSYLYCEDVAEAFEVVLHKGEVGHVYNIGTKRERRVIDVATDICKLFGKDPESSIEFVENRPFNDQRYFLDDQKLKNLGWSERTAWEDGLKKTMEWYIQNPEWWGDVSGALLPHPRMLMMPGGRVPDGSDEKNDSSSNAVQTFTVVTPNNKTGGSSDKAFLKFLIYGKTGWIGGLLGKLCEKQGITYEYGKGRLEDRASLVADIRSIKPTHVFNAAGLTGRPNVDWCESHKPETIRVNVAGTLTLADVCRENDLLMMNFATGCIFEYDAAHPERSGIGFKEEDKPNFTGSFYSKTKAMVEELLREFDNVCTLRVRMPISSDLNNPRNFITKISRYNKVVNIPNSMTILDELLPISIEMAKRNLRGIWNFTNPGVVSHNEILEMYKSYIEPGFKWSNFTVEEQAKVIVAPRSNNEMDGTKLSKEFPEMLPIKEALIKYVFEPNKRT

SEQ ID NO: 20 - DNA, 5240 bp, Thlaspi arvense
  source 1..5240: mol_type = genomic DNA
acccttattttcaatcacagctccccaagatagatcagttaagcaacagcaacacacatatggccattgatgctaagctgttgcaggcgcaatcacagttcggtccagcgggagcagcagcggttgcggtagcggcacaccggaacattggcacaattagttacggcgcagcatcgtagactcatcaaacaaacagcattttcagacacatctttaacttacatcaccctccaaatccaggcaacgcgaaaccaggtgattccggtctcggtctctttatgtaagtattattcagccaggctctgatttaaacaactttgcagtgatattaataaaagactttcagttgtaactcaccagaacaagatcgcttagatcagtctgatcccgggttatcaccggtgattgtttcggttatcttgtttgctccatagtctttgaatttgttataagcgtagttcatcgaagagaagaaaaccgtcgtgattatatacttcttaaacttcaagatcggtcccattactccttaattgttcttcaacaatgatgaatctctttgtctatcagaaaattgattgatctatttggctatatagagagaatcattaggccgaaaattgtggaagtcaacaaaagtcattggtccgtagatctttctcatccgtaaatcaatcttttgcacattataattagccattttattcaatggttaccagtaaaaaagatatgtaaaagataatttcgaattcttgacgccattaaagtgtctatataatttacccgccaatttaagataaccggttttatgggcctgaactcagcacattaaaggttaacatttactataataattcaatgaacttaactccttttcttcaattacatgaaaaagtgcatttttgtctacttgattttttaattgatgaaaaaggaagtaaattaattattccgttacgtgaccttaagcatcagcattgaatcatctgttatgtttaatttcaggtcttttcttgttgaactgatgattgatatcaggttgacatgtgatatttctattcagtctagaattatttgtttttctaactgaacatatgtacgttttatcataaacaaatcagggattttattaaatcccaagtttaaccttccaataaaagaaatcatatttttattcagtttaaatcattttaagaaatatatatcagacaaaaatgcaaaatattttgtttacttcttccacaattaattaatctccttaattatacaaattttattctctttttattttttggaattttcttctattagtatagattttgtgtgaaaaaataaacaaaaaaaagacatcaaatttttatgtcggacgctaagctcacgtaaaatccgtaatatctaagacaagtaagggtaaatttgtcaattgacccctacggttctccgtaactgtctcaggatatatgaggcgcactgttcagagacgctccgtagaccgtagattccctcttcttcctcctctctctctctctctctctctctctctctcttctcatagaagtgtctctctctctctcttaggattcttctctgattctaacctgaattgtgtcggtacgtgatatgttgctctctttttgttgctgctgaaatttccataatgctttaagttaattttgcgaaatgctatacgtgagtaacggacaagtgtacaacatcagacaactgatcttgtttttgttcttttttttagatttctgtgttgtcggtttatgatcccatatgaaaagttcattatttttgttcgtataagatctggctactgaatttattcggttttggcgattggatctggatctgcctttattctgatttcctttcatatgatccgttctgaattttcgaatgatactgtgacgttattgttgttgttgttgcagatacttgatttcaaatggctactacgtataagcctaagaacattctcatcactggagctgctggattcattgcctctcatgttgccaacagattaatccgtagctatccagattacaagatcgttgtgttggacaagcttgattactgttcagatctgaagaatctcgatccttcgttttcttctccaaatttcaagtttgtgaaaggagatatcgcgagtgatgacctcgttaactacctcctcatcactgaaaacatcgacaccatcatgcactttgctgctcaaacccatgttgataactcctttggtaatagctttgagttcaccaagaacaacatttatggtactcatgtcctcttggaagcctgtaaagtaacaggacagatcaggaggtttattcatgtgagcaccgatgaagtctatggagaaaccgatgaggatgctgctgtaggaaaccatgaggcgtctcagcttttacccacaaacccatactcagccactaaggctggtgctgagatgcttgtgatggcttacggtagatcatacggactgccggttattacaactcgtgggaacaatgtttacggtcctaaccagtttcccgaaaaactgattcctaagttcatcttgttggctatgagtgggaagccgcttccgatccacggagatggatctaacgtaaggagttacttatactgtgaagacgttgctgaagcgtttgaggttgttcttcacaaaggagaagtcggtcacgtctacaacatcgggacaaagagagaaagaagagtgatcgatgtggcgacagacatctgcaaacttttcgggaaagatcctgagtcgagcatcgagttcgtggagaatcgaccgtttaacgatcaaaggtacttccttgatgatcagaagctgaagaatctgggttggtcagagcgaaccgcgtgggaagatggactgaagaagacaatggaatggtacattcagaatcctgagtggtggggtgatgtttctggagctttgcttcctcatccgagaatgcttatgatgcccggaggaagagttcctgacggctccgatgagaagaatgactcgtcaagcaacgcggtccagacattcacggttgtaacaccgaacaacaagactggtggttctagtgacaaagctttcttgaagtttttgatctacggtaagactggttggatcggtggtctcttagggaaactatgtgagaagcaagggattacttatgagtatgggaaaggacgtttagaagatagagcctctctcgtcgcggatattcgcagtatcaaaccgacccatgtgtttaacgctgctggtttaactggcagaccaaacgttgactggtgtgaatctcacaaaccagagaccattcgtgtcaatgtcgctggtactttgactctcgctgatgtttgcagagagaatgatctcttgatgatgaacttcgccaccggttgcatattcgagtacgatgctgcacatccagagcgttcgggtattggtttcaaggaagaagacaagccgaatttcactggctctttctactcaaaaaccaaagccatggtaaaatactaatatctataactcatgacagtctcgaaacaaagaagagtgtctttgtttataatctggttctgcttttttctcttcttctttgttcaccaggtcgaggagcttctgagagaatttgacaatgtgtgtaccttgagagtgcggatgccgatctcatcagacctaaacaacccgagaaacttcatcacgaagatctcgcggtacaacaaagtggtgaacatcccgaacagcatgaccatactggacgagcttctgccgatctccatcgagatggcgaagagaaacctaagagggatatggaacttcaccaacccaggggtggtgagccacaacgagatactggagatgtacaagagttacatcgagccagggtttaaatggtccaacttcacagtggaagaacaagcaaaggtcattgttgctcctcgaagcaacaatgaaatggatgggactaaactaagcaaggagttcccagagatgctaccaattaaagaggcgctgatcaaatacgtcttcgaacctaacaagagaacctgagacctgaacagcactcttcgccacaagtgcttacctataactgtttccttttctttctttctctttcaacagaaatgtctttttatgtttactcatcgtcttatgatccttgtaggtagtttcactatattgattctactaaaatatgatttatcattattatttatagagactaaagttttttttttctttctcaaattctacatttcccctcggattttacttactaagagacagtagtacacttataaaaatgaagagccacttactggttgtgatcattagggattccaccaaggcaggttcaaaacacttgaacttgattattaagctatagcctgagaagagaagcaaacaacaagtgttgatttgaaataaaccgaagtatatgatgtgaatttggtcaatattcagggttatagttttcttacgtgaacagttgagggcgggaacgagagagctgagagcgtttaataggggagagaataaggtttcgtagagttgactggggattagcagcgccaccaccaccgccaaatacaggatgtcctcctcctcctgctcttctgtttccaaggtctgttggaattgcgggtgagtcgttggagatgtcgaatggacctgagtttgaactgttctgtcttgctggccaaatctcatctttaggtcctggtgttgcaggagagtaaaacgaccggtctgcgccaaataagtcaacttgatttggagatattaaccaacaatagacttggaatcaaaagaagcactaggctcaaggtagttcattaacctttgcgagggggctctctgttctccatcatgttaactggtgggtttgagaaaaagtcaggttcgtggtgtcgtgggtagaaattgtttgctggttggatggctgtacgtttacatgactcgtattcacttcttagctggtcatacatctcatcgagcttcctcttctgtctggtgtttgaaacaataattacagctgagttagagataaggaacagaaccaggcaaacaaagcgtgtgttaaatcactgaccttgatttctcggagaacttctcttggagctcttgtttatccttggtcaagttttctacctcttgctccatcatctgacacctcttgcccatcttctggtatgctgtatgcacctgctccattttctcgctaaactttgct

SEQ ID NO: 21 - DNA, 1995 bp, Thlaspi arvense
  source 1..1995: mol_type = other DNA
atggctacatataagcccaagaacatcctcatcactggggctgctggattcatagcgtcccatgtcgccaacaggcttgttcgaagctaccctgactacaaaatcgttgtgcttgacaagcttgattactgctcaaacctgaaaaacctcaatccttcgaaatcctctccaaacttcaagtttgtcaagggagacatcgccagtgctgacctcgtcaactaccttctcatcactgaaaacatcgacacgattatgcactttgctgctcagacccatgtcgacaattccttcggtaacagcttcgagtttaccaagaacaatatttacggcacccatgtccttctggaagcttgcaaagtcactgggcagatcaggaggttcatccatgtgagtaccgatgaggtctatggagagactgatgaggatgcttcagtgggaaaccatgaggcttctcagttgctccctacaaacccttactctgccactaaagctggagctgagatgcttgtgatggcatacggtagatcatacgggttgccagttataacgactcgcgggaacaatgtctatggtccgaatcagtttcctgaaaagttgatccctaagttcattctgttggctatgagtgggaagccactgccgatccacggagatggatctaacgtgaggagttacctctactgcgaagatgttgctgaggcgtttgaggttgttctacacaaaggggaagtcaaccatgtctacaatatagggacaacgagagaaaggagagtgattgatgttgccaacgacatctcaaaactctttggaatagaccctgactccaccattcagtttgttgagaaccggccttttaatgaccagaggtacttcctcgatgaccagaagctgaagaagttgggatggtctgaacgaaccacttgggaagaaggactgaaaaagacaatggattggtacactgcgaaccctgagtggtggggagatgtctccggagctctgctgcctcatccacggatgttgatgatgcctggtgatagactctctgatggctctgacgagcgcaaggatgcagacggtaatcagacattcacggtggttactcccaccaaggccggtggttccgcagacaaaacatccttaaagttcctcatctatggcaaaactgggtggctcggtggtctcctaggaaagatatgtgagaagcaagggattccgtacgagtatggaaaagggagactagaagacagagcttcaatcatggcggatattcgcagcgtcaaacctacccatgtcttcaatgccgcgggcttaacaggcaggcctaatgttgactggtgtgagtctcacaaaaccgagactatccgagtcaacgtcgctggtactttgactctggcagatgtttgcagagagaatgatctgttgatgatgaactttgccaccggttgtatatttgagtatgacgctgcacatccagaaggttcagggattggcttcaaggaagaagacaaaccgaatttcaccggttccttctactcaaagacaaaggcaatggtcgaagagcttctaagagagtttgacaacgtatgcaccttgagagtgaggatgccaatctcatccgacttgaacaacccgcgaaacttcatcacaaagatctcgcgttacaacaaagtggtgaacatcccaaacagcatgaccatactcgacgagctcttaccaatctcaatcgagatggcgaagaggaacctacgggggatttggaatttcaccaacccaggagtggtgagtcacaacgagatactagagatgtacaagagctacatcgagccaggtttcaaatggtccaacttcactttagaggaacaggctaaggtcattgtcgcaccacggagcaacaacgagatggatggttttaagctcagcaaggagtttccagagatgctttccatcaaagattcgttgatcaaatacgtcttcgaacccaacaagagaacgtaa

SEQ ID NO: 22 - protein, 664 aa, Thlaspi arvense
MATYKPKNILITGAAGFIASHVANRLVRSYPDYKIVVLDKLDYCSNLKNLNPSKSSPNFKFVKGDIASADLVNYLLITENIDTIMHFAAQTHVDNSFGNSFEFTKNNIYGTHVLLEACKVTGQIRRFIHVSTDEVYGETDEDASVGNHEASQLLPTNPYSATKAGAEMLVMAYGRSYGLPVITTRGNNVYGPNQFPEKLIPKFILLAMSGKPLPIHGDGSNVRSYLYCEDVAEAFEVVLHKGEVNHVYNIGTTRERRVIDVANDISKLFGIDPDSTIQFVENRPFNDQRYFLDDQKLKKLGWSERTTWEEGLKKTMDWYTANPEWWGDVSGALLPHPRMLMMPGDRLSDGSDERKDADGNQTFTVVTPTKAGGSADKTSLKFLIYGKTGWLGGLLGKICEKQGIPYEYGKGRLEDRASIMADIRSVKPTHVFNAAGLTGRPNVDWCESHKTETIRVNVAGTLTLADVCRENDLLMMNFATGCIFEYDAAHPEGSGIGFKEEDKPNFTGSFYSKTKAMVEELLREFDNVCTLRVRMPISSDLNNPRNFITKISRYNKVVNIPNSMTILDELLPISIEMAKRNLRGIWNFTNPGVVSHNEILEMYKSYIEPGFKWSNFTLEEQAKVIVAPRSNNEMDGFKLSKEFPEMLSIKDSLIKYVFEPNKRT

SEQ ID NO: 23 - DNA, 5650 bp, Thlaspi arvense
  source 1..5650: mol_type = genomic DNA
cctttcgtttgcatttttgtgttacggtgtgatatctggtgaggatgtacatatgtggtaaagtggcaataatagtagctatttataaaattttatcataaatattattttttacatgaaactatatataatacaaaatttttaggcaaacaaaaattattagtcaaaaagtataattcaaaactcacttgattcaaatatcggaatcagcgcgctagatggggtgataagatttaccatctcaactaaatgaccatatatatgactccatataaatataatcaaatagttttgatttaataaaacgtttactattatatacgtttaataaaaaagtactttaccagcttttacgtgagttatggaaaaattatgaaatccaagatgtaatcaagggttgctgtccaaaaaaataaaaaaaaaacattagttaagggttgataagacgtagaaataaatagatcgttacgtaaaacatctgcaggaagtgtattgatttgtaaacgttaaaatacttctctctgaccatttattatatgtcagtcgttataagagaaaacaaaacgcacatgttatattgacatgtggacgataatgtatattgacatgtgaagaagccaactccgtacgtaaagcgccatttgcgctgcaaatactgatcctcaactacagtggattcttttctcacaaaaacatagaccgtttcaaatatatgttcccaaacacttgtgagacattctatacaaagtttatcatgcacccttcctttttttttaacgtcaaaatgatcatgtacttctgtcacattatttttgtacattatgaatatatagacatttgtattctctctttcgccgaatacacacatctatatatttgtaaatgtagcaggtttaaattttggagtaaaagaatagttgattttgaccacatagagaactaatggatcaattctcactaatacaaatatttggtgaaagccttagaggtgagaaagtccaaggcccataaaggcctattacggccacccccggtcacgtaaaaccaagcctcgttctcgttgatgaggccgaatataaaaggcatcatcaaatcaaacatgtgcgtaacgtgatatttaatttagcatttgcaagtaatgatcacttctgttttttcttttagtatttagttcttcacttaagttttccacgttatttattaatatacaggaactgctttttcttattttattggaaaaatcatgttttatgtttgttcaattaaaatttcagcacaatttctttttcatttttttatatgaaaactttaaggtagaaatgggaaattgcgaaaccgaatcatgcggacaaaacgaaatttctgcgttgcctatattttttgttggtaatttttaaaacaataaacaattaatttgacgtgataaaaacaaagggacatgaaaaaactctaaaagcgtagtaatggtaatttggtaatttcaaagtccgctggttctccgtaactgtctcaaattaaaaagagggcttactgttttctgacgctcgttagattccctctctttcttcttcattttctcctcttcgtcttcactgctaattcccttgatctctctccctgtcctccaattttccctctctacaaatatcgactccttcttcaatattagattgatcctgatccgattcgagccggtacgtacctgaactgtttctgtttctctgagctaattcgtgaatgtacgaggttctgctgcgttttattttttttgatggtatagttgacatgttttcaggattttttgttgtatactctgatctttgatgcttgtttatcgttttgccattggatctgctgctcgatctgggcaatttctcgcatttgattgctacatttgtcataacttcgggatctggatctaccttttttttctgatcatttagaatttcgctaacagctttagattttcgtacttatcgcgtggatttggcttcccgctacttgttcagctgtatctgttaaaatctcacaaatttttattgaactgaatcatggggttttcaataggatagatctggttgagttgttctcctcagtagctgtttccttccacatttgagcttaatcgatttcatggagtaatacgggtgatcgtgatttcgttaatcacatctgatccgatgacgttcatgatatatatactagccattatttacctgtttgctggatcttttgtccttcgattaaatctggctgtttcgtcattgacgagtgtactgaaagcttttccgaatgcaaatataatgttttgtgttgttgcagattatatatttatcatcacatggctacatataagcccaagaacatcctcatcactggggctgctggattcatagcgtcccatgtcgccaacaggcttgttcgaagctaccctgactacaaaatcgttgtgcttgacaagcttgattactgctcaaacctgaaaaacctcaatccttcgaaatcctctccaaacttcaagtttgtcaagggagacatcgccagtgctgacctcgtcaactaccttctcatcactgaaaacatcgacacgattatgcactttgctgctcagacccatgtcgacaattccttcggtaacagcttcgagtttaccaagaacaatatttacggcacccatgtccttctggaagcttgcaaagtcactgggcagatcaggaggttcatccatgtgagtaccgatgaggtctatggagagactgatgaggatgcttcagtgggaaaccatgaggcttctcagttgctccctacaaacccttactctgccactaaagctggagctgagatgcttgtgatggcatacggtagatcatacgggttgccagttataacgactcgcgggaacaatgtctatggtccgaatcagtttcctgaaaagttgatccctaagttcattctgttggctatgagtgggaagccactgccgatccacggagatggatctaacgtgaggagttacctctactgcgaagatgttgctgaggcgtttgaggttgttctacacaaaggggaagtcaaccatgtctacaatatagggacaacgagagaaaggagagtgattgatgttgccaacgacatctcaaaactctttggaatagaccctgactccaccattcagtttgttgagaaccggccttttaatgaccagaggtacttcctcgatgaccagaagctgaagaagttgggatggtctgaacgaaccacttgggaagaaggactgaaaaagacaatggattggtacactgcgaaccctgagtggtggggagatgtctccggagctctgctgcctcatccacggatgttgatgatgcctggtgatagactctctgatggctctgacgagcgcaaggatgcagacggtaatcagacattcacggtggttactcccaccaaggccggtggttccgcagacaaaacatccttaaagttcctcatctatggcaaaactgggtggctcggtggtctcctaggaaagatatgtgagaagcaagggattccgtacgagtatggaaaagggagactagaagacagagcttcaatcatggcggatattcgcagcgtcaaacctacccatgtcttcaatgccgcgggcttaacaggcaggcctaatgttgactggtgtgagtctcacaaaaccgagactatccgagtcaacgtcgctggtactttgactctggcagatgtttgcagagagaatgatctgttgatgatgaactttgccaccggttgtatatttgagtatgacgctgcacatccagaaggttcagggattggcttcaaggaagaagacaaaccgaatttcaccggttccttctactcaaagacaaaggcaatggtaatatactactacatcacataaccaaatcacatgtgatcctcaaactgtgcaactctgttcataaatcctctgtttctattttcgccaggtcgaagagcttctaagagagtttgacaacgtatgcaccttgagagtgaggatgccaatctcatccgacttgaacaacccgcgaaacttcatcacaaagatctcgcgttacaacaaagtggtgaacatcccaaacagcatgaccatactcgacgagctcttaccaatctcaatcgagatggcgaagaggaacctacgggggatttggaatttcaccaacccaggagtggtgagtcacaacgagatactagagatgtacaagagctacatcgagccaggtttcaaatggtccaacttcactttagaggaacaggctaaggtcattgtcgcaccacggagcaacaacgagatggatggttttaagctcagcaaggagtttccagagatgctttccatcaaagattcgttgatcaaatacgtcttcgaacccaacaagagaacgtaataccctcagtaacacatacacacacacacacttcctctttatctgttcattgttatattattatcttgcaggtagtttcaccactataatgattctactataattttattttgtcatatgattcatttactctttttttggctttctacgtcgaacatgtagctctcttgacgcattctacgtcacaacacattttgttttcattaatattatttattaaacgataaaattgcttgaagtttattactttcactattgattcctccttttagttttcatctcaaaagagcagaggacagagattaagaacgaaacagcattgactgataacttatttccctatgcttttaaacttgaggtttctatttgttacaaaacaatgtctttcataaagttaaatctttctattgcataaatcgaaactgcaaactcaaaatgtaatataaattaaaccttctgtacttcctgtccccaaatcttcaccatacgaccatctaaaagcagaatttttcacactacgaacaacattccataatctgatcatccttgcaacaaagcataccgattcgtaagccttcaatttgaatgaagacgtaaaatgatgaataaaaggtaagagagaggaacagaaaaagctcagcaccttgaaatttgttgttctcttcacatagcttgagcgtattgttgtctagacaatggtggaatttcttgtcccgtcataaaatttaaagtcaaaagtcagtagtagttggtgattgattggctcctgagttcttacaaaggaggagaacacttaaaaaacagagtatgagaatataccttctgcctctgtagacaaccaatcatgtgcacagaacagagcctgtctaatatcagggctcaaggaactctggctatcatcgatcaccggtctcccggagttgaacgttgaatcaggcgcaaggatcgacatcggcgtccccaagatatcgcgtgccatcatagagaggatagggtatctcggcgtatggaccttccagtaattcagaatgttgaactcgccactacgaggaaagattggttcagacaagtacttgtccaagtccgatgttgtgttctggctctgagatgtctcgtggagaaacttgtcgaatcctttcaacctgtctctagtgtccatacctgctctacctaagccagagccagagtaggaagagtcgtccccaacaatggctgagcatatc

SEQ ID NO: 24 - DNA, 1092 bp, Thlaspi arvense
  source 1..1092: mol_type = other DNA
atgggtagacattcttgctgttacaaacaaaagctgaggaaagggctttggtctcctgaagaagacgagaagcttctcaatcacatcacaaatcacggccatggctgctggagctctgtccctaaactcgctggtttgcagagatgcggaaagagttgcagactgagatggatcaattacttgagacctgatttaaagagaggagctttctctccagaggaagaaaatctcatcgtcgagcttcacgctgtcctcggaaacagatggtcacagattgcagcaaggcttccgggaagaaccgataacgagatcaagaatctgtggaattcaagtatcaagaagaaactgaaacaaagaggcattgatccaaacacacacaaacccatctctgaagttgagggctttagcgacaaagacaaaccagcaacaagcgacaataaaagaagcagcaacgatcataagtctccgagttcctcctctgcaaccaaccaagacttcttcctagaaaggccatctgatttctccgactacttcggttttcagaagcttaacttcaactccaacctcggactctctgctgcaactgattcttcactctgctccatcattccggcgcagtttagccccggaaacatgtctggttctgtcttccagactccggtatgcgtaaagccttcaattagtcttcctccggacaacagttcgagcaccgtctccggaggagatcatgtgaaactggctgcacctaattgggaatttcagacaaacaacgcctccagtttcttcgacaatggcggattctcatggtcaatcccaaattcttcttcttcactagtcaaacccaatcataacttcgaagaaatgaaatggtcagagtatttgaacacaccgttcttcaatgggagcactgtacagagtcaaagctcacaaccgatctacatcaaatcagaggcagattacttagccaatgtttcgaacatgacagatccttggagccaaacccagaacgagaatttgggcacaaatgaagctactgacgtgttctccaaggatcttcagagaatggccgtctcctttggtcagtccctttag

SEQ ID NO: 25 - protein, 363 aa, Thlaspi arvense
MGRHSCCYKQKLRKGLWSPEEDEKLLNHITNHGHGCWSSVPKLAGLQRCGKSCRLRWINYLRPDLKRGAFSPEEENLIVELHAVLGNRWSQIAARLPGRTDNEIKNLWNSSIKKKLKQRGIDPNTHKPISEVEGFSDKDKPATSDNKRSSNDHKSPSSSSATNQDFFLERPSDFSDYFGFQKLNFNSNLGLSAATDSSLCSIIPAQFSPGNMSGSVFQTPVCVKPSISLPPDNSSSTVSGGDHVKLAAPNWEFQTNNASSFFDNGGFSWSIPNSSSSLVKPNHNFEEMKWSEYLNTPFFNGSTVQSQSSQPIYIKSEADYLANVSNMTDPWSQTQNENLGTNEATDVFSKDLQRMAVSFGQSL

SEQ ID NO: 26 - DNA, 4198 bp, Thlaspi arvense
  source 1..4198: mol_type = genomic DNA
aaaataattaattctaacttatgacttaaaaaccttgtatacgtctagctaaatcttattttcgacgatcttttttaggattgggtcccaataaacaaatggataaacggtaagagtctaattacgagaggccatgtccagataacgtaagaaaactacaaaaattcaacatgtgaatatttgagggaaagtttgggtaaatggacaaagaatataccctctctattatgactggcttaaaggcaaaaaaagggagaaaattgccaaagagaagtgagtccatttaaatttaaaaatgtataaagcaaacaaaagagagacttaattattctcattcatctgcaaaagaaaccatgtatttaaagcaaaatttctaaattccgttatgtagacatttaattccatttaatcatttctggaaacattaaccaatgatgacaatttcttgctggttataaacctttcccattatttcctttaattgatgcgttcatcttcacaaagatttagtccacatttagcatttgcttttaattcattgcagaagtctttcatgacgacaacaatcaactcttctttgtccacattcttatctagctatacgatctacctcgtgtgttattttaattcttccgttctcactgtaaatcatttttgtatagcgcttccaccgctaactattgaatatcacttttcaatacattaatcgttacaataagtttgtagctgcaagaaaaaatttagactcggatgcatttggtaacatagatatcatataaaacttttaaactttttctcgtcatgcatcactcaaagagtgctatatccttgtcacataccaaaaacgttttaggagcacgcattgcttcaaactctcgtctatgtgcgatttcgatacatttttctaattactctcaagtctcaactaagcacacttaattatggatttcttttttaaaaatagcctatttctcgatttacaccactgtaaatatatttccataaattctatatcgaaccatatactacatgagtatttttaagtgaaaactaattattttgtgacataaaaaacctgatatacgtctaccaaaaaaggttttttttgtaaaccatgacttacgtgaatctccgaaataaaaatctttagaaaagttgttgaggtcacgctggcttttggctgcgtacgtatagagtggtccgtaacatcttcgaggacaaactgaacataaatgagcatgtctccactacttagaaccacacttactattaattttaaaagaagtttttttttttttttatcaattgttgcatttgtatgtatgatcataatgggtccatttggagatgacgaatgtatgatgattagagtgatgtaaaggtcaaaactacatgaactccatctcttaaccctgattattttaccattggtgtgaaccaatctgatgtggaccaatcatattgtttttacaaaagctaaaaaagatgtacatactttttgctatttaatctttaaagagagtatagaatttcaacaaacccttccgaagaaagtgacttttcttagtcctattaatactctctctctctctggagatctgttatttcgttttctccacctttctcttcagattccattaaccttcaaaagttttaaatacatgctctctgctcaaagcgtttttctttcgttacttgtaaagtaaaacacagagctctcttctctttcatcgttcctttgctcagcattgcagctttaataaaccaaaatgggtagacattcttgctgttacaaacaaaagctgaggaaagggctttggtctcctgaagaagacgagaagcttctcaatcacatcacaaatcacggccatggctgctggagctctgtccctaaactcgctggtaacattttcttccttaattcatgggatacaaaacatgaacttaaaaaggctaccttttttgtaataacaattcacaaatctgagtctactacaggtttgcagagatgcggaaagagttgcagactgagatggatcaattacttgagacctgatttaaagagaggagctttctctccagaggaagaaaatctcatcgtcgagcttcacgctgtcctcggaaacaggtaataattcatagaaaacagaggatcatgtttgtgtcttaagcttcctctgtttttaacagaggatcatgtatatcttttaaccttcctctgtttttttatcagatggtcacagattgcagcaaggcttccgggaagaaccgataacgagatcaagaatctgtggaattcaagtatcaagaagaaactgaaacaaagaggcattgatccaaacacacacaaacccatctctgaagttgagggctttagcgacaaagacaaaccagcaacaagcgacaataaaagaagcagcaacgatcataagtctccgagttcctcctctgcaaccaaccaagacttcttcctagaaaggccatctgatttctccgactacttcggttttcagaagcttaacttcaactccaacctcggactctctgctgcaactgattcttcactctgctccatcattccggcgcagtttagccccggaaacatgtctggttctgtcttccagactccggtatgcgtaaagccttcaattagtcttcctccggacaacagttcgagcaccgtctccggaggagatcatgtgaaactggctgcacctaattgggaatttcagacaaacaacgcctccagtttcttcgacaatggcggattctcatggtcaatcccaaattcttcttcttcactagtcaaacccaatcataacttcgaagaaatgaaatggtcagagtatttgaacacaccgttcttcaatgggagcactgtacagagtcaaagctcacaaccgatctacatcaaatcagaggcagattacttagccaatgtttcgaacatgacagatccttggagccaaacccagaacgagaatttgggcacaaatgaagctactgacgtgttctccaaggatcttcagagaatggccgtctcctttggtcagtccctttagctttttttttttcttcttttctttattctaacagatgtagagaacaaaaaaatatacaatacatacatacgtacagtggatttaagtctgtatattccatgagctgtctttatttttacattttttaagtgtgttttatacgtcaaatattcttctattttttgcaaacctttcagtctcatactatatatacacttttatttcttttgttttgttataaagattatgatgcatagaattctcgatgatttcagaggcctgtgtttgcaattaatctgttgaagaacaatgatgaaagtaataaatcagtttctgtctgtttccgtgaacgagttgtaatccagagtcacatccttcaccatttttcagacctgtaatgaattaaaagacaaaaaaggacaaaaacataaaactaaagcaaatcataataaataaactaaagtgggaattagctcaactaataagaagggacacttttttcgaaaggacccgagttttaatacgatgtaaattttttaaaaaaaaagatttctcttttctgaaatcaatgactgatcacatatttgagagattagaaatcgaatacccctaatttcttcgggctattataaactttgaaaaaggtacgtatgtcgtttttgcttagtcttatcagagaactggaattgtccccattgacggcgtcggaatattctttagcggtagaaaattcggaacagttcgagaattttctatttttttgtctgttaaataaaatagttatatgatttgaccttaataaacatgaaggaggtgatgactgatgagaaggtgacttcatttttaatcctaaaaagtcaattgatttattttataacccatatttttttttttagattctaatccaaaacaattacttattacttttttagaaataacctaacgcaataactcgactgataggtaaaactaaggtactataatatgtttgttttgactttaaatttaaagacgatgctatatttttttgaaaatgaaaagaaattgatctatcaaacacataagtctagattcaacagtaattataaaaatagaataaagagagaaaagttaatattttcttggcattatgagaaatcaaatatatttaacctata

SEQ ID NO: 27 - DNA, 939 bp, Thlaspi arvense
  source 1..939: mol_type = other DNA
atgttctcatcactctccaaccacaattcaccacaatcaatggagtcaccacaatacgagatctcttcaagctcttcttctgaaaaacctagatactactttcaatcatctgatatattccccaacctcactcaaaaccctagtaacagcaatacccaaatcgagtcgttaccgcttatcgatgggataaatttaaactcaaaccttaacctaaaccttaagccaccgtatgttgaaaaagaagaggaagagaaagaagaggaggaagatcacgttgatctgagcttatacatcggccttcctagctctgataattcgagaaacggtgttaaactgccgaagaagaaaaatgggaaggacatcatcactcatgacgctggaaaacagatggagaatgaactttccggcaaagcatactggattccggcggtggagcaaattataataggcttcactcatttttcttgccatgtatgcttcaagacattcaatcgctacaacaatcttcagatgcacatgtggggccacggttcacaatacaggaaaggaccagagtcacttaaagggacgcagccacgagcaatgctagggatcccttgttactgctgcgtcgaagggtgtaggaaccacattgaccatcctcgatccaagccgcttaaagacttccgaacgctccaaacacactacaaacgcaaacacggccaaaagccctatgcgtgtcgcatctgcggtaagctgttggctgtcaaaggcgattggcgcacacacgagaagaattgtgggaaacgctgggtttgcgtttgcggttctgactttaaacacaaacgctcccttaaggaccatgttaaggcttttgggcctggtcatgggtcttatctaaccggtttgcttgacgagcaggcctctcattcttctctctctgagaatttgttcttttaa

SEQ ID NO: 28 - protein, 312 aa, Thlaspi arvense
MFSSLSNHNSPQSMESPQYEISSSSSSEKPRYYFQSSDIFPNLTQNPSNSNTQIESLPLIDGINLNSNLNLNLKPPYVEKEEEEKEEEEDHVDLSLYIGLPSSDNSRNGVKLPKKKNGKDIITHDAGKQMENELSGKAYWIPAVEQIIIGFTHFSCHVCFKTFNRYNNLQMHMWGHGSQYRKGPESLKGTQPRAMLGIPCYCCVEGCRNHIDHPRSKPLKDFRTLQTHYKRKHGQKPYACRICGKLLAVKGDWRTHEKNCGKRWVCVCGSDFKHKRSLKDHVKAFGPGHGSYLTGLLDEQASHSSLSENLFF

SEQ ID NO: 29 - DNA, 4025 bp, Thlaspi arvense
  source 1..4025: mol_type = genomic DNA
ttattgtttatcaccagtttggttgtcattaattaataagtaagatttgtgtttagtgacggctgattccgtttctagtgagtcagatgcgagatgattgaaaaccgagaagacgatgactccacaaaataagattttgtttaagttttataattgagttttagcgaaattcgttttcaatttttttttttagctttattttttttattgagaatttaagaattataaaagttttttaggtaaaatttgaagaaattttgattaataaattatttaatgaaatagctttaaattattggttgtagaagatgacataacagttttgaactctactattgattaattatttttgctgatgtggcatattgttttattcttattagttagttttttcataatttaatgatgtggtaatttgttatattcttattaactgattattttgatgattatttttgcttatgtgacaccttttagagagcaggaaatctatccttttatataaaggagattagattttaccgatcatgtattatttagtagccaattccatacgtaaaaaaaaagatttttacaatttggttataaatagcctgcatgttttatcggtcctatcttgattgtatatcgtaaaaaaagatgctgactctaagaaaacgaatttcatatggaccgtagtaacagggcccacgagtaattagggttttaacggctgacattttgatctctcatacatctaagtatctaactagaagtgttgaccgttagagaagaattaaataacttacatacatacaaaaacataagtcgaagaataatcataacagtgcatcttctacaataatgataacaaaaaaagtaaattagaaattagcatttattccaattaatacccatattcgaaaatgcacatggtagaaaagcaaaaaaagcttacgtaaattccaaatattgtcaaacccctgcaatgacaaagttgccaaaaattgaagaggttggtccacacaatttaaggttctttgcttcacactctatttataggcaaagagatgaaacagaggagattaaattgcttcttaacaaaggttgttttcactcaaccacatgccttctcaagtgtctgctgctcacattccccgagattctcatttactttttcctctatttggtacgtactttatattacaattctatttgtttctttgattattcgttttgttcatacttagttatcataaacatacatagttgatcttatattatacagtaaatttgataaatgtttctcttaattaatttactcacgcaatttaaaggagacgattgatacgcgggcctacttacgcacctgcatgattattagttataaaagttattgcaaacattaaattactttgatagctagagagcaattattatataaagctaatttttaattgtagatatacatttagtcgaaagttaaaaagaaaaatgaaatccctaaacaaacgttcccaaatgttctcatcactctccaaccacaattcaccacaatcaatggagtcaccacaatacgagatctcttcaagctcttcttctgaaaaacctagatactactttcaatcatctgatatattccccaacctcactcaaaaccctagtaacagcaatacccaaatcgagtcgttaccgcttatcgatgggataaatttaaactcaaaccttaacctaaaccttaagccaccgtatgttgaaaaagaagaggaagagaaagaagaggaggaagatcacgttgatctgagcttatacatcggccttcctagctctgataattcgagaaacggtgttaaactgccgaagaagaaaaatgggaaggacatcatcactcatgacgctggaaaacagatggagaatgaactttccggcaaagcatactggattccggcggtggagcaaattataataggcttcactcatttttcttgccatgtatgcttcaagacattcaatcgctacaacaatcttcaggtacaaaccaatgttatctcatgcgcattacgtgcatgcataaccaaataaaatcttaattcatatttgaatttgtttgttagagaacaaacggagaaaatcctattcgatttatatgtttataacccccttatctaatgttatgagttagaatgaatttatacatacataatcaaaccctaagttgactaactatatattattttgtagaataattgttaatatagatctgtttggatgcatggttgagatttaattaaaatatactgttaaataaacccaaatttaaaatgaatttaatagtttttctccatataattaattaacgtttcctttaaaatttcatccaaattaataattaatagattacttcagtgaaacaatatgatcgatcaacaataagattgtaatgattaatgaaccattttattagttgttaaacttatatttgattaaaaaaaggtggggggtatttgttatgaaaatttatcttgaaatcgtcagtctaaccattgttatccatttcattttttgttattacatatactgatatacaaatctttgttgacaccaaatatgaattcagatgcacatgtggggccacggttcacaatacaggaaaggaccagagtcacttaaagggacgcagccacgagcaatgctagggatcccttgttactgctgcgtcgaagggtgtaggaaccacattgaccatcctcgatccaagccgcttaaagacttccgaacgctccaaacacactacaaacgcaaacacggccaaaagccctatgcgtgtcgcatctgcggtaagctgttggctgtcaaaggcgattggcgcacacacgagaagaattgtgggaaacgctgggtttgcgtttgcggttctgactttaaacacaaacgctcccttaaggaccatgttaaggcttttgggcctggtcatgggtcttatctaaccggtttgcttgacgagcaggcctctcattcttctctctctgagaatttgttcttttaaaactttgtgcatctatcagtcttttgacgtgtgttgtccgtttatttagtctagaataatgtggtatctaataattctcgtagtgaataatatcataatctacttgatatgagaggtcaacatatttagtcccgcagttaataatatcataatttggtgcaccaactaagggaaatgactatcagccacacttagggattactcattaatcgtagactcataaaagctatatgtttaaaaatgctagtttgtatacatatcattagccacacttagggattacgcataaaccgtagactcataaaatctatatgtttaaaaatgttagtttgtataaaaggagatatatatgaaatgagtaaggaagtcacattcaagagcaagtgtagtgtgctttccgagaaatttcctccacatgtccagacggtacgaaatgccagttaattccaattctatcattattgatctgaatgtgatcgcaaaacatgatttgattagtttcctctctttataatttactaaaataaaatgacgaccatataacatcatttttcagaaggaaattaaaacatatcaagaatattcatgtaaaatagttaaaatatcagttaaaaatgttaccattctatacatattatattttatatacatggactgaattcgacaatattggtaaatatcaataaatccaaaatcctgattatttgtaaatcaataaaatagtattatgatacaaaccaattcatatacggtgattcgaaatttcagtacatcatgaacatggaacaatggattttatgaactgatgagttgtccaacgttcgttacgtgcatgcattcaatgcctcggtgccacattactcaccttttatgtatcctctctccattgtttttttttttttatctaacttattgggtatccaaattcatttttgatccttattttagtgaaaccatgcatgtcctacgtactatcgctcgtcatatttaaaggaacagg

SEQ ID NO: 30 - DNA, 966 bp, Thlaspi arvense
  source 1..966: mol_type = other DNA
atgttctcatcactctccaaccacgattcaccacattcaatggagtcaccagactcaccacaatatgagatctcttcatgctcttcttctgaaaaacctagatactactttcaatcccttgatctcttccccaacctcactcaaaacgcttgtaacaacaataacctaatcgagcctttaccacttatcgatcggatagactcaagctcaaaccttaaccttaaccgtaagccaaaggcattgtatgttgaggaaggagaggaagaggaagaacaggaggaagaggacgtggatgtgagcttacgcatcggccttcctggctctgataatttgagcaacggtgctaaattttcgaagaaaaatgggaaggagatcatcactcacgatgccggaaaacaatcagagaatgaactttccggcaaggcatactggattccagcagtggagcaaattataataggcttcactcatttttcttgtcacgtctgtttcaagacattcaaccgctacaacaatcttcagatgcacatgtggggccacggttcacagtacaggaaaggaccagattcacttaaagggacgcagccacgagccatgctagggatcccttgttactgctgcgtcgaaggctgtaagaaccacattgaccatcctcgctccaagccgctcaaagactttcgaacgctccaaacgcactacaaacgcaaacacggccaaaagccctatgcgtgtcgcatctgcggtaagcttttggctgtcaaaggtgattggcgtacgcatgagaagaattgcgggaaacggtgggtttgcgtttgcggttccgattttaaacacaaacgctccctgaaggatcacgttaaagcttttgggcctggtcatgggtcttatccgaccggtttgtttgatgagcaggcctctaattcttctgtctttgaaagtttgttctgtgtgatcggtgagtattag

SEQ ID NO: 31 - protein, 321 aa, Thlaspi arvense
MFSSLSNHDSPHSMESPDSPQYEISSCSSSEKPRYYFQSLDLFPNLTQNACNNNNLIEPLPLIDRIDSSSNLNLNRKPKALYVEEGEEEEEQEEEDVDVSLRIGLPGSDNLSNGAKFSKKNGKEIITHDAGKQSENELSGKAYWIPAVEQIIIGFTHFSCHVCFKTFNRYNNLQMHMWGHGSQYRKGPDSLKGTQPRAMLGIPCYCCVEGCKNHIDHPRSKPLKDFRTLQTHYKRKHGQKPYACRICGKLLAVKGDWRTHEKNCGKRWVCVCGSDFKHKRSLKDHVKAFGPGHGSYPTGLFDEQASNSSVFESLFCVIGEY

SEQ ID NO: 32 - DNA, 3923 bp, Thlaspi arvense
  source 1..3923: mol_type = genomic DNA
cacgaaacaagttcaattaaatttaacggaaataaatggtaattaatgaaagtttgaattgtattaattactgcttccacgaaacaaccaaaaaaatcatttgacaaagtaatttgtgtacggtattagccacatggggccaatcctctatgtatatcggagttgttttgccaaatgcccaattcttactctagtaaatattaaaccattttgtagatcctaatcttgagtcaactcaaagtcctatgtttggaaactaaaaataagtttaaatcctctagactacgactaagttgtaaaaagaaatgttcaaaattccttagacattgaaattgaatacttcaattaaagaaaattttaccagcatgttcatagtagtagaccaccacagaacaaaattaatagtttttacattgcattcttatataataattttggagtataattgtaattataaacaaaataactaaaagaaaaggaaagtattcttgacatatttataggtactaatttgctagtacgactattaattatggagattaaatctagtatttgactaaccagaaacattttaaaggtaagtgataagttgataacctcgcaattatttttgaaagctattaatcactttagcagaatgtatacaagttctatattaacaagtttatctcaaaatcttgagatcctactaataaatcataacttttctcttattggtatgtcgaatctagtgtttaccaaactagaggtgttgaccgttagagacaattaaacaacttacatacatacaaaagtacaagccgaagaataatagtaataacagtgcattttctacaataattaaaacaaaaaagtatattaaaaattagcatttattccaattaataccaatattcgaaaattaatatggtagaaaagcaaaaagcttacgtaaattccacagattgtcaaaaccctgcaatgaaaaagttgccaaaaattgacgaggttggtccacaaaatttaaggttctttgcttcacactctatttataggcgaagagatgaaacagaggaaattaattactccttaacaaaggttgttttcactcaaccacatgccttctcaagtgtctgctgctcacattccccgagattctcatttacttactcctctatttggtacgtcctttatattacaattctagtattttttttttcattattcgttttgttcatacttcgtttcataaacatatatagttaatcttatattatacagtaactttgataaatatgtatcttaatttactcacgcagtttagagagacgattgatacgtggggactacttacgtacctgcatgattatataagttataaaagttattgcagaacattaaattactttgatagctcgagagcaatcattatataaagctatatttttaatcacaaatatacatctactcgaaagttttttttttaaaaaaaagatgaaatccctaaacaaacgttcccaaatgttctcatcactctccaaccacgattcaccacattcaatggagtcaccagactcaccacaatatgagatctcttcatgctcttcttctgaaaaacctagatactactttcaatcccttgatctcttccccaacctcactcaaaacgcttgtaacaacaataacctaatcgagcctttaccacttatcgatcggatagactcaagctcaaaccttaaccttaaccgtaagccaaaggcattgtatgttgaggaaggagaggaagaggaagaacaggaggaagaggacgtggatgtgagcttacgcatcggccttcctggctctgataatttgagcaacggtgctaaattttcgaagaaaaatgggaaggagatcatcactcacgatgccggaaaacaatcagagaatgaactttccggcaaggcatactggattccagcagtggagcaaattataataggcttcactcatttttcttgtcacgtctgtttcaagacattcaaccgctacaacaatcttcaggtaccaatgttatctcaaccaaattaaaaccagaattcaaattcgtttttttgtttctttatttaataaaaatagactttaatatatatatgtttggatgcatggtaaagaaaatatttattgaatagaccatggtttaaattcaaattacaagtttgattggctatcgttttaatagtttttcctcttataattaactcttcctttaatagttattcaaagagatttcaaccaaattaatacacagatttcttcaatgaaacagtatgatcgatctctaacaagattgtaatgattgatgaaccatgttattattagttaaaataaaattggagtcaaagatatgtgtatttgctgtgaacatttatcttgaatacggcagtcaaaccattttttatcaatttcattttttgtttttacgtatgcaaatctttgttgactccaaatatgaatgcagatgcacatgtggggccacggttcacagtacaggaaaggaccagattcacttaaagggacgcagccacgagccatgctagggatcccttgttactgctgcgtcgaaggctgtaagaaccacattgaccatcctcgctccaagccgctcaaagactttcgaacgctccaaacgcactacaaacgcaaacacggccaaaagccctatgcgtgtcgcatctgcggtaagcttttggctgtcaaaggtgattggcgtacgcatgagaagaattgcgggaaacggtgggtttgcgtttgcggttccgattttaaacacaaacgctccctgaaggatcacgttaaagcttttgggcctggtcatgggtcttatccgaccggtttgtttgatgagcaggcctctaattcttctgtctttgaaagtttgttctgtgtgatcggtgagtattagagtaactgagaggaatgtaactgagagaaaaaagaaaagtaataattaaaataattgaaaataataagtaagagcatctagatagtccttaccaaaaaaaagatcatctagatagtctttccatagtatctgatttatataatactaatataatgtatttatataattaaattataaattaataaagagatgaaccaattcttaacagacatttgcctagagacatatctttattcttaacaaacatttggctagaaacatatctaatagtttcttgtttcaaaaatgtcttcgctttttttctgtttttctcccttcctttttccttattttttttatttttcttattcactaaatatactcccataatatctgctatataatattaatataatatatttatataattaaattaaaaattcataaagagatgaaccaattcttaatagatatttggctaaatacatatttaatatttttttgtttgaaagatatctttgctatttttttctgtttccttctcttcttttcttcttatatttcttattttttttattcaataaatatattttaaaaaacaccaattttcttataagaatatctgaaaataattgagaataattaaattaaatattttcttttagtaaaacttataattatatatatgctaaaaagatatgtgatatttattattctatctttaaagatttttttatcgtgaatcactattttcagttatccaacctaaaatgaatactcagagagcaaccacatcgaaagtgttagagattgaatgaatacagttcttaaaaggtttatttcacattaatgaagtctatcaaaacaaaatttatctaattacatctctataacaaaaatgataattctaaagttaaatgaaaaaaaaaaacaaaaaaatagagagaatttttctttaaaaaaaagataagaaagatcaataaaaccgacttcctcacattataaatagaaaagtcttcat

SEQ ID NO: 33 - DNA, 1707 bp, Thlaspi arvense
  source 1..1707: mol_type = other DNA
atgtcacaatattccttcttctatttcttcctaatctctcttttcctctacgaaaattgcattgcgtatcgctacacattcacggttattgaagctccatatagcaaactgtgtagcacgaagaagattttgaccgttaatggtcagtttcctggaccagtgttaagggcttacaaaggtgacaccatttacgttaacgttcgtaaccaagctagtgaaaatatcacattgcattggcatggtgtagagcagccgagaaacccgtggtcagatggacccgaatacatcacacaatgcccgattcaacccgggtcagattttacgtacaaaattttactttccatcgaagacgcgactgtttggtggcatgcgcatagctcgtggacacgtgccaccgtacacggtctgattttcgtgtatcctcggcctcctgataccctgccttttccagaaccggactacgaagtccccttagtttttggagagtggtggaagagggatgtgagagaagtagtggaggatttcatgaggaacggaggtgaacctaatgtgtccgatgctttgactatcaatgggcatcctggtttcttgtatccttgctctcaatcagatacattcaagctcgtggtagagaagggcaaaacctaccgcattcggatggtaaacgccgcgatgaacctaattctcttcttcgccatcgcgaaccacaaactcaccgtggtcgccgccgatggccactacaccaaacctctaaccgctagttatatcaccatatctcctggccaaacgctagacctgttactatacgccgaccaaagtccagagagcacttataacatggcggccagagcttaccatagcaaccccaacgttgggttcaacaactctaccaccgtcgggatcttacgttactactcttcaaacgacgccggaacgtcttcatcagaacgttacccgtaccttcctggctacaatgacacctcagcagctttcgatttcttcacaaaaatcaaaggcttatactccagagtagctcccgccaaagtttcacgtaggataatcacgacggtttcgataaatctcctcaagtgtcccaacgactcgtgtgcaggcccaaacgggtcgaggttagcggcgagtatgaacaacatatcgttcgtcacaccgagccacgtggacatactaagagcttattaccttcacattaacggcgtttacggaacgcggtttccggagttcccaccgcggatattcaatttcacagcggacgaccaaccgctgtttttgcagactccgaggctggcgacggaggtaaagaagtttcagtacggggagacggttgagattgttatacaagggacgagtttggtaggtggtggaatcgatcatcctatgcatctccatggttttagcttctacgtggttggtttagggtttgggaattttaacgcacgtaaagatccctccaactataatctagacgatcctccttacagaaacacggcgactgtgcccaggaacggttggatcgctatcagattcgtagctgacaatccaggggtttggttcatgcactgtcactttgatagacatcaaacgtggggtatgaatgttgtcttcattgttaagaatggaataaaaccaaatcagaagattctacctccaccgcctggcttaccaccttgtgaccaatttgagaatctataa

SEQ ID NO: 34 - protein, 568 aa, Thlaspi arvense
MSQYSFFYFFLISLFLYENCIAYRYTFTVIEAPYSKLCSTKKILTVNGQFPGPVLRAYKGDTIYVNVRNQASENITLHWHGVEQPRNPWSDGPEYITQCPIQPGSDFTYKILLSIEDATVWWHAHSSWTRATVHGLIFVYPRPPDTLPFPEPDYEVPLVFGEWWKRDVREVVEDFMRNGGEPNVSDALTINGHPGFLYPCSQSDTFKLVVEKGKTYRIRMVNAAMNLILFFAIANHKLTVVAADGHYTKPLTASYITISPGQTLDLLLYADQSPESTYNMAARAYHSNPNVGFNNSTTVGILRYYSSNDAGTSSSERYPYLPGYNDTSAAFDFFTKIKGLYSRVAPAKVSRRIITTVSINLLKCPNDSCAGPNGSRLAASMNNISFVTPSHVDILRAYYLHINGVYGTRFPEFPPRIFNFTADDQPLFLQTPRLATEVKKFQYGETVEIVIQGTSLVGGGIDHPMHLHGFSFYVVGLGFGNFNARKDPSNYNLDDPPYRNTATVPRNGWIAIRFVADNPGVWFMHCHFDRHQTWGMNVVFIVKNGIKPNQKILPPPPGLPPCDQFENL

SEQ ID NO: 35 - DNA, 5054 bp, Thlaspi arvense
  source 1..5054: mol_type = genomic DNA
catgcacgtaagaaactaaatcaacacataaggtaacgaggctcggaatagttgggtttcggatttttatttttaaaaagaaagcatcacctaaccaaaactcataagggcatctccatattaaaaaatacaaattaatagaatggaaaaagaaagatagagacgtatctcgtttgaactttgaaatatgtttagcaacgtatctaattaagtgtcatattctgattagtttatattatttttagatactctatttaagatatgcaccgttaaaggtgttctaaagcatcttcatttactctgatagtatatccaaaacttattataataatataatttatttgtgtaataaaatattaaattattaaaagtgtgatgcatatattaaaaatgacagatattgagaaacatatctcatgtcatgctcttttctttgaaaaacagttcgtaatttctctcattctctctctttctttctaattaatttttttattatccagatattctctgaaataccgttgttgcaaatacttttagaacacctttaacagtgtataatctcaaatagaatatctaagatttttttttattaatataaaaaaattaaactaactaatacttgacacttggtcagatacatttctagataggattctctatctctctccatcctttccattattttgtacattttaattattataaattggtcatatatgactttcagatattattctcgaattttccatcacttaccaacatttgttaaaataattttccgtttaaaatagtttaatagtatatattaacaggttacaggtatgaaaatgactttagtatgagatagggagtcgagagtttttaaaatattcgaatactttagacttctcaaattacccatttaaaaatattcaataacttagacttctcgcattacccaaaataccaaatttgtctgaaaccaagctatatctgaattcttttgtcctgtattttaattactatacttcgaacagtatattcagatatctgaacaattcgttctcacctcttaccttctattactggtttcaatactcgaaataaatgctattgctaaaaagtctgtttgttacttttacactataaatttagaatgttatttcccttaagttgaaagttacgtttgaccgagagatgtcaagtattttcaagagtattacgattcttttcagacatagatattctaattaacttttaaagcttacgatacgaagacaggatttgtgtatgaacatcgatggcataacaacatatcttgaatcttgtccaccagagttatctggggggcagttttgaaaatataaaagatctgtaaggttaataaaaaaaacattatcttgtaattccgtagttcttatatcgaaactgttactaatttgagaaagacgtggagagctagaggcgtctataaatatatattcctctctcagaaatcataatatacctaatttattaaaaaagtctctcaaaatgtcacaatattccttcttctatttcttcctaatctctcttttcctctacgaaaattgcattgcgtatcgctacacattcacggtgagttcaaaattaattaatcaatttagtcaggcgtgagtaaactaacttaaaactgatggtatataggttattgaagctccatatagcaaactgtgtagcacgaagaagattttgaccgttaatggtcagtttcctggaccagtgttaagggcttacaaaggtgacaccatttacgttaacgttcgtaaccaagctagtgaaaatatcacattgcattggtatttcatccaaaaccctttttttcgtcttcttaattatgtaaccattttaaatacaagaacataaacgaaatttcgatggttgaataaaaacaggcatggtgtagagcagccgagaaacccgtggtcagatggacccgaatacatcacacaatgcccgattcaacccgggtcagattttacgtacaaaattttactttccatcgaagacgcgactgtttggtggcatgcgcatagctcgtggacacgtgccaccgtacacggtctgattttcgtgtatcctcggcctcctgataccctgccttttccagaaccggactacgaagtccccttagtttttggtacaaaccaggacatataacaaaagatcagtgaagttgcttttttttttttttttttttttatctctcttaaattaaaattaatttcataaaaacttgacaggagagtggtggaagagggatgtgagagaagtagtggaggatttcatgaggaacggaggtgaacctaatgtgtccgatgctttgactatcaatgggcatcctggtttcttgtatccttgctctcaatcaggtttcttttactttttccctttctcctattaatttcttattttgtttttaatatacagttgtgggataaaaactaattgtggagatgaaataaaatttagggatattgatcattgaaacaaattgtgaaatgattcaaacgagcattttttttttcaagtcaactgtttttaatttgtttttcctcgttttttcaaaagtttcttactaatttagttagttaaacataattaatgtttgatcaaattgtccaaaaattagttaagaacttacgagtggttgataaaaaaaaaatcacgaggcatattaattcaaaccaaaatagttgtgtttgtatttattagttcttaaaaattgtgctcataaatttgaaactagcatttgcatgcatatttatgtttaaaacctagttagtaaagtccgttattgacatgcatacgttacgtatacgtatgtttaacagatacattcaagctcgtggtagagaagggcaaaacctaccgcattcggatggtaaacgccgcgatgaacctaattctcttcttcgccatcgcgaaccacaaactcaccgtggtcgccgccgatggccactacaccaaacctctaaccgctagttatatcaccatatctcctggccaaacgctagacctgttactatacgccgaccaaagtccagagagcacttataacatggcggccagagcttaccatagcaaccccaacgttgggttcaacaactctaccaccgtcgggatcttacgttactactcttcaaacgacgccggaacgtcttcatcagaacgttacccgtaccttcctggctacaatgacacctcagcagctttcgatttcttcacaaaaatcaaaggcttatactccagagtagctcccgccaaagtttcacgtaggataatcacgacggtttcgataaatctcctcaagtgtcccaacgactcgtgtgcaggcccaaacgggtcgaggttagcggcgagtatgaacaacatatcgttcgtcacaccgagccacgtggacatactaagagcttattaccttcacattaacggcgtttacggaacgcggtttccggagttcccaccgcggatattcaatttcacagcggacgaccaaccgctgtttttgcagactccgaggctggcgacggaggtaaagaagtttcagtacggggagacggttgagattgttatacaagggacgagtttggtaggtggtggaatcgatcatcctatgcatctccatggttttagcttctacgtggttggtttagggtttgggaattttaacgcacgtaaagatccctccaactataatctagacgatcctccttacagaaacacggcgactgtgcccaggaacggttggatcgctatcagattcgtagctgacaatccaggtacgtacacttacataaacctctaactttgatttggttcaaatctctttttaatattttgtgtttttgtaggggtttggttcatgcactgtcactttgatagacatcaaacgtggggtatgaatgttgtcttcattgttaagaatggaataaaaccaaatcagaagattctacctccaccgcctggcttaccaccttgtgaccaatttgagaatctataaatgattttatagcatgttgcagtattgtgtttgatgtaataaactactgcatatttacaaaaaaaaatataatcttaaattttgtttttatttaattaattttcacaagtttttctatcgtagcagtcataataaggaaagatactcccaagacaaaacagtgtctgaagtcattattttaaccctgagcctttctttctcataatatcttcaaaagctatagatgtggtgaagtttacctcgctcacactgataagtccatgtcttgtaccatatcatcataatcttgagggacctctgcgtgatggaaacgccctgtgcaagtggagtgatgcatctgtgtaatgtgactctgttgaagtgctatagccttgtggcttctactccagtctcttcggctccaaaggtataacggtggcggcatattgttccactgctctatcgtttgatcatttacatctatcgatccaggcaagtagaacgactacagagcaaaaaaacaaaggaatgtgattgaaatgtattggttatactaaacgagagtttgattcattagtgaacgtacttaccatgccagaaagtaatctcgtgtcttcccaaatcaagtcatactcagctatctcgtcgaccctgtgattgtagaggaaaacaaaggttatgaaaagtttgtaactgacactctatatttgctatttacctttttgtttcacttggtacgatgaggattagaatcttgggtctaaactcgagggccttcctgatgaaaatgttagcaagactggatttgtaaccgaaaggcgggtttaatcccattatctgtttttactcacgaccaagtaatatctcagttagtgaattcaaaaagtgtatttcacctttaggatgttggttgcgttttttaccagtcgagagccatcgggtaactcttgtttcttcacactcaaccaatctctcttctcaaagttgaagttatactgccatggaaacatagtgtttcagaaacatcttcaaacacaacaataaaagagtagtg

SEQ ID NO: 36 - DNA, 1524 bp, Thlaspi arvense
  source 1..1524: mol_type = other DNA
atgagctccacggagacatatgagcctctattgagacggctccactcagattctcagttaaccgtaggttcttcaccggagatagaggagtttctcggccgtcgtagatccacggtgacgccacggtggtggctaaggctggccgtatgggaatcaaagcttctttggacgctctctggagcctccatagtggtctctgtgctgaattacatgctcagcttcgtcaccgttatgttcatcggccatcttggctctcttcagctcgccggcgcatccatcgccaccgtcggtatccaaggcctcgcttacggtatcatgttgggaatggcgagcgcggtccagacagtgtgtggtcaagcgtacggcgcgaggcagtactcatcaatgggaataatttgccaacgagccatggtcttgcacctcgcagctgcggtcctcctcacgttcctctactggtactcgggtccgatcctaaaggcgatgggccaatccgcagccatcgcacgcgagggtcaggtctttgcacgtgggattattccgcagatttatgcttttgccctcgcttgccctatgcagaggttcctccaggctcaaaaaattgtaaaccctttggcttacatgtcactaggagttttcgtgctacacacgctactaacctggctggtaaccaacgtcctgcatttcggcttgctcggtgcagctctggtgctgagtttttcgtggtggcttctcgcggctgtgaatggtctgtatatcgtgatgagcccgagttgcaaggaaacttggaccgggttctcagctagggctttaagagggatttggccttacttcaagctcacgatagcttcagcagtcatgctatgtttggagatatggtacgtccaagggctagtgattatttccggtttactcaccaatcccacaattgccctagacgcaatttcgatttgcatgtattactggaattgggatatgcagttcatgcttggtctaagtgcggcaatcactgtccgagtgagcaacgagctaggagcgggaaacccacgagtggctaagttatcagtggtagtggttaacatcacgacggttgtcatcagcttattcctctgtgtcgttgtgctcgtgttccgcattggccttagtaaagccttcaccagcgacgcagaggttatagctgcagtctctgatctctttcccctgctcgccgtttccattttcttaaacggaatccaaccaattctctctggtgttgccattggaagtgggtggcaagcagtggtggcttatgtgaatcttgttacttactatgtcattggtcttcctattggctgtgttcttggcttcaaaaccagtcttggagttgcggggatctggtgggggatgattgcaggagttatacttcaaaccctaactttgattgttcttacactcagaactaactggaattccgaggtggagaatgcagctcataggttaaaagcttcagcaaatgagagtcaagaaatggctaccgaaggaatctaa

SEQ ID NO: 37 - protein, 507 aa, Thlaspi arvense
MSSTETYEPLLRRLHSDSQLTVGSSPEIEEFLGRRRSTVTPRWWLRLAVWESKLLWTLSGASIVVSVLNYMLSFVTVMFIGHLGSLQLAGASIATVGIQGLAYGIMLGMASAVQTVCGQAYGARQYSSMGIICQRAMVLHLAAAVLLTFLYWYSGPILKAMGQSAAIAREGQVFARGIIPQIYAFALACPMQRFLQAQKIVNPLAYMSLGVFVLHTLLTWLVTNVLHFGLLGAALVLSFSWWLLAAVNGLYIVMSPSCKETWTGFSARALRGIWPYFKLTIASAVMLCLEIWYVQGLVIISGLLTNPTIALDAISICMYYWNWDMQFMLGLSAAITVRVSNELGAGNPRVAKLSVVVVNITTVVISLFLCVVVLVFRIGLSKAFTSDAEVIAAVSDLFPLLAVSIFLNGIQPILSGVAIGSGWQAVVAYVNLVTYYVIGLPIGCVLGFKTSLGVAGIWWGMIAGVILQTLTLIVLTLRTNWNSEVENAAHRLKASANESQEMATEGI

SEQ ID NO: 38 - DNA, 4858 bp, Thlaspi arvense
  source 1..4858: mol_type = genomic DNA
accgtttctttttgttgcgtgtcgagaataatagtcatctatgtgttttatatatagagagtcatagactatagaaaaaatgttataagaggacaaaatttcaataaattgaattagtttaaatttgatcaacaatttttttatcatcttatttaattcttagatgattatagtaaacaactaagatatcccagtatcaatatattcatgcataaatagaatgaaattgtattgggggggggggggaatatacattatttaattatatagattgtcatcaagtaattaaataaaataccaaaatgacattaaccataacaaagtgaatatgctgctgcatatttgtaagaaatcaaaagaaactttgcagcatataattactcgatgactaatacaagtatattgtgttgaaatttgatgtagtgtggaatagttaagattatttagaaaataaaaccacttttaataattacctgaaaatgagtaataatcttctaatttggtggggccatccgacctaatagacaactcattgatttcatcttacgtcagggacagttcataaaatgcaaataattgtctttttttttggtaatgattgtctttaatctttattttgtagattaacagattatattattcctttttctttcttactgttcttcagattatttggatggtttcagttgggcctcaggagcagaccggtaaatgggttggaggactattggtgggccacatttctgaaaagcatttcttcctctcaaaagctcattattatgagtatctttttatacggtagaaaggagtacataagtggtaacataaaatatattctgccaaaaaagttagttgattcttcttaatcactactccttttcttgataattatctacgtgggaaacactatttgtcctccccccatttaatttggttgaaagtcttgagactagaggttggctcaatccaaaatcgttgacgaacgttaggtatcgttatcaactacaactctttttttcactgaggtaccgttatatttatatacctacctagttttactcttgtgcacaaggatatttcggttcggtttgatatctttctcgatcttgaagaaatattaccaatttggagcttatacattcctcggtctggtatcattcaacaaagtttttggtttggtttgtttaacaaataatatgaatgtgtgtttagtcgtcccttaggtatttctcaatctctttcttttaagcttcactttcttaataagccattaagtaacgtaactagagaatggttgttacactatacactaacaaaaatcagaccaaacagtcatgaaagatcttaaccatcaattccgtttcggtcaacgactcgaaccctcagcataaccaaaacaaacagtcgtaatataaacacgcccggtctataactataacaaaataacggcaaaagaaagaaaatacgagaaaaagaagaagacgaacaaacaaacggaccatgagctccacggagacatatgagcctctattgagacggctccactcagattctcagttaaccgtaggttcttcaccggagatagaggagtttctcggccgtcgtagatccacggtgacgccacggtggtggctaaggctggccgtatgggaatcaaagcttctttggacgctctctggagcctccatagtggtctctgtgctgaattacatgctcagcttcgtcaccgttatgttcatcggccatcttggctctcttcagctcgccggcgcatccatcgccaccgtcggtatccaaggcctcgcttacggtatcatggtatgtgctttagagagtaaacgacgttgacgtcgttcgatgttatagcttcacattcatttgcttatcattttgtaatatagtaaatccgggttttgaattaggtttctcaatattttgaccattttatgaataccagcaaccataataaaaatacaaactgtcggatcagttttgttctccatttgagatccgattttggtctttcagatgcaaaccatattaggatacagttcggttttcatgtcggctattttggtccggtttatcatttttgatcaatcttagccttaggcatctcccaactgtttttatgtatcaaatgtactagttgggaatggcgagcgcggtccagacagtgtgtggtcaagcgtacggcgcgaggcagtactcatcaatgggaataatttgccaacgagccatggtcttgcacctcgcagctgcggtcctcctcacgttcctctactggtactcgggtccgatcctaaaggcgatgggccaatccgcagccatcgcacgcgagggtcaggtctttgcacgtgggattattccgcagatttatgcttttgccctcgcttgccctatgcagaggttcctccaggctcaaaaaattgtaaaccctttggcttacatgtcactaggagttttcgtgctacacacgctactaacctggctggtaaccaacgtcctgcatttcggcttgctcggtgcagctctggtgctgagtttttcgtggtggcttctcgcggctgtgaatggtctgtatatcgtgatgagcccgagttgcaaggaaacttggaccgggttctcagctagggctttaagagggatttggccttacttcaagctcacgatagcttcagcagtcatgctatggtaaatgtctttaatctaaacacaaatctgtatgatttgaccggttaaaatttatggtttgaagaaagctgatatataccaatttaaaatgaaatatctgcagtttggagatatggtacgtccaagggctagtgattatttccggtttactcaccaatcccacaattgccctagacgcaatttcgatttggtactcctttcacccgagatttatcatatgccgacgaacctcaacggttacgtcttaacccggttaagtgattttgcagcatgtattactggaattgggatatgcagttcatgcttggtctaagtgcggcaatcacgtaacaaaacaaaattaaaaatggcatgtagtttttaatttaaatgatccatttgcaaaaaccgtgccgtttttgtgtgttttgtgttagtgtccgagtgagcaacgagctaggagcgggaaacccacgagtggctaagttatcagtggtagtggttaacatcacgacggttgtcatcagcttattcctctgtgtcgttgtgctcgtgttccgcattggccttagtaaagccttcaccagcgacgcagaggttatagctgcagtctctgatctctttcccctgctcgccgtttccattttcttaaacggaatccaaccaattctctctggtaaaaacacacacaagaaaaagaggctcttttgtgaattttggtttgttgattgatctttgctctatggattcaaaggtgttgccattggaagtgggtggcaagcagtggtggcttatgtgaatcttgttacttactatgtcattggtcttcctattggctgtgttcttggcttcaaaaccagtcttggagttgcggtataatctcttttactctttctttgtgtttatatgtattgtatgcatcataagagatgggaggtatttcattacaggggatctggtgggggatgattgcaggagttatacttcaaaccctaactttgattgttcttacactcagaactaactggaattccgaggtaaaacaatcaccaaatctctctttttttctctaaatactccaaagtccttacctttactctgcatctcttacaggtggagaatgcagctcataggttaaaagcttcagcaaatgagagtcaagaaatggctaccgaaggaatctaacagcaactctgttcttttctcctctcttttgttggcaagagatatgaaataaataccttctgtttattaggattcagtaacatatttcatttcgttaaactacagacaaaaaataatggacaaactacttaatcctcttctgcaaaatctttcttctgcctttagatgattacaaaaatcaaaactttctcgttgttttcataaccccacaagtttttccgtctgtgagctaacataagccaaagacttttcttgtgttttatcatacaacacagtttctcttgcatcatcatcaccatctccttcatagtcctcctcatcctcatcctcatcctcatcatcactactcacatcgacatcatcatcatcatcatcatcatcatcagatctgtagactccagcaatgatggttgtagtctcatctctgagaccagtaagttctttagcttcctctagctcatcttgagttgaagccaatgacaaaagcacattcttcgctttctgatcaggtggtaccccacaactctccatctccttgtaccaactaagagcgctcccgaaatccttgcacctcccagacgcatccatgatagtcgttatgatggtttgattcgctttgatgccacttaacctcattttctcatatacctccataattttatcaagatcgtttgctttcgcatagccttttatcattgtcccataggtgactatattcggctcaaaaccatctacctttatcctcttgaagaatttctcagcaccctccatgtccgaagcattcacatacgctgataacatagttgtgtaagaccagagatccgggaaaaatctgcaaagggaattatgttttgttaccaatctaaaacagagaagcaacacagttcacatgatagaattattctttacctgtcacgtcgcatgctttgaaaaacggtctttgcttgatccaccattccagaaatagcgaatgcatcaagcaaaatgttataagctttat

SEQ ID NO: 39 - DNA, 2214 bp, Thlaspi arvense
  source 1..2214: mol_type = other DNA
atgcttccattaatggcgataccacttgcgacttgcaggagcatcaactggtcagccacggaaaggattcctgtttcgcttctgttccggagtattcttctccaagacgacgaagtttgtagcgctgtgccactataccggatcctcgatcagaatgacgggcaacttggtcctataagtatggccgaggaatcagacaaaccattgctggatcctgatactctcaacagagaaggaattgacttgggtctgttgccattggaggaggtttttgaatacctaagaacatctccacgggggcttttatctggagatgctgaagaaagattgacgatatttggtcctaacagccttgaagagaaacgggagaacaagtttctgaagttcctaggttttatgtggaatcctttgtcatgggttatggaagctgcagcattgatggccatcgccctagcagatagtgaagtagagactatcagtcttttgctataccatttctgctcagtgctgaccggagaatcgctacctgtgaccaagaagaagggtgagcaagtcttctctggctctacttgtaagcaaggtgagatagaagctgttgtgatagccaccggttcgagcactttctttggtaaaacagcatctttggtggacagcacagatgcaactggacattttcagcaggttctaagcttgtgccagcagaaaaatgagattgcgcaaagagtttatgccatcataaatagatttgcagaaaaaggtttgaggtctcttgctgttgcttatcaggaaattccagagagaagcagcaacagtcctggaggaccatggttgttctgtggtctgttgccactgtttgatcctccaaggcatgacagtgctgaaaccatactgagagctcttaaccttggagtttgtgttaagatgatcaccggtgatcagttggcgattgcaaaggagacaggaaggcgacttgggatgggaaccaatatgtatccttcttcctctttgttaggccacaacaacgatgatcacgaagccattccattggatgagcttattgaaatggcagatggatttgctggagtgttccctgaacacaagtatgagattgtaaagatattacaagaaaagaagcatgtggttggaatgaccggagatggtgtgaatgatgctcctgctctgaaaaaggctgacattggaatagctgtcgctgatgcaacagatgccgcaagaagttctgctgacattgtactaactgagcctggcttaagtgtaattatcagtgctgtcttgaccagcagagccattttccagcgtatgaagaactatacagtatatgcagtctcgatcaccatacgaatagtgctcggttttacacttttagcgttgatatgggaatacgactttccacctttcatggttttgataatcgcaatactcaatgacgggaccatcatgactatctctaaagatcgagtaaggccatctcctacacccgagagttggaagctcaaccagatatttgcgactggaattgtcattggaacataccttgcattggtcactgtcctattctactggatcattgtctctaccaccttcttcgagaaacacttccatgtaaaatcaatcggcaacaacagtgaacaagtctcatccgctctgtatctccaagtaagcatcatcagtcaagcactcatatttgtaacacgtagtcgaagctggtcttttcttgaacgtcccgggactctcctgattttcgccttccttgttgcccaacttgccgctacattgattgctgtctatgccaacatcagctttgctaacatcaccggcattggatggggatgggcaggtgttatatggttatacagtttgattttttacatacctcttgatattataaagttcttcttccactacgcattgagtggagatgcttggaaccttgtatttgaccgtaagacagcatttactaataagaaagattatagaaaagatgacggagcgtccaatgtaaccatctctcagagaagtcactctgcagaagaactcagtggaagtcgttctcgcgcatcttggatcgctgagcagaccagaaggcgtgcagaaaccgccaggctcttggagggacactcggtgtcaaggcatttggaatcagtaatgaagctcaaacaaattgaccccaagatgattcgtgcagacactgtctaa

SEQ ID NO: 40 - protein, 737 aa, Thlaspi arvense
MLPLMAIPLATCRSINWSATERIPVSLLFRSILLQDDEVCSAVPLYRILDQNDGQLGPISMAEESDKPLLDPDTLNREGIDLGLLPLEEVFEYLRTSPRGLLSGDAEERLTIFGPNSLEEKRENKFLKFLGFMWNPLSWVMEAAALMAIALADSEVETISLLLYHFCSVLTGESLPVTKKKGEQVFSGSTCKQGEIEAVVIATGSSTFFGKTASLVDSTDATGHFQQVLSLCQQKNEIAQRVYAIINRFAEKGLRSLAVAYQEIPERSSNSPGGPWLFCGLLPLFDPPRHDSAETILRALNLGVCVKMITGDQLAIAKETGRRLGMGTNMYPSSSLLGHNNDDHEAIPLDELIEMADGFAGVFPEHKYEIVKILQEKKHVVGMTGDGVNDAPALKKADIGIAVADATDAARSSADIVLTEPGLSVIISAVLTSRAIFQRMKNYTVYAVSITIRIVLGFTLLALIWEYDFPPFMVLIIAILNDGTIMTISKDRVRPSPTPESWKLNQIFATGIVIGTYLALVTVLFYWIIVSTTFFEKHFHVKSIGNNSEQVSSALYLQVSIISQALIFVTRSRSWSFLERPGTLLIFAFLVAQLAATLIAVYANISFANITGIGWGWAGVIWLYSLIFYIPLDIIKFFFHYALSGDAWNLVFDRKTAFTNKKDYRKDDGASNVTISQRSHSAEELSGSRSRASWIAEQTRRRAETARLLEGHSVSRHLESVMKLKQIDPKMIRADTV

SEQ ID NO: 41 - DNA, 5382 bp, Thlaspi arvense
  source 1..5382: mol_type = genomic DNA
atgcttccattaatggcgataccacttgcgacttgcaggagcatcaactggtcagccacggaaaggtggtttcaattttcattcgtggaccctttttaaggattcctgtttcgcttctgttccggagtattcttctccaagacgacgaagtttgtagcgctgtgccactataccggatcctcgatcagaatgacgggcaacttggtcgtaacatagtggtttaagttcgtgtgtagctcgtactatgttttgatggtttgctattaccttagaattttaaataattatcttatgtacatcgacgaagttacggtttttgctattgttcactagttccaaggtgtggatcgaatctaggaatgtgggctttgaagtggtacttgtaccgtggattttgaagctataagtatggccgaggaatcagacaaaccattgctggatcctgatactctcaacagagaaggaattgacttggtaaatgatgtgtggttcctttacttttattaaaattcttggattctttagtggcaaaaatggttttgacgcttgagctggacagggtctgttgccattggaggaggtttttgaatacctaagaacatctccacgggggcttttatctggagatgctgaagaaagattgacgatatttggtcctaacagccttgaagagaaacgggtaataaaaagcttatcgtcaaagtttttccatagtgttcctgcctaagacaggagagaagcttactagttctgagatcttattcattatgaacactcttcatttctttttcacatattatccttaggccacacactgatttttctgccaagttgtggttctttacattagctcttgtataatatgttagtgttgtcctaatgacactgaaaacgaaacgatacaggagaacaagtttctgaagttcctaggttttatgtggaatcctttgtcatgggttatggaagctgcagcattgatggccatcgccctagcagatagtgaagtagagactatcagtcttttgctataccatttctgcgtacatgagagtttatgaaatcgtttctgctcttgaaactcatggtgaaaaatgtttattacagagcttaggtcctgactgggaagactttgttggaatcgtttgccttttactgatcaacgcaacaatcagcttctttgaagaaaacaatgctgggaatgctgctggagctcttatggctcgcctggctccaaaaacaagagtctgcttcttcaccttatgcattttcactcttattaccttaaatctgatcaagatccactcttgataggttcttagagatggacagtggcaagagcaagacgcgtctatcttggtacctggtgatattattagcataaagcttggggatatcattcctgcagatgctcgccttcttgaaggagaccccttgaaaattgatcaggcacgcacagattatatttagcgctaagtcacatttcttctctcttagtacattatgtaaagactgtatctgacagaatattcctgcagtcagtgctgaccggagaatcgctacctgtgaccaagaagaagggtgagcaagtcttctctggctctacttgtaagcaaggtgagatagaagctgttgtgatagccaccggttcgagcactttctttggtaaaacagcatctttggtggacagcacagatgcaactggacattttcagcaggttctttattgttccttaactcccttttctggttgaaacagtctgactggtaaaagaccaaaccttgtaaagctgtgaatacctttgcaagaacatgacatgtttctgtgacatgttttccttataggttcttacgtcaattgggaacttctgcatttgctcaattgctgttggaatggttcttgaaatcattgtcatgttccctatacaacatcgctcatacagaattgggatcaataaccttcttgtactactgattggagggatacccattgccatgcccactgtactatctgtcacgcttgccattggatctcatcgactctcacaacaggtgtcgtttctcttgactgattaactgtaacagagtgaaccaagaagaatccaacttttaagcttctgtagaactttttgttagcaatataatatgtgtttcttgttgttttaaaagggtgccatcacgaaaaggatgacggcgatagaggaaatggctgggatggatgtcctctgctgtgataaaactggaacccttaccttgaacagtctcaccgttgatagaaatcttattgaggtaccaaccaatacttcccatgtgacttgcatttcaaagtccaaagagtacagttaacaacagttgcctccatctttacaggttttcgatgactacatggacaaggacacaattttgctgcttgcaggcagagcttcacggttagaaaaccaggatgccatagatgcagcaattgttagcatgcttgctgatccgaaagaggtggagatgtttcttttacataaactctgttttatgaaaatattgtcatcttctttagaagttttacttattagaaaaggttgtttatctttaggcacgtgcaaacattaaagaaattcatttcttgccattcaatcctgtggacaaacgtacagcaataacatatattgactccgatggaaaatggtatcgcgctagcaaaggagctcccgaacaggtaacaaagaatcaccctatactacttggcactttcaaaactgactctagatgtaaaaaaatgaaagttcttttatatataggtccataaaagatatatcatcactgattcaattccaactgtactgtatacataggttctaagcttgtgccagcagaaaaatgagattgcgcaaagagtttatgccatcataaatagatttgcagaaaaaggtttgaggtctcttgctgttgcttatcaggtaaaatatttctgttatcccttttctctcttgatatggtttttattgtaagtgtactatttggggaagaagcttataatgacattagttatactcattcaatcattttaatcattgtttctaggaaattccagagagaagcagcaacagtcctggaggaccatggttgttctgtggtctgttgccactgtttgatcctccaaggcatgacagtgctgaaaccatactgagagctcttaaccttggagtttgtgttaagatgatcaccggtaattctgaaccctagagcaggcttgcttgggaccacagaggaacagacacgctctcatggtgaaaatctgataagtttggataaaaaaaatgtaggtgatcagttggcgattgcaaaggagacaggaaggcgacttgggatgggaaccaatatgtatccttcttcctctttgttaggccacaacaacgatgatcacgaagccattccattggatgagcttattgaaatggcagatggatttgctggagtgttccctggtcatactcacaacacagcgcttatatcttaccgagtttcagattttctctcttttactgatcccagtttcttttgatggctctcatgtttcagaacacaagtatgagattgtaaagatattacaagaaaagaagcatgtggttggaatgaccggagatggtgtgaatgatgctcctgctctgaaaaaggctgacattggaatagctgtcgctgatgcaacagatgccgcaagaagttctgctgacattgtactaactgagcctggcttaagtgtaattatcagtgctgtcttgaccagcagagccattttccagcgtatgaagaactatacagtaagtactaaagacaactatcatctgattccacattgctaaagataagcaaatccatgtaatataggatatgaatttcaagtagtttaatgaaattctgaagtttcttttggtttcctctgcaggtatatgcagtctcgatcaccatacgaatagtggtaaggagcttcaagatacacgatctaacttgctaagttacatctacttgagccttctcttcttatcattgtttcatgcagctcggttttacacttttagcgttgatatgggaatacgactttccacctttcatggttttgataatcgcaatactcaatgacggtaatcttttaatcctctcaatagcttcatgtttgaattgttgatgttaaaaactctaaattcttaacactttcaagtgctcttgtttatctcctacgcaacagggaccatcatgactatctctaaagatcgagtaaggccatctcctacacccgagagttggaagctcaaccagatatttgcgactggaattgtcattggaacataccttgcattggtcactgtcctattctactggatcattgtctctaccaccttcttcgaggtatcttcccgtcgctcgaaagtaatcaaattcgatttgcttaccgagaaaaacgcataaccatgaccatccctgaatcttaaatggctgcagaaacacttccatgtaaaatcaatcggcaacaacagtgaacaagtctcatccgctctgtatctccaagtaagcatcatcagtcaagcactcatatttgtaacacgtagtcgaagctggtcttttcttgaacgtcccgggactctcctgattttcgccttccttgttgcccaacttgtaagaactcttcatgtttaacctttttccatcacagaatactacatacagcatacataggtcttggttttgatttgtccgttttcatgtacacaggccgctacattgattgctgtctatgccaacatcagctttgctaacatcaccggcattggatggggatgggcaggtgttatatggttatacagtttgattttttacatacctcttgatattataaagttcttcttccactacgcattgagtggagatgcttggaaccttgtatttgaccgtaaggttagtgcatgtcttgtcctctgtctcagactttaactctgtttttttcttaaaagacaaagagtgttggttttgtcttgcagacagcatttactaataagaaagattatagaaaagatgacggagcgtccaatgtaaccatctctcagagaagtcactctgcagaagaactcagtggaagtcgttctcgcgcatcttggatcgctgagcagaccagaaggcgtgcagaaaccgccaggttctcttttgtctatacgactttttttgggtttctctttcatttcacatactaccagaaccatctctggtccacagaaaatagaaacttagtttttttgttcatttgataggctcttggagggacactcggtgtcaaggcatttggaatcagtaatgaagctcaaacaaattgaccccaagatgattcgtgcagacactgtctaa

SEQ ID NO: 42 - DNA, 1857 bp, Thlaspi arvense
  source 1..1857: mol_type = other DNA
atggagagtagtgtagttaatcatccattgcaagaagatgagaagggtttttctgatgaagataatgctgtaaataatgagaaagagagtttattgcaaacatctggctctgtagagaatgctcctgaaggttctggtcgttcttcggattggcgtaggggactagaccactgcataactgcacctgttggtctctatggagatatggtaatcgatgacaatgaggttaagtactctcggtccataacagagagattgtcccctgcgagtcataattcaaaattagatcgattatcggagcgggaaaagcaaaaactcattgttgagctagtcagaatacaaaatgacgggaccgtggaagttgatatagataacggtacaccggtatcggagttattggagtttcagccaaccaaagggcagccaacaatcacatatgaaaagtcatttgctgattcctttagatcaattccaagattaaaaattgtgatacttgtggttggaactcgcggtgatgtgcagcctttcttggccatggcaaagcgcctccaggagtttggtcatcgtgttaggttggcaactcatgcaaatttctgctcttttgtacgatctgctggagtagagttctatcccttgggtggtgatcctcgagaactagctggatatatggctagaaataaaggtctgattccttctgggcctggagaaatagcaaaacagagaaaacagttgagggcaattatagagtctcttcttccggcttgcacagagcctgatatgcaaactgctgcctctttcagagctcaagcaataattgcaaaccctcctgcgtatggacatgtgcatgttgctgaagctctaggagtaccaattcacatttttttcacaatgccttggacgccaactcatgaatttccccaccctttggcccgagttcctcaaagtcctgcgtattggctatcatatatagttgttgatctgatggtatggtggagcataaggacatacataaatgattttaggaagaggaagctaaaccttgcacctttcgcatatttcagcacataccatggctcaatttctcacttgcctactgcttacatgtggagtccccatgttgtgccaaaaccaagtgattggggtcctttagttgatgttgttgggtattgtttcttgagccttggatcgaagtaccaacctcgtgaagattttatccactggatagaaagaggatcaccgcccgtatatattggtttcggaagcatgcctcttgacaatccgaaaaaaacaatggatattatactggaaacactgagagatacagaacacagagggatagttgatcgaggttggggtggccttggaaaccttgctgaagttcctgaaaatgtattcctcttggaggactgtcctcatgattggttgtttcctcaatgttcagctgtgattcatcatggaggtgctggaaccacagcgactggactaaaagctgggtgtccaacaacaatcgtgccgttctttggggatcagttcttctggggtgacaggatctatgagaaaggacttgggcctgcgccaataccaatagctcagctcaatgttgagaacctctgcaattccataagattcatgcttcaaccagaggtgaaatcacgagtgatggaactagcgaaagtactggagaacgaggacggtgtagctgcagctgttgatgcattccacaggcatttgccactggctctgccactcccggagtcctcgccggagaaaagacacgaagatgatcgaccagacctgttacagtggttcttcatccagattggtaaaaagtgttgccttccatgtggtggtgtgtga

SEQ ID NO: 43 - protein, 618 aa, Thlaspi arvense
MESSVVNHPLQEDEKGFSDEDNAVNNEKESLLQTSGSVENAPEGSGRSSDWRRGLDHCITAPVGLYGDMVIDDNEVKYSRSITERLSPASHNSKLDRLSEREKQKLIVELVRIQNDGTVEVDIDNGTPVSELLEFQPTKGQPTITYEKSFADSFRSIPRLKIVILVVGTRGDVQPFLAMAKRLQEFGHRVRLATHANFCSFVRSAGVEFYPLGGDPRELAGYMARNKGLIPSGPGEIAKQRKQLRAIIESLLPACTEPDMQTAASFRAQAIIANPPAYGHVHVAEALGVPIHIFFTMPWTPTHEFPHPLARVPQSPAYWLSYIVVDLMVWWSIRTYINDFRKRKLNLAPFAYFSTYHGSISHLPTAYMWSPHVVPKPSDWGPLVDVVGYCFLSLGSKYQPREDFIHWIERGSPPVYIGFGSMPLDNPKKTMDIILETLRDTEHRGIVDRGWGGLGNLAEVPENVFLLEDCPHDWLFPQCSAVIHHGGAGTTATGLKAGCPTTIVPFFGDQFFWGDRIYEKGLGPAPIPIAQLNVENLCNSIRFMLQPEVKSRVMELAKVLENEDGVAAAVDAFHRHLPLALPLPESSPEKRHEDDRPDLLQWFFIQIGKKCCLPCGGV

SEQ ID NO: 44 - DNA, 7708 bp, Thlaspi arvense
  source 1..7708: mol_type = genomic DNA
ctaaaagagcatgagcagcaccgcgatcatcatcggaatagtccgccaccaacgcaattgaactaagaaaggctacaaaactgctttaaatccatcctgctgcttattccttttgcgtgtggccgccagaagaagatgagaaaacttactttcaccattagaaattagaataaagagtcaccgaaagtgaaagtgaataggatattcaccagaccgcctttgagaagcgccagttctgcagatcctgcatctcaatcactcaagataactcccaaatctcaaatcaactccgctaaagaaacttcctcttcgcaatcacgacgatttattaacagaaaagagaaggaattgctctttcgggagaagatccagcataactaacggaaagagtttcatcaaattcgtctggaataaagatgaaaacaagcaaaaggaaaaccgaacgttgtcggagaacttagaatcctataaacggaaaataaaatccgatcaacggaaaagaagatccgattgacggaactataagacagccaaaaagccgatcaaatcggatcaaagaaagaactctctcgctctgaaagattttaaagagagaagagagagagagcccttcaccttgtgccacccgtacttttaagagcatctccaaccatattctattttcaactccaaatgctattttgaagtaaaatcctctccaaccctagtctattttcaactttaaaatagagtaaacctaaattttactctatatttggagtaaatctaaactttactccatcttggaattagacttttttatttgcaaattaatccttgagatttattataattatattttatactatttaatatttataacaaatattataaaactgataattatgaatatttaaatactgcaattattcctacaaaattaaaaaatataataaactttaaaatacaaaataagggctaaaattaagataaacaacataaataaatttaagacaacaaatactaaaaatattaatgataatttttttttattatagtaatgtttaaataaaaattgcatatgcttttttgtgatgttatgtaatttttattatttgataaatatttaagttatagtttttcaaagaaattgtaaataataaaataagtgggatttatttataaattttaaaactaaaaaatatttataataaaatcaaataagattctatttagaatatttctttttagagtaaaaaataaagaaatacattagagtaaaacacaactctattttagagttactctatttttctattttggagtagaaaatgaagaaataattgaagatggtataacaaacgaaaagtcgcattatcttactgttaaattactataattcataatcaattggttttgtttcggtggcatccggcatcccctaatatgattgatttttatcgctgcatttattaaaatatatatatcttcatcctcgatcaccacaattcattgattcaaaagtctccaaaccccttggaagctcaacattacaatctcgccaaattcctcaaaaccagaattttccacagacccagaaacatttctcatcaaagttctctcctttcctgtctcttgaactttctctcctactcactcagttcaagaacaatctttcgatcattgatcagtgatggtagattcaattgttgggtttcatttacttgggcaatggcttttcttttcttttctcttctcttttcgattgattgattggttaattctgtgtctctgtacagtttcgaattgtgtctttcaagttaaagctggatcatttttctagttgatctcatcctcgcgcttaacgtgagagactctctgctctgtaatctttccctgcgttttcttgttttatctgaaacggttaatatagagataaaaaaacccaatttctctgacttttttttctttctttaatatatcatttcttctcccttttgctttttgtataaagtgcagctaactttccttaaggattcactggttggttcaagcactgattcgccgcgtacagcttttggcaggagccatttgcatctctgatcgacatggattagaatagtgtgcagttgtgttgtgtacaactcgctgcatagatgttactttgtggagttcaattcatatgtagtatgtttgttgtttaagaagctgatctttgtgggggcattgggtagtgagatctgttaaattgaagtcggtgatggagagtagtgtagttaatcatccattgcaagaagatgagaagggtttttctgatgaagataatgctgtaaataatgagaaagagagtttattgcaaacatctggctctgtagagaatgctcctgaaggttctggtcgttcttcggattggcgtaggggttagtcctctattggaacacgtgtatttatcttattccaagctttgccatcaaaaccataacttagagcataacaacttatcaagattgtatgttcttgaaggactagaccactgcataactgcacctgttggtctctatggagatatggtaatcgatgacaatgaggttaagtactctcggtccataacagagagattgtcccctgcgagtcataattcaaaattagatcgattatcggagcgggaaaaggtaggaatctgaaccttcattgcaatggatatgttcttcatttgattacaaatttttttggtaacttgaaaacttcttgttattccagcaaaaactcattgttgagctagtcagaatacaaaatgacgggaccgtggaagttgatatagataacggtacaccggtatcggagttattggagtttcagccaaccaaagggcagccaacaatcacatatgaaaagtcatttgctgattcctttagatcaattccaagattaaaaattgtgatacttgtggttggaactcgcggtgatgtgcagcctttcttggccatggcaaagcgcctccaggtagtttcgaaattgctttctcattctttgtatccttttgcgaaattaagattcacagagggaatcattgtgactttacatatgtatattttgtggatgcatgcatatagtacactgcaattgaacaggctcgtatcaaagtgttggcatgtgcctatatcatgtgttctcgtcattttaaatttgtttcatttcttcatcctatcgtcatatgtgttcttgacgcttttcttagcatttggtgagagatttggaactgattggcattgagagaggttaaagttagatattgtttttctctgttgcaggagtttggtcatcgtgttaggttggcaactcatgcaaatttctgctcttttgtacgatctgctggagtagagttctatcccttgggtggtgatcctcgagaactagctggatgtaagaagtcctccttgaaaagattcgtttatattttagtttctcgagttttttttgtttgatgatgaaagctgtcataaattctctctttagcttcatgtgggtatttttgaatgtagatatggctagaaataaaggtctgattccttctgggcctggagaaatagcaaaacagagaaaacagttgagggcaattatagagtctcttcttccggcttgcacagagcctgatatgcaaactgctgcctctttcagagctcaagcaataattgcaaaccctcctgcgtatggtatatccttcgttaactttaaaactctttgatccatcagaacctcattgtttgtaaacctttcttaagcactttttctatgaaactgatggtatggtttttggttctaattataggacatgtgcatgttgctgaagctctaggagtaccaattcacatttttttcacaatgccttggacgtgagttgacttctctgcttttaaacttgccttaacgtgttatttggtttcctgttctcttacatcatcttcatgtaggcaggccaactcatgaatttccccaccctttggcccgagttcctcaaagtcctgcgtattgggtaatgttattctttcttatgaccatatactctctcgaagataatgaggcttattgtttcacaacatttttttgtctcagctatcatatatagttgttgatctgatggtatggtggagcataaggacatacataaatgattttaggaagaggaagctaaaccttgcacctttcgcatatttcagcacataccatggctcaatttctcacttgcctactgcttacatgtggagtccccatgttgtgccaaaaccaagtggtgagattcccgctgcatccccagtacatatattccgctgaggtttatcatatgtattgtagcttcattctggcttctagattaatgttgttcttctggctttgtcaattggcaagaccataatgggttgtcaattttaggctgagctctttatctttccttcggtagatatctgaaagattttgctttttgtttgactaatttgcagattggggtcctttagttgatgttgttgggtattgtttcttgagccttggatcgaagtaccaacctcgtgaagattttatccactggatagaaagaggatcaccgcccgtatatattggtttcggaagcatggtaaactgatgatccttagaaaatatgctcttccttgctttggtgatattcagttataatgcatagtactgatattgttgtttcttctcttttacacaaccaagcctcttgacaatccgaaaaaaacaatggatattatactggaaacactgagagatacagaacacagagggatagttgatcgaggttggggtggccttggaaaccgtaagcagcttctgtaccttctcttttgatgctctgtgtcctgattcctgaactacttttcttctttgcttatacataattttttttatcttcaaacatcttgcagttgctgaagttcctgaaaatgtattcctcttggaggactgtcctcatgattggttgtttcctcaatgttcagctgtggtaacccctttttagattaactacatcatgtctccaaagacattatcttctaatccaggctatttcttgtgttgtggatatgaagattcatcatggaggtgctggaaccacagcgactggactaaaagctggggtaaaacattttgctttcacagaaatgtcctgtagtgaaatcagttttcttgaccatatgaaacctaatggttcctatattcttttgaattctatgatatgtctccagtgtccaacaacaatcgtgccgttctttggggatcagttcttctggggtgacaggatctatgagaaaggacttgggcctgcgccaataccaatagctcagctcaatgttgagaacctctgcaattccataagattcatgcttcaaccagaggtaaacaaacttaaattttccttctttttttccatgtatctcatgcccatgtaggatgtttgagtaaagaaccacagtagaagttaaacacaaacactctttcttgcaaaattaaacaaactaaacaaaacccaaaacctaaagctgtccttttgagttcaaaaaagtagaaagatgtaatcttgtatatacacttaaatattgcttatacagttcatacaaatagaaaatgtcatctttatagttcatagaagtagaaagatgtaatctttatatatacacttagaaattgcttatatagttcatacaaatagaaaaatgtcatctttatagttcatacaaatagaaagatttaatctttatagttcatacaaatagaaagatgtaacttttatgtatatgcgtggatatcgctttatcagttttttaatatgtgaaggccctcgcacaaaaaaaaaaatattatgtgaaagaaagctcggtgcttaatatttgaactatgaagcaactttctatatatatacacaaaactgacattgctttatagttcatacaaaaaaaaagatgtaatcgttatagttagttcatacaaaagaaagatgtgatctttctattttcgttcagtgatgttatgtgaagaaaaattcggtgtttagatttgaactatgaagcatctttctatttatatacacaaaactgatattgttttatactcatacaaatagaaagatgtatgaactataaaaatagaaagcatcatacaaatacaaatagttcatacaaacatcacacacaatgcacactagctcaaagctttttcctctgtttaaaactcataaaacttccaaaggtctctctctagctttgttgtatctcacaaacggaactggaatcggtagaatatgtaaaaccaatcatggcctatccaggtgaaatcacgagtgatggaactagcgaaagtactggagaacgaggacggtgtagctgcagctgttgatgcattccacaggcatttgccactggctctgccactcccggagtcctcgccggagaaaagacacgaagatgatcgaccagacctgttacagtggttcttcatccagattggtaaaaagtgttgccttccatgtggtggtgtgtgataacaaactcccttagatattttgatcttgtctctgcaactcgtttcatttcattcagttgtcaagaatatgattagatttttaacacagctgcaaaagatgggtttggggcatctttataagtttgttgttcagtgagaataagatgatatttgtgtgagtttgtcttaagaacaaagtaccgatctcctttattgtatacttaaaacccattcgaaacagaatctcccacgtcaaactacatttctcagcttgtaggcattggatttcatcagctcctgagcatgtgccagatgacccttcatatgatctgttaagtttcagtggctcaaaacggcacctttaagagaagcttgaagtatcaaaacgtgagattaaaacggaagttgcagaaacttgcagaaagcagagtatgagagattgagagaagaagaagggagaagggaacacatacaaatatttaacgagttcacgcccataacacgctatatctcaccaagactaagctggaaatccactagatatcagagagaatacatatttagagacgaacaagtgaccgttttaatatctttcactagcacttaaaattcactatgttaaatcaattaaaaccagaaaaaaaacaatagctaaacttatgctaagatgtgtttttctctccactctcactagcgactacattgtgtctatctcgttctcttcctcatgtgtactacaatctctctcacgtcttcagcttcactttatagtgacaacaacattagacctaaagcaccttgccaaacgccaaaacagcttcctatagatgcgtttgcttttttatcatatcttagaggcaaatactccttagcttttaaattcacaacaagacaaaagcaagaggctctccttgtggtcccaaaagtaactcaatccaatatgaactcaccaaagtaatcatagttatgccttgagttacttgacttgaatttgcttgagcgacaagttctcgtcttcacaaatctccacctgagaacatgatgttcaagccaaacgacatacactcttgagaaagatatagaacgccttcttctagcttatggattctaatcttggtttctgagtatgattacccagtcttgatactaagcagatttaaataccataaaactgatagatccttgctggatttaa

SEQ ID NO: 45 - DNA, 732 bp, Thlaspi arvense
  source 1..732: mol_type = other DNA
atgggaagagggaagatagagataaagaagatagagaatcagacagcgaggcaagtgaccttctgcaagaggagaactggtcttatcaagaagactaatgagctctctgttctctgcgatgctcacattggtctcatcgtcttctcctccaccggaaagctctcgcagtactgttccgaacccctcaggatgcctcagctcattgaccgatacttgaagaccagtggaatgcgacttcctgatcctaatgacggccgggaggaattgtaccaagagatggaagtactaaaaagagagacatgtaagcttgagcttcgtctgcgtccataccatggacatgacttaacctcccttcctccacacgagctcgatggtctcgagcaacagctcgaacattctgtccttaaagtccgcgagcgtaagaatgagttgatgcagcaacagttggagaatctaagcagaaagaggcggatgctagaagaagataacaacaatatgtaccgtttgcttcatgagcatcgtaacgcggttgaatttcagcaagctgggatagagacgaaaccaggggagtatcaacagtttctagagcagcttcagtactataatgatcatcagcaacaaccaaacagtgttcttcagcttgctacgcttccttctgagattgatcctaattaccatctccagcttgctcagcctaatcttcaaaacgatccaacggccaagattgattag

SEQ ID NO: 46 - protein, 243 aa, Thlaspi arvense
MGRGKIEIKKIENQTARQVTFCKRRTGLIKKTNELSVLCDAHIGLIVFSSTGKLSQYCSEPLRMPQLIDRYLKTSGMRLPDPNDGREELYQEMEVLKRETCKLELRLRPYHGHDLTSLPPHELDGLEQQLEHSVLKVRERKNELMQQQLENLSRKRRMLEEDNNNMYRLLHEHRNAVEFQQAGIETKPGEYQQFLEQLQYYNDHQQQPNSVLQLATLPSEIDPNYHLQLAQPNLQNDPTAKID

SEQ ID NO: 47 - DNA, 5332 bp, Thlaspi arvense
  source 1..5332: mol_type = genomic DNA
ttacatttcaaacagatttgacataacatgtaatattgcttaggacatttgtgttcatcacgtccgtctttcaatgaccaattaatgctgttttgtttgtttgttttaaccacgttttagcaaaagtacatttatacaggacttttttaatccgctcgttacttaatcgacaaatatataatgtccctcaatactatttggtatatattttttacaaaacatgccactgaaaatgattcagttgtatatgttcatatcatcacataattgtgttcaacctgatgtagcggctgattactctatgcacaatgttagaaaatctgaatattaactcgatgatctaaataccaatttcttttccagaattttaatacgttcgagtttcagcataaaagcttttactcacaccacttgtttccccttgcgttgtgtggcaatgtcgctgtataaatgtacatattccttttgttttcctccaaaaagtttattaatgaaattcagattctacgatataataataaataatgttacttcaaaaataaaagagtgtgccaatatggactgtgcttttaccatgagggatttaaactcgattttttttttgttacactgaagttgatgaatatagacattaaattaactcgaatagacaggaaaaatccgatgtccaaaaaaaaagacaggaaagagatatcacaaataatctaacaaaactattatggctaagtatcacatttttagatatatcaacggttcaaagcccgatccatactgtcatacgtaaaaaaatattgttttggcaaaactacatataaggtgatgttactatagaaataaaaccaaattaagaggaaggtgggtaagaaaaaataagagagagtcactttcaagtattgttacattttgtcttttcccatttggctatctctctcttttgccttttcccttttgtggtaactttattttccctataacattttttcattaagtttccatttatggattattttctagttgcgtcaagcatggaatatcaaagaaattagttcgagatttgactaaaaagggtcatttctgctaaataaattactaacactgccattaggccaatcacatgtctagtaacaatttgacatttcacttactattgtaacttttgatagatattgagactttacaaaaaaatattttaagaaaattttgttgaagaaaaaaacttgaatatcattcactataaaaaaaaggaaaaaatgtataggtttttgttacaatactgaacgtaaattgtgaccatgattccataaagcagtaacatttcaaactctaaaaattgttgatattaaaaacttgaatatcatccactataaaaaaaaggaaaaaatgtataggtttttgttacaatactgaacgtaaattgtgaccatgattccataaagcagtaacatttcaaactctaaaaattgttgatattaatctagtttacagaaaaagtagaagaaagaaaaaatgaaattagaaaatgttgagctgacatcacacgccacacacagaattgtatagaaaagaggaagtgtaattaagcatattcttccgcattaacctctctcctctctgtgtcatccaacctcatatactactgatctccatttccagatccccaagaacacaactcatcaacaagtactttaaatactctatctctctctttagagatctctctttctctctctctctctctctctctctctctctctctttctctctgtttctcactaattactctctacctctcttacatacacaaacacaatctctctcgcttctctctaattcacacatcaagataaaagaatcaaaccatccttgaaatgaatcctgtaattaattataggatttcagtttttgagttttttgttcttaatttggttttgtagttaattagggtttctttatagtttatctaccttgcatatatatatgtatgacatagacttacatgacactgaatcaggaggaagaggaaggaacgaataagaggaagaggagagagatgggaagagggaagatagagataaagaagatagagaatcagacagcgaggcaagtgaccttctgcaagaggagaactggtcttatcaagaagactaatgagctctctgttctctgcgatgctcacattggtctcatcgtcttctcctccaccggaaagctctcgcagtactgttccgaacccctcaggttaacttcttcttcctctccctctctcgaattagggtttcagagatctatacatacatgtgtatgtattatctaattaaatgagtaaataagagatatatagctcgtgcttgtgaacagacaattctcatcattagtttctgaagttagcaggtatcatgaatactatgtttcagattttaatttgacccagaagttaagaatctctctgatgctatatatatatatatatatatatatatatatttacttttgcagtatttgatttgtatatatctgtagatgcatgtatataatcattgtttattgatatcggtcaaattctgtaatttctacacctgccaagcaaagagatgttttttcaaagatttttcatttcttgatcaaccttttttcccatataatgtttacgacatatatatatatatacctagtatatatataagtcttatttgaatcattcgatataagtaccattaattataaaggatttttattaaaagttgtaaatctaagtcatgaaccagaagacgaatttattcacatctagcctaacaatataagaagaaaggtatgctgatatagtttgaattttgctatcataaaacaaaaatggggaaaatgtatactctctccgtttttttatataaaatattttatgaattgttttttgttcaaaaatagttgatgttctcacatatctatgcagaaattaattgcattttattgattttaagtgtttaaattttgtatattgtttttttattggttgaattgttttggaattaatgactaaaacatgttttgttttggaaatatacaaaattaaatgatttcttaatctatataaaaaaaccttaaacatcgtatataaaaaaacggagggagtatgttatttgatttttgtgttcctccaatgatgattaaagtcttgacgatgtacgattaaagatactatttgataacaatttattattaccaatgttgaataggatgcctcagctcattgaccgatacttgaagaccagtggaatgcgacttcctgatcctaatgacggccgggtaatatatatatacacgcatacttattcctttgtcttagccaattcaaaacaaagaatataacattctcacaaaaatcaataatcatttggagttttttgtgtgtatatataggaggaattgtaccaagagatggaagtactaaaaagagagacatgtaagcttgagcttcgtctgcgtccataccatggacatgacttaacctcccttcctccacacgagctcgatggtctcgagcaacagctcgaacattctgtccttaaagtccgcgagcgtaaggtaacgtaatatatgttcacatcaatatacatattctcttaaaactatagtgattattacacttttgtttgatctctcttttctatctctactgttaataaattgaagaatgagttgatgcagcaacagttggagaatctaagcagaaaggtcgctctctaattaatcattcttttgataagtactcttaattttattttcctctaattagtcatcttttataccgcggatttaatgatcattaccgtgtctatataaatatatgatcagaggcggatgctagaagaagataacaacaatatgtaccgtttggtaagtttggttactagagaacgtttaatttggttgcacattttcggtttgtgtgacataattattcaacgtattaattgcagcttcatgagcatcgtaacgcggttgaatttcagcaagctgggatagagacgaaaccaggggagtatcaacagtttctagagcagcttcagtactataatgatcatcagcaacaaccaaacagtgttcttcagcttgctacgcttccttctgagattgatcctaattaccatctccagcttgctcagcctaatcttcaaaacgatccaacggccaagattgattagtcctcaaaagtgaatcatttatgtcttttattactacctattttgattatagccaatgccttcttctgtgtctgttttgtgtggttatggaaacctaatattgtttgaagtacaattcacttgaaaagcgtttatggtctttctttgattaaataatttaatcttcattatcacacatttgccaactagagatcaactgtttatgtaatcgcagattttgagatacatttttggccatagaaagagtgggagacacatgagtaaactattcttaggttgttgacaaaaggaagaaccaacacctcagaatcttaataatgtgtgatcgacaagcttatcaaggaccttcactgaaaatagattttatatatttcagacagattagatcgcaatcccaaaaatagctcttataaactcagccaagattgcaaaaattcaatcaacttctgtagggtattgcaagggacgatcaagaagcaggaaaagagttctggaagaagaatcttcctttcctcttttcctcttcaatctgttttcatcataaagacgagaaaaaattgaatacttggcttcttgatcgctcgaataaccatcatcatcatctagatcccccaaacgctgcgttttttgttggctgaaccgtctacatccatgacaggaggatattttatatccgagagtggccatggaaaagagtaccaagaaggccgtgttactgcttttgtcgtgatctcctgcattgtggctgcaatgggaggtctcctcttcggttacgatatcggtatctcaggtttgtttcttcccaaccaagaaaccccaagatttctccttctctcttcttctttctcttctcatcatggcgggatatatttttttcaggaggagtgacatcaatggatgagtttctaacgagattcttccccgacgtgcaacgccaaaggcaacacaatacagggcatgaaacagagtattgcaaattcgacaatgagcttctcactctcttcacctcctctctctacctcgcggctctattcgcttccttcctcgcttcaacgatcacaaggctttttggccggaaaatctcaatgaagatcggaggtctcgcttttctctccggagctcttctcaacggt

SEQ ID NO: 48 - DNA, 1071 bp, Thlaspi arvense
  source 1..1071: mol_type = other DNA
atggctgcagtagaaagagtggagagtttagccaaaagcggaatcaaatctatcccaaaagattacgttcgtccgaaagaagagctcgagagcatcaacgacgttttccaagaagagaagaaagaagaaggtcctcaagtccccaccatcgatctacaagacatcgagtcagaagacgaaacgatccgcgagaagtgcacagaggagctgaggaaggcggctatggattggggagtgatgcatttgatcaaccatggtataccggtcgatctaatggagcgtgtgaagaaaaccggagaagagtttttcggttctcctgtggaagtgaaggagaagtatgccaacgatcaagccacagggaagattcaagggtatggaagtaagttggctaacaacgcgagcggacagttggagtggcaagattacttcttccatcttgtttatcctgaagataagagagatctaacactttggcccaagacaccaagtgattacattgaagcaacgagtgagtacgcgaagtgtcttcgtttgctagcgacaaaagtcttcaaggctctttctatcggtctagggttagagcctgaccgtttagagagagaagtgggtggtttagaagagcttcttctacagatgaagatcaattattacccaaaatgccctcagcctgagctagcacttggcgtggaagctcacaccgacgttagcgccttaaccttcattctacacaacatggttccaggtttgcagctattctacgagggcaaatgggtcattgcaaaatgtgtccccgactcgattgtgatgcacattggagacactctagagattcttagtaatggcaagtataagagtatacttcatcgtgggttggtgaacaaggagaaggttagggtttcttgggctgtgttttgtgagccaccaaaggaaaagattgttcttaaaccgttgccggagttggtgactgttgagtctccggctaagtttcctccaaggacatttgcacaacatgtcgagcataagttgtttaggaaggaacaagaggaattggtgtctgagaaaaaaagttga

SEQ ID NO: 49 - protein, 356 aa, Thlaspi arvense
MAAVERVESLAKSGIKSIPKDYVRPKEELESINDVFQEEKKEEGPQVPTIDLQDIESEDETIREKCTEELRKAAMDWGVMHLINHGIPVDLMERVKKTGEEFFGSPVEVKEKYANDQATGKIQGYGSKLANNASGQLEWQDYFFHLVYPEDKRDLTLWPKTPSDYIEATSEYAKCLRLLATKVFKALSIGLGLEPDRLEREVGGLEELLLQMKINYYPKCPQPELALGVEAHTDVSALTFILHNMVPGLQLFYEGKWVIAKCVPDSIVMHIGDTLEILSNGKYKSILHRGLVNKEKVRVSWAVFCEPPKEKIVLKPLPELVTVESPAKFPPRTFAQHVEHKLFRKEQEELVSEKKS

SEQ ID NO: 50 - DNA, 4065 bp, Thlaspi arvense
  source 1..4065: mol_type = genomic DNA
gtaaagtagacagctttttggaatttgcagagattatggtacaggaataaacactgaatcgagattatagccactgaatcaatcaaagccttgagcaaatgcgattgagagctgaaatttaacagggtttcgagccacaatactataaactagtgactgaaaaacttcgatcactaaagcttcagctagatttggtggaagaagaaatctaccactaaattctaaaaggctccatctttgtagaatcaattgtgaacggattctaggtaaaggatgaaaattgaagacctgattgctctgtggtggcttttgcaggcaataagaaggatcttcttctcaaggaaatcgatcttccagggctgagctgatcccattgagtcctcggcgacgacgacgacggaggagaaggagaagagaaagaagtggtgggtttgcgagaaacggcggagaaaagtcgagggcttgtcaaattgaacaacatcttgctacccattttccccgggagaagcaaggagagatccttttcctctgttttccgggaaggaacctgtggttgaagatgagttactgtgagcttcaggttccttctgatttttttattttattttaattcaatattttattatttatttatttaatttagtagagaggatttggagggaagaaattaggaaagataagagaggtgtggagatgaattcctaggcagatctctgatattttttccccctctcatcttaaagaaaaagaatatccacgtcagcaataaatatcccacctttctgtattttttgtaactttataagaattttatttactttaatattttttaaatgatacagtgatttctctttgtatataaaaaactttgaagtactaatttactttagacaaacaaatgtgatattattatttcctttgttcagttgatcttttatacaattagtctttttgaaactgaaaccagtcaaatactcaaaatgtttttagtgatgctaaaaattacagaaattatgataaaatgtggacattaaaaataaaataaaaaggtggataatgtacagacacctatattgattgaactatttaaaggtggacacgtggagatacgatttaggcacgtgcacacggacgcagaagaaacgccaccaaaagtctgacgttgatagtcatcggtttaactctattgggcttcttttttatgggcttttaaatccaaagcccttaccaagctaggacatactgtagtaacttctcttccagaattaaaagaaaacttttttgaccgttggatctcaaggatggtgaaaccatcagtcaacctctctcgttgacctgaccgtgaagtgtgttgtcactcactcacctgttcttcctccctacccaaccggtagctccacacttcctaattccttgattaattcttaattctaatggaaaattaatataattatctttgttatataagaaagcctctgcatatatttcatttgacatgcaacaaaatcggcaagaagaatagtagaacaaagtatttattcgttagttatcttacacactgttttttcctctgctttattaagtttctttacttacttactctgtttctttgctctgttttagcttttaaaagaagacaataaagatggctgcagtagaaagagtggagagtttagccaaaagcggaatcaaatctatcccaaaagattacgttcgtccgaaagaagagctcgagagcatcaacgacgttttccaagaagagaagaaagaagaaggtcctcaagtccccaccatcgatctacaagacatcgagtcagaagacgaaacgatccgcgagaagtgcacagaggagctgaggaaggcggctatggattggggagtgatgcatttgatcaaccatggtataccggtcgatctaatggagcgtgtgaagaaaaccggagaagagtttttcggttctcctgtggaagtgaaggagaagtatgccaacgatcaagccacagggaagattcaagggtatggaagtaagttggctaacaacgcgagcggacagttggagtggcaagattacttcttccatcttgtttatcctgaagataagagagatctaacactttggcccaagacaccaagtgattacatgtaagcttttgattcgtttgttttatcatttataaaacaaagttcttgctttggttatagtaacgttttttggatgattgtagtgaagcaacgagtgagtacgcgaagtgtcttcgtttgctagcgacaaaagtcttcaaggctctttctatcggtctagggttagagcctgaccgtttagagagagaagtgggtggtttagaagagcttcttctacagatgaagatcaattattacccaaaatgccctcagcctgagctagcacttggcgtggaagctcacaccgacgttagcgccttaaccttcattctacacaacatggttccaggtttgcagctattctacgagggcaaatgggtcattgcaaaatgtgtccccgactcgattgtgatgcacattggagacactctagagattcttagtaatggcaagtataagagtatacttcatcgtgggttggtgaacaaggagaaggttagggtttcttgggctgtgttttgtgagccaccaaaggaaaagattgttcttaaaccgttgccggagttggtgactgttgagtctccggctaagtttcctccaaggacatttgcacaacatgtcgagcataagttgtttaggaaggaacaagaggaattggtgtctgagaaaaaaagttgaagtttgagtctaatatgagtaaaaactccatgttaaagtttctcgtttcttttgtgtttatgtctttatcctgtatttgatgcgtcttgttgaagatgacacgaaatatttctaccgattgtgaaattgttaaaaatttcactctattataagttggttttatgtatcgccgaagtgacagatgttggaagaaatctagtcattggaaactgtattacattcgtgctaattgcatttcttttcaagtttaaaccaaattagtggaacgtctccggttctagtctgtgtgacttagttatagcttggtgaatagtaaaggaagctcagtaaatacgagtaacatagaaagatatttatgaaccacattgttgtattaaggacttgagaatattctgatttacatttccagtttgttcttttttgttatgctactaactgtaaaaaaactactcttctccctcctttaatgataattggcattccctgcttggaaagagttcactctattttccttgaagaccttaaaaccaagaatagattgcacaactcaatgattagtgttggaaaatagaaaaaaaaaaatcaaaaattgagtttcaagtttcacaaggctgcacctttggttgacgaaatcttgtgagagatccattgttttgctggagctccgatttgatagagagctgcacaggtttaatacgggtcaagagagcgtatacaaataaactagagtgtgtttaagaaagatccattacatcaaaccatgagctgtaccttgctgaaaagatctgttggtaaatctggctgaactctcttttccgaatgaaaactaaactcctgtgtttgcattcccaaaacagtttgcatcctcatcaggtaactcaattttacagacatacagaagatcaagcgcaaaaagaataattggtaaagactaccataccaaaggtactgttgtttctcgcttgctgtttttgaaaatgcccatgtctcctctgcttgagagtatctgttttgcaggagtgtgaaactatgtaaggtgtgacacgtataattaacgcaagcgaaatgagactcgagaaaggataataccttcttgttcagaggacgagctttaaaaacgtgttttccctccgagacatcatgcttaggtatatccataacgcttggtctgcaagaaaaaaatacacttttatgtttacattcacttcaaccacaagttgaagtgagaaatcaagcaatccttcttaatgttccatgtgactttat

SEQ ID NO: 51 - DNA, 645 bp, Thlaspi arvense
  source 1..645: mol_type = other DNA
atggttgtgaagctatacgggcaggtaacggcagcttgtccacagagggtcttgctttgttttctggagaaagaaattgaatttgagattgttcatatcgatcttgatacatttgagcagaaaaaaccagaacatcttcttcgtcagccatttggtcaagttccagccatagaagatggagatttcaagctttttgaatcaagagccattgcgagatactacgcgaccaagtactcggaccaaggcacgaaccttttgggcaagtctctagagcaccgagccatcgtggatcagtgggccgatgttgagacccattacttcaacgttctggcccaccccattgtgattaacctagtcatcaagcctaggttaggcgaagaatgtgacgtcgttttggtcaaggacctcaaggtgaagcttgaggaagttttggacatatacgagaaccggcttgcttcgaaccggtttttggctggtgatgaattcaccatggctgatttgacgcacatgccagctatgcggtatttgatgggtataatcgatataaaccggatggtcaaggctcgggtgaatatgaaccggtggtgggaagagattacggctagaccggcttggaagaagcttatggtgatggctggttcttga

SEQ ID NO: 52 - protein, 214 aa, Thlaspi arvense
MVVKLYGQVTAACPQRVLLCFLEKEIEFEIVHIDLDTFEQKKPEHLLRQPFGQVPAIEDGDFKLFESRAIARYYATKYSDQGTNLLGKSLEHRAIVDQWADVETHYFNVLAHPIVINLVIKPRLGEECDVVLVKDLKVKLEEVLDIYENRLASNRFLAGDEFTMADLTHMPAMRYLMGIIDINRMVKARVNMNRWWEEITARPAWKKLMVMAGS

SEQ ID NO: 53 - DNA, 3574 bp, Thlaspi arvense
  source 1..3574: mol_type = genomic DNA
ttaaatgtcggattccaattgagttaagtaagtctcatctatatgtaaatgggtttttggaatagtatcatcttataatcattttacacagaatcaaagttattagccttgctaaatctaggttgtattgatcgaatgatcttcgaaaaaactcagttagctgtaaatgctttgcagggtatgttaatgaatgaaaatctacataatcacatccctcttgaactaatatgtctgtttatagatcaaaaacaagttaggcatgtgaaagttttgtaatcttgttctggttatggtatttgtgcaagctttcgaactcgtgtataaaggttttcttctcattttcatgttacaacaacgcagagatctcaggtcaaggttaccaccacttcagatccactcacacgatgctcttatccaagaagtccagctttggatctcggcttcacttcagctatttttctaatgatggctcagataatcgtcagcgtcggaagcggctgtctctgttgtagaaaaggtcctgctccttccagatctaattggattatcgccttaacctgcttcgttgtttcctggtaatcctcatcatttctttctcctatcgagctttcctacttcacaattttgctggacagacacaagtgacgaatctttgtgtttactcttaggttcacttttgtgatagctttcctcttgctgctaaccggagctgcactcaacgatgaacacactgaggagtcaatgtatgccggttactactcctgctacattgtgaaaccgggagttttctctaccggttctttgctttcgcttctcactgttgccctcgggattgtctactatttgtgtttgacttcgagtaaacaaaacgttgctgacacagcgacgacggcgaaccgaggaggaggtatagcaatgggacagcctcagattccggagagagtggaagatcctgtctttgttcatgaagatacttacatgagaagacagttcacttaaaaacagaacatggctttctttggatacacgttaggttttaggatgataattagataaacaagagatgctgttttttttttttggggattttatctttgtgattttagtatgtgaaactaagaccatgaaacttggtagctggtaatgatgattaatgatgattgataacgtacagaaaaccaaacaaacgtctccttttacttatctatgtgaatttaaagtggttgttgggaagtgttcacaaaaatcagaaattgaaataaataattaacctatccaccggtccgaccaaacacgggacatctaatagaaatcaattttgtttatctcgaatcataagacgaaaactactgaaatttttatgttaataagtttgtagagcaactttggatgatatccaccgttagtggaacaaccaccacatgctctacccaaccagcacaacaaccagctccttttaaatgtttttgagtctaataaaatgccaacacatctactactctcacttcttcacatttataaataagatccagagaagcaattttaaaataacacattgaaattgtttcaaagcttatttttttttaaatttatatcaataaaaatttggttgcaaagttattgtaacgcttatagaatggttgtgaagctatacgggcaggtaacggcagcttgtccacagagggtcttgctttgttttctggagaaagaaattgaatttgagattgttcatatcgatcttgatacatttgagcagaaaaaaccagaacatcttcttcgtcaggtcaaacattttatattttctaattttgaaaagtcatgaattgtatttaatatcattaatgttttcttttagccatttggtcaagttccagccatagaagatggagatttcaagctttttggtaagatcctaataacagcattgtaaaacattctttaatacttgttttatatcattaatatgtagattgtgttttgaaatttggcgtgtgtgctcagaatcaagagccattgcgagatactacgcgaccaagtactcggaccaaggcacgaaccttttgggcaagtctctagagcaccgagccatcgtggatcagtgggccgatgttgagacccattacttcaacgttctggcccaccccattgtgattaacctagtcatcaagcctaggttaggcgaagaatgtgacgtcgttttggtcaaggacctcaaggtgaagcttgaggaagttttggacatatacgagaaccggcttgcttcgaaccggtttttggctggtgatgaattcaccatggctgatttgacgcacatgccagctatgcggtatttgatgggtataatcgatataaaccggatggtcaaggctcgggtgaatatgaaccggtggtgggaagagattacggctagaccggcttggaagaagcttatggtgatggctggttcttgaattatttcgaatttatggtgatctgaaccaaataagcttcatattttctgtactattttctttatctatgttttgtaagtttcaattgataaaataaatttacttttaaagatttaaattcgttaatattttctttatctatgttttgtaagtttcaattgataaaataaatttacttttaaagatttaaattcgttaattctcaattttaaaggggactatagatttacagttatcattttgttacgtattactacaaattgctgaattgttatagaactttttttccaattgtttgtgaacctaatactttaaatctgaatagacatcatgtatttaattatttcccatgttatattttcatctagtatatatagttcattcatttgtagccatgcagatgcacaatgaatctcgattttttttttttttgtgcgagcacaatgaatctcgatctcttagtgtttttgaattcagtaacttctttgcatctttcactaaactatctctccaaccaaaaaaattcatatttcttcagcagccaagagagaaataaaaaatttcaaaaattactttttacatagagaaaaagaagggaacatccgcccatttatatgtatattagttaacatgataaaaaatccgaccctaagttttttcattaatcacaaaagccctctctttggttgtttttcttggcttctctcattcatgtcgacttagaagaagaagctaatcttgagcttgaagtctttagcactgattttgcataagccaatggcaaagctgcaattttcttggctttccctacataagctctctttgtaaaattgttgtaatcattcgcttcaatctcgtccagtatcctcctgtataatagcagcgatgcccatacctgaaaaaattgcacagccaagtgtaagggggttaaatcgatccaaacaaaaaagctttggggcgaaaacaaaacaaaaatgtaaacggtaaagtgtaaacgtgggggcttaagagtgttgttagagacacttaccggccatctgcttgcggcgtcgagctccgtgacgcctttctcagcttcgtcgaagaacattcttgctcgtttaagctgcattttcatgaagttt

SEQ ID NO: 54 - DNA, 1155 bp, Thlaspi arvense
  source 1..1155: mol_type = other DNA
atggttagtcacaaagagaccgtgtgtgtaacaggcgcatcgggattcatcggttcatggcttgttatgcgattattggagcgtggttactttgtccgtgccactgttcgcgaccccggaaatttgaagaaagtgcaacatcttgttgatttacctaacgccaagacgcaactcactctatggaaagccgatttatctgatgaaggaagctacgatgacgccataaacggatgcgacggcgttttccatgtagcaactcccatggattttgaatcaacggatccggaaaacgaagtgataaaaccaacagtgaatggagtgttggggataatgaaagcttgtgataaggcaaaaacagtacgaagaatcatctttacttcttctgccggaactgttaatgtcgaggaacatcagaaaaatgtctacgttgaaaatgattggagtgatcttgactttatcatgtccaaaaagatgaccggatggatgtatttcttgtcgaaaactttagccgagaaagcagcgtgggattatgcgaaggaaaatggattagacttcattagtataattcctacattggtgatcggtccattcataacaacatctatgccgcctagcctcatcaccgcgctctctcctatcactcggaacgaggcacattactcgatcataagacaagggcagtacgtgcatttggacgacttatgcaatgctcatatattcttgtacgaacaagctgatgccaagggacgttatgtttgttcctctcacgatgccacgattcttagtatctctgaatttattaggaaaaagtaccccgagtataacgtgccttcaacgtttgaaggtgtggatgaaaatctagagagcattgtgttcagttcgaagaagctgattgatatgggatttagctttaagtatagtctcgaggagatgttggtcgaatcgattgagacatgtcgtcaaaagggttttctcccggtttctttaccagatccatcaatatttgaggacaaagttccgactagtgatgacaagattgagcacaaaaccggagctggtttacccgatgatgtggtgccctgtaagaagacagaaccggtggtaatccgcgagaaaaccgatgcttgcatgccggcagagcagatgtgtgcttag

SEQ ID NO: 55 - protein, 384 aa, Thlaspi arvense
MVSHKETVCVTGASGFIGSWLVMRLLERGYFVRATVRDPGNLKKVQHLVDLPNAKTQLTLWKADLSDEGSYDDAINGCDGVFHVATPMDFESTDPENEVIKPTVNGVLGIMKACDKAKTVRRIIFTSSAGTVNVEEHQKNVYVENDWSDLDFIMSKKMTGWMYFLSKTLAEKAAWDYAKENGLDFISIIPTLVIGPFITTSMPPSLITALSPITRNEAHYSIIRQGQYVHLDDLCNAHIFLYEQADAKGRYVCSSHDATILSISEFIRKKYPEYNVPSTFEGVDENLESIVFSSKKLIDMGFSFKYSLEEMLVESIETCRQKGFLPVSLPDPSIFEDKVPTSDDKIEHKTGAGLPDDVVPCKKTEPVVIREKTDACMPAEQMCA

SEQ ID NO: 56 - DNA, 4705 bp, Thlaspi arvense
  source 1..4705: mol_type = genomic DNA
cctccgttattatggagccttgtaattagtgttcagaaaatcaatcccaacaatattatctaatattttctatagaaaaaatatagtttaacaagtgtttagatgcctcatatcaaactctctaagattgtgtttctaatctagtactaagtacaagtccaatgactccaaccacaatcatatttattctacacatgaggggtgaaattttaattgttaaataaaaaaatatagatacaattattctattctatagtttatatgttgacaaagaaatctttggtaaattttatttttaaaagtcaaaaagatatttgttaaaagtattgttgtttgaggaaatgctccaaaataatccagaataagaaaataatatgaaacggtactccattgagaaaaaactgtgaaaataacccatattttatgattttttttaaataccagtgctacatttctaactatttttacttgtagtctaatggcatactgaatgcagagtactggcagactgattggtcttacaattgaatatagactattggcagactaaatgcaaattactgacagactaacgacagattaaaagcatattagtggatcctgcttatggatcatttgaaaaaggttcatgtttggtaacaaaattaccaaatgaataatttcaaaaattatcccatttgagtaaagtatatttttatttttggctaatttcttctttgaattaacccaaattatggtgtttgtaaattgtaactgtgatttttttttacatcaagaagtgaatggttgacaaaaaaaaaagaatgattaaggtttaaatactaaactcgtatatttaaattataaacttttcgaattcattttttttaattttatcaatctttagaaaaatattatatgtttctagaaagtttctataaattctaatgtgtttaccattaaaaatatattatttattttcctcatttgaaatatcaatttatttatatataactcataattttaaaaatttatatatcaactcatgtcaaaattttaatttcatatcagtttatttcaataatgtttttacacgtattaaaatctaatcaattacactcttttattattaacaaatttgacgtattaaattttatatgataaattttgttaacgtattaaaataatataaactcttcttgtagtttagtaacaaaataaaaaaattacaaaaaacaataagtaagaaaaggaaacttcaactcttgtcgctatctcactaaacaaacaagcaaacccattcggcgtagttcacccaccagtacaactaaaactatatcctaaaaaataataaaatcaaacttaccagtttgtcacgtaccacacaacccagtccttcgccaaccaacgttcctcacgtgcttcgccggttggtactcacgtgaccggcagctttctaatagcaattctcaatacatatataatctcttcataccaaagctacatatatagtctcttcataccaaagctacatagcaaagtctatcccaaagcacagtccatctttataatacacaaaaatggttagtcacaaagagaccgtgtgtgtaacaggcgcatcgggattcatcggttcatggcttgttatgcgattattggagcgtggttactttgtccgtgccactgttcgcgaccccggtacgtatatatgttcttacaaactaactcgttaattaatttttcctaagattaattaaatctatgtgtggctaatttacgggttttattgggttatttatataggaaatttgaagaaagtgcaacatcttgttgatttacctaacgccaagacgcaactcactctatggaaagccgatttatctgatgaaggaagctacgatgacgccataaacggatgcgacggcgttttccatgtagcaactcccatggattttgaatcaacggatccggaagtaagttataatatgaacctcttttaggtttcatatcaaccctaaaagatcttgttggttaaatttttttttttttttaatcagaacgaagtgataaaaccaacagtgaatggagtgttggggataatgaaagcttgtgataaggcaaaaacagtacgaagaatcatctttacttcttctgccggaactgttaatgtcgaggaacatcagaaaaatgtctacgttgaaaatgattggagtgatcttgactttatcatgtccaaaaagatgaccggatgggtaaatatatataaattatatatcaaacatcacactaaccctaagtttattcttcttcatagttatttatgttttaataaaatgtttttggcagatgtatttcttgtcgaaaactttagccgagaaagcagcgtgggattatgcgaaggaaaatggattagacttcattagtataattcctacattggtgatcggtccattcataacaacatctatgccgcctagcctcatcaccgcgctctctcctatcactcgtgagctctcacttaatttctactctttttgtaaactaagagatttcttgaccttaggccaggtcttgctcataaaatcaatgtccactgagcaatattctattttataagcctaataatcataaatggcaaggaaaacaacctatttttttttaaagaaccttaacgtctaaccaaaaattacaaaaagttatatggacccaatgcaaatacatctttggcacatgccaagaaccggatcgtaggaagatctttctggctagcgactagagcatgtcaactagtctcttctatcttccatcttcttttgttggaatttgaaatgttaattttttttaaaaacggtgaaaatgtttcagggaacgaggcacattactcgatcataagacaagggcagtacgtgcatttggacgacttatgcaatgctcatatattcttgtacgaacaagctgatgccaagggacgttatgtttgttcctctcacgatgccacgattcttagtatctctgaatttattaggaaaaagtaccccgagtataacgtgccttcaacgtaagatttatagatttaaattacggagtttaagccttgttttgcttaagcaatcaagatcgtttgctgaaaaactatttggaacaggtttgaaggtgtggatgaaaatctagagagcattgtgttcagttcgaagaagctgattgatatgggatttagctttaagtatagtctcgaggagatgttggtcgaatcgattgagacatgtcgtcaaaagggttttctcccggtttctttaccagatccatcaatatttgaggacaaagttccgactagtgatgacaagattgagcacaaaaccggagctggtttacccgatgatgtggtgccctgtaagaagacagaaccggtggtaatccgcgagaaaaccgatgcttgcatgccggcagagcagatgtgtgcttagagatttaaccggtatctattatatatcaattgtcgtatcgttttagtattggatgtgtgttttgaatttgttactttctgaatcgtagattattattgaagggtggtatggactgattctgatagtaacatgattgagtgtaacattatgaacttttacatatttaagaagcagagtgatatttaaacaatgttgccttgagtcaaattagtcgtgtaatgtcgcttgaatgcttccataatctataattagacaatttcaacatctcaatcgcaggcatgcatttcttaacaaagagttatatattcggtggtcactggaaatattttatacatatataatataatttaactactatgcagattacagagtataagaaaacaattcttggctaaatagattttcagttacaaaataaagaaaaaccaaatgactgaactttttttatttgaagaacaaaaaatgaaaatttagtcgttcgagttaatttacggatcctatcagctaaaaataatttagttctgttgagatgtccatgctttttttggaatttggattttcctttttccatatgtgaaacctttccatataccaaaaactctatcatcaaactacccagcctttgtatctctatgccaaaaaaaaaaaattaaacaaaatctttaatttgaagtcggactgtcggagtatatggtttttcttgtacgtacgttttccaaatgcttcagtaaattgctcttcgaagtctttcatcgtcagctggaaagaaatacaaaagtgattcctcttgtgcctcaaatgttcttttgtagcttaggagaggatattgggagatgggttttaaagaatttttcaaattttgagattctattgtttataaatttttaaaatcttaatagttaatattgttattggttgaaagattttaaaattctatccaaaatcctttgttatttaaaaaatttagcttttaaagattttatgatttattaaaatcttgtgttattggaacatgaattttaaacaatctaacttataaaataattctttcaaaatactacctatatagcttagattctcaaagtcattataataaaatattttgatagattttttaaatataaaaactctttccaaatttaacaaatattttttacaagtttaacaaatctcccaactcttgaaatcaatcaaaactttataatttcatctcttaatgaccctcccttactctttgctttttgttgtttgtttctcaattc

SEQ ID NO: 57 - DNA, 1188 bp, Thlaspi arvense
  source 1..1188: mol_type = other DNA
atggtgatgggtacacaaccgtcgttggaagagatcagaaaggcacagagagcggatggccccgcaggcatcttggggataggcacggccaaccctgcgaaccatgtgatccaggcagagtatccggactactacttccgcatcaccaacagtgagcacatgactgacctcaaggagaagttcaagcgcatgtgcgacaagtcgatgatacggaaacggcacatgcacctgacggaggagttcctgaaggagaatccggacatgtgcgcctacatggctccttctcttgatgtgaggcaggacatcgtggtggtcgaggtccctaagctagggaaagaggcggcagtgaaggccatcaaggagtggggtcagcccaagtccaagatcacccacgtcgtcttctgcactacatccggagttgacatgcctggtgctgactaccagctcaccaagctcctcggtcttcgcccttccgtcaagcgtctcatgatgtaccagcaaggttgctacgccggcggcactgtcctccgactcgccaaggacctcgctgagaataaccgtggtgctcgtgtccttgtcgtctgctccgagatcacagccgtcaccttccgtggcccctctgacacacacctcgactccctcgttggtcaggctctcttcagtgacggtgctgccgcgctcattgttggtgcggaccctgatgcctccgtgggagagaagcctatcttcgagatggtgtctgctgcacagaccatcctcccagactcggacggagccatagatggacacttgagggaagttgggctcaccttccatctcctcaaggacgtccctgggctcatctcgaagaacatagagaagagtctagaagaagcgtttaaaccgctcgggataagtgactggaactctctcttttggatagctcaccctggaggtcctgcgatcctggaccaggttgagttaaagctaggactcaaggaagagaagatgagggccacgcgtcacgtgctgagcgagtacggaaacatgtcgagcgcgtgcgttctcttcattatggacgagatgaggaggaagtccaaggaggatggtgtggccacgacaggagaagggttggagtggggtgtcttgtttggtttcggaccaggtctcaccgtagagacagtcgtcttgcacagcgtccctgtttga

SEQ ID NO: 58 - protein, 395 aa, Thlaspi arvense
MVMGTQPSLEEIRKAQRADGPAGILGIGTANPANHVIQAEYPDYYFRITNSEHMTDLKEKFKRMCDKSMIRKRHMHLTEEFLKENPDMCAYMAPSLDVRQDIVVVEVPKLGKEAAVKAIKEWGQPKSKITHVVFCTTSGVDMPGADYQLTKLLGLRPSVKRLMMYQQGCYAGGTVLRLAKDLAENNRGARVLVVCSEITAVTFRGPSDTHLDSLVGQALFSDGAAALIVGADPDASVGEKPIFEMVSAAQTILPDSDGAIDGHLREVGLTFHLLKDVPGLISKNIEKSLEEAFKPLGISDWNSLFWIAHPGGPAILDQVELKLGLKEEKMRATRHVLSEYGNMSSACVLFIMDEMRRKSKEDGVATTGEGLEWGVLFGFGPGLTVETVVLHSVPV

SEQ ID NO: 59 - DNA, 4151 bp, Thlaspi arvense
  source 1..4151: mol_type = genomic DNA
cgaatccgcatagagaagctgaagctcaggtttctcaattatttcttctttctttttcaaaaggcttatcattgacttgtctctgtttttttttttttttttttgtgatcattgattcagtctctccaacttgatgaaaaagataaccatccaagagcccacctttgagagaattattgtagtatacaggtacaagagtagagtaatggtgaaatctttggagggatgtgagtttgattctcattttggctttggattcacatacacgcaggagagtttcagggaagagagaatcagaaaggaacatatatgtgaaacacttcaagagcattcctatggctgatatggaaattgtgcttgtaagcatccattaaccaacactttgtgctcaaatgtatcttactaattataaattaactgattgctcataacggcacagccagagaagaaaaatccaggtcttacgccactggactgggtcaagtttcttgtctctgctgccattggactggtcagttctgctacactattctaaagactttaataatcagactctgaaaattttgatttctcaaactctgcttttacaggtcacagtggttagttcagtgagcctaaaaaaaactgacatcagagtcattgctgccatacttagcacggtcgtggcctactgcgttaaaacatatttcacgtaatctacactcaataatcagacaacaccctcgcttatagctaaattaatccttaattagctctgtctcttcctctgtatgaaatgtaggttccagagaaacttggtagattatcagagccttatcacaagatctgtgtatgataagcagctagacagtggaagaggcactctgcttcacctctgcgatgaagtcatccaacaagaggtgctaataaatagtccttttttcttatttttcttatgtcatattcttgtgttttgctaattaaaaaactgatcaaacgcaggttaaagaggtcattatttccttcttcatgctgataaagcaagggcgtcccacgagcaaggaggagcttgacatgcaaagtgaagcattcatcaaagaagaattcaacgaaagttgcaatttcgatgtggatgatgctgtcaagaagcttgagaagcttggacttgtctctcgtgtgagtctccttcatctctcttctataatcttttctttttctccacgcatatgcttgtatatactcagtaagtaaactaatattgtgaaaatggaaagggttggtcaggattcagaagacaagtatagatgcgtgaatatgaaggaagcaaacgagataatgggaacaacgacggaagagatggtactcaaggcaagaagaggtggtgaatatgaagatgaagaggcagcagagactgagccacggatgaatcctcaagatgaactcacagcaaaggaagaacgttatcaatctcaattagacgagttcgagaccttgtggttgtaaaaagatttgacgtcattcaagacaaataaatttgatattgtattaaagaaaaagaaaaaaagacataaaggcagacaaattaattgaaaggacccatcaacaatgagtccaccacatttcacatttcacactaaatgaattctcccttaattatttcatacataatttatattaaaatgaaaaacataagactcgatgatggaaagtatgtgtaggtaggtaggcatataagaggagagcgctctgtatggtgatgggtacacaaccgtcgttggaagagatcagaaaggcacagagagcggatggccccgcaggcatcttggggataggcacggccaaccctgcgaaccatgtgatccaggcagagtatccggactactacttccgcatcaccaacagtgagcacatgactgacctcaaggagaagttcaagcgcatgtgtgagtatccctcttaatactccctattttgtatctcttcatttcttttggcatatggttcccatagttaacaattactgtaacaggcgacaagtcgatgatacggaaacggcacatgcacctgacggaggagttcctgaaggagaatccggacatgtgcgcctacatggctccttctcttgatgtgaggcaggacatcgtggtggtcgaggtccctaagctagggaaagaggcggcagtgaaggccatcaaggagtggggtcagcccaagtccaagatcacccacgtcgtcttctgcactacatccggagttgacatgcctggtgctgactaccagctcaccaagctcctcggtcttcgcccttccgtcaagcgtctcatgatgtaccagcaaggttgctacgccggcggcactgtcctccgactcgccaaggacctcgctgagaataaccgtggtgctcgtgtccttgtcgtctgctccgagatcacagccgtcaccttccgtggcccctctgacacacacctcgactccctcgttggtcaggctctcttcagtgacggtgctgccgcgctcattgttggtgcggaccctgatgcctccgtgggagagaagcctatcttcgagatggtgtctgctgcacagaccatcctcccagactcggacggagccatagatggacacttgagggaagttgggctcaccttccatctcctcaaggacgtccctgggctcatctcgaagaacatagagaagagtctagaagaagcgtttaaaccgctcgggataagtgactggaactctctcttttggatagctcaccctggaggtcctgcgatcctggaccaggttgagttaaagctaggactcaaggaagagaagatgagggccacgcgtcacgtgctgagcgagtacggaaacatgtcgagcgcgtgcgttctcttcattatggacgagatgaggaggaagtccaaggaggatggtgtggccacgacaggagaagggttggagtggggtgtcttgtttggtttcggaccaggtctcaccgtagagacagtcgtcttgcacagcgtccctgtttgacttttacaattcaagtcttttagagtttgatcgatgagtgagattgtgtactatgcaagttatgtatatttgatggcaagcggagagtgggagtttatattaacgagagaaagggagaagagagagtgtggtaggttagatggacgggcagatgaagcactacgtgtctatgtgttagctcccttttatgtggttctccttcttgcttcccttttatttcgttacttaccaagaatattgaatggtggtttttttattgattttacgtatattcgcaacaacaagtcatattaatttctatgtgcgtaattattatatattcgatgtatatacatgtaaagatacgtacggcctactggagaggttagttgtatagattttcccacacgtgcatacttaactccatcattagctcctactaatctaattttccttcttaatatacctgataatcctataactaactaaaaattacattaggtacgtctcgttttctctctcccaccccatcatgatgatagtttgaatctgctcctttttcggcttccaacaacgcaagatgcatttcgcatcccatcataatgatatttgtgttgttgctgttctttatgttagactaataaaagatgcatttgtaagcttttgcctcattaattttattcggaaaaaaattgaatatgcgtaatatcacatcgttttttgttagtattcatttattcaattcatgtcttaataatgttgtagatatttttattggaaaaataatatcaatgggcccataaaagaaggtgggccctagagctggttatgcttagccatgtgggcagaatataaccagagtgtgttgtcattgtggtaagtaggggcactccaatgcgggtgtttttatcaacccggcccggcccaaagcctatccgtcgaaaacccgtgtccatcaaaaactcgccaaactagcggttatatttagggttgggcaaattatccgttatatttgattcgatctgctatttgtttcgattcgattcgaaaaatccagatatccatagctttacggagcaaagcaaatactaaattttgatattcgttaaaaacggagcaaatcacaaatattaaaattttaagagtcggatatccgatctgctctaata

SEQ ID NO: 60 - DNA, 759 bp, Thlaspi arvense
  source 1..759: mol_type = other DNA
atgtcttcttccgcatgtccgtcaccgttaccctcagtcagcaaacttcatgtcgattccgttacttttccaccgtccgtcaattcaccggcttcctccaatcccctattcctcggtggcgcaggggtgcgagggttagatattcaaggaaagtttgtgattttcaccgtcatcggagtttacctagacgctgtcgccgtcccgtcactctctgttaagtgggagggcaaaactacagaagagttaacggaatccgtcccttttttccgtgaaatcgtcacaggtgcgtttgagaaattcataaaggtgacgatgaaactgccgttaacgggacagcagtattcggagaaagtaacggagaattgtgtggcgatttggaaatcgttagggatttacacagagagtgaagctaaagctgtggagagatttttggaagtcttcaaggaccaaactttcgctcctggtgcatccatcctcttcgctctctcccctaacggctccctcacggttgcgttttcgaaagacgatagcattcctgaaaccggaaaagcggtgatcgagaataaattgttggcagaggcagttcttgaatcaataattggaaagaagggtgtgtctcctgggactaggctgagtatagcagagaggttagctaagctgatgaagaagaagaaggtcgaagaagatgcatcatcactgactgatcaagaggaagctacagatctctccctcggagataaattggccaaagagaactga

SEQ ID NO: 61 - protein, 252 aa, Thlaspi arvense
MSSSACPSPLPSVSKLHVDSVTFPPSVNSPASSNPLFLGGAGVRGLDIQGKFVIFTVIGVYLDAVAVPSLSVKWEGKTTEELTESVPFFREIVTGAFEKFIKVTMKLPLTGQQYSEKVTENCVAIWKSLGIYTESEAKAVERFLEVFKDQTFAPGASILFALSPNGSLTVAFSKDDSIPETGKAVIENKLLAEAVLESIIGKKGVSPGTRLSIAERLAKLMKKKKVEEDASSLTDQEEATDLSLGDKLAKEN

SEQ ID NO: 62 - DNA, 3963 bp, Thlaspi arvense
  source 1..3963: mol_type = genomic DNA
ttccccacaaacaatgtgtgtgtcagctatatatttatgggaaggctgaaacgtttaaatactagcctctgcatcgtttgttgtaattttgtgataaaattgtaacatatttaatcgttttatctctaggtacttttatggaatattgtaaaagaattctatttttgtgtaaaatccaaattagcgtattatacttgaatacacaagcatttcggcacatagttcaattggggttaattcatgaatcatttttaattcaaaaatttcgacccatcaaaattagacaatgaccaaagaaattataaaaaatgagatgatgtttgaaaatgtttagtgaggaagtgaaggtatagattatagacgtttattgtcaaatttcaacggatgttatatacgttgttaaatttaaaacaactttagaatatatatggcgcgtgattttgttaaatcgactttggtaggaaaatgttattttgcgattttgtcaagaaaacgtaattttgtgattttgaccaaaaaaaatgttatttacagtaatagaaaaaaataattttataatttaaaaaacatgatttttgattttattgaaattttttttttttaattttagtgagaagtgattgcacatttttaatgggaaaattttctacaattttaattaaaaaaatgatttcagcataattttagtaaaaaaattgtgattttacagttttataaaaaaatatacgtttttatttttttgaaataattgaaaaatctcatttatattatgttgatttattcatctgaaatttgcatttaaatattctatctaaataaaagtattttaattatttgttattttaaaatagattatttccattttttatcaataaacaaccccatatgttgttaaacaaagaaagaaaggacaatctatatttcttagttatttttattattatattttctttattctttattctctttatttatattatttttataatgttcattaattaaaacctacctcttacagaacttttttgggttgttttaaaaggatcagacatagtgtaaactaaaaaattaaactgaaccaaaccaaactatgtcttatacttatcaagtaatatacactacatgataagcttaaactagattctatctttatcataaattaattttatctttatcacattgtggtctacataaatcctcattacataagtatcttaattaaatcttctagattcttccttaacagtaaaccaagattaaaaatgatctgatttgaactgataaaacctaaactaaaaagaaattggcatacctaccgactctaaagcggtcagagttcccgcaaccaccaaaattataaaccactgaatcttccaatcaacaaaaccacgtgtttacccatccaacactcgtaagctattgctagttgctacctacctccatcttctcttataattaccaatctccatcaaattcttttttacttttttttacattataatcaaacctaacaccctcaaagtcaaaaccatgtcttcttccgcatgtccgtcaccgttaccctcagtcagcaaacttcatgtcgattccgttacttttccaccgtccgtcaattcaccggcttcctccaatcccctattcctcggtggcgcaggttcgagtgctgtttaattcatttgctcttgcagcattcttttttttttttttaaatgcgttttttgttgcctctttgagtttctctgtttcttgctaacttacgcaggggtgcgagggttagatattcaaggaaagtttgtgattttcaccgtcatcggagtttacctagacgctgtcgccgtcccgtcactctctgttaagtgggagggcaaaactacagaagagttaacggaatccgtcccttttttccgtgaaatcgtcacaggtgcttgtcatgcaacaaactgttttaagtcaaaaagggattttaatttgtttagaccaaactatttgaccgtcattaatttattattaccatttttagttaattatgatttttttttgtttttgggcacgattaggtgcgtttgagaaattcataaaggtgacgatgaaactgccgttaacgggacagcagtattcggagaaagtaacggagaattgtgtggcgatttggaaatcgttagggatttacacagagagtgaagctaaagctgtggagagatttttggaagtcttcaaggaccaaactttcgctcctggtgcatccatcctcttcgctctctcccctaacggctccctcacggtacttcttgtcctatcacacagctttgcgtttgcgtttacattactattacgaactgtttacaatgaaacgcaaattaatgtagaaatagcgtttaaaacgaactgtgcccaaaacatgtatttttaagtaagatttggttttaaaaattgttttacgtgtattaaacgcaattgacgttagaaaaacagtcgtaggttgtaaaatgtctttgttgtgaaaaaaaaatcgttttgcaggttgcgttttcgaaagacgatagcattcctgaaaccggaaaagcggtgatcgagaataaattgttggcagaggcagttcttgaatcaataattggaaagaagggtgtgtctcctgggactaggctgagtatagcagagaggttagctaagctgatgaagaagaagaaggtcgaagaagatgcatcatcactgactgatcaagaggaagctacagatctctccctcggagataaattggccaaagagaactgatcctatgccgagatttttcttggtttctgagggattttatgtttctgttatatttaatcctattccatcgcatgtttaatttatctctgttcgtaagaataattaaataacctcatggtattggatcaaagtttccaaacaaaacaaaattgtattgtcaaatatttaatacaagccaaacttgataaacatttagttctaggcttgatcacacggatccgcaaggttaagtaattggttaaccgaagggaagggaaaacacctacacgaatcccggaccgggcctaaattcttttaactagaacacggcccaatctgtagaccagttcggcccattgtagtatcaaaaatattccataaacgaaatcatttgatttcaaatggaggaaatcattaaattagcagacgcggaaaaccactatctcatcaaaataaattgcgaaatttattgaataaactaatgaatcaataaataaatgaaatggtccaaccatctaaaaattgattttctaagatgtcactgtatcaatatcacccattcatgttcatataaaccctacccgccagcataatgcatattgagtattgacgacttataaacaaaagaagaaatcacttacagaaaaatgatttcttgaggaaatagatcacaggatgtgtatgttgattaatgacctagggtacaataatgcagtttgattcactactagacccataattttttttttttaaaaataaaaagggctttcatgacccataaaaattattattatctttttttcccataaaaattatttgataattgtttacgtgtttgtttgttttctcgttcatattgatatttctctcatccgaattcttgcattttcaacgtgtcaattatctttttaaaactacgtaaatactattatgataccttgtaggcttgtactgaatatttgtgagtattttaggctttataaattcttatgccgactttgttatcaagccttcgacacattttctgtggcgttcttgagactataaaatttgggagacgattgaaccattttgtttttatctataatggtttttcttttgtatcctttatttgattttttttcttctttttttggctggttctagagaccttcttagccacagtgattcttctgtcatcagttcatcaaatcctgaaaagagcatcatagc

SEQ ID NO: 63 - DNA, 1239 bp, Thlaspi arvense
  source 1..1239: mol_type = other DNA
atggctccagggactctcaccgagctcgccggagaggctaagctcaactctaaattcgtccgggacgaggacgaacgtcccaaggtggcatacaacaagtttagcgacgatatcccggtgatatctctcgccggactcgacgatgttggtgggaaaagaggagagatctgccgtaagatcgttgaggcttgcgagaattggggcgtgttccaggtggtcgatcatggtgtcgataccaatttggtagaggatatgactcgcctcgctcgcgacttctttgctttaccacccgaagagaaacttagtttcgacatgtctggtggtaagaaaggcggcttcatcgtctctagtcaccttcagggagagactgtgcaagattggagagagatcgtgacgtacttctcgtacccggtgagaaacagagactactcacggtggccagataagccggaagggtgggtgaaagtgacggaggagtacagcgacaaactgatgggtttagcttgtaagcttcttgaggttttgtctgaagctatggggctcgagaaagaagcacttaccaatgcttgcgtcgatatggaccaaaagatagttgttaattattaccctaaatgccctcagcctgatctcaccctcggactcaagcgtcacactgatcctggaaccatcactttgctgctccaagaccaggtcggtggattacaagccacacgcgacgatggcaaaacatggataacggttcagccaattgagggagcttttgtcgtgaatctcggcgaccatggtcactatttgagcaacgggaggttcaagaacgcggatcatcaggcggtggtgaattccaactcgagcaggctatctatagccacgtttcagaatccggcgcaggatgcaaccgtgtatccgcttaaagttagagaaggagagaagccgatcttggaggagccaatcacttttgcagagatgtataagagaaagatgggaaaagatctggagctggctcgcctcaagaagcttgcgaaagaagaaaatgaccagaagctggccaaagaagaacatgacaagaacctggccaaagaagaaaatgatcagaagctggctaaagaagaacatgaccagaagctggccaaagaagaacatgacaagagccttgccaaagaagaaaattaccaaaagctggccaaagatgaacatagccacacggaagctgttaagcgtctcggccaaatcctcgcttag

SEQ ID NO: 64 - protein, 412 aa, Thlaspi arvense
MAPGTLTELAGEAKLNSKFVRDEDERPKVAYNKFSDDIPVISLAGLDDVGGKRGEICRKIVEACENWGVFQVVDHGVDTNLVEDMTRLARDFFALPPEEKLSFDMSGGKKGGFIVSSHLQGETVQDWREIVTYFSYPVRNRDYSRWPDKPEGWVKVTEEYSDKLMGLACKLLEVLSEAMGLEKEALTNACVDMDQKIVVNYYPKCPQPDLTLGLKRHTDPGTITLLLQDQVGGLQATRDDGKTWITVQPIEGAFVVNLGDHGHYLSNGRFKNADHQAVVNSNSSRLSIATFQNPAQDATVYPLKVREGEKPILEEPITFAEMYKRKMGKDLELARLKKLAKEENDQKLAKEEHDKNLAKEENDQKLAKEEHDQKLAKEEHDKSLAKEENYQKLAKDEHSHTEAVKRLGQILA

SEQ ID NO: 65 - DNA, 4251 bp, Thlaspi arvense
  source 1..4251: mol_type = genomic DNA
aaaatgtagggaaaaaaaaacagagagaatcagatacagagagacgaaatccgaatcggagtctatctatctacttgaaattggtgacagaagaggaacagagaattgctaataaaattctaagataggcacaaaaaaacaagaacaagtttcatttggaacaagaagatgactgaaagaaactgcaagaagagaatcatggaaagacaaaacatacctaatgaaaagggaattttagagtcagaatcagagttactgattgaaaagatagcctgcgatctagtgactcttcttgctgatgatggagtctccattaggatcttgatcgtcttgcaagcaacaacggctaaagatcaagtgaaagaatttctgggaaaatcaatctgaatttcaatatctgagatatcaataaagaagagaaaggggataaacaattgcgaatctcttaggtagcagtattataggtatggggaaaaggttaccgtttgaaataaactagccgttgcgtctaaacggaaggaaggagccgtaatactagccgttgggtccattctctcatggaaagaaatcaagaatggttaaagacttaaagtagctgtttgggttgaaatctcagtacgttaggggcttttacggattaagaaggctgcgattaatagctcggcccatttatctctctgttgcgagttgcaagctgctaaaagttttataagcttttttattcggttatttgccaatcgtttaaattactcctatgatttataaatcttggaatgtgtgtatgagacgaagtattcattgttttcaatctatggtgtctgttttatgttttgcttttttttttttaattaaatatacaactcacaattcacaagccatgacaaaacatatcaaaatgttgataagagtaatgaaaactaaatacactagaaaagtcagatccaacatttcgtcttctcggattaaggacgatataaatataatatatatagtgaaaaaaaggtttttcttctctgatctcaatgggattatgtacaaataaccatgcaaaattgatgatcatttggatttttgtagtgcaaacccgtaacgtaacaatttttgccatgtgaattcaccgagaacgaccattttttttctttttttaataaaaaaatatgcaacccattttttaagacgtggcattaaattcaccgtaaaaaacatttaactatattgggcatggtgttaaagcaactttactagaaacgatttatgtacacaatggaatgtagcgcagaaaatatgatttattagaaagaaattaaagacagaagcacgtataggaagttgagtaactgcgtgtttctagaaacagaacggacggtatagtactgtggtaggtagcgagcgacctcttcgttcgtcagtcttcacaacctttgaaaggtttttcagctaccagtcatctccttatatattggttacctcttttatctctctttataaacttaattagtcttttgcctttgtaaccaaacactcacaaaaaaatataaaaatggctccagggactctcaccgagctcgccggagaggctaagctcaactctaaattcgtccgggacgaggacgaacgtcccaaggtggcatacaacaagtttagcgacgatatcccggtgatatctctcgccggactcgacgatgttggtgggaaaagaggagagatctgccgtaagatcgttgaggcttgcgagaattggggcgtgttccaggtggtcgatcatggtgtcgataccaatttggtagaggatatgactcgcctcgctcgcgacttctttgctttaccacccgaagagaaacttagtttcgacatgtctggtggtaagaaaggcggcttcatcgtctctagtcaccttcaggtaaagccacacaatttacgttacgttttcatgcgactcaaacttttatactgtagacttaattagacctataatcacatttcgggccgcaaaaatacgaattatgttttgatcttgtagttaaatacgaaataatgatgataaacgcagggagagactgtgcaagattggagagagatcgtgacgtacttctcgtacccggtgagaaacagagactactcacggtggccagataagccggaagggtgggtgaaagtgacggaggagtacagcgacaaactgatgggtttagcttgtaagcttcttgaggttttgtctgaagctatggggctcgagaaagaagcacttaccaatgcttgcgtcgatatggaccaaaagatagttgttaattattaccctaaatgccctcagcctgatctcaccctcggactcaagcgtcacactgatcctggaaccatcactttgctgctccaagaccaggtcggtggattacaagccacacgcgacgatggcaaaacatggataacggttcagccaattgagggagcttttgtcgtgaatctcggcgaccatggtcacgtacgtcagtatactctctcaatctctctgcttatatttttctccgtttgtgattttgacttggccaaacttgcttgtctattgaagtatttgagcaacgggaggttcaagaacgcggatcatcaggcggtggtgaattccaactcgagcaggctatctatagccacgtttcagaatccggcgcaggatgcaaccgtgtatccgcttaaagttagagaaggagagaagccgatcttggaggagccaatcacttttgcagagatgtataagagaaagatgggaaaagatctggagctggctcgcctcaagaagcttgcgaaagaagaaaatgaccagaagctggccaaagaagaacatgacaagaacctggccaaagaagaaaatgatcagaagctggctaaagaagaacatgaccagaagctggccaaagaagaacatgacaagagccttgccaaagaagaaaattaccaaaagctggccaaagatgaacatagccacacggaagctgttaagcgtctcggccaaatcctcgcttagagtccttgttgctccgctgtgttggtttcggtttggttttgtaatttgttttatcgtcaagttaacgaacgtggtgtgtttgagtttcttctcaatatagaaataatgacaagtaatgcaattgtacttgctctgtttgtttggttactttttatgtcagaagcacatacattactttctcgctattcgtgtggatgtaaatttaataagataatgacggttaaaccggtagtaggaccattttatttctttatggtttctttacgccacgtgtccgtctaaaagaaacttaccttgaaaaagtgaataattcatccctctttttcaagtttcgatttttttttctcttttcgagtcattttgttctaatcaacgacgacgcgacggagatgaatccttttcacggtgccgacgggaagcaaagaccggcgatgtatccggacatcgatcaatcaattccggataatcctttcgctcagacaaacccttatgccgcttctgcccctaatctctacccttctccctcctcgaacaatctcgggcctaatcttttcccggaccacggagatgcatccaacaaccagtcaccgtctgctccgcctcaagcgacggaggaggttctcatccgtgtcccgggctccattctcaaccttatcgacaaatcctacagcgtcgaactcgcgtgcggtgacttcaccatcgttcgaatcgtccagggccagaacatcgtcgccgttctcgccaacgtcgccgatgagattcaatggccgttgaacaagagcgaggtagcagcgaaggtcgatgggtcgcactatttcttttcaatccacccgccaaaggaagagggtcacggatctgggtccgactccgatggtgagaagcaggggaaaaagagcaatccgaaaccggaggacgaaattctcaattacggattgaccattgcttcgaaagggcaagagaacgtattaaacgagctcgaccgggttctccgggactattgctgcttcacggagcagaggatgtctgaaaaggcgaaggagacgggagaggaggtgctgggaaactccatggctgcggcgacttcgccggaggagctgaagggtgagaggaaagacatcgtggagggtcaatgcgcggcgtattggaccacactcgcgcctaacatcgaggattacagtagcaagactgctaagttgatagcttccgggtcaggtcagctgatcagagggatactt

SEQ ID NO: 66 - DNA, 1545 bp, Thlaspi arvense
  source 1..1545: mol_type = other DNA
atggccactctcttactcacaatcctcctccccactttcctcttcctcctcgtcctcctcctttctctccgccgcaaccacaaccgcagtagccgtctcccaccaggcccaaaaccatggcccatcctcggaaacctccctcacatgggtcctaaaccccatcgaaccctagccgccatggtaaccacctacggtccaatcctccacctccgattagggttctccaacgtcgtggttgctgcgtctaaatccgtggccgaacagttcttcaaaatccatgatgccaatttcgctagccgaccaccaaattcaggagccaaacacatggcatataactatcaagatcttgtctttgcgccttacggacaacgatggagaatgttgaggaagattagttctgttcatttattttcagctaaagctcttgaagattacaagcatgttcggcaggaagaggtaggaacgctcacgcgcgagctagtggatgcaggcacgaaacccgtaaacttaggccagttggtgaacatgtgtgtggtcaacgcgcttggaagagagatgatcggacggcgtctgttcggcgccggagctgatcacaaagcggaggagtttcgatcgatggtgacggaaatgatggctctcgccggagtattcaacctcggagatttcgtgccggctctggattggttagatttacaaggcgttgctggtaaaatgaaacggctacacaaaagattcgacacttttctatcgtcgattttgaaggagcacgagatgatgcacggtcaagatcaaaagcataaagatatgctcagcactttaatctcgctcaagggaactgattttgacggtgacggcggaagcctaacggatactgagatcaaagccttgctcttgaacatgtttacggctggaactgacacgtcagcaagtacggtggactgggccatagctgaactgatacgacacccggatgcaatgaccagagcccaagaagaacttgattcagttgtaggccgcgataggcccattaacgagtcagacctttctcggcttccttatcttcaggcggttatcaaagagaatttcaggcttcatccgccgacaccactctcgttaccacacatcgcatcagagagctgtgagatcaacggctaccatatcccgaaaggatcgactcttttaacaaacatatgggccatagcccgtgacccggaacaatggtccgacccgttatcgtttcgacccgagagatttttacagggtggagaaaaatccggcgtcgatgtgaaaggaagcgatttcgagcttataccgttcggagccgggaggagaatctgcgctgggctcagtttagggctacggatgattcagttactgacggcgacgctggttcacggatttgattgggaattggccggaggaattccgccggagaagctgaatatggaggagacttatgggattactctgcaaagagcagttcctttggtggtgcatcctaagccaaggttggctcccagtgtttacgaactcgggtcgcgctaa

SEQ ID NO: 67 - protein, 514 aa, Thlaspi arvense
MATLLLTILLPTFLFLLVLLLSLRRNHNRSSRLPPGPKPWPILGNLPHMGPKPHRTLAAMVTTYGPILHLRLGFSNVVVAASKSVAEQFFKIHDANFASRPPNSGAKHMAYNYQDLVFAPYGQRWRMLRKISSVHLFSAKALEDYKHVRQEEVGTLTRELVDAGTKPVNLGQLVNMCVVNALGREMIGRRLFGAGADHKAEEFRSMVTEMMALAGVFNLGDFVPALDWLDLQGVAGKMKRLHKRFDTFLSSILKEHEMMHGQDQKHKDMLSTLISLKGTDFDGDGGSLTDTEIKALLLNMFTAGTDTSASTVDWAIAELIRHPDAMTRAQEELDSVVGRDRPINESDLSRLPYLQAVIKENFRLHPPTPLSLPHIASESCEINGYHIPKGSTLLTNIWAIARDPEQWSDPLSFRPERFLQGGEKSGVDVKGSDFELIPFGAGRRICAGLSLGLRMIQLLTATLVHGFDWELAGGIPPEKLNMEETYGITLQRAVPLVVHPKPRLAPSVYELGSR

SEQ ID NO: 68 - DNA, 7303 bp, Thlaspi arvense
  source 1..7303: mol_type = genomic DNA
ctctttttcgtttaaaaataaatataaaatcagttctttatgaaattcaaatgcggtctatgatccataaacgtggccttggcatttacccgaatcccatccgtctccatcatttgcctttcgatcgtatatggaagttggaacgacgtcgacgccaattctgcggtaatcgtaatagtattaaaattgtggagccaacggaaacacaatgcatttttgcatttccatgcacacctttgtttaattttctaaagagaaattagtatatatataatttgtattgatctaatttttttaaatccagttcgactttgaaggaatttaagttcgacttgtatataattcttgtcaagacctcgatcccgcatccagtaataaaataataatgattgcaaaggacaacactaataaagaaaatgctataacgagaaagaattctgaaagacgtactaacgaaaattgtgtcctagtgaccataacaggagtatcatccaacactatgaaccacatatcttacctacccttcacgagtactctccagctaccacgattaacgataaatatatggtccagagaatttccgaatgatccgctaatattcgaataactgaaattatcaagcagtgagtttaattttttgtaaccgtatatctttttagccttttaaaatgataaactcatttatgaattaattgaatatatattacgtttaacccatccattcatattgtcacatatttttgaattttgttaacttcctttttatttcttttcgtattttctcaaaatcatatgtagtcattatatatacacacaaaaaaaagagatagatattgactaaaaggtagtgaaaaattacaaatctatagacattacaccataaaaaccatttttcaatagacaaatatatggttttactatgtgttgcgggaatcaacggaatcaacttgatgttagtatttacaaatagacgataaatcttctaaaattaattataaacacgtgaaagcttaaagacattgtgtaatatcttctgataatttttaatgttcaagacagtattttgattatgaagcttggtcgaaaccaaaaacaaaaatcaaaagacaagaagaattgaagaagtgaagaacacaacgtttcgttttaaaccatacaaaaaagtggttcacgatgtgatcttaaatgtatatctctttaataatcacttttccgttgaaaaggagaggaaaaaatcactgtagacttagtttttggaaagtatttctcatccccttttcgcaaggggattgtgtttttttttatcgaaaatacatggtccatggttaaatgggtcaagagtataatttagtactataattttataatcaaaatgttctaagttctatcttatatttatataaaaatagaagaagatgttctaacttatatcatattaattagtggctttacttaaccaaaagattgttacttatatttttcaacctacgttctactaacgactaagtattcagtaagatatatagctacctttcatagtattaatcaaatcttacgaaccagaaagctcacctaccattcgactctctttcgcttccaacttattctacataagataagattttctcatctacatattcgtatgtttgacgtcgtggtgggatccatgatttatccactttaacaatagaaaacaaaaacctaatcagagaaatataagctcttatgttttaaaaggaaaaaagcaatggaaattgaagctttttaaccaacaaaaaaaccagagaaatatacattattataattttatatattctgtcaagacgataattatcaatgtatatgtgtactaataatgttattactcgattacacccgtagttaataagccacttaaaattaactatttacaaaaaaaaaaaatcttttggtgactttgatttgatggtgtgaaaatctacatctcattcttcagtattcagatgattataacaaaatgttttttttctaaacttgcatttccgataatctaatactaaaaaatgtatcggcagaaagaatactagcttgaaaaacctttttataaaaaagaaaagtaaatatactagctaatggtgcccaacaggagatcgaagtggtgatgtttaattagttaaaggtaaaagaaaacctatttctaacttttgatgaaacaataaaaacaaaaaaatctttctaacctaaccgagacatgcatagatagattattggatttcgcaaaaaaaaaaaaatcaccctttatttatagcttatgtttgttattcctcatttctcacttaccattcaaacccaacactatggccactctcttactcacaatcctcctccccactttcctcttcctcctcgtcctcctcctttctctccgccgcaaccacaaccgcagtagccgtctcccaccaggcccaaaaccatggcccatcctcggaaacctccctcacatgggtcctaaaccccatcgaaccctagccgccatggtaaccacctacggtccaatcctccacctccgattagggttctccaacgtcgtggttgctgcgtctaaatccgtggccgaacagttcttcaaaatccatgatgccaatttcgctagccgaccaccaaattcaggagccaaacacatggcatataactatcaagatcttgtctttgcgccttacggacaacgatggagaatgttgaggaagattagttctgttcatttattttcagctaaagctcttgaagattacaagcatgttcggcaggtaacagtattagttataaacgttattctcatttcctaacgctataactcacctatatatagagatagtcatgccgttaatttttatatttatgattagtttattttatatcattatttaactgtggtacgaactctagaatttaataaaataaatttagagaagtacgtatagagatttttaatggtggagtggcgtttttttgtttagtattatgttttcagtgttgataaaataaccaaaaaataataatgttagtaatcgttaaaacacaaaacaaattttgttgataaaacgagatttatgactttttatcaacagattttgttttgaaaaacgagaactagaacataatactataacaagttccaatcctgtagaactagtcaccaagtcataaaactggaacttttttatcaaaaaatattgtttcgtttttcacgatttgcaacctttttcgttattttaacaatattggaaacattgcaacctataaaccccaatttaaacgagtaaaacaaaaaaaaaatactaaagtaggcctaagtgcaactgtgcaatactgtcgttgccatagacgtacagtacgatgtatccttgataataccatggaaaaatggaaagttcatcagaaacccaaggacaaaatacttcaatatgtatggaccacatttttccttaaataagatgtatcaacgagtcaccacgagacacgagtgattcactttcagtagtataagattgtttttgcattttcgtttaaaaaaatgtagatgaacatacaagatgatcctgacaatttatttataggtagattacttttcattgatggaacaattgaatatacaaaaatgtaaactagacttcagaattttaagtttaggggttaaagtaacttaactagggtctaaagtgtatataggctttatatttgagcttaggatttagatattggttaattagtggattttaatcgatttaaatttagaagcaagattatttgttattaagttattactttttaaaatcatagttaaagtcatgtgttaggggtttaataaattctaaatattagttgaaatttaatgttattaatttttataagaaatcgattttacattcgattttagtttttaacatctttgtaagtgcttttgagttactaaagcaactttcttatttaaaaacaggcttattgaattttttttaaaaattacgttttgaaagcatttgagtaattgtaaatcttaagtaaatttataaatcaattataaccctaactaaaatttattaatcaactaaacttcatacaccaataatcctacttagagttttataaggtttttgctgttaatcaaacatcaagatttaaaaatgagtaaaataaattccaaaatcaactaatatacccaaaattttccatttatagtttaagtagagcaaaattgaattttacaggaagaggtaggaacgctcacgcgcgagctagtggatgcaggcacgaaacccgtaaacttaggccagttggtgaacatgtgtgtggtcaacgcgcttggaagagagatgatcggacggcgtctgttcggcgccggagctgatcacaaagcggaggagtttcgatcgatggtgacggaaatgatggctctcgccggagtattcaacctcggagatttcgtgccggctctggattggttagatttacaaggcgttgctggtaaaatgaaacggctacacaaaagattcgacacttttctatcgtcgattttgaaggagcacgagatgatgcacggtcaagatcaaaagcataaagatatgctcagcactttaatctcgctcaagggaactgattttgacggtgacggcggaagcctaacggatactgagatcaaagccttgctcttggttcgtataacgatcaattaattgtagtattaatttcatactttatgaaaagttattgattccttcttaaatacagaacatgtttacggctggaactgacacgtcagcaagtacggtggactgggccatagctgaactgatacgacacccggatgcaatgaccagagcccaagaagaacttgattcagttgtaggccgcgataggcccattaacgagtcagacctttctcggcttccttatcttcaggtatacccttaaccgggaattaggaattgtcttggttaacgagctctattgttaatccggtttaaacggttttgttttaaaaacaggcggttatcaaagagaatttcaggcttcatccgccgacaccactctcgttaccacacatcgcatcagagagctgtgagatcaacggctaccatatcccgaaaggatcgactcttttaacaaacatatgggccatagcccgtgacccggaacaatggtccgacccgttatcgtttcgacccgagagatttttacagggtggagaaaaatccggcgtcgatgtgaaaggaagcgatttcgagcttataccgttcggagccgggaggagaatctgcgctgggctcagtttagggctacggatgattcagttactgacggcgacgctggttcacggatttgattgggaattggccggaggaattccgccggagaagctgaatatggaggagacttatgggattactctgcaaagagcagttcctttggtggtgcatcctaagccaaggttggctcccagtgtttacgaactcgggtcgcgctaaacctaagtttgcttgccagcaaaggtaggtcttgcacggaggttaaaaagcttgtttctggaatttcctcaaataaagtttaaaatagcgtaatgtggtccggagtataaggctatgttatctgcgtcgtcgatccgatgccgaggaagaagacgatggctctcgaaagcaaacctgatccgcggacccgacccgttttatacgactaagattttcattcataatagtatatgataattttaaattttaaatttttatcgtgtaatttttacagtactgaattttgtattaaagcatcttccttactgtaccagatgcatttacaactctagatttttttctgccagcaaaatcagatttttccatcttttttatatatattaaagtggaacaccactacaacctgcaattctgcaacacatgttacattacacattcatttggcgttttccaataagttataaacagtgaatgtttgtagacaatagacaattataaacagtaaatcatgtttcccctctgttttcaaaagtgaaaaagtttctaaatatgtatatgtattatactttaataactcgtcggaccatactattcccaccttctaattaaccttgtatacactggtttaccaacaccatgtctcttccttgttcaaaaaaactccatgtctctttaattactttttttcttcttctcgaaatttgttgataatagaaactagtcgaagtttctctttaattctgttttcatttaatataagcgtcgttgttataatttcaaatttcaaaaaggtacttacaagttcacacggagagctacaataatggaaaagctgactcaagaagggctagaaaagaaacaagagtcacggaacaagtagtcactttcaatctcagtatacagtacactagtgtctgcttgcatctctctctctctctctctctctctcttggtctaaaaatatcagaagagaaaatctctctatctatttatctctctttccctttctctttcaacaagacaatagtgacgacatttgtgtttccatggctgttctggttctctatctcctcggtttcctcatggctggccactgtagtaagaaactctcgctcttcactacattacttatctctctcttttttttaaatgtgtctattgatgggaactaaatttcaataaaattctttcggctcttagctagttatcactacatctcttaagttcacgaccctcaaaaagaaggtttcctcaaatcttcttggcttcacacttacaatttgtttcatttggtaggcgcgacgtggtgtgtgtgcaaaacaggactgagtgactcagtgctacaaaagacattagactatgcttgcgggaatggagctgactgtaacccaactcacccaaaagggtcttgcttcaaccccgacaatgttagggctcattgtaactatgctgtcaatagcttctatcaaaagaaaggtcaagcttctgaatcttgtaatttcactggaactgccactcctaccacaactgatcccagtaagtttccctcagaaatctgatgcttttactgtgattgtttacaactctaaatagtttttggagtcacagaaagtccaccgtcattttggttacttaaaatgatttggtattagagattagtgaatattaaagtttaaagtaacaatttggttttagtaatgtatgaggaggatctgatttggttacagtacactaaatgtttttttttttgtgtgtgtgcttttttgctttgatgggtgaacattttgtcacaggctactcag

SEQ ID NO: 69 - DNA, 1581 bp, Thlaspi arvense
  source 1..1581: mol_type = other DNA
atggatgaatcaagtatttttacggcagagaaagtgatcggagctgagaaaagagagcttcaagggctgcttaaggcggcggtgcaatctgtggagtggacttatagtctcttctggcaactttgtcctcaacaaagggttttgctgtgggagaatggatactacaacggtgcaataaagacgaggaagacaactcagccggcggaagtgacggcggaagaggctgcgttagagaggagtcagcagctaagggaactttacgaggcccttttggccggagagtcctcatcggaagctagggcatgcacggcattatcgccggaggatctgacggagactgaatggttttatctaatgtgtgtctctttctctttccctcctccttccgggatgccaggaaaggcgtatgcgaggaggaaacacgtatggctatgtggtgcaaatgaggttgacagtaaaatcttttctagggctattctcgcaaagagtgccaaaatccagcagacagtggtttgcattcccatgcttgatggcgttgtggaactaggcacaacgaacaaggtaaaagaagatatagcgtttgttgagctcataaagagttttttccataaccaccccaagtcaaacccaaaagctgctctttctgaacactccatcaacgaagagcacgaagaagacgaagaacaagaagaagaagaagaagaagaagtagaagaagaaatgacaatgtcagaggagataaggcttggctctcctgatgatgatgacgtctccaatcaaaacctactctctgatttccatgtagaatcaacccacactttagacacacacatggacatgatgaatctaatggaggagggtggaaactattctcagacagtatcaacacttcttatgtcacaacccacgagtcttttttcagattcagtttccacatcttcttacatccaatcatcatttgccacatggaaggctgataattttaaagagcatcagcgagtggaaactaaatcgacgtcgtcgtcgcaatggatgctcaaacacataatcttgagagttcctttactccacgaccacactaaagaaaagaggctgcctcgagaagagcttaatcacgtggtggcagagcgccgcaggagagagaagctgaatgagagattcataacactgagatcattggttccctttgtgaccaagatggataaagtctcaattcttggagacaccatcaactacgtaaaccatcttcgaaatagggtccaagagctggagactaatcatcacgaacaaaaacataagcggatgcgtagctgtaagggaaaaacgtgggaagaggtcgttgaggtttccatcatagagagtgatgttttgttagagatgagatgcgagtaccgagatggtctattgctcgacatccttcaggttcttaaggaacatggtatagagactactgcagttcataccgcggtgaacgagcgtgatttcgaggccgagataagggctatggtgagagggaagaaaccaagcattgctgaggtcaaaagagccatccatcaaactatatccaatattaaactatag

SEQ ID NO: 70 - protein, 526 aa, Thlaspi arvense
MDESSIFTAEKVIGAEKRELQGLLKAAVQSVEWTYSLFWQLCPQQRVLLWENGYYNGAIKTRKTTQPAEVTAEEAALERSQQLRELYEALLAGESSSEARACTALSPEDLTETEWFYLMCVSFSFPPPSGMPGKAYARRKHVWLCGANEVDSKIFSRAILAKSAKIQQTVVCIPMLDGVVELGTTNKVKEDIAFVELIKSFFHNHPKSNPKAALSEHSINEEHEEDEEQEEEEEEEVEEEMTMSEEIRLGSPDDDDVSNQNLLSDFHVESTHTLDTHMDMMNLMEEGGNYSQTVSTLLMSQPTSLFSDSVSTSSYIQSSFATWKADNFKEHQRVETKSTSSSQWMLKHIILRVPLLHDHTKEKRLPREELNHVVAERRRREKLNERFITLRSLVPFVTKMDKVSILGDTINYVNHLRNRVQELETNHHEQKHKRMRSCKGKTWEEVVEVSIIESDVLLEMRCEYRDGLLLDILQVLKEHGIETTAVHTAVNERDFEAEIRAMVRGKKPSIAEVKRAIHQTISNIKL

SEQ ID NO: 71 - DNA, 5726 bp, Thlaspi arvense
  source 1..5726: mol_type = genomic DNA
atctaatcaagagaagctagctaacaatatcgaagggaagacatgaacacatcctcacttttgcctaatcgaatgaaagctaaaaatggatctagggtttaagggatctaacgatggaaagcaaaggactcaagagaacggcggctaggaacggcggaacgacggcggctctcctcagcggcggcggtcggcggcgaaaacgaacggcggcggcggcttgctcggttagggttcctaggttatatctctgagtgctttgggagttatgatggaaaacctaattctctaactctgtttatatagggaagactcaggaaaaatcctaatatccttttctcttgggcttctgacacatgaacctttccttttcctattgagcctagatccaggacgttacaactagaatcagaatcgaacaacaagcgtatgcgcttaagaaatgatttttactcacactatatgggcgcgcatggcattgtcgtaagaattaaataagcttcgtcccactccttaatggatttacgcacacagtcaatccacgtggttgtcataactaaatataattggtgaaaaaactaatttaaagacaaagtaagaagcggaaaccgaaggaaaagccaaacaacattatgtttatcgacaaaaaagccaaaacaacatttaatgttaatttttgtccaaaccaggaatacatcactcatacggtcatatataccataccccaaattgtatgtactacatgtgtacgtaactgatttatgtatatctatctatttctcttttattgtaggggtcaaaatctacctatcgatatttataaataggattttataagacattgttaaaatggaaaacatggtagctacttggccagcgattaacatcaataattaaaaatacgaattgtgaaacatctcactctcttccttttatcacaccaaaccacttctctttctttacttaccggtcaggtcaacaattctaccattccctttatttagtttttttttttcatctatctctcttttcatttttaacttttaaaaaatattagtccgaaaatcgcactcttttatattcgttgatgggcattaaaatattgtaaaaattaaaaaaaatgtgtaaattaaaacgcaatttgtttgcacctgcagcagtagtaacacacaagtcaaagcaatgtctgttttctcttgtatgtcggttagctattttatgtactgaaatatgttattctttctgaccaaaacatattaagaaatttgcattctgtaatttgatttatccaatcagtagaggacacgtaaccaagataattagatatttttattctatctgtatactactaattcatccaacgtctgttggacgaccaaccagtcaaaactcataaaagtcaacttttactacatcgtgaattttttggtcatgcatttatatacacatacatggaagaaaaaacaatactttacctatgtcaaaatgctgcaaaagcattaagatggtatgtatacatacatattgatataacagtggtcccatatatcattttaaatcatcataaagagtatccatcttctttcatattaacatccccttcaaagttataagatttttctctcttcattagagagagagagagagagaattaacacaagttttaatctccgggaaagatggatgaatcaagtatttttacggcagagaaagtgatcggagctgagaaaagagagcttcaagggctgcttaaggcggcggtgcaatctgtggagtggacttatagtctcttctggcaactttgtcctcaacaaaggttcttttttttttttaataaatttcatcgatctctcacaataaaaaccctaaattttatatcatttattattatatgtttaactacataattatcagtattttaaccgtccatgtgctttatttggttccatttctgtctcatattttacttgaggttcagactgccgagcacatctctcgtttgtctcgaatctgtgagactttttcgtttattggcacttctgtgtcaattgagttatactgaagtaattatatgtttaaatgaattagggttttgctgtgggagaatggatactacaacggtgcaataaagacgaggaagacaactcagccggcggaagtgacggcggaagaggctgcgttagagaggagtcagcagctaagggaactttacgaggcccttttggccggagagtcctcatcggaagctagggcatgcacggcattatcgccggaggatctgacggagactgaatggttttatctaatgtgtgtctctttctctttccctcctccttccgggtacccaactctctctctctctctctctctctctctctctctctctctctctctctctctcttttgtctatactgaagtttcttaatttatctttttatcatctcctactgaagacaaaaatagtattgtgtgttaaatgcgaatcacgaatattgtggaagcattaaaaacaaactgaggaggttgagttactgaaagaagaaatgtattggagttgatgaaacgtacactccattttagtgaacataattggaccgttgagattcttatttttttgctgattgattatctaaagtagaagcataaatagataatacataaatgcataacaaattgtgttagttatgggtatagttaatgctttttctctatgagaggaaaaaaaaaaaaatatataaatgtggaagtaataattttgtaggatgccaggaaaggcgtatgcgaggaggaaacacgtatggctatgtggtgcaaatgaggttgacagtaaaatcttttctagggctattctcgcaaaggtctatttcctttttcatttaccactactctatgcatctacttctctacctatttatatatctcatctttcaaattaattaattttctgtctttattttcttggatgctccttctacatcggtcggttccttaatggttagagtgccaaaatccaggtaaacgttgtctttattgattaattctaattttgagtaatattttacatttattttacatgtttgaaaattgttttgtgataaaaaaaaagcagacagtggtttgcattcccatgcttgatggcgttgtggaactaggcacaacgaacaaggtacggcgtagttatctttttatatatgcataaccaaatggttaagaaaaaggttagaagagaaatagatcatgcttaagttttatcagttaaattaaaaatgtaaaaataagatattatgttcattaataatgtatagtccctgttagttaaaaaaaagaataaaatatttaaccatttgaagtcataatataaaaatattgtttttggagatagtacataattctcacaataaaaaaaataacaaagggatgattaagggaaggagttggatacatgttgtttgtctgtgtgtgtgaaggtaaaagaagatatagcgtttgttgagctcataaagagttttttccataaccaccccaagtcaaacccaaaagctgctctttctgaacactccatcaacgaagagcacgaagaagacgaagaacaagaagaagaagaagaagaagaagtagaagaagaaatgacaatgtcagaggagataaggcttggctctcctgatgatgatgacgtctccaatcaaaacctactctctgatttccatgtagaatcaacccacactttaggtatacacttatacattaaattagttaacgatatcattacacgtatctatttattttgttaacaagaaatttaaaaatattcgccatttctttgttatgtctaaagaaaatctataaaattttatgaatagacacacacatggacatgatgaatctaatggaggagggtggaaactattctcagacagtatcaacacttcttatgtcacaacccacgagtcttttttcagattcagtttccacatcttcttacatccaatcatcatttgccacatggaaggctgataattttaaagagcatcagcgagtggaaactaaatcgacgtcgtcgtcgcaatggatgctcaaacacataatcttgagagttcctttactccacgaccacactaaagaaaagaggctgcctcgagaagagcttaatcacgtggtggcagagcgccgcaggagagagaagctgaatgagagattcataacactgagatcattggttccctttgtgaccaagatggataaagtctcaattcttggagacaccatcaactacgtaaaccatcttcgaaatagggtccaagagctggagactaatcatcacgaacaaaaacataagcggatgcgtagctgtaagggaaaaacgtgggaagaggtcgttgaggtttccatcatagagagtgatgttttgttagagatgagatgcgagtaccgagatggtctattgctcgacatccttcaggttcttaaggaacatggtatagagactactgcagttcataccgcggtgaacgagcgtgatttcgaggccgagataagggctatggtgagagggaagaaaccaagcattgctgaggtcaaaagagccatccatcaaactatatccaatattaaactatagtttaagactctaacaatattgatgccaactctagaaaaggacaactgaacttattttgttttaagccttggctatattacattatcagttttacacttctacgtatacacaactttaatttttctatattactacatgcatactagatgttagaaatatcttatataagcatacatattaaattagttatgcgatatttaaaattaatgtatataaatattcagtttcaaagcttacgaatacgtaaaattaatcaatacaaaccgaaaccaaaaagccacttctcatctcaaaatgttaattacaaatttacaataagccgaatcactatctaaaaagcttttgggatcccgagacccaaaacatttcttcgtataagtgcaacaattatcgagtgtgatgagacacgtaaaaagcaaggatcgggacaacgattttcggctatatagtagtttctcatatctgactttattagcaaattactacataaaattgcttttaagtatgattaacggaacaagtataatgcgtttatttaattacagatctggctaaatgtaatatggtatcaaagctggaaagacaaatagtctaaggtttggaatttttcatctgtctataaaattcttaagacactgatagatcattaacttattttggagtcaccaatggacaaatcaataactattgatgtccaaaacccacaagacaagcctattttttttgcacgtgcaagtacaccggtggaagaattcatttgtatactgaatctgaaattataaaagattagaattggttgaagaatttacttcaaaacaagctagaagatggtgttatttaaataaacaatgttaaattatatcaatgactttcaaattttatcaaaacattttttgaaagagaatcacgcacaaagtatttcgaattacaaaacaattttttgcaataaattttatagttaaagcaaattttgtcaattattgaaaaaaattacttagataaaatatctaatttttttttttaaacaatgtctctataaaagatggattagccaagaaaatctgatggatgctacaacgcagggttggagatatggtgctgacactacat

SEQ ID NO: 72 - DNA, 2583 bp, Thlaspi arvense
  source 1..2583: mol_type = other DNA
atggaagggaactctttaagttcatcttccttagtttcagccaatcgggtgggtcaatgtgacaatcttgagcatagtagaatgacttgttctcgaaatttcattgagatgcatttgactgaccagctgagaaaaactcagatagtgaacgagaccaataaggatcttgttgtcgaggcactgagatcaatcgcggagatattgacttatggcgatcagcacgaccctttattctttgaattttttatggagaagcaagtaatgggagagtttgtacgtattttgagggttagcaagacagtaacagtttccgttcagttgttgcaaaccatgagtattatgatccagaacctaaaaagtgaacaagccatctactacttgttcagtaacgaatatgtaaattatttgataacatatacatttgacttccaacatgaagagcttctatcttactacatatccttcctaagagctgttagtgggaaactaaaccagcatacaatatcgttgcttttgaagaccgagaacgatgtagtagtttcttttcccctttacgtcgagggcataaaatttgcatttcatgaagagaacatgatacgcactgcagttcgtgccctgactcttaatgtgtatcatgttggcgatgaatctgtgaatgattatgtagttagtccaccgcacactgagtacttttcaaaattagttacatttttccaaaagcaatgcatggatctaagtgcaatggtgttgaacactctaaagagcccatcccgagactcaggtggaaaattgtttgctgccgttgatgggatcgaggacacgctgtactactttagtgatgttatctctgctggcatacctgatatcgggaggctgataacagatcacattctacagcatctaactctcccacttcttctcccgtctttgtgctctgaggctgataaatcagttgatcctgtgacttctctctatctgctctgttgcatcgtgcggatagttaaaatcaaagatttggcgaatttgactgctgctacttttttctgccctgtagaagctttcatttcaagttccctagtgaaacctaatagtagcttggctcctgaacgtcttacatatggaaatgggcatccagacaatggtgttgctgaggaaacagttcaacagtgtccaagcactgcagtctcgagtgaatatggaaattcccacgtttgcagtgaaaatactacgaaaagcatcttcaacaattcacgtattacgtttagggatactttacttcaatatatttctgagggagatgatgtgcaagctcagggttccttgtttgtgctagccacgttgttgcagacaaaagaacttgaagagtcaatgctagatgcttttggcattcttcctcagcgtaagcagcacaaaaagcttttgctgcaatctttggttggggaagacactggtgaagaacaactgttttcaccacaaaatggttccatgagagatggcttaagcagcgaacttgattggtatctacggaggttggaggagcagtttggagtatgctgttcactgcctggggctgcaatgtgcccgcgtgtacatagacatcaggtggtggatgcattggtcattcttctctgccgtgaaaacatatctgcagaaacattatgggatggagggtggcttttacggcagttgcttccttatagcgaggcagagtttaatcgtaaacatctcaaaatgctgaatgattcatatgagaagtgcacaagtgcactaatccgggaggttaaaggtacctggcctgatctactcatcacggtgctgcttgatgagtggaaaaagttgatcgaagctccatcccctcaaaaagagcctaaatctgttcttctccagctggataaatcctcttctagtggtaacactgttagcgaatcatcattcacagccggtgaaaaactgtgcgaggtggtgaaggtttttgtgcttcttcaccaactccagatcttctcgcttggtaggcccttgccagagcagcctcctatccatcctcctgcagacagatctgaaacgtctcgcgccacaagtgctggtttggatgtttcagtccccaaaactggcaccgaagtgaagctagttgatgctgtacactgtaggattgcctttgaaagaggcaaggagcggaatttctcgtttctagcattatcatctggtgtgtctgggtggattgtccttgctgaagaatcgctttcgaagccagatcacggaaccgtccgtgttaccgcacctttagccggctgcaaaccccggatagatgaaaagcacccaagatggctacacttgaagatccggccatcgacgttaccattcttggatccaacaaagcgaggagtctatgagaagctcaagtccaaaggtctagtagacgggagatggacattagcattcagagacgaagagtcttgttactctgcttactcaatggttgtacatgagatcgatctacaatgcagcgaggttgaaaggaggttaaagccattgttcgaccttgagagaaaccagcaagatcaatcaaacgttgcttctctatag

SEQ ID NO: 73 - protein, 860 aa, Thlaspi arvense
MEGNSLSSSSLVSANRVGQCDNLEHSRMTCSRNFIEMHLTDQLRKTQIVNETNKDLVVEALRSIAEILTYGDQHDPLFFEFFMEKQVMGEFVRILRVSKTVTVSVQLLQTMSIMIQNLKSEQAIYYLFSNEYVNYLITYTFDFQHEELLSYYISFLRAVSGKLNQHTISLLLKTENDVVVSFPLYVEGIKFAFHEENMIRTAVRALTLNVYHVGDESVNDYVVSPPHTEYFSKLVTFFQKQCMDLSAMVLNTLKSPSRDSGGKLFAAVDGIEDTLYYFSDVISAGIPDIGRLITDHILQHLTLPLLLPSLCSEADKSVDPVTSLYLLCCIVRIVKIKDLANLTAATFFCPVEAFISSSLVKPNSSLAPERLTYGNGHPDNGVAEETVQQCPSTAVSSEYGNSHVCSENTTKSIFNNSRITFRDTLLQYISEGDDVQAQGSLFVLATLLQTKELEESMLDAFGILPQRKQHKKLLLQSLVGEDTGEEQLFSPQNGSMRDGLSSELDWYLRRLEEQFGVCCSLPGAAMCPRVHRHQVVDALVILLCRENISAETLWDGGWLLRQLLPYSEAEFNRKHLKMLNDSYEKCTSALIREVKGTWPDLLITVLLDEWKKLIEAPSPQKEPKSVLLQLDKSSSSGNTVSESSFTAGEKLCEVVKVFVLLHQLQIFSLGRPLPEQPPIHPPADRSETSRATSAGLDVSVPKTGTEVKLVDAVHCRIAFERGKERNFSFLALSSGVSGWIVLAEESLSKPDHGTVRVTAPLAGCKPRIDEKHPRWLHLKIRPSTLPFLDPTKRGVYEKLKSKGLVDGRWTLAFRDEESCYSAYSMVVHEIDLQCSEVERRLKPLFDLERNQQDQSNVASL

SEQ ID NO: 74 - DNA, 7185 bp, Thlaspi arvense
  source 1..7185: mol_type = genomic DNA
cgtggatggaggaagggtttctcgtcgtgttcgtcgcgaaagatggttcctcttctgcgccgccaccgccggagatcgaggagaatcgcaacgtgagagtcgtggaaatcaccggtgatgaatgaatgaataattatgtctttaaaacttcaaaatctgtgtattatatgaacagagtaatcatgttgtgatcgtgctgctgttttcgtatgtaatagtgaaagttgcataaaagcccttaaactaatcaaagttttcaaaataacccatcatttaagaaaactataaaacgatcaaaattaatgtaaaatctacatttgagcttccgactacaacatttattcgattcaatttcccttttaataatctaacaaattttccaaatttcaacaaatctcgaaccgaatgattatttgattcaaagacaaactattatgttttcgctacaacccaaaacgatgaatttaagtgtacagtcggaattgtattactgtatagattttaaattagatgggacatttgtttaaacaatttaattaagtgagggttattttacaactttgctatattttgaggggttttgttataattttgtgacttaatagcaagagtcgtctttgaaggaaccgttgtgacgtggcggtcttcaacactcgaatggtcgatcgtaaaaataaatgttttccctaattaaaatgccatagacggatccccccattctaaagattctttctttgaattcgatattgaacccgacccggatccgaatctggatacttgacccaacgccagctcaacgccccacttcggtgcttgcttctattcgtctctccgtcaacaattctgttgtttaccggaatacctagagccttcgagaaattcaaacacgacgcagatatcattctttcgcttacgctattgatttgtatgattttgtcgtcggtgaagcaatccgaaccggaactggaatcggatttcatcaggacttgtggggttccctttaatcgaggagcaaccatggaattggggttttcgcgggagtgaaggatgatccagagaagactggattcagaggattgatccgataatcatgtggttctccttcttaagacccagagatcgattctccttggtcgaactcaggttaaatttttttttgtttgatcgggtcgatcccgcaacaagttccatttgcgatatatatctctgtttcgtttgatccctattgtgactaagattagcggatttttgtgaattctggccttaaaatgtgtcttttaagggtggttgagaggtttttcgtcgtaatctctttggtgtgaatgacttgttctcgaaatttcattgagattttagtgtacgacaagtatttgttcggtgattgtaagcgttgaaattttgagttttttcgtcgtagtctcttcggaattagaatgggcagtttgcagttatctgttagggttttcgagaatttgaacatttgatcgcttgaatggtgtcatggaagggaactctttaagttcatcttccttagtttcagccaatcgggtgggtcaatgtgacaatcttgagcatagtagaatgacttgttctcgaaatttcattgagatgttagtgtacgacaagtatttgttcggtgattataccagatgatgaagcataaacgttgaaactttgggttttgtttttgtaggcatttgactgaccagctgagaaaaactcagatagtgaacgagaccaataaggtcagtgggataaaagtctttttcactttagcaactttgtcttggcattactgttctgttttttccttgtggattcgatctttgtttaccgttttgaaggatcttgttgtcgaggcactgagatcaatcgcggagatattgacttatggcgatcagcacgaccctttattctttgagtgagagtctttatgtcaattatcagtcaatgcccttcattttcttattggcatatatgctaataatactttgcgctcgttgcagattttttatggagaagcaagtaatgggagagtttgtacgtattttgagggttagcaagacagtaacagtttccgttcagttgttgcaaaccatgagtattatgatccagaacctaaaaagtgaacaagccatctgtgagttcatcagaagcagtgtatattttgtctttgataattcgtaatgattatagcctattgatgatcttcttttgaaactacttgcagactacttgttcagtaacgaatatgtaaattatttgataacatatacatttgacttccaacatgaagagcttctatcttactacatatccttcctaaggtacattcttctgttgttgacctcggcttcaggaagtacatgttgactgtatctggtaactgttttgttttctttttgtagagctgttagtgggaaactaaaccagcatacaatatcgttgcttttgaagaccgagaacgtgagtattctttaagttgcatcttccttaaacttctataatagtcctttatggattttttttttctgccatattttaattctgcgtttctgcgtctaggatgtagtagtttcttttcccctttacgtcgagggcataaaatttgcatttcatgaagagaacatgatacgcactgcagttcgtgccctgactcttaatgtgtatcatggtaagtcactcagtcctttcgatttgtcactttaatgactcagaagcttttagcaatgtttctgatgcctttagttttttttttcttttcgcagttggcgatgaatctgtgaatgattatgtagttagtccaccgcacactgagtacttttcaaaattagttacatttttccaaaagcaatgcatggatctaagtgcaatggtgttgaacactctaaagtaagattcactgcatcttcatttcccagggcaataatatcgtgttaaatacgtatcatatccccttttcatctattgactcattagttatattcttctgaaagatttccatttactttgtctaaaggagcccatcccgagactcaggtggaaaattgtttgctgccgttgatgggatcgaggacacgctgtactactttagtgatgttatctctgctggcatacctgatatcgggaggctgataacagatcacattctacagcatctaactctcccacttcttctcccgtctttgtgctctgaggctgtaaatgtataacatatctactttttcgatttattttgtccttttgtgctaattttgtaagccttgttagttttttctatgcaagagtacaatttctaatgtcagtatactgtttgttctgtggttatttcaggataaatcagttgatcctgtgacttctctctatctgctctgttgcatcgtgcggatagttaaaatcaaagatttggcgaatttgactgctgctacttttttctgccctgtagaagctttcatttcaagttccctagtgaaacctaatagtagcttggctcctgaacgtcttacatatggaaatgggcatccagacaatggtgttgctgaggaaacagttcaacagtgtccaagcactgcagtctcgagtgaatatggaaattcccacgtttgcagtgaaaatactacgaaaagcatcttcaacaattcacgtattacgtttaggtaacatgttatctaacaacctgagtgaatttgagatagttgctttttacactccttaagctgtcttaatcataatatattcctatatctctccgaagctgatgttccttttgtaaatagggatactttacttcaatatatttctgagggagatgatgtgcaagctcagggttccttgtttgtgctagccacgttgttgcagacaaaaggtattggtagtggctttgtgcatctccttattttatttctagttttgacagggaaattcgcatctcacgcttacattctctttgtggtagaacttgaagagtcaatgctagatgcttttggcattcttcctcagcgtaagcagcacaaaaagcttttgctggtgagtatctgtcattattctttatcttctgctcttttccagcaaattccaaggcagattgccagggaaattcgcatctcatggtttatggaccgtctactatagtctggaccaaaaatataagctttacttcttggatagctaaacttaatttggtggtcatctctgacagcaatctttggttggggaagacactggtgaagaacaactgttttcaccacaaaatggttccatgagagatggcttaagcagcgaacttgattggtatctacggaggttggaggtacttcagtcactgcatatcttagaattttgcaaacacgttctacttctccatctctttggtgttgtgttaaattgtgattgacttactcattcaagtaccctcaacaggagcagtttggagtatgctgttcactgcctggggctgcaatgtgcccgcgtgtacatagacatcaggtaaattacgaatgtttgtaaacctaaattattagcctcgcttcttctgaaaagtgaaaattccatctgcttgagttaggttctttcttcatcacagagcaagttcttgtcttgaatcaatgaaaaaattgtggtataggtggtggatgcattggtcattcttctctgccgtgaaaacatatctgcagaaacattatgggatggagggtggcttttacggcagttgcttccttatagcgaggcagagtttaatcgtaaacatctcaaaatgctgaatgtatgtgtgttgcttttaagatgttgacactgttacactctccctttcgtcattatttaccagtttcctgctgatgtcaggattcatatgagaagtgcacaagtgcactaatccgggaggttaaaggtacctggcctgatctactcatcacggtgctgcttgatgagtggaaaaagtgtaaaagaggcaagtaaagaagcaaaatgtttggattttgattctaaatttacatgttcagtgaatctaataccaaatctcttgtgacagtgatcgaagctccatcccctcaaaaagagcctaaatctgttcttctccagctggataaatcctcttctagtggtagaatttttgttttacaatcaatgtgaatgatatagacactcccttgttcagttcctgctaatgcaaaccgttaacaactgaacttttacaggtaacactgttagcgaatcatcattcacagccggtgaaaaactgtgcgaggtggtgaaggtaagtccattgtgttccctctgtattttcaatcagcgcttgtcgttgatgtgtaaatgctacagaaatctgagaatggagcattttactccttaggtttttgtgcttcttcaccaactccagatcttctcgcttggtaggcccttgccagagcagcctcctatccatcctcctgcagacagatctgaaacgtctcgcgccacaagtgctggtttggatgtttcagtccccaaaactggcaccgaagtgaagctaggttagcacatgatgctctttatgcttgcttagttcaacatctaccaaaccgacaccatgtccgtagttaaactgatgtttgaaatttcccggtgcagttgatgctgtacactgtaggattgcctttgaaagaggcaaggagcggaatttctcgtttctagcattatcatctggtgtgtctgggtggattgtccttgctgaagaatcgctttcgaagccagatcacggaaccgtccgtgttaccgcacctttagccggctgcaaagtacgtgctcacctacattgtctttttttttgtaacgatattgcttgtgaacaccacttacaaggacagatataatcatgatgttggcatagagaaatgagctatcttttgtttggtattcagccccggatagatgaaaagcacccaagatggctacacttgaagatccggccatcgacgttaccattcttggatccaacaaagcgaggagtctatgagaagctcaagtccaaaggtctagtagacgggagatggacattagcattcagagacgaagagtcttgttactctgcttactcaatggttgtacatgagatcgatctacaatgcagcgaggttgaaaggaggttaaagccattgttcgaccttgagagaaaccagcaagatcaatcaaacgttgcttctctatagctcttgggtttgtttttgttttattcattaaattttttgtttcttctttgtaatgttgctataatgtgataatatcgttgtatatttgaaagtgatagtgaatttcagtttttatcacacaaaaatatgactagtgtgagtgtcgagaactctgcttactcttataattctgtgattctgcgtctcttcttgttgaatatgaaaccctaaaacaaatgaacccttactcttctttatgcatcctgtagctgtcaacgagagcagttttgtatgagttacggacactctgtttccagatggagagagaagcaatcaccgtccgtattttgagcaatcctctttttaacgcagctaatggatgcaacattggcttttagacttgtaactatgtctctctctctctctctcttccttcagccgcagtttaaaagacccacatacagtaccacatcatacctcagatgtgaatggtttgtcttcactaaaaggtttgctggaaccaaaacctaaacaggaaacataactccttgacccacagtaaattaaactaccagaatcactctgaaagaagttcctcgaccagaaatatccaaaagccacataaacagggtctggtcagacataacagtggcaacatcgtaataagaaagatgccaagaagttgcagaggctaatgtttgaaaaaaaaagaagccatgagagaccaaaattaagagaatttgtaattaatacagtactcaggaaaagagtttcaaccacttgcgccaacaaactagatagacattgttatccaacacacaaactcatgtccaaccaaaagatagagagataaagagacattatccaacacaacacatgtccaaataaaagagataacagataaaagatagaagagtgggttctccttttcttactacaaacacccatgaattcgattccctactttcggccaagtaccctgaaacacaacacaaaactgaattgttatacaaaactatgt

SEQ ID NO: 75 - DNA, 1026 bp, Thlaspi arvense
  source 1..1026: mol_type = other DNA
atggataactcagctccggattctttgtccagatcggaaaccgccgtcacctacgattctccttacccactctacgccatggccttctcttccatcggtactccctccggccaccgaatcgccgtcggaagcttcctcgaggattacaacaaccgcatcgacattctctccttcgattccgactccatgacggtgaagcctctcccgaatctctccttcgatcatccttatcctcccacaaagctgatgttcagccctccctccctccgtcgtccctccgccggcgatctcctcgcttcctccggcgatttcctccgtttatgggagatcagtgaagattcctccaccgtcgagcctgtctcggtgctcaacaacagcaagacgagcgagttctgcgcgccgttgacctccttcgactggaacgacgtcgagccgaaacgcctgggaacctgcagcatcgacacgacctgcacgatttgggacatcgagaagtgcgtggtggagacgcagctcatagcgcacgataaggaggtccacgacatcgcttggggagaagctagggttttcgcgtcggtctccgccgacggatccgtcaggatcttcgatctacgcgacaaggagcattccaccatcatctacgagagtcctcagcccgatacgcctctcctaagactcgcctggaacaaacaagacctgaggtacatggcgacgatcctgatggattcgaataaggtcgtgattctcgacattcgctcgccgacgatgcctgtcgccgagctcgaacggcaccaggctagcgtcaacgccatagcttgggctccacagagctgcaaacacatctgctctgctggtgacgacacgcaggctctcatctgggagctcccgactgtagctggacccaacggcattgatccgatgtcggtttactcagccggctcggagataaaccagttgcagtggtcctcttcacagcctgattggattggcatcgctttcgctaacaaaatgcagctccttagagtttga

SEQ ID NO: 76 - protein, 341 aa, Thlaspi arvense
MDNSAPDSLSRSETAVTYDSPYPLYAMAFSSIGTPSGHRIAVGSFLEDYNNRIDILSFDSDSMTVKPLPNLSFDHPYPPTKLMFSPPSLRRPSAGDLLASSGDFLRLWEISEDSSTVEPVSVLNNSKTSEFCAPLTSFDWNDVEPKRLGTCSIDTTCTIWDIEKCVVETQLIAHDKEVHDIAWGEARVFASVSADGSVRIFDLRDKEHSTIIYESPQPDTPLLRLAWNKQDLRYMATILMDSNKVVILDIRSPTMPVAELERHQASVNAIAWAPQSCKHICSAGDDTQALIWELPTVAGPNGIDPMSVYSAGSEINQLQWSSSQPDWIGIAFANKMQLLRV

SEQ ID NO: 77 - DNA, 4435 bp, Thlaspi arvense
  source 1..4435: mol_type = genomic DNA
acacatatctaatactataaaaaaaggtgtatagcgtccgcgaaactcatgtcttccataatcattaatcaaaaaccgatatctctaatcaagatgcatttgacaagaaaaaagaatcaaaatgcattgccaagaaaaaaagaatcaagatgcatgattgtttggtgagtaaacgagacatcttaattttaatataacaattcgttccttgtttttttttttcctgtatcgtacgtgattcatgtgttcaactgttttgttgtcatctcatgtgttagttaaattctatcttattgattttaatacatagatatttcggtgcagcgcaaaaacattattatatttcggtgtagccgcatttagcacaatcatacctaaatattaccaaattgtgctccactatcttacgtgattcatgtgttaaactgttttttctttcctgtggtctaccaaaattaagtttttaattgcaaagacgattgccaattttaattgacgatctaatttgtcacagataacataattatctgatggcgtataagttataagctcttttattttttgaacaaaatatttttgttcttagctgagctgggaaatgtcgtatttaaagtattaaacctataatctcttcggtaatatgttaaataaatctgttttttcaggtcgttagtaaattatttcggctacagacgccatatcaaataatatatcaggttgctgtgaatgagtatctcaatttgcatgctaagaactatataaactgtattaacttttatcttaataccatgagtaagtcgaattatcgatctatctattatttttatttttaaacgtgtggcctgattgataaaataaacttgtggtcatatcaaatctgaaactggagtaaacgtgggattggggatgaagaaattagggcatgtcaacgtcttgggacttaccgtcatgtcccttcactgtaatattggacctatcattttcttccttatcatcttagttttttttgtcgtctcatcctctttaaaataaagtaaaagtaattaacactattatattttctcacaaaattagatattatatgctcttttcaaaaaaatgttaggcatctaacatgatatttttgagatagaaaatgacacaaatactcttcaccccaacctcacgcatatctctatatttattacatcgctattacacacattacacatagtattcatgtacatgtctatttacgcaaaggatcacacgttccacaaaccatttgctaaatcctaaatgagtagtaacaagatattgtccgtctcaaaacaaaatatatatttgtagagaatatcataattttagtatcgtcttcaaaatggtttgaaaatgttattgactttttgtagacaacattttaatctgtgtgtttgggaaagaaatgtggaaagctcgcttagcgttgaaaaggcctactatgtaaagacacaaggcccaaaaatgcgttgaaaggcccactatcaatagatattgattgacacagagggtttagcatgcagtcaaaatatcgcactggacactgaccatagaactttctgtcattttcctctgaaaaacggagatgtcgccgtgaagaatccaaaaatcgaatcgaatcagatcaaaccattccacattttcgtgcagagataatggataactcagctccggattctttgtccagatcggaaaccgccgtcacctacgattctccttacccactctacgccatggccttctcttccatcggtactccctccggccaccgaatcgccgtcggaagcttcctcgaggattacaacaaccgcatcgacattctctccttcgattccgactccatgacggtgaagcctctcccgaatctctccttcgatcatccttatcctcccacaaagctgatgttcagccctccctccctccgtcgtccctccgccggcgatctcctcgcttcctccggcgatttcctccgtttatgggagatcagtgaagattcctccaccgtcgagcctgtctcggtgctcaacaacagcaagacgagcgagttctgcgcgccgttgacctccttcgactggaacgacgtcgagccgaaacgcctgggaacctgcagcatcgacacgacctgcacgatttgggacatcgagaagtgcgtggtggagacgcagctcatagcgcacgataaggaggtccacgacatcgcttggggagaagctagggttttcgcgtcggtctccgccgacggatccgtcaggatcttcgatctacgcgacaaggagcattccaccatcatctacgagagtcctcagcccgatacgcctctcctaagactcgcctggaacaaacaagacctgaggtacatggcgacgatcctgatggattcgaataaggtcgtgattctcgacattcgctcgccgacgatgcctgtcgccgagctcgaacggcaccaggctagcgtcaacgccatagcttgggctccacagagctgcaaacacatctgctctgctggtgacgacacgcaggctctcatctgggagctcccgactgtagctggacccaacggcattgatccgatgtcggtttactcagccggctcggagataaaccagttgcagtggtcctcttcacagcctgattggattggcatcgctttcgctaacaaaatgcagctccttagagtttgaggttaggttttatatttaactatgaagtcgatgatatgaatgatatcacctggttaggcctaatgaattcgcaaagaaagttgaactgaaaactcacttgaatgctttcatggctggctattacagattgtcttgtagctataagagaactttgttagtaaatgatctcacagttgctgtaatggctgataaaatgatattcatgtagacgatgattgggtacaaaacacctttgtactttgtgcttcaggtttttgcaactcatatagagaatctagattgaacaataacattgcacatgtagaaaatcaaataacatttccttattatatacatctcgcttgatgtcagatgcagatggtgaagtggtcaaaatcagatttagcatagacccgatgtgacaagtaggttcggtgcacgcgcactctcgcgtcttgggtcagcaagcaatgcctctgtatctacctgattgtaactaaaactgatttcatttgatgaaccaaatgccactgttatctttctgttttgtgtataaaccccaaccagaatttattgcggtttctggtgtttagatttgaagtggaagcttattacagtataatgcaccctgtctttcctttgttgggtattcttcggataaaacagctacttgtcatcggttatttagcatctaaacaaagcaattataaaatatgtgttacaggttccaacttcgaacacctgtttttagtcagagttttttttttgtattttgcaaattaacttcaagtgacaagcaaattctcaatttattataccttcttcgtttgagaaaacctctgaacgtccgactgttatatttctctatctcattctttacaaagagataaatttatgttaaacttctctatttaccatttttaaaatttcatataaccaatttacataactttggagaacgttgatattcatattttccatttaataaaatgaataaaaatagaaaatttagcttaagggaaaggaaaatatgtgtcagattcttgatttcacaaaaccctacaagcaaccccctctacatataaatagcaacgtccttgtaacttaaaaggcaagtgataataatagtgcaaaaagatttgaaaaaaaaggttagagagaatgtccaccagcgagcttgcctgcacatatgccgctctaatcctccacgatgatgggattgacatcaccgttagttttctcttctctctaattctcaattttaacctctttttgatctagtttctactctttttctttgctcttcatgcatgtacttatatatgttgtagttgcgaatttcgtttatatagtttcatgtcggtaactttcttgtttattgtggatttactaggccgagaagatatcaaagctggtgaaagcagccaacgtgaatgttgaatcatactggcctagcctctttgctaagctatgtgcgaagaagaatattgacgatctcatcatgaatgttggagccagtggtggtggtgaggcagctccggttgcaaccaacgttcctccaactgctcaagcagctccagcagttgaggagacaaagaagaagaaggtatatcctattgtctttctaacagtcttagcgttattgcaatccaaatcatcaactatataatttaacaagcttatgattaaaactaaccaatgggaatattgttttaaaaattctcaggaggaggtgaaggaagagagtgaagatgaca

SEQ ID NO: 78 - DNA, 1275 bp, Thlaspi arvense
  source 1..1275: mol_type = other DNA
atggaggtgaaagagagtgaaagagtggtaatagccaaaccagtggcttcaaggccttcatgctctagcttcaggactttcactgagcttctgactgattcagctactgtgtctcctcaatcgaattgccacgagattgtagacgctgccattagaccaaagactctcaggtttaaccagccagctgcagctgcggtctcatgtccacgggctaaagaaaatggcaatggaaagtcttgtgatgacacagatggcggaaactacgtcgtttacaaacctaaagcaaagcttgtctccaaagcaaccgtctctgtgttggctaacatggggaatcgtcaacagacttggagacaacccgaagcagtagcgtatgggaagagtgtgagtcaaggtactggtcctaatctagtccagagagtttcatcctttacagaaacagagacatcggtcggggacagatcatctgtggacggatacaactggaggaaatacggacagaagcaagttaaaggaagtgagtgtccaagaagctattacaaatgcacacacccgaaatgtccggtgaagaagaaagtagagaggtcattgggaggtcaggtctcagagattgtgtatcaaggtgagcataatcactcgaagccgtcttgtccacttccacggcgcgcttcgtcatcatcctcttcagggtttcagaaaccaccaaaagggcttgtctctgaaggatcaatgggacaagaccctaatagtaatgccttttatcatcatcctctttggagcaatcaaagcaatgactcgtctaagatgtatgagggttgtgttgtaactccattcgagttcgctgttccaagatcggcgaattcaaccggcggaacttcggattccggttgtcgaagtagccagtgtgatgaaggcagcaatggaggagagcttgatgatccaagcagaagcaaaagaagcaggaagaacgagaagcaatcaagtgaagcaggagtatcgcaaggttcggtggaatcagacagtcttgaagatggatttaggtggagaaaatacggacagaaagttgttggaggcaatgcgtatccaagaagttattacagatgcacgagcgcgaattgcagagcaaggaaacacgtcgagagagcgagtgatgatccaagagcttttattacaacctacgaaggtaaacacaatcaccatttgctcttgagacctccaccttcgtctacggttcttcttccctttaactccacacaacattctaatcaagccatttga

SEQ ID NO: 79 - protein, 424 aa, Thlaspi arvense
MEVKESERVVIAKPVASRPSCSSFRTFTELLTDSATVSPQSNCHEIVDAAIRPKTLRFNQPAAAAVSCPRAKENGNGKSCDDTDGGNYVVYKPKAKLVSKATVSVLANMGNRQQTWRQPEAVAYGKSVSQGTGPNLVQRVSSFTETETSVGDRSSVDGYNWRKYGQKQVKGSECPRSYYKCTHPKCPVKKKVERSLGGQVSEIVYQGEHNHSKPSCPLPRRASSSSSSGFQKPPKGLVSEGSMGQDPNSNAFYHHPLWSNQSNDSSKMYEGCVVTPFEFAVPRSANSTGGTSDSGCRSSQCDEGSNGGELDDPSRSKRSRKNEKQSSEAGVSQGSVESDSLEDGFRWRKYGQKVVGGNAYPRSYYRCTSANCRARKHVERASDDPRAFITTYEGKHNHHLLLRPPPSSTVLLPFNSTQHSNQAI

SEQ ID NO: 80 - DNA, 5443 bp, Thlaspi arvense
  misc_feature 887: note = n is a, c, g, or t
  source 1..5443: mol_type = genomic DNA
ttgaatgtgatatatgatattgcggctggccgagctggctggtttaagtactcaaccagacagtaaagtaaaacagccgcatagattgaaatctcgtggaacgtataaccagctcctgtctgtcctagaattggcggttcgggatagaactgttccttacatctcttggaatctccggttgagttgatgctaattgtatcactacttgtgatgtgatctagaaacaaacatagcttatgttttgcgtttgcggtctctgagaaatcgttggggttctatgattcttctggcctgacaattaaaatcattttatggacccaattgaaagactaaaccggacgcagcctattgcaatttaaagaacaataacgagcatgtaggttagaaaccggtttgtagttccacttgagtcgaaactgtactacttgaaaaatttgggttttagacttaaactggtttcaagctccttttatctagggtggagagaacttgttaggaaaaaaaacaaattgttgtaatgcgcggaacggatcgacttatgctctataaaagtctgcggacgcagccaatattaaaggcatgttattataagaaaatgtcttgcggatgcaaaattaaggtaaaataaaacttctgttttaaactgtaactgtgtgtacattgattatgctcaaacaaaccaccttcttaacgaatctttaaggaggtgttattggttcttatattttaatggatttgagaatctaaaccaaattcagtattattggtttttgtattttaaaatttatattgaaatatagtgttattagttttatgattttaaaattcataatgaaatacagtgttattggttctattattttagaatctaaatattataaggattnaagaaaatgtcttgcggatgcaaaattaaggtaaaataaaacttctgttttaaactgtaactgtgtgtacattgattatgctcaaacaaaccaccttcttaacgaatctttaaggaggtgttattggtttttatattttaatggatttgagaatctaaaccaaattcagtattattattttaaaatttatattgaaatatagtgttattagttttatgattttaaaatccataatgaaatacagtgttattgtatctatcattttagaatctaaatattataaggatttgagttttaattgaatttgaatggatttggaaggattttcatgactaaaatataaagatccaaatacaaagtctaattttggtatttaaatagatttgattttttttttattttattgattttgaaatcaataaatttatcaaatccaaaaaagatttataaatctaccaaaatacaagaaccaataacccctagtaagtaatccagcaaactgtttgtataatgtcacctctaatagtagttgaaaattacaaactaataattgtttaactttcataaatgtttctgttaatggataattcataatattttttgtattgtgatactttattatattcatgcgaataataatattttagtttcggttcaatataaacttctgaaattgggacaacagcaacgtgataatattatatatcttcttatttctgacaatggagaggggtgaaatcgagaatgaaccggtttaaatttcggtacggttcagttcactttgtctaaacgagttggtatggttcacgcgtgctttacttctaacaagacaagctcgcgcgcgtgtgtcaacaaccaaccaaagtcactttggccgctggagcctcaaccaaaattcgaaacgacgccgtttctttggccgcgtttccaactaactttcaaaggcctataaaactcaactaacgttcaaccaaaactatctgtctcttctctgtctttcattttcatcgccttctttcatcactatagactagctcatctaaagtacggaccttgatccatccaacgtaccctaccttgacacgtgtcccttgacagtgtgtcggcaagactcaacgaactgaaccgatacgacggatacatcaacgcccaccttaatgaaaaacccgaattcggatcttcctaaagggttttgcctcaaactccttttttgaacttcagattctgcatcatcatctctctcaccgtgagtaacttacttatgtcctctcttttgcgtcacttatggttttacatttgtattcatcttttgggtttttgatttggaatgattcagaacctaatcacaactgtatcggcgcatgtgggtatcatcaagtttcttttttttttttttccggcatcatcaagtttctttctttttgctatagtttgcatcaaactttccaaggctctatatatagatcgagattatgtattgttggatttgatgcttctcaccgtccaaatccaatcttttgttcctctccttttaaaaccttctcgatacttgacttaagactctagaaaatgagctccgattcagaatctgaatctcttataaatttgattgaggctatgtgaagctaatgtgttgatttttaatctgtggaacatttttcaggttgaatcaaagctttttgactggaaacaattttgggtggtaaggttggaacaatggaggtgaaagagagtgaaagagtggtaatagccaaaccagtggcttcaaggccttcatgctctagcttcaggactttcactgagcttctgactgattcagctactgtgtctcctcaatcgaattgccacgagattgtagacgctgccattagaccaaagactctcaggtttaaccagccagctgcagctgcggtctcatgtccacgggtgattcatcttattaatctcttggcaatataatatatcttcttatttctgaatcttctgcattttagcactgactcgtataagtttttctcataatcttaggctaaagaaaatggcaatggaaagtcttgtgatgacacagatggcggaaactacgtcgtttacaaacctaaagcaaagcttgtctccaaagcaaccgtctctgtgttggctaacatggtaagttgtttctagtgctacaaagatcaagaatttctcggaattagtttcttaactctgtttttgttttagcttcaggggaatcgtcaacagacttggagacaacccgaagcagtagcgtatgggaagagtgtgagtcaaggtactggtcctaatctagtccagagagtttcatcctttacagaaacagagacatcggtcggggacagatcatctgtggacggatacaactggaggaaatacggacagaagcaagttaaaggaagtgagtgtccaagaagctattacaaatgcacacacccgaaatgtccggtgaagaagaaagtagagaggtcattgggaggtcaggtctcagagattgtgtatcaaggtgagcataatcactcgaagccgtcttgtccacttccacggcgcgcttcgtcatcatcctcttcagggtttcagaaaccaccaaaagggcttgtctctgaaggatcaatgggacaagaccctaatagtaatgccttttatcatcatcctctttggagcaatcaaagcaatgactcgtctaagatgtatgagggttgtgttgtaactccattcgagttcgctgttccaagatcggcgaattcaaccggcggaacttcggattccggttgtcgaagtagccagtgtgatgaaggcagcaatggaggagagcttgatgatccaagcagaagcaaaagaaggtataatattagagagctttgaatagtttcaaaacaccaatcttcttcgtttactgttacattgacttttatgaataataatatacagcaggaagaacgagaagcaatcaagtgaagcaggagtatcgcaaggttcggtggaatcagacagtcttgaagatggatttaggtggagaaaatacggacagaaagttgttggaggcaatgcgtatccaagaagttattacagatgcacgagcgcgaattgcagagcaaggaaacacgtcgagagagcgagtgatgatccaagagcttttattacaacctacgaaggtaaacacaatcaccatttgctcttgagacctccaccttcgtctacggttcttcttccctttaactccacacaacattctaatcaagccatttgatgaatgatggtatattgatacattacttcttcaatcttcatagcaacattagttcatcattttcttgttgttgcactgtgaatttatttattttacatcaaaattgtaaggagaagcaaaatagttgttatttaacaaacgaaaaaaaaagcaaataaaaagagtgttatattttaggtttaacaacttatgttcccatgttgtagctttcttctgttagtatattgggtttgatctacagtagtggtaaaaagaaactacttttactaatcacaaaaacagtaaatgtaaaacgcaacacacacttaccgcttaataaatcatttgaagcttaaccaccaattagttgaaatacaaacatgaaaggtttggttacaattgatttcatggcaataaacaatttttatttaggaaaatagcagaaaatcggaatatttaatttggagttaagaaccattgaagatggaaaccatatcactttaatgtatcagctttctaattagaaatataaagatgaaatattcttaaatatgaaaccgtttgatcaaagatcccaagtcgataaagcgtcaaaacttgattaaaggtagagaaattttctgaaacatatccaaagctaacgaaaacagcacaaaaaaaatgtctttggagatataatgcaaactcagggcaaaggaagatcccttaacgattggccttggcaacacgctcaatctcatctttcttcttgatagcatagctgcaaagacaagacaaagatgcatctcatcagctactaaagtaacacaaatgtgaagccatttaatagacaagacgatgtagagaatttgttttataaaacctgttggaagatcccttggcagcattgatgagttcatcagcaaggcactcagcgattgtcttgacgtttctaaacgcagcctcacgtgcaccagtggtgatcaagaagattgcttggttcacacgtcttagaggagagatatcaacggcctgcctcctaaccacaccagcagatccaatcctggtagcatcttctctcggaccactgtctcaccaaaaataaacgaacatcatgagaaaagaggttcataacaacacaacaagaaagtgagagggtttcagtatcaccacatgtttgatttacttacctgttaacaatggcatcaatgataacctgaatcgggttctggtcagacaagagatggatgatctccatggcgtgcttgatgatcctgacggccatcagcttcttaccgttgttccttccgtgcatcatgagagagttcgtgagcctctc

SEQ ID NO: 81 - DNA, 404 bp, Thlaspi arvense
  source 1..404: mol_type = other DNA
caaacacacgctcggacgcatattacacatgttcatacacttaatactcgctgttttgaattgatgttttaggaatatatatgtagctatctgatcggtcagtattttcacaggtcgtgatatgattcaattagcttccgactcattcatccaaataccgagtcgccaaaattcaaactagactcgttaaatgaatgaatgatgcggtagacaaattggatcattgattctctttgataatactcaccgatcagacagctctcttttgtattccaattttcttgattaatctttcctgcacaaaaacatgcttgatccactaagtgacatatatgctgccttcgtatatatagttctggtaaaattaacattttgggtttatctttatttaaggcatcgccatg

SEQ ID NO: 82 - DNA, 404 bp, Thlaspi arvense
  source 1..404: mol_type = other DNA
caaacacacgctcggacgcatattacacatgttcatacacttaatactcgctgttttgaattgatgttttaggaatatatatgtaggaacgtattacctacacattttcacaggtcgtgatatgattcaattagcttccgactcattcatccaaataccgagtcgccaaaattcaaactagactcgttaaatgaatgaatgatgcggtagacaaattggatcattgattctctttgataatgtgaaggtaatacgctcctctcttttgtattccaattttcttgattaatctttcctgcacaaaaacatgcttgatccactaagtgacatatatgctgccttcgtatatatagttctggtaaaattaacattttgggtttatctttatttaaggcatcgccatg

SEQ ID NO: 83 - DNA, 404 bp, Thlaspi arvense
  source 1..404: mol_type = other DNA
caaacacacgctcggacgcatattacacatgttcatacacttaatactcgctgttttgaattgatgttttaggaatatatatgtagtcagctccgagttatcaattttcacaggtcgtgatatgattcaattagcttccgactcattcatccaaataccgagtcgccaaaattcaaactagactcgttaaatgaatgaatgatgcggtagacaaattggatcattgattctctttgataattgaaaactcggagccgactctcttttgtattccaattttcttgattaatctttcctgcacaaaaacatgcttgatccactaagtgacatatatgctgccttcgtatatatagttctggtaaaattaacattttgggtttatctttatttaaggcatcgccatg

SEQ ID NO: 84 - DNA, 404 bp, Thlaspi arvense
  source 1..404: mol_type = other DNA
caaacacacgctcggacgcatattacacatgttcatacacttaatactcgctgttttgaattgatgttttaggaatatatatgtaggaacttgacagtataatcttttcacaggtcgtgatatgattcaattagcttccgactcattcatccaaataccgagtcgccaaaattcaaactagactcgttaaatgaatgaatgatgcggtagacaaattggatcattgattctctttgataagattttactgtcaagctcctctcttttgtattccaattttcttgattaatctttcctgcacaaaaacatgcttgatccactaagtgacatatatgctgccttcgtatatatagttctggtaaaattaacattttgggtttatctttatttaaggcatcgccatg

SEQ ID NO: 85 - DNA, 1998 bp, Thlaspi arvense
  source 1..1998: mol_type = genomic DNA
ctataaaatataatatttagcaccttgacaggattgtcagttattatattgttagagtgataaagatcatcatcacgtacatataaagagattataagataaaaataattttcggtactgtaggttttctgcaatttaaattatttaaaatatgtaattgagaaaatattcggtcgcctggtttatatagtcaagtgttacgaaaacatgtttgttttgtatgcaatttttgttttacttatttgagacataaatgagttattttataatgggctgttacagatatgtttaattaatataaattattggtttttaacttgttgattttttatttttatttttcaagctttagaaactgatgccacgtggcattgtgggagagagttttttttgcttaggtggatagcctaagaagccccaaataatcctttttatttagtatagattagtcacggcttccacgaaacaagttcaattaaatttaacggaaataaatggtaattaatgaaagtttgaattgtattaattactgcttccacgaaacaaccaaaaaaatcatttgacaaagtaatttgtgtacggtattagccacatggggccaatcctctatgtatatcggagttgttttgccaaatgcccaattcttactctagtaaatattaaaccattttgtagatcctaatcttgagtcaactcaaagtcctatgtttggaaactaaaaataagtttaaatcctctagactacgactaagttgtaaaaagaaatgttcaaaattccttagacattgaaattgaatacttcaattaaagaaaattttaccagcatgttcatagtagtagaccaccacagaacaaaattaatagtttttacattgcattcttatataataattttggagtataattgtaattataaacaaaataactaaaagaaaaggaaagtattcttgacatatttataggtactaatttgctagtacgactattaattatggagattaaatctagtatttgactaaccagaaacattttaaaggtaagtgataagttgataacctcgcaattatttttgaaagctattaatcactttagcagaatgtatacaagttctatattaacaagtttatctcaaaatcttgagatcctactaataaatcataacttttctcttattggtatgtcgaatctagtgtttaccaaactagaggtgttgaccgttagagacaattaaacaacttacatacatacaaaagtacaagccgaagaataatagtaataacagtgcattttctacaataattaaaacaaaaaagtatattaaaaattagcatttattccaattaataccaatattcgaaaattaatatggtagaaaagcaaaaagcttacgtaaattccacagattgtcaaaaccctgcaatgaaaaagttgccaaaaattgacgaggttggtccacaaaatttaaggttctttgcttcacactctatttataggcgaagagatgaaacagaggaaattaattactccttaacaaaggttgttttcactcaaccacatgccttctcaagtgtctgctgctcacattccccgagattctcatttacttactcctctatttggtacgtcctttatattacaattctagtattttttttttcattattcgttttgttcatacttcgtttcataaacatatatagttaatcttatattatacagtaactttgataaatatgtatcttaatttactcacgcagtttagagagacgattgatacgtggggactacttacgtacctgcatgattatataagttataaaagttattgcagaacattaaattactttgatagctcgagagcaatcattatataaagctatatttttaatcacaaatatacatctactcgaaagttttttttttaaaaaaaagatgaaatccctaaacaaacgttcccaaatgttctcatcactctccaaccacgattcaccacattca

SEQ ID NO: 86 - DNA, 1978 bp, Thlaspi arvense
  source 1..1978: mol_type = genomic DNA
agtaactgagaggaatgtaactgagagaaaaaagaaaagtaataattaaaataattgaaaataataagtaagagcatctagatagtccttaccaaaaaaaagatcatctagatagtctttccatagtatctgatttatataatactaatataatgtatttatataattaaattataaattaataaagagatgaaccaattcttaacagacatttgcctagagacatatctttattcttaacaaacatttggctagaaacatatctaatagtttcttgtttcaaaaatgtcttcgctttttttctgtttttctcccttcctttttccttattttttttatttttcttattcactaaatatactcccataatatctgctatataatattaatataatatatttatataattaaattaaaaattcataaagagatgaaccaattcttaatagatatttggctaaatacatatttaatatttttttgtttgaaagatatctttgctattttttttctgtttctttctcttcttttcttcttatatttcttattttttttattcaataaatatattttaaaaaacaccaattttcttataagaatatctgaaaataattgagaataattaaattaaatattttcttttagtaaaacttataattatatatatgctaaaaagatatgtgatatttattattctatctttaaagatttttttatcgtgaatcactattttcagttatccaacctaaaatgaatactcagagagcaaccacatcgaaagtgttagagattgaatgaatacagttcttaaaaggtttatttcacattaatgaagtctatcaaaacaaaatttatctaattacatctctataacaaaaatgataattctaaagttaaatgaaaaaaaaaaacaaaaaaatagagagaatttttctttaaaaaaaagataagaaagatcaataaaaccgacttcctcacattataaatagaaaagtcttcataatttgaagattcaatccgaaaatccctaaaattctagaaagtaagaccaaatgttcaaagttttctagtttaattttttcaagtgttcttacacacagtttagcaaaacgtgattgttaagctatctttgtaatcactctgagcttttgagtaataatgagatttaattttttaaacacacaaccttatattgctttttttctttgagtgatatcttggttaacaattgacgtcgtctgtagaaaataaagaataaattcttaagcaaaacaaggtttagagatgagctctccgaataagagcaatcaacacactcaaatccctacctttgatgagcacagcaacccccattgtcattggaaatcaaacaccacctccaccactagccacatgaacattgacccttgtctctaccggtgatcttgctgctgcaattcaacccgccctaaaaatcgatcacctaagaccttagttccaaattcgataacttgcaagctcagcaagcaagggatcaggaacaactcaacctcatggcaacctcggccactaaacaagttgcaccacttggacgaagacttgtctttgagacacccaccgtccacatcgtagcaagagccacaacagacacccaagcaaacaagacgaatgtcccagccctaactaatgaagcgttacatgccaaggtgggttatgaagtctcacctgccaaggtgggttagacgaatgtctctctgttagacacctccacttgaccacttgtttgaggatggtaaggagtagcaaccttatgcttaacaccatgcttccttagcagattctcaaaaactttgttgatgaagtggcttcctccatcacttataacacaccttggaacaccaaaccttgggaagatgattatcttgaaaagtttcagcacaaccctagcatcatttgttggactggctatggcttcaacccactttgagacatagtctac

SEQ ID NO: 87 - DNA, 1424 bp, Thlaspi arvense
  source 1..1424: mol_type = genomic DNA
tgctttgggagttatgatggaaaacctaattctctaactctgtttatatagggaagactcaggaaaaatcctaatatccttttctcttgggcttctgacacatgaacctttccttttcctattgagcctagatccagaacgttacaactagaatcagaatcgaacaacaagcgtatgcgcttaagaaatgatttttactcacactatatgggcgcgcatggcattgtcgtaagaattaaataagcttcgtcccactccttattggatttacgcacacagtcaatccacgtggttgtcataactaaatataattggtgaaaaaactaatttaaagacaaagtaagaagcggaaaccgaaggaaaagccaaacaacattatgtttatcgacaaaaaagccaaaacaacatttaatgttaatttttgtccaaaccaggaatacatcactcatacggtcatatataccataccccaaattgtatgtactacatgtgtacgtaactgatttatgtatatctatctatttctcttttattgtaggggtcaaaatctacctatcgatatttataaataggattttataagacattgttaaaatggaaaacatggtagctacttggccagcgattaacatcaataattaaaaatacgaattgtgaaacatctcactctcttccttttatcacaccaaaccacttctctttctttacttaccggtcaggtcaacaattctaccattccctttatttagtttttttttttcatctatctctcttttcatttttaacttttaaaaaatattagtccgaaaatcgcactcttttatattcgttgatgggcattaaaatattgtaaaaattaaaaaaaatgtgtaaattaaaacgcaatttgtttgcacctgcagcagtagtaacacacaagtcaaagcaatgtctgttttctcttgtatgtcggttagctattttatgtactgaaatatgttattctttctgaccaaaacatattaagaaatttgcattctgtaatttgatttatccaatcagtagaggacacgtaaccaagataattagatatttttattctatctgtatactactaattcatccaacgtctgttggacgaccaaccagtcaaaactcataaaagtcaacttttactacatcgtgaattttttggtcatgcatttatatacacatacatggaagaaaaaacaatactttacctatgtcaaaatgctgcaaaagcattaagatggtatgtatacatacatattgatataacagtggtcccatatatcattttaaatcatcataaagagtatccatcttctttcatattaacatccccttcaaagttataagatttttctctcttcattagagagagagagagagagaattaacacaagttttaatctccgggaaag

SEQ ID NO: 88 - DNA, 1982 bp, Thlaspi arvense
  source 1..1982: mol_type = genomic DNA
tttaagactctaacaatattgatgccaactctagaaaaggacaactgaacttattttgttttaagccttggctatattacattatcagttttacacttctacgtatacacaactttaatttttctatattactacatgcatactagatgttagaaatatcttatataagcatacatattaaattagttatgcgatatttaaaattaatgtatataaatattcagtttcaaagcttacgaatacgtaaaattaatcaatacaaaccgaaaccaaaaagccacttctcatctcaaaatgttaattacaaatttacaataagccgaatcactatctaaaaagcttttgggatcccgagacccaaaacatttcttcgtataagtgcaacaattatcgagtgtgatgagacacgtaaaaagcaaggatcgggacaacgattttcggctatatagtagtttctcatatctgactttattagcaaattactacataaaattgcttttaagtatgattaacggaacaagtataatgcgtttatttaattacagatctggctaaatgtaatatggtatcaaagctggaaagacaaatagtctaaggtttggaatttttcatctgtctataaaattcttaagacactgatagatcattaacttattttggagtcaccaatggacaaatcaataactattgatgtccaaaacccacaagacaagcctattttttttgcacgtgcaagtacaccggtggaagaattcatttgtatactgaatctgaaattataaaagattagaattggttgaagaatttacttcaaaacaagctagaagatggtgttatttaaataaacaatgttaaattatatcaatgactttcaaattttatcaaaacattttttgaaagagaatcacgcacaaagtatttcgaattacaaaacaattttttgcaataaattttatagttaaagcaaattttgtcaattattgaaaaaaattacttagataaaatatctaatttttttttttaaacaatgtctctataaaagatggattagccaagaaaatctgatggatgctacaacgcagggttggagatatggtgctgacactacatactattaattggttgatagaatcggtaaatatagatatgaatatcgaaatggagacaacaggaaactcaaccgtatggaaggaataaaatagaggaactttaaagagaacttgaggatatacaaacagatgactcacgtatgcaagagaagcttaatgagataacaaataactaaaggatgcgtatcgggatgagaaacaattctggcaacagaagagcagaaacttatggaacaaatgtggagattttaatacataattttataatacttcaacaaagcaacggaggactataaacagaatagtgggactacatgatagtcagggtgtatggataacttaggttgcatggaaactccctccgaggtacgtttctcgcttccgaaacgtttcggaaaccgaaactctcggaagctcgtcggaaacacaaaaatcacgtttcctaaaaattctaatttgtgaatactttggaaacacgtttccattttaaaaacacatgtttccattttggaaagaagataaaaactaattttttttgttttatgaaataaatagataattataaaaattagatttaaatgatcaatttaattatttatagtaaataataattgatttggtaactaaaattaattttgatattattaagtttgaaaattattctttccatgaattagaattagagatagtttggttaatgaaactaataaaattgataataaagaaaatcttctaaatttttgactttacatattttaatttttatagtttaataattatgtaaaaattatatattagattttgttgatttaaatattctacttataacataattagatctttaataattaatatatatatatacacatttcc

SEQ ID NO: 89 - DNA, 24 bp, Thlaspi arvense
  source 1..24: mol_type = other DNA
attgtatatcatgatccatggcga

SEQ ID NO: 90 - DNA, 24 bp, Thlaspi arvense
  source 1..24: mol_type = other DNA
aaactcgccatggatcatgatata

SEQ ID NO: 91 - DNA, 24 bp, Thlaspi arvense
  source 1..24: mol_type = other DNA
attgatctgatggatttggaaggt

SEQ ID NO: 92 - DNA, 24 bp, Thlaspi arvense
  source 1..24: mol_type = other DNA
aaacaccttccaaatccatcagat

SEQ ID NO: 93 - DNA, 24 bp, Thlaspi arvense
  source 1..24: mol_type = other DNA
attgttcgtgctgatgaatcttct

SEQ ID NO: 94 - DNA, 24 bp, Thlaspi arvense
  source 1..24: mol_type = other DNA
aaacagaagattcatcagcacgaa

SEQ ID NO: 95 - DNA, 24 bp, Thlaspi arvense
  source 1..24: mol_type = other DNA
attgacaacggtgcaataaagacg

SEQ ID NO: 96 - DNA, 24 bp, Thlaspi arvense
  source 1..24: mol_type = other DNA
aaaccgtctttattgcaccgttgt

SEQ ID NO: 97 - DNA, 24 bp, Thlaspi arvense
  source 1..24: mol_type = other DNA
attggcatgccctagcttccgatg

SEQ ID NO: 98 - DNA, 24 bp, Thlaspi arvense
  source 1..24: mol_type = other DNA
aaaccatcggaagctagggcatgc

SEQ ID NO: 99 - DNA, 24 bp, Thlaspi arvense
  source 1..24: mol_type = other DNA
attgatgcacggcattatcgccgg

SEQ ID NO: 100 - DNA, 24 bp, Thlaspi arvense
  source 1..24: mol_type = other DNA
aaacccggcgataatgccgtgcat

SEQ ID NO: 101 - DNA, 24 bp, Thlaspi arvense
  source 1..24: mol_type = other DNA
attgagtttcctggaccagtgtta

SEQ ID NO: 102 - DNA, 24 bp, Thlaspi arvense
  source 1..24: mol_type = other DNA
aaactaacactggtccaggaaact

SEQ ID NO: 103 - DNA, 24 bp, Thlaspi arvense
  source 1..24: mol_type = other DNA
attgccatcgaagacgcgactgtt

SEQ ID NO: 104 - DNA, 24 bp, Thlaspi arvense
  source 1..24: mol_type = other DNA
aaacaacagtcgcgtcttcgatgg

SEQ ID NO: 105 - DNA, 24 bp, Thlaspi arvense
  source 1..24: mol_type = other DNA
attggttctctgcgatgctcacat

SEQ ID NO: 106 - DNA, 24 bp, Thlaspi arvense
  source 1..24: mol_type = other DNA
aaacatgtgagcatcgcagagaac

SEQ ID NO: 107 - DNA, 24 bp, Thlaspi arvense
  source 1..24: mol_type = other DNA
attggaccgatacttgaagaccag

SEQ ID NO: 108 - DNA, 24 bp, Thlaspi arvense
  source 1..24: mol_type = other DNA
aaacctggtcttcaagtatcggtc

SEQ ID NO: 109 - DNA, 20 bp, Thlaspi arvense
  source 1..20: mol_type = other DNA
cggaagaggctgcgttagag

SEQ ID NO: 110 - DNA, 20 bp, Thlaspi arvense
  source 1..20: mol_type = other DNA
gcagctaagggaactttacg

SEQ ID NO: 111 - DNA, 20 bp, Thlaspi arvense
  source 1..20: mol_type = other DNA
cggaagaggctgcgttagag

SEQ ID NO: 112 - DNA, 20 bp, Thlaspi arvense
  source 1..20: mol_type = other DNA
caggaaaggcgtatgcgagg

SEQ ID NO: 113 - DNA, 20 bp, Thlaspi arvense
  source 1..20: mol_type = other DNA
cgccgtcggaagcttcctcg

SEQ ID NO: 114 - DNA, 20 bp, Thlaspi arvense
  source 1..20: mol_type = other DNA
caaacaagacctgaggtaca

SEQ ID NO: 115 - DNA, 20 bp, Thlaspi arvense
  source 1..20: mol_type = other DNA
agcattccaccatcatctac

SEQ ID NO: 116 - DNA, 20 bp, Thlaspi arvense
  source 1..20: mol_type = other DNA
tcgactggaacgacgtcgag

SEQ ID NO: 117 - DNA, 1188 bp, Thlaspi arvense
  source 1..1188: mol_type = genomic DNA
atggtgatgggtacacaaccgtcgttggaagagatcagaaaggcacagagagcggatggccccgcaggcatcttggggataggcacggccaaccctgcgaaccatgtgatccaggcagagtatccggactactacttccgcatcaccaacagtgagcacatgactgacctcaaggagaagttcaagcgcatgtgcgacaagtcgatgatacggaaacggcacatgcacctgacggaggagttcctgaaggagaatccggacatgtgcgcctacatggctccttctcttgatgtgaggcaggacatcgtggtggtcgaggtccctaagctagggaaagaggcggcagtgaaggccatcaaggagtggggtcagcccaagtccaagatcacccacgtcgtcttctgcactacatccggagttgacatgcctggtgctgactaccagctcaccaagctcctcggtcttcgcccttccgtcaagcgtctcatgatgtaccagcaaggttgctacgccggcggcactgtcctccgactcgccaaggacctcgctgagaataaccgtggtgctcgtgtccttgtcgtctgctccaagatcacagccgtcaccttccgtggcccctctgacacacacctcgactccctcgttggtcaggctctcttcagtgacggtgctgccgcgctcattgttggtgcggaccctgatgcctccgtgggagagaagcctatcttcgagatggtgtctgctgcacagaccatcctcccagactcggacggagccatagatggacacttgagggaagttgggctcaccttccatctcctcaaggacgtccctgggctcatctcgaagaacatagagaagagtctagaagaagcgtttaaaccgctcgggataagtgactggaactctctcttttggatagctcaccctggaggtcctgcgatcctggaccaggttgagttaaagctaggactcaaggaagagaagatgagggccacgcgtcacgtgctgagcgagtacggaaacatgtcgagcgcgtgcgttctcttcattatggacgagatgaggaggaagtccaaggaggatggtgtggccacgacaggagaagggttggagtggggtgtcttgtttggtttcggaccaggtctcaccgtagagacagtcgtcttgcacagcgtccctgtttga

SEQ ID NO: 118 - protein, 395 aa, Thlaspi arvense
MVMGTQPSLEEIRKAQRADGPAGILGIGTANPANHVIQAEYPDYYFRITNSEHMTDLKEKFKRMCDKSMIRKRHMHLTEEFLKENPDMCAYMAPSLDVRQDIVVVEVPKLGKEAAVKAIKEWGQPKSKITHVVFCTTSGVDMPGADYQLTKLLGLRPSVKRLMMYQQGCYAGGTVLRLAKDLAENNRGARVLVVCSKITAVTFRGPSDTHLDSLVGQALFSDGAAALIVGADPDASVGEKPIFEMVSAAQTILPDSDGAIDGHLREVGLTFHLLKDVPGLISKNIEKSLEEAFKPLGISDWNSLFWIAHPGGPAILDQVELKLGLKEEKMRATRHVLSEYGNMSSACVLFIMDEMRRKSKEDGVATTGEGLEWGVLFGFGPGLTVETVVLHSVPV

SEQ ID NO: 119 - DNA, 1188 bp, Thlaspi arvense
  source 1..1188: mol_type = genomic DNA
atggtgatgggtacacaaccgtcgttggaagagatcagaaaggcacagagagcggatggccccgcaggcatcttggggataggcacggccaaccctgcgaaccatgtgatccaggcagagtatccggactactacttccgcatcaccaacagtgagcacatgactgacctcaaggagaagttcaagcgcatgtgcgacaagtcgatgatacggaaacggcacatgcacctgacggaggagttcctgaaggagaatccggacatgtgcgcctacatggctccttctcttgatgtgaggcaggacatcgtggtggtcgaggtccctaagctagggaaagaggcggcagtgaaggccatcaaggagtggggtcagcccaagtccaagatcacccacgtcgtcttctgcactacatccggagttgacatgcctggtgctgactaccagctcaccaagctcctcggtcttcgcccttccgtcaagcgtctcatgatgtaccagcaaggttgctacgccggcggcactgtcctccgactcgccaaggacctcgctgagaataaccgtggtgctcgtgtccttgtcgtctgctccgagatcacagccgtcaccttccgtggcccctctgacacacacctcgactccctcgttggtcaggctctcttcagtgacggtgctgccgcgctcattgttggtgcggaccctgatgcctccgtgggagagaagcctatcttcgagatggtgtctgctgcacagaccatcctcccagactcggacggagccatagatggacacttgagggaagttgggctcaccttccatctcctcaaggacgtccctgggctcatctcgaagaacatagagaagagtctagaagaagcgtttaaaccgctcgggataagtgactgaaactctctcttttggatagctcaccctggaggtcctgcgatcctggaccaggttgagttaaagctaggactcaaggaagagaagatgagggccacgcgtcacgtgctgagcgagtacggaaacatgtcgagcgcgtgcgttctcttcattatggacgagatgaggaggaagtccaaggaggatggtgtggccacgacaggagaagggttggagtggggtgtcttgtttggtttcggaccaggtctcaccgtagagacagtcgtcttgcacagcgtccctgtttga

SEQ ID NO: 120 - protein, 300 aa, Thlaspi arvense
MVMGTQPSLEEIRKAQRADGPAGILGIGTANPANHVIQAEYPDYYFRITNSEHMTDLKEKFKRMCDKSMIRKRHMHLTEEFLKENPDMCAYMAPSLDVRQDIVVVEVPKLGKEAAVKAIKEWGQPKSKITHVVFCTTSGVDMPGADYQLTKLLGLRPSVKRLMMYQQGCYAGGTVLRLAKDLAENNRGARVLVVCSEITAVTFRGPSDTHLDSLVGQALFSDGAAALIVGADPDASVGEKPIFEMVSAAQTILPDSDGAIDGHLREVGLTFHLLKDVPGLISKNIEKSLEEAFKPLGISD

SEQ ID NO: 121 - DNA, 1239 bp, Thlaspi arvense
  source 1..1239: mol_type = genomic DNA
atggctccagggactctcaccgagctcgccggagaggctaagctcaactctaaattcgtccgggacgaggacgaacgtcccaaggtggcatacaacaagtttagcgacgatatcccggtgatatctctcgccggactcgacgatgttggtgggaaaagaggagagatctgccgtaagatcgttgaggcttgcgagaattggggcgtgttccaggtggtcgatcatggtgtcgataccaatttggtagaggatatgactcgcctcgctcgcgacttctttgctttaccacccgaagagaaacttagtttcgacatgtctggtggtaagaaaggcggcttcatcgtctctagtcaccttcagggagagactgtgtaagattggagagagatcgtgacgtacttctcgtacccggtgagaaacagagactactcacggtggccagataagccggaagggtgggtgaaagtgacggaggagtacagcgacaaactgatgggtttagcttgtaagcttcttgaggttttgtctgaagctatggggctcgagaaagaagcacttaccaatgcttgcgtcgatatggaccaaaagatagttgttaattattaccctaaatgccctcagcctgatctcaccctcggactcaagcgtcacactgatcctggaaccatcactttgctgctccaagaccaggtcggtggattacaagccacacgcgacgatggcaaaacatggataacggttcagccaattgagggagcttttgtcgtgaatctcggcgaccatggtcactatttgagcaacgggaggttcaagaacgcggatcatcaggcggtggtgaattccaactcgagcaggctatctatagccacgtttcagaatccggcgcaggatgcaaccgtgtatccgcttaaagttagagaaggagagaagccgatcttggaggagccaatcacttttgcagagatgtataagagaaagatgggaaaagatctggagctggctcgcctcaagaagcttgcgaaagaagaaaatgaccagaagctggccaaagaagaacatgacaagaacctggccaaagaagaaaatgatcagaagctggctaaagaagaacatgaccagaagctggccaaagaagaacatgacaagagccttgccaaagaagaaaattaccaaaagctggccaaagatgaacatagccacacggaagctgttaagcgtctcggccaaatcctcgcttag

SEQ ID NO: 122 - protein, 124 aa, Thlaspi arvense
MAPGTLTELAGEAKLNSKFVRDEDERPKVAYNKFSDDIPVISLAGLDDVGGKRGEICRKIVEACENWGVFQVVDHGVDTNLVEDMTRLARDFFALPPEEKLSFDMSGGKKGGFIVSSHLQGETV

SEQ ID NO: 123 - DNA, 1239 bp, Thlaspi arvense
  source 1..1239: mol_type = genomic DNA
atggctccagggactctcaccgagctcgccggagaggctaagctcaactctaaattcgtccgggacgaggacgaacgtcccaaggtggcatacaacaagtttagcgacgatatcccggtgatatctctcgccggactcgacgatgttggtgggaaaagaggagagatctgccgtaagatcgttgaggcttgcgagaattggggcgtgttccaggtggtcgatcatggtgtcgataccaatttggtagaggatatgactcgcctcgctcgcgacttctttgctttaccacccgaagagaaacttagtttcgacatgtctggtggtaagaaaggcggcttcatcgtctctagtcaccttcagggagagactgtgcaagattggagagagatcgtgacgtacttctcgtacccggtgagaaacagagactactcacggtggccagataagccggaagggtgggtgaaagtgacggaggagtacagcgacaaactgatgggtttagcttgtaagcttcttgaggttttgtctgaagctatggggctcgagaaagaagcacttaccaatgcttgcgtcgatatggaccaaaagatagttgttaattattaccctaaatgccctcagcctgatctcaccctcggactcaagcgtcacactgatcctggaaccatcactttgctgctccaagaccaggtcggtggattacaagccacacgcgacgatggcaaaacatggataacggttcagccaattgagggagcttttgtcgtgaatctcggcgaccatggtcactatttgagcaacgggaggttcaagaacgcggatcatcaggcggtggtgaattccaactcgagcaggctatctatagccacgtttcagaatctggcgcaggatgcaaccgtgtatccgcttaaagttagagaaggagagaagccgatcttggaggagccaatcacttttgcagagatgtataagagaaagatgggaaaagatctggagctggctcgcctcaagaagcttgcgaaagaagaaaatgaccagaagctggccaaagaagaacatgacaagaacctggccaaagaagaaaatgatcagaagctggctaaagaagaacatgaccagaagctggccaaagaagaacatgacaagagccttgccaaagaagaaaattaccaaaagctggccaaagatgaacatagccacacggaagctgttaagcgtctcggccaaatcctcgcttag

SEQ ID NO: 124 - protein, 412 aa, Thlaspi arvense
MAPGTLTELAGEAKLNSKFVRDEDERPKVAYNKFSDDIPVISLAGLDDVGGKRGEICRKIVEACENWGVFQVVDHGVDTNLVEDMTRLARDFFALPPEEKLSFDMSGGKKGGFIVSSHLQGETVQDWREIVTYFSYPVRNRDYSRWPDKPEGWVKVTEEYSDKLMGLACKLLEVLSEAMGLEKEALTNACVDMDQKIVVNYYPKCPQPDLTLGLKRHTDPGTITLLLQDQVGGLQATRDDGKTWITVQPIEGAFVVNLGDHGHYLSNGRFKNADHQAVVNSNSSRLSIATFQNLAQDATVYPLKVREGEKPILEEPITFAEMYKRKMGKDLELARLKKLAKEENDQKLAKEEHDKNLAKEENDQKLAKEEHDQKLAKEEHDKSLAKEENYQKLAKDEHSHTEAVKRLGQILA

SEQ ID NO: 125 - DNA, 1545 bp, Thlaspi arvense
  source 1..1545: mol_type = genomic DNA
atggccactctcttactcacaatcctcctccccactttcctcttcctcctcgtcctcctcctttctctccgccgcaaccacaaccgcagtagccgtctcccaccaggcccaaaaccatggcccatcctcggaaacctccctcacatgggtcctaaaccccatcgaaccctagccgccatggtaaccacctacggtccaatcctccacctccgattagggttctccaacgtcgtggttgctgcgtctaaatccgtggccgaacagttcttcaaaatccatgatgccaatttcgctagccgaccaccaaattcaagagccaaacacatggcatataactatcaagatcttgtctttgcgccttacggacaacgatggagaatgttgaggaagattagttctgttcatttattttcagctaaagctcttgaagattacaagcatgttcggcaggaagaggtaggaacgctcacgcgcgagctagtggatgcaggcacgaaacccgtaaacttaggccagttggtgaacatgtgtgtggtcaacgcgcttggaagagagatgatcggacggcgtctgttcggcgccggagctgatcacaaagcggaggagtttcgatcgatggtgacggaaatgatggctctcgccggagtattcaacctcggagatttcgtgccggctctggattggttagatttacaaggcgttgctggtaaaatgaaacggctacacaaaagattcgacacttttctatcgtcgattttgaaggagcacgagatgatgcacggtcaagatcaaaagcataaagatatgctcagcactttaatctcgctcaagggaactgattttgacggtgacggcggaagcctaacggatactgagatcaaagccttgctcttgaacatgtttacggctggaactgacacgtcagcaagtacggtggactgggccatagctgaactgatacgacacccggatgcaatgaccagagcccaagaagaacttgattcagttgtaggccgcgataggcccattaacgagtcagacctttctcggcttccttatcttcaggcggttatcaaagagaatttcaggcttcatccgccgacaccactctcgttaccacacatcgcatcagagagctgtgagatcaacggctaccatatcccgaaaggatcgactcttttaacaaacatatgggccatagcccgtgacccggaacaatggtccgacccgttatcgtttcgacccgagagatttttacagggtggagaaaaatccggcgtcgatgtgaaaggaagcgatttcgagcttataccgttcggagccgggaggagaatctgcgctgggctcagtttagggctacggatgattcagttactgacggcgacgctggttcacggatttgattgggaattggccggaggaattccgccggagaagctgaatatggaggagacttatgggattactctgcaaagagcagttcctttggtggtgcatcctaagccaaggttggctcccagtgtttacgaactcgggtcgcgctaa

SEQ ID NO: 126 - protein, 514 aa, Thlaspi arvense
MATLLLTILLPTFLFLLVLLLSLRRNHNRSSRLPPGPKPWPILGNLPHMGPKPHRTLAAMVTTYGPILHLRLGFSNVVVAASKSVAEQFFKIHDANFASRPPNSRAKHMAYNYQDLVFAPYGQRWRMLRKISSVHLFSAKALEDYKHVRQEEVGTLTRELVDAGTKPVNLGQLVNMCVVNALGREMIGRRLFGAGADHKAEEFRSMVTEMMALAGVFNLGDFVPALDWLDLQGVAGKMKRLHKRFDTFLSSILKEHEMMHGQDQKHKDMLSTLISLKGTDFDGDGGSLTDTEIKALLLNMFTAGTDTSASTVDWAIAELIRHPDAMTRAQEELDSVVGRDRPINESDLSRLPYLQAVIKENFRLHPPTPLSLPHIASESCEINGYHIPKGSTLLTNIWAIARDPEQWSDPLSFRPERFLQGGEKSGVDVKGSDFELIPFGAGRRICAGLSLGLRMIQLLTATLVHGFDWELAGGIPPEKLNMEETYGITLQRAVPLVVHPKPRLAPSVYELGSR

SEQ ID NO: 127 - DNA, 1581 bp, Thlaspi arvense
  source 1..1581: mol_type = genomic DNA
atggatgaatcaagtatttttacggcaaagaaagtgatcggagctgagaaaagagagcttcaagggctgcttaaggcggcggtgcaatctgtggagtggacttatagtctcttctggcaactttgtcctcaacaaagggttttgctgtgggagaatggatactacaacggtgcaataaagacgaggaagacaactcagccggcggaagtgacggcggaagaggctgcgttagagaggagtcagcagctaagggaactttacgaggcccttttggccggagagtcctcatcggaagctagggcatgcacggcattatcgccggaggatctgacggagactgaatggttttatctaatgtgtgtctctttctctttccctcctccttccgggatgccaggaaaggcgtatgcgaggaggaaacacgtatggctatgtggtgcaaatgaggttgacagtaaaatcttttctagggctattctcgcaaagagtgccaaaatccagcagacagtggtttgcattcccatgcttgatggcgttgtggaactaggcacaacgaacaaggtaaaagaagatatagcgtttgttgagctcataaagagttttttccataaccaccccaagtcaaacccaaaagctgctctttctgaacactccatcaacgaagagcacgaagaagacgaagaacaagaagaagaagaagaagaagaagtagaagaagaaatgacaatgtcagaggagataaggcttggctctcctgatgatgatgacgtctccaatcaaaacctactctctgatttccatgtagaatcaacccacactttagacacacacatggacatgatgaatctaatggaggagggtggaaactattctcagacagtatcaacacttcttatgtcacaacccacgagtcttttttcagattcagtttccacatcttcttacatccaatcatcatttgccacatggaaggctgataattttaaagagcatcagcgagtggaaactaaatcgacgtcgtcgtcgcaatggatgctcaaacacataatcttgagagttcctttactccacgaccacactaaagaaaagaggctgcctcgagaagagcttaatcacgtggtggcagagcgccgcaggagagagaagctgaatgagagattcataacactgagatcattggttccctttgtgaccaagatggataaagtctcaattcttggagacaccatcaactacgtaaaccatcttcgaaatagggtccaagagctggagactaatcatcacgaacaaaaacataagcggatgcgtagctgtaagggaaaaacgtgggaagaggtcgttgaggtttccatcatagagagtgatgttttgttagagatgagatgcgagtaccgagatggtctattgctcgacatccttcaggttcttaaggaacatggtatagagactactgcagttcataccgcggtgaacgagcgtgatttcgaggccgagataagggctatggtgagagggaagaaaccaagcattgctgaggtcaaaagagccatccatcaaactatatccaatattaaactatag

SEQ ID NO: 128 - protein, 526 aa, Thlaspi arvense
MDESSIFTAKKVIGAEKRELQGLLKAAVQSVEWTYSLFWQLCPQQRVLLWENGYYNGAIKTRKTTQPAEVTAEEAALERSQQLRELYEALLAGESSSEARACTALSPEDLTETEWFYLMCVSFSFPPPSGMPGKAYARRKHVWLCGANEVDSKIFSRAILAKSAKIQQTVVCIPMLDGVVELGTTNKVKEDIAFVELIKSFFHNHPKSNPKAALSEHSINEEHEEDEEQEEEEEEEVEEEMTMSEEIRLGSPDDDDVSNQNLLSDFHVESTHTLDTHMDMMNLMEEGGNYSQTVSTLLMSQPTSLFSDSVSTSSYIQSSFATWKADNFKEHQRVETKSTSSSQWMLKHIILRVPLLHDHTKEKRLPREELNHVVAERRRREKLNERFITLRSLVPFVTKMDKVSILGDTINYVNHLRNRVQELETNHHEQKHKRMRSCKGKTWEEVVEVSIIESDVLLEMRCEYRDGLLLDILQVLKEHGIETTAVHTAVNERDFEAEIRAMVRGKKPSIAEVKRAIHQTISNIKL

SEQ ID NO: 129 - DNA, 1581 bp, Thlaspi arvense
  source 1..1581: mol_type = genomic DNA
atggatgaatcaagtatttttacggcagagaaagtgatcggagctgagaaaagagagcttcaagggctgcttaaggcggcggtgcaatctgtggagtggacttatagtctcttctggcaactttgtcctcaacaaagggttttgctgtgggagaatggatactacaacggtgcaataaagacgaggaagacaactcagccggcggaagtgacggcggaagaggctgcgttagagaggagtcagcagctaagggaactttacgaggcccttttggccggagagtcctcatcggaagctagggcatgcacggcattatcgccggaggatctgacggagactgaatggttttatctaatgtgtgtctctttctctttccctcctccttccgggatgccaggaaaggcgtatgcgaggaggaaacacgtatggctatgtggtgcaaatgaggttgacagtaaaatcttttctagggctattctcgcaaagagtgccaaaatccagcagacagtggtttgcattcccatgcttgatggcgttgtggaactaggcacaacgaacaaggtaaaagaagatatagcgtttgttgagctcataaagagttttttccataaccaccccaagtcaaacccaaaagctgctctttctgaacactccatcaacgaagagcacgaagaagacgaagaacaagaagaagaagaagaagaagaagtagaagaagaaatgacaatgtcagaggagataaggcttggctctcctgatgatgatgacgtctccaatcaaaacctactctctgatttccatgtagaatcaacccacactttagacacacacatggacatgatgaatctaatggaggagggtggaaactattctcagacagtatcaacacttcttatgtcacaacccacgagtcttttttcagattcagtttccacatcttcttacatctaatcatcatttgccacatggaaggctgataattttaaagagcatcagcgagtggaaactaaatcgacgtcgtcgtcgcaatggatgctcaaacacataatcttgagagttcctttactccacgaccacactaaagaaaagaggctgcctcgagaagagcttaatcacgtggtggcagagcgccgcaggagagagaagctgaatgagagattcataacactgagatcattggttccctttgtgaccaagatggataaagtctcaattcttggagacaccatcaactacgtaaaccatcttcgaaatagggtccaagagctggagactaatcatcacgaacaaaaacataagcggatgcgtagctgtaagggaaaaacgtgggaagaggtcgttgaggtttccatcatagagagtgatgttttgttagagatgagatgcgagtaccgagatggtctattgctcgacatccttcaggttcttaaggaacatggtatagagactactgcagttcataccgcggtgaacgagcgtgatttcgaggccgagataagggctatggtgagagggaagaaaccaagcattgctgaggtcaaaagagccatccatcaaactatatccaatattaaactatag

SEQ ID NO: 130 - protein, 316 aa, Thlaspi arvense
MDESSIFTAEKVIGAEKRELQGLLKAAVQSVEWTYSLFWQLCPQQRVLLWENGYYNGAIKTRKTTQPAEVTAEEAALERSQQLRELYEALLAGESSSEARACTALSPEDLTETEWFYLMCVSFSFPPPSGMPGKAYARRKHVWLCGANEVDSKIFSRAILAKSAKIQQTVVCIPMLDGVVELGTTNKVKEDIAFVELIKSFFHNHPKSNPKAALSEHSINEEHEEDEEQEEEEEEEVEEEMTMSEEIRLGSPDDDDVSNQNLLSDFHVESTHTLDTHMDMMNLMEEGGNYSQTVSTLLMSQPTSLFSDSVSTSSYI

SEQ ID NO: 131 - DNA, 1581 bp, Thlaspi arvense
  source 1..1581: mol_type = genomic DNA
atggatgaatcaagtatttttacggcagagaaagtgatcggagctgagaaaagagagcttcaagggctgcttaaggcggcggtgcaatctgtggagtggacttatagtctcttctggcaactttgtcctcaacaaagggttttgctgtgggagaatggatactacaacggtgcaataaagacgaggaagacaactcagccggcggaagtgacggcggaagaggctgcgttagagaggagtcagcagctaagggaactttacgaggcccttttggccggagagtcctcatcggaagctagggcatgcacggcattatcgccggaggatctgacggagactgaatggttttatctaatgtgtgtctctttctctttccctcctccttccgggatgccaggaaaggcgtatgcgaggaggaaacacgtatggctatgtggtgcaaatgaggttgacagtaaaatcttttctagggctattctcgcaaagagtgccaaaatccagcagacagtggtttgcattcccatgcttgatggcgttgtggaactaggcacaacgaacaaggtaaaagaagatatagcgtttgttgagctcataaagagttttttccataaccaccccaagtcaaacccaaaagctgctctttctgaacactccatcaacgaagagcacgaagaagacgaagaacaagaagaagaagaagaagaagaagtagaagaagaaatgacaatgtcagaggagataaggcttggctctcctgatgatgatgacgtctccaatcaaaacctactctctgatttccatgtagaatcaacccacactttagacacacacatggacatgatgaatctaatggaggagggtggaaactattctcagacagtatcaacacttcttatgtcacaacccacgagtcttttttcagattcagtttccacatcttcttacatccaatcatcatttgccacatgaaaggctgataattttaaagagcatcagcgagtggaaactaaatcgacgtcgtcgtcgcaatggatgctcaaacacataatcttgagagttcctttactccacgaccacactaaagaaaagaggctgcctcgagaagagcttaatcacgtggtggcagagcgccgcaggagagagaagctgaatgagagattcataacactgagatcattggttccctttgtgaccaagatggataaagtctcaattcttggagacaccatcaactacgtaaaccatcttcgaaatagggtccaagagctggagactaatcatcacgaacaaaaacataagcggatgcgtagctgtaagggaaaaacgtgggaagaggtcgttgaggtttccatcatagagagtgatgttttgttagagatgagatgcgagtaccgagatggtctattgctcgacatccttcaggttcttaaggaacatggtatagagactactgcagttcataccgcggtgaacgagcgtgatttcgaggccgagataagggctatggtgagagggaagaaaccaagcattgctgaggtcaaaagagccatccatcaaactatatccaatattaaactatag

SEQ ID NO: 132 - protein, 322 aa, Thlaspi arvense
MDESSIFTAEKVIGAEKRELQGLLKAAVQSVEWTYSLFWQLCPQQRVLLWENGYYNGAIKTRKTTQPAEVTAEEAALERSQQLRELYEALLAGESSSEARACTALSPEDLTETEWFYLMCVSFSFPPPSGMPGKAYARRKHVWLCGANEVDSKIFSRAILAKSAKIQQTVVCIPMLDGVVELGTTNKVKEDIAFVELIKSFFHNHPKSNPKAALSEHSINEEHEEDEEQEEEEEEEVEEEMTMSEEIRLGSPDDDDVSNQNLLSDFHVESTHTLDTHMDMMNLMEEGGNYSQTVSTLLMSQPTSLFSDSVSTSSYIQSSFAT

SEQ ID NO: 133 - DNA, 1582 bp, Thlaspi arvense
  source 1..1582: mol_type = genomic DNA
atggatgaatcaagtatttttacggcagagaaagtgatcggagctgagaaaagagagcttcaagggctgcttaaggcggcggtgcaatctgtggagtggacttatagtctcttctggcaactttgtcctcaacaaagggttttgctgtgggagaatggatactacaacggtgcaataaagaacgaggaagacaactcagccggcggaagtgacggcggaagaggctgcgttagagaggagtcagcagctaagggaactttacgaggcccttttggccggagagtcctcatcggaagctagggcatgcacggcattatcgccggaggatctgacggagactgaatggttttatctaatgtgtgtctctttctctttccctcctccttccgggatgccaggaaaggcgtatgcgaggaggaaacacgtatggctatgtggtgcaaatgaggttgacagtaaaatcttttctagggctattctcgcaaagagtgccaaaatccagcagacagtggtttgcattcccatgcttgatggcgttgtggaactaggcacaacgaacaaggtaaaagaagatatagcgtttgttgagctcataaagagttttttccataaccaccccaagtcaaacccaaaagctgctctttctgaacactccatcaacgaagagcacgaagaagacgaagaacaagaagaagaagaagaagaagaagtagaagaagaaatgacaatgtcagaggagataaggcttggctctcctgatgatgatgacgtctccaatcaaaacctactctctgatttccatgtagaatcaacccacactttagacacacacatggacatgatgaatctaatggaggagggtggaaactattctcagacagtatcaacacttcttatgtcacaacccacgagtcttttttcagattcagtttccacatcttcttacatccaatcatcatttgccacatggaaggctgataattttaaagagcatcagcgagtggaaactaaatcgacgtcgtcgtcgcaatggatgctcaaacacataatcttgagagttcctttactccacgaccacactaaagaaaagaggctgcctcgagaagagcttaatcacgtggtggcagagcgccgcaggagagagaagctgaatgagagattcataacactgagatcattggttccctttgtgaccaagatggataaagtctcaattcttggagacaccatcaactacgtaaaccatcttcgaaatagggtccaagagctggagactaatcatcacgaacaaaaacataagcggatgcgtagctgtaagggaaaaacgtgggaagaggtcgttgaggtttccatcatagagagtgatgttttgttagagatgagatgcgagtaccgagatggtctattgctcgacatccttcaggttcttaaggaacatggtatagagactactgcagttcataccgcggtgaacgagcgtgatttcgaggccgagataagggctatggtgagagggaagaaaccaagcattgctgaggtcaaaagagccatccatcaaactatatccaatattaaactatag

SEQ ID NO: 134 - protein, 99 aa, Thlaspi arvense
MDESSIFTAEKVIGAEKRELQGLLKAAVQSVEWTYSLFWQLCPQQRVLLWENGYYNGAIKNEEDNSAGGSDGGRGCVREESAAKGTLRGPFGRRVLIGS

SEQ ID NO: 135 - DNA, 1579 bp, Thlaspi arvense
  source 1..1579: mol_type = genomic DNA
atggatgaatcaagtatttttacggcagagaaagtgatcggagctgagaaaagagagcttcaagggctgcttaaggcggcggtgcaatctgtggagtggacttatagtctcttctggcaactttgtcctcaacaaagggttttgctgtgggagaatggatactacaacggtgcaataaacgaggaagacaactcagccggcggaagtgacggcggaagaggctgcgttagagaggagtcagcagctaagggaactttacgaggcccttttggccggagagtcctcatcggaagctagggcatgcacggcattatcgccggaggatctgacggagactgaatggttttatctaatgtgtgtctctttctctttccctcctccttccgggatgccaggaaaggcgtatgcgaggaggaaacacgtatggctatgtggtgcaaatgaggttgacagtaaaatcttttctagggctattctcgcaaagagtgccaaaatccagcagacagtggtttgcattcccatgcttgatggcgttgtggaactaggcacaacgaacaaggtaaaagaagatatagcgtttgttgagctcataaagagttttttccataaccaccccaagtcaaacccaaaagctgctctttctgaacactccatcaacgaagagcacgaagaagacgaagaacaagaagaagaagaagaagaagaagtagaagaagaaatgacaatgtcagaggagataaggcttggctctcctgatgatgatgacgtctccaatcaaaacctactctctgatttccatgtagaatcaacccacactttagacacacacatggacatgatgaatctaatggaggagggtggaaactattctcagacagtatcaacacttcttatgtcacaacccacgagtcttttttcagattcagtttccacatcttcttacatccaatcatcatttgccacatggaaggctgataattttaaagagcatcagcgagtggaaactaaatcgacgtcgtcgtcgcaatggatgctcaaacacataatcttgagagttcctttactccacgaccacactaaagaaaagaggctgcctcgagaagagcttaatcacgtggtggcagagcgccgcaggagagagaagctgaatgagagattcataacactgagatcattggttccctttgtgaccaagatggataaagtctcaattcttggagacaccatcaactacgtaaaccatcttcgaaatagggtccaagagctggagactaatcatcacgaacaaaaacataagcggatgcgtagctgtaagggaaaaacgtgggaagaggtcgttgaggtttccatcatagagagtgatgttttgttagagatgagatgcgagtaccgagatggtctattgctcgacatccttcaggttcttaaggaacatggtatagagactactgcagttcataccgcggtgaacgagcgtgatttcgaggccgagataagggctatggtgagagggaagaaaccaagcattgctgaggtcaaaagagccatccatcaaactatatccaatattaaactatag

SEQ ID NO: 136 - protein, 98 aa, Thlaspi arvense
MDESSIFTAEKVIGAEKRELQGLLKAAVQSVEWTYSLFWQLCPQQRVLLWENGYYNGAINEEDNSAGGSDGGRGCVREESAAKGTLRGPFGRRVLIGS

SEQ ID NO: 137 - DNA, 1582 bp, Thlaspi arvense
  source 1..1582: mol_type = genomic DNA
atggatgaatcaagtatttttacggcagagaaagtgatcggagctgagaaaagagagcttcaagggctgcttaaggcggcggtgcaatctgtggagtggacttatagtctcttctggcaactttgtcctcaacaaagggttttgctgtgggagaatggatactacaacggtgcaataaaggacgaggaagacaactcagccggcggaagtgacggcggaagaggctgcgttagagaggagtcagcagctaagggaactttacgaggcccttttggccggagagtcctcatcggaagctagggcatgcacggcattatcgccggaggatctgacggagactgaatggttttatctaatgtgtgtctctttctctttccctcctccttccgggatgccaggaaaggcgtatgcgaggaggaaacacgtatggctatgtggtgcaaatgaggttgacagtaaaatcttttctagggctattctcgcaaagagtgccaaaatccagcagacagtggtttgcattcccatgcttgatggcgttgtggaactaggcacaacgaacaaggtaaaagaagatatagcgtttgttgagctcataaagagttttttccataaccaccccaagtcaaacccaaaagctgctctttctgaacactccatcaacgaagagcacgaagaagacgaagaacaagaagaagaagaagaagaagaagtagaagaagaaatgacaatgtcagaggagataaggcttggctctcctgatgatgatgacgtctccaatcaaaacctactctctgatttccatgtagaatcaacccacactttagacacacacatggacatgatgaatctaatggaggagggtggaaactattctcagacagtatcaacacttcttatgtcacaacccacgagtcttttttcagattcagtttccacatcttcttacatccaatcatcatttgccacatggaaggctgataattttaaagagcatcagcgagtggaaactaaatcgacgtcgtcgtcgcaatggatgctcaaacacataatcttgagagttcctttactccacgaccacactaaagaaaagaggctgcctcgagaagagcttaatcacgtggtggcagagcgccgcaggagagagaagctgaatgagagattcataacactgagatcattggttccctttgtgaccaagatggataaagtctcaattcttggagacaccatcaactacgtaaaccatcttcgaaatagggtccaagagctggagactaatcatcacgaacaaaaacataagcggatgcgtagctgtaagggaaaaacgtgggaagaggtcgttgaggtttccatcatagagagtgatgttttgttagagatgagatgcgagtaccgagatggtctattgctcgacatccttcaggttcttaaggaacatggtatagagactactgcagttcataccgcggtgaacgagcgtgatttcgaggccgagataagggctatggtgagagggaagaaaccaagcattgctgaggtcaaaagagccatccatcaaactatatccaatattaaactatag

SEQ ID NO: 138 - protein, 99 aa, Thlaspi arvense; identical to SEQ ID NO: 134

SEQ ID NO: 139 - DNA, 1707 bp, Thlaspi arvense
  source 1..1707: mol_type = genomic DNA
atgtcacaatattccttcttctatttcttcctaatctctcttttcctctacgaaaattgcattgcgtatcgctacacattcacggttattgaagctccatatagcaaactgtgtagcacgaagaagattttgaccgttaatggtcagtttcctggaccagtgttaagggcttacaaaggtgacaccatttacgttaacgttcgtaaccaagctagtgaaaatatcacattgcattggcatggtgtagagcagccgagaaacccgtggtcagatggacccgaatacatcacacaatgcccgattcaacccgggtcagattttacgtacaaaattttactttccatcgaagacgcgactgtttgatggcatgcgcatagctcgtggacacgtgccaccgtacacggtctgattttcgtgtatcctcggcctcctgataccctgccttttccagaaccggactacgaagtccccttagtttttggagagtggtggaagagggatgtgagagaagtagtggaggatttcatgaggaacggaggtgaacctaatgtgtccgatgctttgactatcaatgggcatcctggtttcttgtatccttgctctcaatcagatacattcaagctcgtggtagagaagggcaaaacctaccgcattcggatggtaaacgccgcgatgaacctaattctcttcttcgccatcgcgaaccacaaactcaccgtggtcgccgccgatggccactacaccaaacctctaaccgctagttatatcaccatatctcctggccaaacgctagacctgttactatacgccgaccaaagtccagagagcacttataacatggcggccagagcttaccatagcaaccccaacgttgggttcaacaactctaccaccgtcgggatcttacgttactactcttcaaacgacgccggaacgtcttcatcagaacgttacccgtaccttcctggctacaatgacacctcagcagctttcgatttcttcacaaaaatcaaaggcttatactccagagtagctcccgccaaagtttcacgtaggataatcacgacggtttcgataaatctcctcaagtgtcccaacgactcgtgtgcaggcccaaacgggtcgaggttagcggcgagtatgaacaacatatcgttcgtcacaccgagccacgtggacatactaagagcttattaccttcacattaacggcgtttacggaacgcggtttccggagttcccaccgcggatattcaatttcacagcggacgaccaaccgctgtttttgcagactccgaggctggcgacggaggtaaagaagtttcagtacggggagacggttgagattgttatacaagggacgagtttggtaggtggtggaatcgatcatcctatgcatctccatggttttagcttctacgtggttggtttagggtttgggaattttaacgcacgtaaagatccctccaactataatctagacgatcctccttacagaaacacggcgactgtgcccaggaacggttggatcgctatcagattcgtagctgacaatccaggggtttggttcatgcactgtcactttgatagacatcaaacgtggggtatgaatgttgtcttcattgttaagaatggaataaaaccaaatcagaagattctacctccaccgcctggcttaccaccttgtgaccaatttgagaatctataa

SEQ ID NO: 140 - protein, 120 aa, Thlaspi arvense
MSQYSFFYFFLISLFLYENCIAYRYTFTVIEAPYSKLCSTKKILTVNGQFPGPVLRAYKGDTIYVNVRNQASENITLHWHGVEQPRNPWSDGPEYITQCPIQPGSDFTYKILLSIEDATV

SEQ ID NO: 141 - DNA, 1707 bp, Thlaspi arvense
  source 1..1707: mol_type = genomic DNA
atgtcacaatattccttcttctatttcttcctaatctctcttttcctctacgaaaattgcattgcgtatcgctacacattcacggttattgaagctccatatagcaaactgtgtagcacgaagaagattttgaccgttaatggtcagtttcctggaccagtgttaagggcttacaaaggtgacaccatttacgttaacgttcgtaaccaagctagtgaaaatatcacattgcattggcatggtgtagagcagccgagaaacccgtggtcagatggacccgaatacatcacacaatgcccgattcaacccgggtcagattttacgtacaaaattttactttccatcgaagacgcgactgtttggtggcatgcgcatagctcgtggacacgtgccaccgtacacggtctgattttcgtgtatcctcggcctcctgataccctgccttttccagaaccggactacgaagtccccttagtttttggagagtggtggaagagggatgtgagagaagtagtggaggatttcatgaggaacggaggtgaacctaatgtgtccgatgctttgactatcaatgggcatcctggtttcttgtatccttgctctcaatcagatacattcaagctcgtggtagagaagggcaaaacctaccgcatttggatggtaaacgccgcgatgaacctaattctcttcttcgccatcgcgaaccacaaactcaccgtggtcgccgccgatggccactacaccaaacctctaaccgctagttatatcaccatatctcctggccaaacgctagacctgttactatacgccgaccaaagtccagagagcacttataacatggcggccagagcttaccatagcaaccccaacgttgggttcaacaactctaccaccgtcgggatcttacgttactactcttcaaacgacgccggaacgtcttcatcagaacgttacccgtaccttcctggctacaatgacacctcagcagctttcgatttcttcacaaaaatcaaaggcttatactccagagtagctcccgccaaagtttcacgtaggataatcacgacggtttcgataaatctcctcaagtgtcccaacgactcgtgtgcaggcccaaacgggtcgaggttagcggcgagtatgaacaacatatcgttcgtcacaccgagccacgtggacatactaagagcttattaccttcacattaacggcgtttacggaacgcggtttccggagttcccaccgcggatattcaatttcacagcggacgaccaaccgctgtttttgcagactccgaggctggcgacggaggtaaagaagtttcagtacggggagacggttgagattgttatacaagggacgagtttggtaggtggtggaatcgatcatcctatgcatctccatggttttagcttctacgtggttggtttagggtttgggaattttaacgcacgtaaagatccctccaactataatctagacgatcctccttacagaaacacggcgactgtgcccaggaacggttggatcgctatcagattcgtagctgacaatccaggggtttggttcatgcactgtcactttgatagacatcaaacgtggggtatgaatgttgtcttcattgttaagaatggaataaaaccaaatcagaagattctacctccaccgcctggcttaccaccttgtgaccaatttgagaatctataa

SEQ ID NO: 142 - protein, 568 aa, Thlaspi arvense
MSQYSFFYFFLISLFLYENCIAYRYTFTVIEAPYSKLCSTKKILTVNGQFPGPVLRAYKGDTIYVNVRNQASENITLHWHGVEQPRNPWSDGPEYITQCPIQPGSDFTYKILLSIEDATVWWHAHSSWTRATVHGLIFVYPRPPDTLPFPEPDYEVPLVFGEWWKRDVREVVEDFMRNGGEPNVSDALTINGHPGFLYPCSQSDTFKLVVEKGKTYRIWMVNAAMNLILFFAIANHKLTVVAADGHYTKPLTASYITISPGQTLDLLLYADQSPESTYNMAARAYHSNPNVGFNNSTTVGILRYYSSNDAGTSSSERYPYLPGYNDTSAAFDFFTKIKGLYSRVAPAKVSRRIITTVSINLLKCPNDSCAGPNGSRLAASMNNISFVTPSHVDILRAYYLHINGVYGTRFPEFPPRIFNFTADDQPLFLQTPRLATEVKKFQYGETVEIVIQGTSLVGGGIDHPMHLHGFSFYVVGLGFGNFNARKDPSNYNLDDPPYRNTATVPRNGWIAIRFVADNPGVWFMHCHFDRHQTWGMNVVFIVKNGIKPNQKILPPPPGLPPCDQFENL

SEQ ID NO: 143 - DNA, 1708 bp, Thlaspi arvense
  source 1..1708: mol_type = genomic DNA
atgtcacaatattccttcttctatttcttcctaatctctcttttcctctacgaaaattgcattgcgtatcgctacacattcacggttattgaagctccatatagcaaactgtgtagcacgaagaagattttgaccgttaatggtcagtttcctggaccagtgtttaagggcttacaaaggtgacaccatttacgttaacgttcgtaaccaagctagtgaaaatatcacattgcattggcatggtgtagagcagccgagaaacccgtggtcagatggacccgaatacatcacacaatgcccgattcaacccgggtcagattttacgtacaaaattttactttccatcgaagacgcgactgtttggtggcatgcgcatagctcgtggacacgtgccaccgtacacggtctgattttcgtgtatcctcggcctcctgataccctgccttttccagaaccggactacgaagtccccttagtttttggagagtggtggaagagggatgtgagagaagtagtggaggatttcatgaggaacggaggtgaacctaatgtgtccgatgctttgactatcaatgggcatcctggtttcttgtatccttgctctcaatcagatacattcaagctcgtggtagagaagggcaaaacctaccgcattcggatggtaaacgccgcgatgaacctaattctcttcttcgccatcgcgaaccacaaactcaccgtggtcgccgccgatggccactacaccaaacctctaaccgctagttatatcaccatatctcctggccaaacgctagacctgttactatacgccgaccaaagtccagagagcacttataacatggcggccagagcttaccatagcaaccccaacgttgggttcaacaactctaccaccgtcgggatcttacgttactactcttcaaacgacgccggaacgtcttcatcagaacgttacccgtaccttcctggctacaatgacacctcagcagctttcgatttcttcacaaaaatcaaaggcttatactccagagtagctcccgccaaagtttcacgtaggataatcacgacggtttcgataaatctcctcaagtgtcccaacgactcgtgtgcaggcccaaacgggtcgaggttagcggcgagtatgaacaacatatcgttcgtcacaccgagccacgtggacatactaagagcttattaccttcacattaacggcgtttacggaacgcggtttccggagttcccaccgcggatattcaatttcacagcggacgaccaaccgctgtttttgcagactccgaggctggcgacggaggtaaagaagtttcagtacggggagacggttgagattgttatacaagggacgagtttggtaggtggtggaatcgatcatcctatgcatctccatggttttagcttctacgtggttggtttagggtttgggaattttaacgcacgtaaagatccctccaactataatctagacgatcctccttacagaaacacggcgactgtgcccaggaacggttggatcgctatcagattcgtagctgacaatccaggggtttggttcatgcactgtcactttgatagacatcaaacgtggggtatgaatgttgtcttcattgttaagaatggaataaaaccaaatcagaagattctacctccaccgcctggcttaccaccttgtgaccaatttgagaatctataa

SEQ ID NO: 144 - protein, 60 aa, Thlaspi arvense
MSQYSFFYFFLISLFLYENCIAYRYTFTVIEAPYSKLCSTKKILTVNGQFPGPVFKGLQR

SEQ ID NO: 145 - DNA, 1708 bp, Thlaspi arvense
  source 1..1708: mol_type = genomic DNA
atgtcacaatattccttcttctatttcttcctaatctctcttttcctctacgaaaattgcattgcgtatcgctacacattcacggttattgaagctccatatagcaaactgtgtagcacgaagaagattttgaccgttaatggtcagtttcctggaccagtgattaagggcttacaaaggtgacaccatttacgttaacgttcgtaaccaagctagtgaaaatatcacattgcattggcatggtgtagagcagccgagaaacccgtggtcagatggacccgaatacatcacacaatgcccgattcaacccgggtcagattttacgtacaaaattttactttccatcgaagacgcgactgtttggtggcatgcgcatagctcgtggacacgtgccaccgtacacggtctgattttcgtgtatcctcggcctcctgataccctgccttttccagaaccggactacgaagtccccttagtttttggagagtggtggaagagggatgtgagagaagtagtggaggatttcatgaggaacggaggtgaacctaatgtgtccgatgctttgactatcaatgggcatcctggtttcttgtatccttgctctcaatcagatacattcaagctcgtggtagagaagggcaaaacctaccgcattcggatggtaaacgccgcgatgaacctaattctcttcttcgccatcgcgaaccacaaactcaccgtggtcgccgccgatggccactacaccaaacctctaaccgctagttatatcaccatatctcctggccaaacgctagacctgttactatacgccgaccaaagtccagagagcacttataacatggcggccagagcttaccatagcaaccccaacgttgggttcaacaactctaccaccgtcgggatcttacgttactactcttcaaacgacgccggaacgtcttcatcagaacgttacccgtaccttcctggctacaatgacacctcagcagctttcgatttcttcacaaaaatcaaaggcttatactccagagtagctcccgccaaagtttcacgtaggataatcacgacggtttcgataaatctcctcaagtgtcccaacgactcgtgtgcaggcccaaacgggtcgaggttagcggcgagtatgaacaacatatcgttcgtcacaccgagccacgtggacatactaagagcttattaccttcacattaacggcgtttacggaacgcggtttccggagttcccaccgcggatattcaatttcacagcggacgaccaaccgctgtttttgcagactccgaggctggcgacggaggtaaagaagtttcagtacggggagacggttgagattgttatacaagggacgagtttggtaggtggtggaatcgatcatcctatgcatctccatggttttagcttctacgtggttggtttagggtttgggaattttaacgcacgtaaagatccctccaactataatctagacgatcctccttacagaaacacggcgactgtgcccaggaacggttggatcgctatcagattcgtagctgacaatccaggggtttggttcatgcactgtcactttgatagacatcaaacgtggggtatgaatgttgtcttcattgttaagaatggaataaaaccaaatcagaagattctacctccaccgcctggcttaccaccttgtgaccaatttgagaatctataa

SEQ ID NO: 146 - protein, 60 aa, Thlaspi arvense; identical to SEQ ID NO: 144

SEQ ID NO: 147 - DNA, 1700 bp, Thlaspi arvense
  source 1..1700: mol_type = genomic DNA
atgtcacaatattccttcttctatttcttcctaatctctcttttcctctacgaaaattgcattgcgtatcgctacacattcacggttattgaagctccatatagcaaactgtgtagcacgaagaagattttgaccgttaatggtcagtttcctggttaagggcttacaaaggtgacaccatttacgttaacgttcgtaaccaagctagtgaaaatatcacattgcattggcatggtgtagagcagccgagaaacccgtggtcagatggacccgaatacatcacacaatgcccgattcaacccgggtcagattttacgtacaaaattttactttccatcgaagacgcgactgtttggtggcatgcgcatagctcgtggacacgtgccaccgtacacggtctgattttcgtgtatcctcggcctcctgataccctgccttttccagaaccggactacgaagtccccttagtttttggagagtggtggaagagggatgtgagagaagtagtggaggatttcatgaggaacggaggtgaacctaatgtgtccgatgctttgactatcaatgggcatcctggtttcttgtatccttgctctcaatcagatacattcaagctcgtggtagagaagggcaaaacctaccgcattcggatggtaaacgccgcgatgaacctaattctcttcttcgccatcgcgaaccacaaactcaccgtggtcgccgccgatggccactacaccaaacctctaaccgctagttatatcaccatatctcctggccaaacgctagacctgttactatacgccgaccaaagtccagagagcacttataacatggcggccagagcttaccatagcaaccccaacgttgggttcaacaactctaccaccgtcgggatcttacgttactactcttcaaacgacgccggaacgtcttcatcagaacgttacccgtaccttcctggctacaatgacacctcagcagctttcgatttcttcacaaaaatcaaaggcttatactccagagtagctcccgccaaagtttcacgtaggataatcacgacggtttcgataaatctcctcaagtgtcccaacgactcgtgtgcaggcccaaacgggtcgaggttagcggcgagtatgaacaacatatcgttcgtcacaccgagccacgtggacatactaagagcttattaccttcacattaacggcgtttacggaacgcggtttccggagttcccaccgcggatattcaatttcacagcggacgaccaaccgctgtttttgcagactccgaggctggcgacggaggtaaagaagtttcagtacggggagacggttgagattgttatacaagggacgagtttggtaggtggtggaatcgatcatcctatgcatctccatggttttagcttctacgtggttggtttagggtttgggaattttaacgcacgtaaagatccctccaactataatctagacgatcctccttacagaaacacggcgactgtgcccaggaacggttggatcgctatcagattcgtagctgacaatccaggggtttggttcatgcactgtcactttgatagacatcaaacgtggggtatgaatgttgtcttcattgttaagaatggaataaaaccaaatcagaagattctacctccaccgcctggcttaccaccttgtgaccaatttgagaatctataa

SEQ ID NO: 148 - protein, 52 aa, Thlaspi arvense
MSQYSFFYFFLISLFLYENCIAYRYTFTVIEAPYSKLCSTKKILTVNGQFPG

SEQ ID NO: 149 - DNA, 1520 bp, Thlaspi arvense
  source 1..1520: mol_type = genomic DNA
atgagctccacggagacatatgagcctctattgagacggctccactcagattctcagttaaccgtaggttcttcaccggagatagaggagtttctcggccgtcgtagatccacggtgacgccacggtggtggctaaggctggccgtatgggaatcaaagcttctttggacgctctctggagcctccatagtggtctctgtgctgaattacatgctcagcttcgtcaccgttatgttcatcggccatcttggctctcttcagctcgccggcgcatccatcgccaccgtcggtatccaaggcctcgcttacggtatcatgttgggaatggcgagcgcggtccagacagtgtgtggtcaagcgtacggcgcgaggcagtactcatcaatgggaataatttgccaacgagccatggtcttgcacctcgcagctgcggtcctcctcacgttcctctactggtactcgggtccgatcctaaaggcgatgggccaatccgcagccatcgcacgcgagggtcaggtctttgcacgtgggattattccgcagatttatgcttttgccctcgcttgccctatgcagaggttcctccaggctcaaaaaattgtaaacccttttacatgtcactaggagttttcgtgctacacacgctactaacctggctggtaaccaacgtcctgcatttcggcttgctcggtgcagctctggtgctgagtttttcgtggtggcttctcgcggctgtgaatggtctgtatatcgtgatgagcccgagttgcaaggaaacttggaccgggttctcagctagggctttaagagggatttggccttacttcaagctcacgatagcttcagcagtcatgctatgtttggagatatggtacgtccaagggctagtgattatttccggtttactcaccaatcccacaattgccctagacgcaatttcgatttgcatgtattactggaattgggatatgcagttcatgcttggtctaagtgcggcaatcactgtccgagtgagcaacgagctaggagcgggaaacccacgagtggctaagttatcagtggtagtggttaacatcacgacggttgtcatcagcttattcctctgtgtcgttgtgctcgtgttccgcattggccttagtaaagccttcaccagcgacgcagaggttatagctgcagtctctgatctctttcccctgctcgccgtttccattttcttaaacggaatccaaccaattctctctggtgttgccattggaagtgggtggcaagcagtggtggcttatgtgaatcttgttacttactatgtcattggtcttcctattggctgtgttcttggcttcaaaaccagtcttggagttgcggggatctggtgggggatgattgcaggagttatacttcaaaccctaactttgattgttcttacactcagaactaactggaattccgaggtggagaatgcagctcataggttaaaagcttcagcaaatgagagtcaagaaatggctaccgaaggaatctaa

SEQ ID NO: 150 - protein, 207 aa, Thlaspi arvense
MSSTETYEPLLRRLHSDSQLTVGSSPEIEEFLGRRRSTVTPRWWLRLAVWESKLLWTLSGASIVVSVLNYMLSFVTVMFIGHLGSLQLAGASIATVGIQGLAYGIMLGMASAVQTVCGQAYGARQYSSMGIICQRAMVLHLAAAVLLTFLYWYSGPILKAMGQSAAIAREGQVFARGIIPQIYAFALACPMQRFLQAQKIVNPFTCH

SEQ ID NO: 151 - DNA, 1524 bp, Thlaspi arvense
  source 1..1524: mol_type = genomic DNA
atgagctccacggagacatatgagcctctattgagacggctccactcagattctcagttaaccgtaggttcttcaccggagatagaggagtttctcggccgtcgtagatccacggtgacgccacggtggtggctaaggctggccgtatgggaatcaaagcttctttggacgctctctggagcctccatagtggtctctgtgctgaattacatgctcagcttcgtcaccgttatgttcatcggccatcttggctctcttcagctcgccggcgcatccatcgccaccgtcggtatccaaggcctcgcttacggtatcatgttgggaatggcgagcgcggtccagacagtgtgtggtcaagcgtacggcgcgaggcagtactcatcaatgggaataatttgccaacgagccatggtcttgcacctcgcagctgcggtcctcctcacgttcctctactggtactcgggtccgatcctaaaggcgatgggccaatccgcagccatcgcacgcgagggtcaggtctttgcacgtgggattattccgcagatttatgcttttgccctcgcttgccctatgcagaggttcctccaggctcaaaaaattgtaaaccctttggcttacatgtcactaggagttttcgtgctacacacgctactaacctggctggtaaccaacgtcctgcatttcggcttgctcggtgcagctctggtgctgagtttttcgtggtggcttctcgcggctgtgaatggtctgtatatcgtgatgagcccgagttgcaaggaaacttggaccgggttctcagctagggctttaagagggatttggccttacttcaagctcacgatagcttcagcagtcatgctatgtttggagatatggtacgtccaagggctagtgattatttccggtttactcaccaatcccacaattgccctagacgcaatttcgatttgcatgtattactggaattgggatatgcagttcatgcttggtctaagtgcggcaatcactgtccgagtgagcaacgagctaggagcgggaaacccacgagtggctaagttatcagtggtagtggttaacatcacgacggttgtcatcagcttattcctctgtgtcgttgtgctcgtgttccgcattggccttagtaaagccttcaccagcgacgcagaggttatagctgcagtctctgatctctttcccctgctcgccgtttccattttcttaaacggaatccaaccaattctctctagtgttgccattggaagtgggtggcaagcagtggtggcttatgtgaatcttgttacttactatgtcattggtcttcctattggctgtgttcttggcttcaaaaccagtcttggagttgcggggatctggtgggggatgattgcaggagttatacttcaaaccctaactttgattgttcttacactcagaactaactggaattccgaggtggagaatgcagctcataggttaaaagcttcagcaaatgagagtcaagaaatggctaccgaaggaatctaa

SEQ ID NO: 152 - protein, 507 aa, Thlaspi arvense
MSSTETYEPLLRRLHSDSQLTVGSSPEIEEFLGRRRSTVTPRWWLRLAVWESKLLWTLSGASIVVSVLNYMLSFVTVMFIGHLGSLQLAGASIATVGIQGLAYGIMLGMASAVQTVCGQAYGARQYSSMGIICQRAMVLHLAAAVLLTFLYWYSGPILKAMGQSAAIAREGQVFARGIIPQIYAFALACPMQRFLQAQKIVNPLAYMSLGVFVLHTLLTWLVTNVLHFGLLGAALVLSFSWWLLAAVNGLYIVMSPSCKETWTGFSARALRGIWPYFKLTIASAVMLCLEIWYVQGLVIISGLLTNPTIALDAISICMYYWNWDMQFMLGLSAAITVRVSNELGAGNPRVAKLSVVVVNITTVVISLFLCVVVLVFRIGLSKAFTSDAEVIAAVSDLFPLLAVSIFLNGIQPILSSVAIGSGWQAVVAYVNLVTYYVIGLPIGCVLGFKTSLGVAGIWWGMIAGVILQTLTLIVLTLRTNWNSEVENAAHRLKASANESQEMATEGI

SEQ ID NO: 153 - DNA, 2214 bp, Thlaspi arvense
  source 1..2214: mol_type = genomic DNA
atgcttccattaatggcgataccacttgcgacttgcaggagcatcaactggtcagccacggaaaggattcctgtttcgcttctgttccggagtattcttctccaagacgacgaagtttgtagcgctgtgccactataccggatcctcgatcagaatgacgggcaacttggtcctataagtatggccgaggaatcagacaaaccattgctggatcctgatactctcaacagagaaggaattgacttgggtctgttgccattggaggaggtttttgaatacctaagaacatctccacgggggcttttatctggagatgctgaagaaagattgacgatatttggtcctaacagccttgaagagaaacgggagaacaagtttctgaagttcctaggttttatgtggaatcctttgtcatgggttatggaagctgcagcattgatggccatcgccctagcagatagtgaagtagagactatcagtcttttgctataccatttctgctcagtgctgaccggagaatcgctacctgtgaccaagaagaagggtgagcaagtcttctctggctctacttgtaagcaaggtgagatagaagctgttgtgatagccaccggttcgagcactttctttggtaaaacagcatctttggtggacagcacagatgcaactggacattttcagcaggttctaagcttgtgccagcagaaaaatgagattgcgcaaagagtttatgccatcataaatagatttgcagaaaaaggtttgaggtctcttgctgttgcttatcaggaaattccagagagaagcagcaacagtcctggaggaccatggttgttctgtggtctgttgccactgtttgatcctccaaggcatgacagtgctgaaaccatactgagagctcttaactttggagtttgtgttaagatgatcaccggtgatcagttggcgattgcaaaggagacaggaaggcgacttgggatgggaaccaatatgtatccttcttcctctttgttaggccacaacaacgatgatcacgaagccattccattggatgagcttattgaaatggcagatggatttgctggagtgttccctgaacacaagtatgagattgtaaagatattacaagaaaagaagcatgtggttggaatgaccggagatggtgtgaatgatgctcctgctctgaaaaaggctgacattggaatagctgtcgctgatgcaacagatgccgcaagaagttctgctgacattgtactaactgagcctggcttaagtgtaattatcagtgctgtcttgaccagcagagccattttccagcgtatgaagaactatacagtatatgcagtctcgatcaccatacgaatagtgctcggttttacacttttagcgttgatatgggaatacgactttccacctttcatggttttgataatcgcaatactcaatgacgggaccatcatgactatctctaaagatcgagtaaggccatctcctacacccgagagttggaagctcaaccagatatttgcgactggaattgtcattggaacataccttgcattggtcactgtcctattctactggatcattgtctctaccaccttcttcgagaaacacttccatgtaaaatcaatcggcaacaacagtgaacaagtctcatccgctctgtatctccaagtaagcatcatcagtcaagcactcatatttgtaacacgtagtcgaagctggtcttttcttgaacgtcccgggactctcctgattttcgccttccttgttgcccaacttgccgctacattgattgctgtctatgccaacatcagctttgctaacatcaccggcattggatggggatgggcaggtgttatatggttatacagtttgattttttacatacctcttgatattataaagttcttcttccactacgcattgagtggagatgcttggaaccttgtatttgaccgtaagacagcatttactaataagaaagattatagaaaagatgacggagcgtccaatgtaaccatctctcagagaagtcactctgcagaagaactcagtggaagtcgttctcgcgcatcttggatcgctgagcagaccagaaggcgtgcagaaaccgccaggctcttggagggacactcggtgtcaaggcatttggaatcagtaatgaagctcaaacaaattgaccccaagatgattcgtgcagacactgtctaa

SEQ ID NO: 154 - protein, 737 aa, Thlaspi arvense
MLPLMAIPLATCRSINWSATERIPVSLLFRSILLQDDEVCSAVPLYRILDQNDGQLGPISMAEESDKPLLDPDTLNREGIDLGLLPLEEVFEYLRTSPRGLLSGDAEERLTIFGPNSLEEKRENKFLKFLGFMWNPLSWVMEAAALMAIALADSEVETISLLLYHFCSVLTGESLPVTKKKGEQVFSGSTCKQGEIEAVVIATGSSTFFGKTASLVDSTDATGHFQQVLSLCQQKNEIAQRVYAIINRFAEKGLRSLAVAYQEIPERSSNSPGGPWLFCGLLPLFDPPRHDSAETILRALNFGVCVKMITGDQLAIAKETGRRLGMGTNMYPSSSLLGHNNDDHEAIPLDELIEMADGFAGVFPEHKYEIVKILQEKKHVVGMTGDGVNDAPALKKADIGIAVADATDAARSSADIVLTEPGLSVIISAVLTSRAIFQRMKNYTVYAVSITIRIVLGFTLLALIWEYDFPPFMVLIIAILNDGTIMTISKDRVRPSPTPESWKLNQIFATGIVIGTYLALVTVLFYWIIVSTTFFEKHFHVKSIGNNSEQVSSALYLQVSIISQALIFVTRSRSWSFLERPGTLLIFAFLVAQLAATLIAVYANISFANITGIGWGWAGVIWLYSLIFYIPLDIIKFFFHYALSGDAWNLVFDRKTAFTNKKDYRKDDGASNVTISQRSHSAEELSGSRSRASWIAEQTRRRAETARLLEGHSVSRHLESVMKLKQIDPKMIRADTV

SEQ ID NO: 155 - DNA, 2214 bp, Thlaspi arvense
  source 1..2214: mol_type = genomic DNA
atgcttccattaatggcgataccacttgcgacttgcaggagcatcaactggtcagccacggaaaggattcctgtttcgcttctgttccggagtattcttctccaagacgacgaagtttgtagcgctgtgccactataccggatcctcgatcagaatgacgggcaacttggtcctataagtatggccgaggaatcagacaaaccattgctggatcctgatactctcaacagagaaggaattgacttgggtctgttgccattggaggaggtttttgaatacctaagaacatctccacgggggcttttatctggagatgctgaagaaagattgacgatatttggtcctaacagccttgaagagaaacgggagaacaagtttctgaagttcctaggttttatgtggaatcctttgtcatgggttatggaagctgcagcattgatggccatcgccctagcagatagtgaagtagagactatcagtcttttgctataccatttctgctcagtgctgaccggagaatcgctacctgtgaccaagaagaagggtgagcaagtcttctctggctctacttgtaagcaaggtgagatagaagctgttgtgatagccaccggttcgagcactttctttggtaaaacagcatctttggtggacagcacagatgcaactggacattttcagcaggttctaagcttgtgccagcagaaaaatgagattgcgcaaagagtttatgccatcataaatagatttgcagaaaaaggtttgaggtctcttgctgttgcttatcaggaaattccagagagaagcagcaacagtcctggaggaccatggttgttctgtggtctgttgccactgtttgatcctccaaggcatgacagtgctgaaaccatactgagagctcttaaccttggagtttgtgttaagatgatcaccggtgatcagttggcgattgcaaaggagacaggaaggtgacttgggatgggaaccaatatgtatccttcttcctctttgttaggccacaacaacgatgatcacgaagccattccattggatgagcttattgaaatggcagatggatttgctggagtgttccctgaacacaagtatgagattgtaaagatattacaagaaaagaagcatgtggttggaatgaccggagatggtgtgaatgatgctcctgctctgaaaaaggctgacattggaatagctgtcgctgatgcaacagatgccgcaagaagttctgctgacattgtactaactgagcctggcttaagtgtaattatcagtgctgtcttgaccagcagagccattttccagcgtatgaagaactatacagtatatgcagtctcgatcaccatacgaatagtgctcggttttacacttttagcgttgatatgggaatacgactttccacctttcatggttttgataatcgcaatactcaatgacgggaccatcatgactatctctaaagatcgagtaaggccatctcctacacccgagagttggaagctcaaccagatatttgcgactggaattgtcattggaacataccttgcattggtcactgtcctattctactggatcattgtctctaccaccttcttcgagaaacacttccatgtaaaatcaatcggcaacaacagtgaacaagtctcatccgctctgtatctccaagtaagcatcatcagtcaagcactcatatttgtaacacgtagtcgaagctggtcttttcttgaacgtcccgggactctcctgattttcgccttccttgttgcccaacttgccgctacattgattgctgtctatgccaacatcagctttgctaacatcaccggcattggatggggatgggcaggtgttatatggttatacagtttgattttttacatacctcttgatattataaagttcttcttccactacgcattgagtggagatgcttggaaccttgtatttgaccgtaagacagcatttactaataagaaagattatagaaaagatgacggagcgtccaatgtaaccatctctcagagaagtcactctgcagaagaactcagtggaagtcgttctcgcgcatcttggatcgctgagcagaccagaaggcgtgcagaaaccgccaggctcttggagggacactcggtgtcaaggcatttggaatcagtaatgaagctcaaacaaattgaccccaagatgattcgtgcagacactgtctaa

SEQ ID NO: 156 - protein, 322 aa, Thlaspi arvense
MLPLMAIPLATCRSINWSATERIPVSLLFRSILLQDDEVCSAVPLYRILDQNDGQLGPISMAEESDKPLLDPDTLNREGIDLGLLPLEEVFEYLRTSPRGLLSGDAEERLTIFGPNSLEEKRENKFLKFLGFMWNPLSWVMEAAALMAIALADSEVETISLLLYHFCSVLTGESLPVTKKKGEQVFSGSTCKQGEIEAVVIATGSSTFFGKTASLVDSTDATGHFQQVLSLCQQKNEIAQRVYAIINRFAEKGLRSLAVAYQEIPERSSNSPGGPWLFCGLLPLFDPPRHDSAETILRALNLGVCVKMITGDQLAIAKETGR

SEQ ID NO: 157 - DNA, 2214 bp, Thlaspi arvense
  source 1..2214: mol_type = genomic DNA
atgcttccattaatggcgataccacttgcgacttgcaggagcatcaactggtcagccacggaaaggattcctgtttcgcttctgttccggagtattcttctccaagacgacgaagtttgtagcgctgtgccactataccggatcctcgatcagaatgacgggcaacttggtcctataagtatggccgaggaatcagacaaaccattgctggatcctgatactctcaacagagaaggaattgacttgggtctgttgccattggaggaggtttttgaatacctaagaacatctccacgggggcttttatctggagatgctgaagaaagattgacgatatttggtcctaacagccttgaagagaaacgggagaacaagtttctgaagttcctaggttttatgtggaatcctttgtcatgggttatggaagctgcagcattgatggccatcgccctagcagatagtgaagtagagactatcagtcttttgctataccatttctgctcagtgctgaccggagaatcgctacctgtgaccaagaagaagggtgagcaagtcttctctggctctacttgtaagcaaggtgagatagaagctgttgtgatagccaccggttcgagcactttctttggtaaaacagcatctttggtggacagcacagatgcaactggacattttcagcaggttctaagcttgtgccagcagaaaaatgagattgcgcaaagagtttatgccatcataaatagatttgcagaaaaaggtttgaggtctcttgctgttgcttatcaggaaattccagagagaagcagcaacagtcctggaggaccatggttgttctgtggtctgttgccactgtttgatcctccaaggcatgacagtgctgaaaccatactgagagctcttaaccttggagtttgtgttaagatgatcaccggtgatcagttggcgattgcaaaggagacaggaaggcgacttgggatgggaaccaatatgtatccttcttcctctttgttaggccacaacaacgatgatcacgaagccattccattggatgagcttattgaaatggcagatggatttgctggagtgttccctgaacacaagtatgagattgtaaagatattacaagaaaagaagcatgtggttggaatgaccagagatggtgtgaatgatgctcctgctctgaaaaaggctgacattggaatagctgtcgctgatgcaacagatgccgcaagaagttctgctgacattgtactaactgagcctggcttaagtgtaattatcagtgctgtcttgaccagcagagccattttccagcgtatgaagaactatacagtatatgcagtctcgatcaccatacgaatagtgctcggttttacacttttagcgttgatatgggaatacgactttccacctttcatggttttgataatcgcaatactcaatgacgggaccatcatgactatctctaaagatcgagtaaggccatctcctacacccgagagttggaagctcaaccagatatttgcgactggaattgtcattggaacataccttgcattggtcactgtcctattctactggatcattgtctctaccaccttcttcgagaaacacttccatgtaaaatcaatcggcaacaacagtgaacaagtctcatccgctctgtatctccaagtaagcatcatcagtcaagcactcatatttgtaacacgtagtcgaagctggtcttttcttgaacgtcccgggactctcctgattttcgccttccttgttgcccaacttgccgctacattgattgctgtctatgccaacatcagctttgctaacatcaccggcattggatggggatgggcaggtgttatatggttatacagtttgattttttacatacctcttgatattataaagttcttcttccactacgcattgagtggagatgcttggaaccttgtatttgaccgtaagacagcatttactaataagaaagattatagaaaagatgacggagcgtccaatgtaaccatctctcagagaagtcactctgcagaagaactcagtggaagtcgttctcgcgcatcttggatcgctgagcagaccagaaggcgtgcagaaaccgccaggctcttggagggacactcggtgtcaaggcatttggaatcagtaatgaagctcaaacaaattgaccccaagatgattcgtgcagacactgtctaa

SEQ ID NO: 158 - protein, 737 aa, Thlaspi arvense
MLPLMAIPLATCRSINWSATERIPVSLLFRSILLQDDEVCSAVPLYRILDQNDGQLGPISMAEESDKPLLDPDTLNREGIDLGLLPLEEVFEYLRTSPRGLLSGDAEERLTIFGPNSLEEKRENKFLKFLGFMWNPLSWVMEAAALMAIALADSEVETISLLLYHFCSVLTGESLPVTKKKGEQVFSGSTCKQGEIEAVVIATGSSTFFGKTASLVDSTDATGHFQQVLSLCQQKNEIAQRVYAIINRFAEKGLRSLAVAYQEIPERSSNSPGGPWLFCGLLPLFDPPRHDSAETILRALNLGVCVKMITGDQLAIAKETGRRLGMGTNMYPSSSLLGHNNDDHEAIPLDELIEMADGFAGVFPEHKYEIVKILQEKKHVVGMTRDGVNDAPALKKADIGIAVADATDAARSSADIVLTEPGLSVIISAVLTSRAIFQRMKNYTVYAVSITIRIVLGFTLLALIWEYDFPPFMVLIIAILNDGTIMTISKDRVRPSPTPESWKLNQIFATGIVIGTYLALVTVLFYWIIVSTTFFEKHFHVKSIGNNSEQVSSALYLQVSIISQALIFVTRSRSWSFLERPGTLLIFAFLVAQLAATLIAVYANISFANITGIGWGWAGVIWLYSLIFYIPLDIIKFFFHYALSGDAWNLVFDRKTAFTNKKDYRKDDGASNVTISQRSHSAEELSGSRSRASWIAEQTRRRAETARLLEGHSVSRHLESVMKLKQIDPKMIRADTV

SEQ ID NO: 159 - DNA, 733 bp, Thlaspi arvense
  source 1..733: mol_type = genomic DNA
atgggaagagggaagatagagataaagaagatagagaatcagacagcgaggcaagtgaccttctgcaagaggagaactggtcttatcaagaagactaatgagctctctgttctctgcgatgctcacattggtctcatcgtcttctcctccaccggaaagctctcgcagtactgttccgaacccctcaggatgcctcagctcattgaccgatacttgaagacccagtggaatgcgacttcctgatcctaatgacggccgggaggaattgtaccaagagatggaagtactaaaaagagagacatgtaagcttgagcttcgtctgcgtccataccatggacatgacttaacctcccttcctccacacgagctcgatggtctcgagcaacagctcgaacattctgtccttaaagtccgcgagcgtaagaatgagttgatgcagcaacagttggagaatctaagcagaaagaggcggatgctagaagaagataacaacaatatgtaccgtttgcttcatgagcatcgtaacgcggttgaatttcagcaagctgggatagagacgaaaccaggggagtatcaacagtttctagagcagcttcagtactataatgatcatcagcaacaaccaaacagtgttcttcagcttgctacgcttccttctgagattgatcctaattaccatctccagcttgctcagcctaatcttcaaaacgatccaacggccaagattgattag

SEQ ID NO: 160 - protein, 80 aa, Thlaspi arvense
MGRGKIEIKKIENQTARQVTFCKRRTGLIKKTNELSVLCDAHIGLIVFSSTGKLSQYCSEPLRMPQLIDRYLKTQWNATS

SEQ ID NO: 161 - DNA, 733 bp, Thlaspi arvense
  source 1..733: mol_type = genomic DNA
atgggaagagggaagatagagataaagaagatagagaatcagacagcgaggcaagtgaccttctgcaagaggagaactggtcttatcaagaagactaatgagctctctgttctctgcgatgctcacattggtctcatcgtcttctcctccaccggaaagctctcgcagtactgttccgaacccctcaggatgcctcagctcattgaccgatacttgaagacgcagtggaatgcgacttcctgatcctaatgacggccgggaggaattgtaccaagagatggaagtactaaaaagagagacatgtaagcttgagcttcgtctgcgtccataccatggacatgacttaacctcccttcctccacacgagctcgatggtctcgagcaacagctcgaacattctgtccttaaagtccgcgagcgtaagaatgagttgatgcagcaacagttggagaatctaagcagaaagaggcggatgctagaagaagataacaacaatatgtaccgtttgcttcatgagcatcgtaacgcggttgaatttcagcaagctgggatagagacgaaaccaggggagtatcaacagtttctagagcagcttcagtactataatgatcatcagcaacaaccaaacagtgttcttcagcttgctacgcttccttctgagattgatcctaattaccatctccagcttgctcagcctaatcttcaaaacgatccaacggccaagattgattag

SEQ ID NO: 162 - protein, 80 aa, Thlaspi arvense; identical to SEQ ID NO: 160

SEQ ID NO: 163 - DNA, 733 bp, Thlaspi arvense
  source 1..733: mol_type = genomic DNA
atgggaagagggaagatagagataaagaagatagagaatcagacagcgaggcaagtgaccttctgcaagaggagaactggtcttatcaagaagactaatgagctctctgttctctgcgatgctcacattggtctcatcgtcttctcctccaccggaaagctctcgcagtactgttccgaacccctcaggatgcctcagctcattgaccgatacttgaagactcagtggaatgcgacttcctgatcctaatgacggccgggaggaattgtaccaagagatggaagtactaaaaagagagacatgtaagcttgagcttcgtctgcgtccataccatggacatgacttaacctcccttcctccacacgagctcgatggtctcgagcaacagctcgaacattctgtccttaaagtccgcgagcgtaagaatgagttgatgcagcaacagttggagaatctaagcagaaagaggcggatgctagaagaagataacaacaatatgtaccgtttgcttcatgagcatcgtaacgcggttgaatttcagcaagctgggatagagacgaaaccaggggagtatcaacagtttctagagcagcttcagtactataatgatcatcagcaacaaccaaacagtgttcttcagcttgctacgcttccttctgagattgatcctaattaccatctccagcttgctcagcctaatcttcaaaacgatccaacggccaagattgattag

SEQ ID NO: 164 - protein, 80 aa, Thlaspi arvense; identical to SEQ ID NO: 160

SEQ ID NO: 165 - DNA, 1005 bp, Thlaspi arvense
  source 1..1005: mol_type = genomic DNA
atggataactcagctccggattctttgtccagatcggaaaccgccgtcacctacgattctccttacccactctacgccatggccttctcttccatcggtactccctccggccaccgaatcgccgtcggaagcttcctcgaggattacaacaaccgcatcgacattctctccttcgattccgactccatgacggtgaagcctctcccgaatctctccttcgatcatccttatcctcccacaaagctgatgttcagccctccctccctccgtcgtccctccgccggcgatctcctccgtttatgggagatcagtgaagattcctccaccgtcgagcctgtctcggtgctcaacaacagcaagacgagcgagttctgcgcgccgttgacctccttcgactggaacgacgtcgagccgaaacgcctgggaacctgcagcatcgacacgacctgcacgatttgggacatcgagaagtgcgtggtggagacgcagctcatagcgcacgataaggaggtccacgacatcgcttggggagaagctagggttttcgcgtcggtctccgccgacggatccgtcaggatcttcgatctacgcgacaaggagcattccaccatcatctacgagagtcctcagcccgatacgcctctcctaagactcgcctggaacaaacaagacctgaggtacatggcgacgatcctgatggattcgaataaggtcgtgattctcgacattcgctcgccgacgatgcctgtcgccgagctcgaacggcaccaggctagcgtcaacgccatagcttgggctccacagagctgcaaacacatctgctctgctggtgacgacacgcaggctctcatctgggagctcccgactgtagctggacccaacggcattgatccgatgtcggtttactcagccggctcggagataaaccagttgcagtggtcctcttcacagcctgattggattggcatcgctttcgctaacaaaatgcagctccttagagtttga

SEQ ID NO: 166 - protein, 334 aa, Thlaspi arvense
MDNSAPDSLSRSETAVTYDSPYPLYAMAFSSIGTPSGHRIAVGSFLEDYNNRIDILSFDSDSMTVKPLPNLSFDHPYPPTKLMFSPPSLRRPSAGDLLRLWEISEDSSTVEPVSVLNNSKTSEFCAPLTSFDWNDVEPKRLGTCSIDTTCTIWDIEKCVVETQLIAHDKEVHDIAWGEARVFASVSADGSVRIFDLRDKEHSTIIYESPQPDTPLLRLAWNKQDLRYMATILMDSNKVVILDIRSPTMPVAELERHQASVNAIAWAPQSCKHICSAGDDTQALIWELPTVAGPNGIDPMSVYSAGSEINQLQWSSSQPDWIGIAFANKMQLLRV

SEQ ID NO: 167 - DNA, 1026 bp, Thlaspi arvense
  source 1..1026: mol_type = genomic DNA
atggataactcagctccggattctttgtccagatcggaaaccgccgtcacctacgattctccttacccactctacgccatggccttctcttccatcggtactccctccggccaccgaatcgccgtcggaagcttcctcgaggattacaacaaccgcatcgacattctctccttcgattccgactccatgacggtgaagcctctcccgaatctctccttcgatcatccttatcctcccacaaagctgatgttcagccctccctccctccgtcgtccctccgccggcgatctcctcgcttccttcggcgatttcctccgtttatgggagatcagtgaagattcctccaccgtcgagcctgtctcggtgctcaacaacagcaagacgagcgagttctgcgcgccgttgacctccttcgactggaacgacgtcgagccgaaacgcctgggaacctgcagcatcgacacgacctgcacgatttgggacatcgagaagtgcgtggtggagacgcagctcatagcgcacgataaggaggtccacgacatcgcttggggagaagctagggttttcgcgtcggtctccgccgacggatccgtcaggatcttcgatctacgcgacaaggagcattccaccatcatctacgagagtcctcagcccgatacgcctctcctaagactcgcctggaacaaacaagacctgaggtacatggcgacgatcctgatggattcgaataaggtcgtgattctcgacattcgctcgccgacgatgcctgtcgccgagctcgaacggcaccaggctagcgtcaacgccatagcttgggctccacagagctgcaaacacatctgctctgctggtgacgacacgcaggctctcatctgggagctcccgactgtagctggacccaacggcattgatccgatgtcggtttactcagccggctcggagataaaccagttgcagtggtcctcttcacagcctgattggattggcatcgctttcgctaacaaaatgcagctccttagagtttga

SEQ ID NO: 168 - protein, 341 aa, Thlaspi arvense
MDNSAPDSLSRSETAVTYDSPYPLYAMAFSSIGTPSGHRIAVGSFLEDYNNRIDILSFDSDSMTVKPLPNLSFDHPYPPTKLMFSPPSLRRPSAGDLLASFGDFLRLWEISEDSSTVEPVSVLNNSKTSEFCAPLTSFDWNDVEPKRLGTCSIDTTCTIWDIEKCVVETQLIAHDKEVHDIAWGEARVFASVSADGSVRIFDLRDKEHSTIIYESPQPDTPLLRLAWNKQDLRYMATILMDSNKVVILDIRSPTMPVAELERHQASVNAIAWAPQSCKHICSAGDDTQALIWELPTVAGPNGIDPMSVYSAGSEINQLQWSSSQPDWIGIAFANKMQLLRV

SEQ ID NO: 169 - DNA, 1026 bp, Thlaspi arvense
  source 1..1026: mol_type = genomic DNA
atggataactcagctccggattctttgtccagatcggaaaccgccgtcacctacgattctccttacccactctacgccatggccttctcttccatcggtactccctccggccaccgaatcgccgtcggaagcttcctcgaggattacaacaaccgcatcgacattctctccttcgattccgactccatgacggtgaagcctctcccgaatctctccttcgatcatccttatcctcccacaaagctgatgttcagccctccctccctccgtcgtccctccgccggcgatctcctcgcttcctccggcgatttcctccgtttatgggagatcagtgaagattcctccaccgtcgagcctgtctcggtgctcaacaacagcaagacgagcgagttctgcgcgccgttgacctccttcgactggaacgacgtcgagccgaaacgcctgggaacctgcagcatcgacacgacctgcacgatttgggacatcgagaagtgcgtggtggagacgcagctcatagcgcacgataaggaggtccacgacatcgcttgggaagaagctagggttttcgcgtcggtctccgccgacggatccgtcaggatcttcgatctacgcgacaaggagcattccaccatcatctacgagagtcctcagcccgatacgcctctcctaagactcgcctggaacaaacaagacctgaggtacatggcgacgatcctgatggattcgaataaggtcgtgattctcgacattcgctcgccgacgatgcctgtcgccgagctcgaacggcaccaggctagcgtcaacgccatagcttgggctccacagagctgcaaacacatctgctctgctggtgacgacacgcaggctctcatctgggagctcccgactgtagctggacccaacggcattgatccgatgtcggtttactcagccggctcggagataaaccagttgcagtggtcctcttcacagcctgattggattggcatcgctttcgctaacaaaatgcagctccttagagtttga

SEQ ID NO: 170 - protein, 341 aa, Thlaspi arvense
MDNSAPDSLSRSETAVTYDSPYPLYAMAFSSIGTPSGHRIAVGSFLEDYNNRIDILSFDSDSMTVKPLPNLSFDHPYPPTKLMFSPPSLRRPSAGDLLASSGDFLRLWEISEDSSTVEPVSVLNNSKTSEFCAPLTSFDWNDVEPKRLGTCSIDTTCTIWDIEKCVVETQLIAHDKEVHDIAWEEARVFASVSADGSVRIFDLRDKEHSTIIYESPQPDTPLLRLAWNKQDLRYMATILMDSNKVVILDIRSPTMPVAELERHQASVNAIAWAPQSCKHICSAGDDTQALIWELPTVAGPNGIDPMSVYSAGSEINQLQWSSSQPDWIGIAFANKMQLLRV

SEQ ID NO: 171 - DNA, 1917 bp, Thlaspi arvense
  source 1..1917: mol_type = other DNA
atgatggatggaatggttactgaacaaaacagaatatctgttccggagaatctgaaaaaacagctcgcagtttcagttcgaagaattcaatggagttacgcaatcttctggtctatttctgcttctcagcctggagtgttagaatggggagatggatactataatggagatatcaaaacgaggaagacgattctagcatcggagatcaaagctgatcagcttggtttacgaaggagcgagcaacttagggagctttacgagtctctttctgtcgctgaatcttcttcctccggcgtcgccgccggatctcaggtcactagacgagcttctgccgccgcactctcgccggaagatctcgccgacacagagtggtactacttggtttgtatgtctttcgtcttcaacatcggtgaaggaatgcctggacgaacgtttgcgaacagtgaaccgatatggttgtgcaacgctcacaccgcagatagtaaagtctttagccgctctcttctggcaaaaagtgcttcggttgtgacagtgatttgcttcccgtttcttggaggagtcgttgagatcggtactacagaacatatcatagaggacatgaatgtaatacaatgcgtgaagacatcattcctcgaagctccagatccatacgcttcactgttaccaacaagatccgattatcacatcgacaacgttctcgatccgcaacagatcctaggtgacgagatttacgcgcctatgtttggtactgagacttttccggcgacttctcctagcagaactaccagcaggttcgatcctgaacacgagcaagtagcagaagatcatgactcgttcatggccgaaggaatcaatggaggagcttctcaggttcaaagctggcagttcatggacgaagagcttagtaactgcgttcaccaatcgcttaattccagtgattgcgtctctcaaacgtttgttaaagcagcggctggacgagtttcttgcaacgcaagaaaaggaagggctcaaaggttagggcatattcaagagcggcagagaaatgtgaaaatgttgtcttttgatccaagaaacgatgacgttcattaccaaagtgtgatctccacaatttttaagaccaaccatcagttaattctcggaccgcagttccggaattgcgataagcggtcaagcttcacgaggtggaagaaattatcgtcatcatcatctggaaccgcgtcaatcgtatcaccgtcacaaggaatgttaaagaagattcttttcgaggttcctcgagtgcaccagaaagagaagttgttgttggattcaccagggatcggggatgaaaccacgaaccacgcggttttagagaagaaacggcgtgagaaattgaacgaacggttcatgatcttgagatcaatcattccatcaatcaataagatcgataaagtatcaattcttgacgatacgatagagtatcttcaagaactggaaagacgtgttcaagaactagaatcttgcagagaatcaaccgatacagaaacacgtgggacaatgacagtgaagaggaagaaatctcacgacgcaggggaaagaacttcagccaactgcacaaacaatgaaaccggaaacgggaagagagttcaggttggagaaaccgagccggcagagaccgattataccggtttaactgataatttaaggatcggttcgtttggtaatgaggtcgttattgagcttagatgtgcttggagagaaggagtattgcttgagataatggatgtcattagtgatctcaacttagattctcattcggtacaatcctcgacaggagatggtttactctgcttaaccgtcaactgcaagcacaagggttcaaaaatgacgacaacaggaatgatcaaagaggcacttcaaaaggttgcatggatctgttga

SEQ ID NO: 172 - protein, 638 aa, Thlaspi arvense
MMDGMVTEQNRISVPENLKKQLAVSVRRIQWSYAIFWSISASQPGVLEWGDGYYNGDIKTRKTILASEIKADQLGLRRSEQLRELYESLSVAESSSSGVAAGSQVTRRASAAALSPEDLADTEWYYLVCMSFVFNIGEGMPGRTFANSEPIWLCNAHTADSKVFSRSLLAKSASVVTVICFPFLGGVVEIGTTEHIIEDMNVIQCVKTSFLEAPDPYASLLPTRSDYHIDNVLDPQQILGDEIYAPMFGTETFPATSPSRTTSRFDPEHEQVAEDHDSFMAEGINGGASQVQSWQFMDEELSNCVHQSLNSSDCVSQTFVKAAAGRVSCNARKGRAQRLGHIQERQRNVKMLSFDPRNDDVHYQSVISTIFKTNHQLILGPQFRNCDKRSSFTRWKKLSSSSSGTASIVSPSQGMLKKILFEVPRVHQKEKLLLDSPGIGDETTNHAVLEKKRREKLNERFMILRSIIPSINKIDKVSILDDTIEYLQELERRVQELESCRESTDTETRGTMTVKRKKSHDAGERTSANCTNNETGNGKRVQVGETEPAETDYTGLTDNLRIGSFGNEVVIELRCAWREGVLLEIMDVISDLNLDSHSVQSSTGDGLLCLTVNCKHKGSKMTTTGMIKEALQKVAWIC

SEQ ID NO: 173 - DNA, 3577 bp, Thlaspi arvense
  source 1..3577: mol_type = genomic DNA
atgatgtaaagagttgcaggtttttcttttctttttttgtttgctataattttaaccccaaaaaaaaaactcactttttctaaatcaggacaaaaatgaaattgatccttttgttttctttttccattttgtatggtttcatgaaaatttagggatggaatggttactgaacaaaacagaatatctgttccggagaatctgaaaaaacagctcgcagtttcagttcgaagaattcaatggagttacgcaatcttctggtctatttctgcttctcagcctgggtgagtttcttaatcactatccttgaaactgatcagttttgttatttttgaaggttcaaatctctactagggggaaaaaaatgaatttcgaattttcattgctaaagcctttgtctgaagctagaagtgcttttggttctgccttaaaaattattaaaactttgataaaaagattactgatttaatttgggaaattttgatttattctgcttctaagttccatcaatgaagttcttcaactcaagacaatgttctaagtcgatttgagttttaggttgatactgtcttagagattattagaaattttataagtggaaatagtgagaccttattagttacaaaaaaaactcaaaacaaagattaattatggttttttttttcttaaaattcaattttcttttgtcttttttttgtgtgtggataattcgggccggaaaccgattaatctcagagtgtgcaagttcgttgggttcttgaagttcttcattagtttcttactgattcgattcgattttttgttttttattgtttgaaccaaaagagtgttagaatggggagatggatactataatggagatatcaaaacgaggaagacgattctagcatcggagatcaaagctgatcagcttggtttacgaaggagcgagcaacttagggagctttacgagtctctttctgtcgctgaatcttcttcctccggcgtcgccgccggatctcaggtcactagacgagcttctgccgccgcactctcgccggaagatctcgccgacacagagtggtactacttggtttgtatgtctttcgtcttcaacatcggtgaagggtaattgcgtctatttatctttcggcattgacatttactatgtgcgtcgtcatgttcggattgatcttgtcagtgaaataaataaaaaaaagacaaaatacccttttattacatgtatgtctggatattagactttttggtaaaaaactaaaaagttttaactagaaaccaaaaattattattttccacaatcgtttgaaatttcttttttttttcttttttttttggtttggtttggttcagtttagggtttttttggattttcagatttttaggtcctggagaaaagaagtccaagatcggtttggttaagtcaaattttaaaatgatttggataattggtcttggtttggtttttaattaaaaattaatcaaaatgaaaatatataattagatttaatcattattataaattttgtaaatgcttaatgaaatgaatttcgatttattcagttctgttacaccaaatatgcgtttggttttgctttttatgcatggcatttccgtcttttcacgtatctagctattcattcacagaatgcctggacgaacgtttgcgaacagtgaaccgatatggttgtgcaacgctcacaccgcagatagtaaagtctttagccgctctcttctggcaaaagttagttgtattatattgtagttgctatataacatttctttttttgcgactgcaaacgcttaaattaatcgttttttttgtgtgtttgtgtgttttgtgcctgtttagagtgcttcggttgtgacagtgatttgcttcccgtttcttggaggagtcgttgagatcggtactacagaacatgtaaggcaaaatttccattttctgtcacaatttgagaatagttataaaacaaccactagttaagtttataacagtgcgaactaattcatcagaccgacgaattaaggtataaagttatgatacaaaaagtttaaagacttatcttgttgtgtgttttatcccgtagatcatagaggacatgaatgtaatacaatgcgtgaagacatcattcctcgaagctccagatccatacgcttcactgttaccaacaagatccgattatcacatcgacaacgttctcgatccgcaacagatcctaggtgacgagatttacgcgcctatgtttggtactgagacttttccggcgacttctcctagcagaactaccagcaggttcgatcctgaacacgagcaagtagcagaagatcatgactcgttcatggccgaaggaatcaatggaggagcttctcaggttcaaagctggcagttcatggacgaagagcttagtaactgcgttcaccaatcgcttaattccagtgattgcgtctctcaaacgtttgttaaagcagcggctggacgagtttcttgcaacgcaagaaaaggaagggctcaaaggttagggcatattcaagagcggcagagaaatgtgaaaatgttgtcttttgatccaagaaacgatgacgttcattaccaaagtgtgatctccacaatttttaagaccaaccatcagttaattctcggaccgcagttccggaattgcgataagcggtcaagcttcacgaggtggaagaaattatcgtcatcatcatctggaaccgcgtcaatcgtatcaccgtcacaaggaatgttaaagaagattcttttcgaggttcctcgagtgcaccagaaagagaagttgttgttggattcaccagggatcggggatgaaaccacgaaccacgcggttttagagaagaaacggcgtgagaaattgaacgaacggttcatgatcttgagatcaatcattccatcaatcaataaggtatatataaccgaatcttcaaaaattcaaattcatattatgtaaccagagttaactaattctaggtttgacattttcaatagatcgataaagtatcaattcttgacgatacgatagagtatcttcaagaactggaaagacgtgttcaagaactagaatcttgcagagaatcaaccgatacagaaacacgtgggacaatgacagtgaagaggaagaaatctcacgacgcaggggaaagaacttcagccaactgcacaaacaatgaaaccggaaacgggaagagagttcaggttggagaaaccgagccggcagagaccgattataccggtttaactgataatttaaggatcggttcgtttggtaatgaggtcgttattgagcttagatgtgcttggagagaaggagtattgcttgagataatggatgtcattagtgatctcaacttagattctcattcggtacaatcctcgacaggagatggtttactctgcttaaccgtcaactgcaaggtacagcctttaacctaatttttgcttaaccgggataaggttaacatggattgatatattgtgaaatgttggtttcagcacaagggttcaaaaatgacgacaacaggaatgatcaaagaggcacttcaaaaggttgcatggatctgttga

SEQ ID NO: 174 - DNA, 1917 bp, Thlaspi arvense
  source 1..1917: mol_type = genomic DNA
atgatggatggaatggttactgaacaaaacagaatatctgttccggagaatctgaaaaaacagctcgcagtttcagttcgaagaattcaatggagttacgcaatcttctggtctatttctgcttctcagcctggagtgttagaatggggagatggatactataatggagatatcaaaacgaggaagacgattctagcatcggagatcaaagctgatcagcttggtttacgaaggagcgagcaacttaggaagctttacgagtctctttctgtcgctgaatcttcttcctccggcgtcgccgccggatctcaggtcactagacgagcttctgccgccgcactctcgccggaagatctcgccgacacagagtggtactacttggtttgtatgtctttcgtcttcaacatcggtgaaggaatgcctggacgaacgtttgcgaacagtgaaccgatatggttgtgcaacgctcacaccgcagatagtaaagtctttagccgctctcttctggcaaaaagtgcttcggttgtgacagtgatttgcttcccgtttcttggaggagtcgttgagatcggtactacagaacatatcatagaggacatgaatgtaatacaatgcgtgaagacatcattcctcgaagctccagatccatacgcttcactgttaccaacaagatccgattatcacatcgacaacgttctcgatccgcaacagatcctaggtgacgagatttacgcgcctatgtttggtactgagacttttccggcgacttctcctagcagaactaccagcaggttcgatcctgaacacgagcaagtagcagaagatcatgactcgttcatggccgaaggaatcaatggaggagcttctcaggttcaaagctggcagttcatggacgaagagcttagtaactgcgttcaccaatcgcttaattccagtgattgcgtctctcaaacgtttgttaaagcagcggctggacgagtttcttgcaacgcaagaaaaggaagggctcaaaggttagggcatattcaagagcggcagagaaatgtgaaaatgttgtcttttgatccaagaaacgatgacgttcattaccaaagtgtgatctccacaatttttaagaccaaccatcagttaattctcggaccgcagttccggaattgcgataagcggtcaagcttcacgaggtggaagaaattatcgtcatcatcatctggaaccgcgtcaatcgtatcaccgtcacaaggaatgttaaagaagattcttttcgaggttcctcgagtgcaccagaaagagaagttgttgttggattcaccagggatcggggatgaaaccacgaaccacgcggttttagagaagaaacggcgtgagaaattgaacgaacggttcatgatcttgagatcaatcattccatcaatcaataagatcgataaagtatcaattcttgacgatacgatagagtatcttcaagaactggaaagacgtgttcaagaactagaatcttgcagagaatcaaccgatacagaaacacgtgggacaatgacagtgaagaggaagaaatctcacgacgcaggggaaagaacttcagccaactgcacaaacaatgaaaccggaaacgggaagagagttcaggttggagaaaccgagccggcagagaccgattataccggtttaactgataatttaaggatcggttcgtttggtaatgaggtcgttattgagcttagatgtgcttggagagaaggagtattgcttgagataatggatgtcattagtgatctcaacttagattctcattcggtacaatcctcgacaggagatggtttactctgcttaaccgtcaactgcaagcacaagggttcaaaaatgacgacaacaggaatgatcaaagaggcacttcaaaaggttgcatggatctgttga

SEQ ID NO: 175 - protein, 638 aa, Thlaspi arvense
MMDGMVTEQNRISVPENLKKQLAVSVRRIQWSYAIFWSISASQPGVLEWGDGYYNGDIKTRKTILASEIKADQLGLRRSEQLRKLYESLSVAESSSSGVAAGSQVTRRASAAALSPEDLADTEWYYLVCMSFVFNIGEGMPGRTFANSEPIWLCNAHTADSKVFSRSLLAKSASVVTVICFPFLGGVVEIGTTEHIIEDMNVIQCVKTSFLEAPDPYASLLPTRSDYHIDNVLDPQQILGDEIYAPMFGTETFPATSPSRTTSRFDPEHEQVAEDHDSFMAEGINGGASQVQSWQFMDEELSNCVHQSLNSSDCVSQTFVKAAAGRVSCNARKGRAQRLGHIQERQRNVKMLSFDPRNDDVHYQSVISTIFKTNHQLILGPQFRNCDKRSSFTRWKKLSSSSSGTASIVSPSQGMLKKILFEVPRVHQKEKLLLDSPGIGDETTNHAVLEKKRREKLNERFMILRSIIPSINKIDKVSILDDTIEYLQELERRVQELESCRESTDTETRGTMTVKRKKSHDAGERTSANCTNNETGNGKRVQVGETEPAETDYTGLTDNLRIGSFGNEVVIELRCAWREGVLLEIMDVISDLNLDSHSVQSSTGDGLLCLTVNCKHKGSKMTTTGMIKEALQKVAWIC

SEQ ID NO: 176 - DNA, 1917 bp, Thlaspi arvense
  source 1..1917: mol_type = genomic DNA
atgatggatggaatggttactgaacaaaacagaatatctgttccggagaatctgaaaaaacagctcgcagtttcagttcgaagaattcaatggagttacgcaatcttctggtctatttctgcttctcagcctggagtgttagaatggggagatggatactataatggagatatcaaaacgaggaagacgattctagcatcggagatcaaagctgatcagcttggtttacgaaggagcgagcaacttagggagctttacgagtctctttctgtcgctgaatcttcttcctccggcgtcgccgccggatctcaggtcactagacgagcttctgccgccgcactctcgccggaagatctcgccgacacaaagtggtactacttggtttgtatgtctttcgtcttcaacatcggtgaaggaatgcctggacgaacgtttgcgaacagtgaaccgatatggttgtgcaacgctcacaccgcagatagtaaagtctttagccgctctcttctggcaaaaagtgcttcggttgtgacagtgatttgcttcccgtttcttggaggagtcgttgagatcggtactacagaacatatcatagaggacatgaatgtaatacaatgcgtgaagacatcattcctcgaagctccagatccatacgcttcactgttaccaacaagatccgattatcacatcgacaacgttctcgatccgcaacagatcctaggtgacgagatttacgcgcctatgtttggtactgagacttttccggcgacttctcctagcagaactaccagcaggttcgatcctgaacacgagcaagtagcagaagatcatgactcgttcatggccgaaggaatcaatggaggagcttctcaggttcaaagctggcagttcatggacgaagagcttagtaactgcgttcaccaatcgcttaattccagtgattgcgtctctcaaacgtttgttaaagcagcggctggacgagtttcttgcaacgcaagaaaaggaagggctcaaaggttagggcatattcaagagcggcagagaaatgtgaaaatgttgtcttttgatccaagaaacgatgacgttcattaccaaagtgtgatctccacaatttttaagaccaaccatcagttaattctcggaccgcagttccggaattgcgataagcggtcaagcttcacgaggtggaagaaattatcgtcatcatcatctggaaccgcgtcaatcgtatcaccgtcacaaggaatgttaaagaagattcttttcgaggttcctcgagtgcaccagaaagagaagttgttgttggattcaccagggatcggggatgaaaccacgaaccacgcggttttagagaagaaacggcgtgagaaattgaacgaacggttcatgatcttgagatcaatcattccatcaatcaataagatcgataaagtatcaattcttgacgatacgatagagtatcttcaagaactggaaagacgtgttcaagaactagaatcttgcagagaatcaaccgatacagaaacacgtgggacaatgacagtgaagaggaagaaatctcacgacgcaggggaaagaacttcagccaactgcacaaacaatgaaaccggaaacgggaagagagttcaggttggagaaaccgagccggcagagaccgattataccggtttaactgataatttaaggatcggttcgtttggtaatgaggtcgttattgagcttagatgtgcttggagagaaggagtattgcttgagataatggatgtcattagtgatctcaacttagattctcattcggtacaatcctcgacaggagatggtttactctgcttaaccgtcaactgcaagcacaagggttcaaaaatgacgacaacaggaatgatcaaagaggcacttcaaaaggttgcatggatctgttga

SEQ ID NO: 177 - protein, 638 aa, Thlaspi arvense
MMDGMVTEQNRISVPENLKKQLAVSVRRIQWSYAIFWSISASQPGVLEWGDGYYNGDIKTRKTILASEIKADQLGLRRSEQLRELYESLSVAESSSSGVAAGSQVTRRASAAALSPEDLADTKWYYLVCMSFVFNIGEGMPGRTFANSEPIWLCNAHTADSKVFSRSLLAKSASVVTVICFPFLGGVVEIGTTEHIIEDMNVIQCVKTSFLEAPDPYASLLPTRSDYHIDNVLDPQQILGDEIYAPMFGTETFPATSPSRTTSRFDPEHEQVAEDHDSFMAEGINGGASQVQSWQFMDEELSNCVHQSLNSSDCVSQTFVKAAAGRVSCNARKGRAQRLGHIQERQRNVKMLSFDPRNDDVHYQSVISTIFKTNHQLILGPQFRNCDKRSSFTRWKKLSSSSSGTASIVSPSQGMLKKILFEVPRVHQKEKLLLDSPGIGDETTNHAVLEKKRREKLNERFMILRSIIPSINKIDKVSILDDTIEYLQELERRVQELESCRESTDTETRGTMTVKRKKSHDAGERTSANCTNNETGNGKRVQVGETEPAETDYTGLTDNLRIGSFGNEVVIELRCAWREGVLLEIMDVISDLNLDSHSVQSSTGDGLLCLTVNCKHKGSKMTTTGMIKEALQKVAWIC

SEQ ID NO: 178 - DNA, 1917 bp, Thlaspi arvense
  source 1..1917: mol_type = genomic DNA
atgatggatggaatggttactgaacaaaacagaatatctgttccggagaatctgaaaaaacagctcgcagtttcagttcgaagaattcaatggagttacgcaatcttctggtctatttctgcttctcagcctggagtgttagaatggggagatggatactataatggagatatcaaaacgaggaagacgattctagcatcggagatcaaagctgatcagcttggtttacgaaggagcgagcaacttagggagctttacgagtctctttctgtcgctgaatcttcttcctccggcgtcgccgccggatctcaggtcactagacgagcttctgccgccgcactctcgccggaagatctcgccgacacagagtggtactacttggtttgtatgtctttcgtcttcaacatcggtgaaggaatgcctggacgaacgtttgcgaacagtgaaccgatatggttgtgcaacgctcacaccgcagatagtaaagtctttagccgctctcttctggcaaaaagtgcttcggttgtgacagtgatttgcttcccgtttcttggaggagtcgttgagatcggtactacagaacatatcatagaggacatgaatgtaatacaatgcgtgaagacatcattcctcgaagctccagatccatacgcttcactgttaccaacaagatccgattatcacatcgacaacgttctcgatccgcaacagatcctaggtgacgagatttacgcgcctatgtttggtactgagacttttccggcgacttctcctagcagaactaccagcaggttcgatcctgaacacgagcaagtagcagaagatcatgactcgttcatggccgaaggaatcaatggaggagcttctcaggttcaaagctggcagttcatggacgaagagcttagtaactgcgttcaccaatcgcttaattccagtgattgcgtctctcaaacgtttgttaaagcagcggctggacgagtttcttgcaacgcaagaaaaggaagggctcaaaggttagggcatattcaagagcggcagagaaatgtgaaaatgttgtcttttgatccaagaaacgatgacgttcattaccaaagtgtgatctccacaatttttaagaccaaccatcagttaattctcggaccgcagttccggaattgcgataagcggtcaagcttcacgaggtggaagaaattatcgtcatcatcatctggaaccgcgtcaatcgtatcaccgtcacaaggaatgttaaagaagattcttttcgaggttcctcgagtgcaccagaaagagaagttgttgttggattcaccagggatcggggatgaaaccacgaaccacgcggttttagagaagaaacggcgtgagaaattgaacgaacggttcatgatcttgagatcaatcattccatcaatcaataagatcgataaagtatcaattcttgacgatacgatagagtatcttcaagaactggaaagacgtgttcaagaactagaatcttgcagagaatcaaccgatacagaaacacgtgggacaatgacagtgaagaggaagaaatctcacgacgcaggggaaagaacttcagccaactgcacaaacaatgaaaccggaaacgggaagagagttcaggttggagaaaccgagccggcagagaccgattataccggtttaactaataatttaaggatcggttcgtttggtaatgaggtcgttattgagcttagatgtgcttggagagaaggagtattgcttgagataatggatgtcattagtgatctcaacttagattctcattcggtacaatcctcgacaggagatggtttactctgcttaaccgtcaactgcaagcacaagggttcaaaaatgacgacaacaggaatgatcaaagaggcacttcaaaaggttgcatggatctgttga

SEQ ID NO: 179 - protein, 638 aa, Thlaspi arvense
MMDGMVTEQNRISVPENLKKQLAVSVRRIQWSYAIFWSISASQPGVLEWGDGYYNGDIKTRKTILASEIKADQLGLRRSEQLRELYESLSVAESSSSGVAAGSQVTRRASAAALSPEDLADTEWYYLVCMSFVFNIGEGMPGRTFANSEPIWLCNAHTADSKVFSRSLLAKSASVVTVICFPFLGGVVEIGTTEHIIEDMNVIQCVKTSFLEAPDPYASLLPTRSDYHIDNVLDPQQILGDEIYAPMFGTETFPATSPSRTTSRFDPEHEQVAEDHDSFMAEGINGGASQVQSWQFMDEELSNCVHQSLNSSDCVSQTFVKAAAGRVSCNARKGRAQRLGHIQERQRNVKMLSFDPRNDDVHYQSVISTIFKTNHQLILGPQFRNCDKRSSFTRWKKLSSSSSGTASIVSPSQGMLKKILFEVPRVHQKEKLLLDSPGIGDETTNHAVLEKKRREKLNERFMILRSIIPSINKIDKVSILDDTIEYLQELERRVQELESCRESTDTETRGTMTVKRKKSHDAGERTSANCTNNETGNGKRVQVGETEPAETDYTGLTNNLRIGSFGNEVVIELRCAWREGVLLEIMDVISDLNLDSHSVQSSTGDGLLCLTVNCKHKGSKMTTTGMIKEALQKVAWIC

SEQ ID NO: 180 - DNA, 1041 bp, Thlaspi arvense
  source 1..1041: mol_type = genomic DNA
atgacaatcttggatcagaccgttgtaacaaccggatcgaagaaggcttgtgtcatcggtggcacaggaaacttagcttctactctcatcaagcatttgcttcaaagtggctacaaagttaacactacagttagagatccagagaatgagaagaaaatggctcacttaagggtacttcaagaacttggggacctcaagatcttcaaggcggaatttactgatgaagagagtttcgattcaccagtttcgggctgtgattacgttttccatgtcgcaacgcctatcaactttacatctgaagatcccgagaaagacatgatcaagccaaggatacaaggagtgaccaatgtgttgaaatcttgcttaaaatcgaaatcagtcaagcgtgtgatctacacttcttcagctgctgcggtttccatcaacaatctttctggacctggacttgtgatgaacgaagaaaactggactgaccttgattatctcacaaaggagaagccgtttaactggggctacccagtgtcaaagatactagcagaaaaggcagcttgtaaatttgcggaagagaacaagatcgatctagttaccgtgattccggcactcatatccggaaaatctctcctctcggatcctcctccgagcagctcatttctctctatgtctttaatcaccgggaatgaaatgtatctgaaaggtctcaaggaaatgcagaagcaatctggctccatctcgttcagccacgtgaaggatttggctcgtgcccatttgtttcttgcggagaaagaaactgcgtctggtcgttacatttgctgtacttacaacacaagtgttccggagattgcagattttctcaggcagagatatcctaagtacaatgtgctgtctgaattcgaagagtgcttatcaagtgcgaagctgacgctatcttcggaaaaactcatcaatgaaggctttcgattcgaatatgggattaatgagatctatgatgagatgatagagcacttcgagtccaaaggattaatcaaagctaaagaatcttga

SEQ ID NO: 181 - protein, 346 aa, Thlaspi arvense
MTILDQTVVTTGSKKACVIGGTGNLASTLIKHLLQSGYKVNTTVRDPENEKKMAHLRVLQELGDLKIFKAEFTDEESFDSPVSGCDYVFHVATPINFTSEDPEKDMIKPRIQGVTNVLKSCLKSKSVKRVIYTSSAAAVSINNLSGPGLVMNEENWTDLDYLTKEKPFNWGYPVSKILAEKAACKFAEENKIDLVTVIPALISGKSLLSDPPPSSSFLSMSLITGNEMYLKGLKEMQKQSGSISFSHVKDLARAHLFLAEKETASGRYICCTYNTSVPEIADFLRQRYPKYNVLSEFEECLSSAKLTLSSEKLINEGFRFEYGINEIYDEMIEHFESKGLIKAKES

SEQ ID NO: 182 - DNA, 1188 bp, Thlaspi arvense
  source 1..1188: mol_type = genomic DNA
atggtgatgggtacacaaccgtcgttggaagagatcagaaaggcacagagagcggatggccccgcaggcatcttggggataggcacggccaaccctgcgaaccatgtgatccaggcagagtatccggactactacttccgcatcaccaacagtgagcacatgactgacctcaaggagaagttcaagcgcatgtgcgacaagtcgatgatacggaaacggcacatgcacctgacggaggagttcctgaaggagaatccggacatgtgcgcctacatggctccttctcttgatgtgaggcaggacatcgtggtggtcgaggtccctaagctagggaaagaggcggcagtgaaggccatcaaggagtggggtcagcccaagtccaagatcacccacgtcgtcttctgcactacatccggagttgacatgcctggtgctgactaccagctcaccaagctcctcggtcttcgcccttccgtcaagcgtctcatgatgtaccagcaaggttgctacgccggcggcactgtcctccgactcgccaaggacctcgctgagaataaccgtggtgctcgtgtccttgtcgtctgctccgagatcacagccgtcaccttccgtggcccctctgacacacacctcgactccctcgttggtcaggctctcttcagtgacggtgctgccgcgctcattgttggtgcggaccctgatgcctccgtgggagagaagcctatcttcgagatggtgtctgctgcacagaccatcctcccagactcggacggagccatagatggacacttgagggaagttgggctcaccttccatctcctcaaggacgtccctgggctcatctcgaagaacatagagaagagtctagaagaagcgtttaaaccgctcgggataagtgactggaactctctcttttggatagctcaccctgaaggtcctgcgatcctggaccaggttgagttaaagctaggactcaaggaagagaagatgagggccacgcgtcacgtgctgagcgagtacggaaacatgtcgagcgcgtgcgttctcttcattatggacgagatgaggaggaagtccaaggaggatggtgtggccacgacaggagaagggttggagtggggtgtcttgtttggtttcggaccaggtctcaccgtagagacagtcgtcttgcacagcgtccctgtttga

SEQ ID NO: 183 - protein, 395 aa, Thlaspi arvense
MVMGTQPSLEEIRKAQRADGPAGILGIGTANPANHVIQAEYPDYYFRITNSEHMTDLKEKFKRMCDKSMIRKRHMHLTEEFLKENPDMCAYMAPSLDVRQDIVVVEVPKLGKEAAVKAIKEWGQPKSKITHVVFCTTSGVDMPGADYQLTKLLGLRPSVKRLMMYQQGCYAGGTVLRLAKDLAENNRGARVLVVCSEITAVTFRGPSDTHLDSLVGQALFSDGAAALIVGADPDASVGEKPIFEMVSAAQTILPDSDGAIDGHLREVGLTFHLLKDVPGLISKNIEKSLEEAFKPLGISDWNSLFWIAHPEGPAILDQVELKLGLKEEKMRATRHVLSEYGNMSSACVLFIMDEMRRKSKEDGVATTGEGLEWGVLFGFGPGLTVETVVLHSVPV

SEQ ID NO: 184 - DNA, 70 bp, synthetic construct
  misc_feature 1..70: note = synthetic, Figure 5A (top strand)
  source 1..70: mol_type = other DNA
agatagaagaagagcttgaagagatcttaatttctactgttgtagatacaccgtttctcgaattatcaga

SEQ ID NO: 185 - DNA, 70 bp, synthetic construct
  misc_feature 1..70: note = synthetic, Figure 5A (bottom strand)
  source 1..70: mol_type = other DNA
tagatctgataattcgagaaacggtgtatctacaacagtagaaattaagatctcttcaagctcttcttct

SEQ ID NO: 186 - DNA, 70 bp, synthetic construct
  misc_feature 1..70: note = synthetic, Figure 5B (top strand)
  source 1..70: mol_type = other DNA
agattccccggtctcaagtagttcttctaatttctactgttgtagatcaaggagattatggaggcggatt

SEQ ID NO: 187 - DNA, 70 bp, synthetic construct
  misc_feature 1..70: note = synthetic, Figure 5B (bottom strand)
  source 1..70: mol_type = other DNA
tagaaatccgcctccataatctccttgatctacaacagtagaaattagaagaactacttgagaccgggga

SEQ ID NO: 188 - DNA, 70 bp, synthetic construct
  misc_feature 1..70: note = synthetic, Figure 5C (top strand)
  source 1..70: mol_type = other DNA
agatcgaggcccttttggccggagagttaatttctactgttgtagatttgcaccgttgtagtatccattc

SEQ ID NO: 189 - DNA, 70 bp, synthetic construct
  misc_feature 1..70: note = synthetic, Figure 5C (bottom strand)
  source 1..70: mol_type = other DNA
tagagaatggatactacaacggtgcaaatctacaacagtagaaattaactctccggccaaaagggcctcg

SEQ ID NO: 190 - DNA, 70 bp, synthetic construct
  misc_feature 1..70: note = synthetic, Figure 5D (top strand)
  source 1..70: mol_type = other DNA
agatctgtgggagaatggatactacaataatttctactgttgtagatgccggagagtcctcatcggaagc

SEQ ID NO: 191 - DNA, 70 bp, synthetic construct
  misc_feature 1..70: note = synthetic, Figure 5D (bottom strand)
  source 1..70: mol_type = other DNA
tagagcttccgatgaggactctccggcatctacaacagtagaaattattgtagtatccattctcccacag

SEQ ID NO: 192 - DNA, 70 bp, synthetic construct
  misc_feature 1..70: note = synthetic, Figure 5E (top strand)
  source 1..70: mol_type = other DNA
agattacgtaaaatctgacccgggttgtaatttctactgttgtagatgtgtatcctcggcctcctgatac

SEQ ID NO: 193 - DNA, 70 bp, synthetic construct
  misc_feature 1..70: note = synthetic, Figure 5E (bottom strand)
  source 1..70: mol_type = other DNA
tagagtatcaggaggccgaggatacacatctacaacagtagaaattacaacccgggtcagattttacgta

SEQ ID NO: 194 - DNA, 70 bp, synthetic construct
  misc_feature 1..70: note = synthetic, Figure 5F (top strand)
  source 1..70: mol_type = other DNA
agatggtgcaagaccatggctcgttggtaatttctactgttgtagatctactggtactcgggtccgatcc

SEQ ID NO: 195 - DNA, 70 bp, synthetic construct
  misc_feature 1..70: note = synthetic, Figure 5F (bottom strand)
  source 1..70: mol_type = other DNA
tagaggatcggacccgagtaccagtagatctacaacagtagaaattaccaacgagccatggtcttgcacc

SEQ ID NO: 196 - DNA, 70 bp, synthetic construct
  misc_feature 1..70: note = synthetic, Figure 5G (top strand)
  source 1..70: mol_type = other DNA
agataattatgactcgcaggggacaattaatttctactgttgtagatccgctccgataatcgatctaatt

SEQ ID NO: 197 - DNA, 70 bp, synthetic construct
  misc_feature 1..70: note = synthetic, Figure 5G (bottom strand)
  source 1..70: mol_type = other DNA
tagaaattagatcgattatcggagcggatctacaacagtagaaattaattgtcccctgcgagtcataatt